European Patent Application EP 4 678 741 A1, published January 14, 2026. Title: RESPIRATORY SYNCYTIAL VIRUS MRNA VACCINE, AND PREPARATION METHOD THEREFOR AND USE THEREOF. Applicant: Hangzhou Tianlong Pharmaceutical Co., Ltd. Application EP. The sequence listing filed with the application follows.

SEQUENCE LISTING (225 sequences)

SEQ ID NO: 1 - protein, 574 aa, Orthopneumovirus hominis
MELLILKANAITTILTAVTFCFASGQNITEEFYQSTCSAVSKGYLSALRTGWYTSVITIELSNIKENKCNGTDAKVKLIKQELDKYKNAVTELQLLMQSTPPTNNRARRELPRFMNYTLNNAKKTNVTLSKKRKRRFLGFLLGVGSAIASGVAVSKVLHLEGEVNKIKSALLSTNKAVVSLSNGVSVLTSKVLDLKNYIDKQLLPIVNKQSCSISNIETVIEFQQKNNRLLEITREFSVNAGVTTPVSTYMLTNSELLSLINDMPITNDQKKLMSNNVQIVRQQSYSIMSIIKEEVLAYVVQLPLYGVIDTPCWKLHTSPLCTTNTKEGSNICLTRTDRGWYCDNAGSVSFFPQAETCKVQSNRVFCDTMNSLTLPSEINLCNVDIFNPKYDCKIMTSKTDVSSSVITSLGAIVSCYGKTKCTASNKNRGIIKTFSNGCDYVSNKGMDTVSVGNTLYYVNKQEGKSLYVKGEPIINFYDPLVFPSDEFDASISQVNEKINQSLAFIRKSDELLHNVNAGKSTTNIMITTIIIVIIVILLSLIAVGLLLYCKARSTPVTLSKDQLSGINNIAFSN

SEQ ID NO: 2 - DNA, 1841 bp, synthetic construct
  source 1..1841: mol_type = other DNA
agcggctcggccattttgtcccagtcagtccggaggctgcggctgcagaagtaccgcctgcggagtaactgcaaaggccaccatggaactgctgatcctgaaggccaacgccatcaccaccatcctgaccgccgtgaccttctgttttgccagcggccagaacatcaccgaggaattctaccagagcacctgtagcgccgtgtccaagggatatctgggcgcccttagaaccggctggtacaccagcgtgatcaccatcgagctgagcaacatcaaagaaaacaagtgcaacggcaccgacgccaaagtgaagctgatcaagcaagagctggacaagtacaagaatgccgtgaccgacctgcagctgctgatgcagtctacaccagccacaggctctggcagcgccatttgttctggtgtcgccgtgtgcaaagtgctgcacctggaaggcgaagtgaacaagatcaagagcgccctgctgagcaccaacaaggccgtggtgtctctgagcaatggcgtgtccgtgctgaccatcaaggtgctggacctgaagaactacatcgacaaacagctgctgcccatcgtcaacaagcagtcctgcagcatccccaacatcgagacagtgatcgagttccagcagaagaacaaccggctgctggaaatcacccgcgagttctctgtgaatgccggcgtgaccacacctgtgtccacctacatgctgaccaacagcgagctgctgagcctgatcaacgacatgcccatcaccaacgaccagaaaaagctgatgagcaacaacgtgcagatcgtgcggcagcagagctacagcatcatgtgcattatcaaagaagaggtgctggcctacgtggtgcagctgcctctgtatggcgtgatcgataccccttgctggaagctgcacacaagccctctgtgcaccaccaacaccaaagagggcagcaacatctgcctgaccagaaccgacagaggctggtactgcgataatgccggcagcgtctcattcttcccacaagccgagacatgcaaggtgcagagcaaccgggtgttctgcgacaccatgaatagcagaaccctgccttccgaagtgaatctgtgcaacgtggacatcttcaaccctaagtacgactgcaagatcatgaccagcaagaccgacgtgtccagcagtgtgatcacctcactgggcgccatcgtgtcctgttacggcaagaccaagtgcaccgccagcaacaagaaccggggcatcatcaagaccttcagcaacggctgcgactacgtgtccaacaaaggcgtggacaccgtgtctgtgggcaacaccctgtactgcgtgaacaaacaagagggccagtctctgtacgtgaagggcgagcccatcatcaacttctacgaccctctggtgttccccagcagcgagttcgatgccagcatcagccaagtgaacgagaagatcaatcagagcctggccttcatcagaaagtccgatgagctgctgcacaacgtgaacgccggcaagtccaccaccaatatcatgatcacgaccatcatcatcgtgattatcgtgatcctgctgtccctgatcgccgtgggcctgctgctttattgataataggctggagcctcggtggccatgcttcttgccccttgggcctccccccagcccctcctccccttcctgcacccgtacccccgtggtctttgaataaagtctgagtgggcggcaaaaaaaaaaaaaaaaaaaaaaaaaaaaaaaaaaaaaaaaaaaaaaaaaaaaaaaaaaaaaaaaaaaaaaaaaaaaaaaaaaaaaaaaaaaaaaaaaaaaaaaaaaaaaa

SEQ ID NO: 3 - DNA, 1539 bp, synthetic construct
  source 1..1539: mol_type = other DNA
atggaactgctgatcctgaaggccaacgccatcaccaccatcctgaccgccgtgaccttctgttttgccagcggccagaacatcaccgaggaattctaccagagcacctgtagcgccgtgtccaagggatatctgggcgcccttagaaccggctggtacaccagcgtgatcaccatcgagctgagcaacatcaaagaaaacaagtgcaacggcaccgacgccaaagtgaagctgatcaagcaagagctggacaagtacaagaatgccgtgaccgacctgcagctgctgatgcagtctacaccagccacaggctctggcagcgccatttgttctggtgtcgccgtgtgcaaagtgctgcacctggaaggcgaagtgaacaagatcaagagcgccctgctgagcaccaacaaggccgtggtgtctctgagcaatggcgtgtccgtgctgaccatcaaggtgctggacctgaagaactacatcgacaaacagctgctgcccatcgtcaacaagcagtcctgcagcatccccaacatcgagacagtgatcgagttccagcagaagaacaaccggctgctggaaatcacccgcgagttctctgtgaatgccggcgtgaccacacctgtgtccacctacatgctgaccaacagcgagctgctgagcctgatcaacgacatgcccatcaccaacgaccagaaaaagctgatgagcaacaacgtgcagatcgtgcggcagcagagctacagcatcatgtgcattatcaaagaagaggtgctggcctacgtggtgcagctgcctctgtatggcgtgatcgataccccttgctggaagctgcacacaagccctctgtgcaccaccaacaccaaagagggcagcaacatctgcctgaccagaaccgacagaggctggtactgcgataatgccggcagcgtctcattcttcccacaagccgagacatgcaaggtgcagagcaaccgggtgttctgcgacaccatgaatagcagaaccctgccttccgaagtgaatctgtgcaacgtggacatcttcaaccctaagtacgactgcaagatcatgaccagcaagaccgacgtgtccagcagtgtgatcacctcactgggcgccatcgtgtcctgttacggcaagaccaagtgcaccgccagcaacaagaaccggggcatcatcaagaccttcagcaacggctgcgactacgtgtccaacaaaggcgtggacaccgtgtctgtgggcaacaccctgtactgcgtgaacaaacaagagggccagtctctgtacgtgaagggcgagcccatcatcaacttctacgaccctctggtgttccccagcagcgagttcgatgccagcatcagccaagtgaacgagaagatcaatcagagcctggccttcatcagaaagtccgatgagctgctgcacaacgtgaacgccggcaagtccaccaccaatatcatgatcacgaccatcatcatcgtgattatcgtgatcctgctgtccctgatcgccgtgggcctgctgctttattgataatag

SEQ ID NO: 4 - protein, 510 aa, synthetic construct
MELLILKANAITTILTAVTFCFASGQNITEEFYQSTCSAVSKGYLGALRTGWYTSVITIELSNIKENKCNGTDAKVKLIKQELDKYKNAVTDLQLLMQSTPATGSGSAICSGVAVCKVLHLEGEVNKIKSALLSTNKAVVSLSNGVSVLTIKVLDLKNYIDKQLLPIVNKQSCSIPNIETVIEFQQKNNRLLEITREFSVNAGVTTPVSTYMLTNSELLSLINDMPITNDQKKLMSNNVQIVRQQSYSIMCIIKEEVLAYVVQLPLYGVIDTPCWKLHTSPLCTTNTKEGSNICLTRTDRGWYCDNAGSVSFFPQAETCKVQSNRVFCDTMNSRTLPSEVNLCNVDIFNPKYDCKIMTSKTDVSSSVITSLGAIVSCYGKTKCTASNKNRGIIKTFSNGCDYVSNKGVDTVSVGNTLYCVNKQEGQSLYVKGEPIINFYDPLVFPSSEFDASISQVNEKINQSLAFIRKSDELLHNVNAGKSTTNIMITTIIIVIIVILLSLIAVGLLLY

SEQ ID NO: 5 - RNA, 1841 nt, synthetic construct
  source 1..1841: mol_type = other RNA
agcggctcggccattttgtcccagtcagtccggaggctgcggctgcagaagtaccgcctgcggagtaactgcaaaggccaccatggaactgctgatcctgaaggccaacgccatcaccaccatcctgaccgccgtgaccttctgttttgccagcggccagaacatcaccgaggaattctaccagagcacctgtagcgccgtgtccaagggatatctgggcgcccttagaaccggctggtacaccagcgtgatcaccatcgagctgagcaacatcaaagaaaacaagtgcaacggcaccgacgccaaagtgaagctgatcaagcaagagctggacaagtacaagaatgccgtgaccgacctgcagctgctgatgcagtctacaccagccacaggctctggcagcgccatttgttctggtgtcgccgtgtgcaaagtgctgcacctggaaggcgaagtgaacaagatcaagagcgccctgctgagcaccaacaaggccgtggtgtctctgagcaatggcgtgtccgtgctgaccatcaaggtgctggacctgaagaactacatcgacaaacagctgctgcccatcgtcaacaagcagtcctgcagcatccccaacatcgagacagtgatcgagttccagcagaagaacaaccggctgctggaaatcacccgcgagttctctgtgaatgccggcgtgaccacacctgtgtccacctacatgctgaccaacagcgagctgctgagcctgatcaacgacatgcccatcaccaacgaccagaaaaagctgatgagcaacaacgtgcagatcgtgcggcagcagagctacagcatcatgtgcattatcaaagaagaggtgctggcctacgtggtgcagctgcctctgtatggcgtgatcgataccccttgctggaagctgcacacaagccctctgtgcaccaccaacaccaaagagggcagcaacatctgcctgaccagaaccgacagaggctggtactgcgataatgccggcagcgtctcattcttcccacaagccgagacatgcaaggtgcagagcaaccgggtgttctgcgacaccatgaatagcagaaccctgccttccgaagtgaatctgtgcaacgtggacatcttcaaccctaagtacgactgcaagatcatgaccagcaagaccgacgtgtccagcagtgtgatcacctcactgggcgccatcgtgtcctgttacggcaagaccaagtgcaccgccagcaacaagaaccggggcatcatcaagaccttcagcaacggctgcgactacgtgtccaacaaaggcgtggacaccgtgtctgtgggcaacaccctgtactgcgtgaacaaacaagagggccagtctctgtacgtgaagggcgagcccatcatcaacttctacgaccctctggtgttccccagcagcgagttcgatgccagcatcagccaagtgaacgagaagatcaatcagagcctggccttcatcagaaagtccgatgagctgctgcacaacgtgaacgccggcaagtccaccaccaatatcatgatcacgaccatcatcatcgtgattatcgtgatcctgctgtccctgatcgccgtgggcctgctgctttattgataataggctggagcctcggtggccatgcttcttgccccttgggcctccccccagcccctcctccccttcctgcacccgtacccccgtggtctttgaataaagtctgagtgggcggcaaaaaaaaaaaaaaaaaaaaaaaaaaaaaaaaaaaaaaaaaaaaaaaaaaaaaaaaaaaaaaaaaaaaaaaaaaaaaaaaaaaaaaaaaaaaaaaaaaaaaaaaaaaaaa

SEQ ID NO: 6 - DNA, 1841 bp, synthetic construct
  source 1..1841: mol_type = other DNA
agcggctcggccattttgtcccagtcagtccggaggctgcggctgcagaagtaccgcctgcggagtaactgcaaaggccaccatggaactgctgatcctgaaggccaacgccatcaccaccatcctgaccgccgtgaccttctgttttgccagcggccagaacatcaccgaggaattctaccagagcacctgtagcgccgtgtccaagggatatctgggcgcccttagaaccggctggtaccacagcgtgatcaccatcgagctgagcaacatcaaagaaaacaagtgcaacggcaccgacgccaaagtgaagctgatcaagcaagagctggacaagtacaagaatgccgtgaccgacctgcagctgctgatgcagtctacaccagccacaggctctggcagcgccatttgttctggtgtcgccgtgtgcaaagtgctgcacctggaaggcgaagtgaacaagatcaagagcgccctgctgagcaccaacaaggccgtggtgtctctgagcaatggcgtgtccgtgctgaccttcaaggtgctggacctgaagaactacatcgacaaacagctgctgcccatcgtcaacaagcagtcctgcagcatccccaacatcgagacagtgatcgagttccagcagaagaacaaccggctgctggaaatcacccgcgagttctctgtgaatgccggcgtgaccacacctgtgtccacctacatgctgaccaacagcgagctgctgagcctgatcaacgacatgcccatcaccaacgaccagaaaaagctgatgagcaacaacgtgcagatcgtgcggcagcagagctacagcatcatgtgcattatcaaagaagaggtgctggcctacgtggtgcagctgcctctgtatggcgtgatcgataccccttgctggaagctgcacacaagccctctgtgcaccaccaacaccaaagagggcagcaacatctgcctgaccagaaccgacagaggctggtactgcgataatgccggcagcgtctcattcttcccacaagccgagacatgcaaggtgcagagcaaccgggtgttctgcgacaccatgaatagcagaaccctgccttccgaagtgaatctgtgcaacgtggacatcttcaaccctaagtacgactgcaagatcatgaccagcaagaccgacgtgtccagcagtgtgatcacctcactgggcgccatcgtgtcctgttacggcaagaccaagtgcaccgccagcaacaagaaccggggcatcatcaagaccttcagcaacggctgcgactacgtgtccaacaaaggcgtggacaccgtgtctgtgggcaacaccctgtactgcgtgaacaaacaagagggccagtctctgtacgtgaagggcgagcccatcatcaacttctacgaccctctggtgttccccagcagcgagttcgatgccagcatcagccaagtgaacgagaagatcaatcagagcctggccttcatcagaaagtccgatgagctgctgcacaacgtgaacgccggcaagtccaccaccaatatcatgatcacgaccatcatcatcgtgattatcgtgatcctgctgtccctgatcgccgtgggcctgctgctttattgataataggctggagcctcggtggccatgcttcttgccccttgggcctccccccagcccctcctccccttcctgcacccgtacccccgtggtctttgaataaagtctgagtgggcggcaaaaaaaaaaaaaaaaaaaaaaaaaaaaaaaaaaaaaaaaaaaaaaaaaaaaaaaaaaaaaaaaaaaaaaaaaaaaaaaaaaaaaaaaaaaaaaaaaaaaaaaaaaaaaa

SEQ ID NO: 7 - DNA, 1539 bp, synthetic construct
  source 1..1539: mol_type = other DNA
atggaactgctgatcctgaaggccaacgccatcaccaccatcctgaccgccgtgaccttctgttttgccagcggccagaacatcaccgaggaattctaccagagcacctgtagcgccgtgtccaagggatatctgggcgcccttagaaccggctggtaccacagcgtgatcaccatcgagctgagcaacatcaaagaaaacaagtgcaacggcaccgacgccaaagtgaagctgatcaagcaagagctggacaagtacaagaatgccgtgaccgacctgcagctgctgatgcagtctacaccagccacaggctctggcagcgccatttgttctggtgtcgccgtgtgcaaagtgctgcacctggaaggcgaagtgaacaagatcaagagcgccctgctgagcaccaacaaggccgtggtgtctctgagcaatggcgtgtccgtgctgaccttcaaggtgctggacctgaagaactacatcgacaaacagctgctgcccatcgtcaacaagcagtcctgcagcatccccaacatcgagacagtgatcgagttccagcagaagaacaaccggctgctggaaatcacccgcgagttctctgtgaatgccggcgtgaccacacctgtgtccacctacatgctgaccaacagcgagctgctgagcctgatcaacgacatgcccatcaccaacgaccagaaaaagctgatgagcaacaacgtgcagatcgtgcggcagcagagctacagcatcatgtgcattatcaaagaagaggtgctggcctacgtggtgcagctgcctctgtatggcgtgatcgataccccttgctggaagctgcacacaagccctctgtgcaccaccaacaccaaagagggcagcaacatctgcctgaccagaaccgacagaggctggtactgcgataatgccggcagcgtctcattcttcccacaagccgagacatgcaaggtgcagagcaaccgggtgttctgcgacaccatgaatagcagaaccctgccttccgaagtgaatctgtgcaacgtggacatcttcaaccctaagtacgactgcaagatcatgaccagcaagaccgacgtgtccagcagtgtgatcacctcactgggcgccatcgtgtcctgttacggcaagaccaagtgcaccgccagcaacaagaaccggggcatcatcaagaccttcagcaacggctgcgactacgtgtccaacaaaggcgtggacaccgtgtctgtgggcaacaccctgtactgcgtgaacaaacaagagggccagtctctgtacgtgaagggcgagcccatcatcaacttctacgaccctctggtgttccccagcagcgagttcgatgccagcatcagccaagtgaacgagaagatcaatcagagcctggccttcatcagaaagtccgatgagctgctgcacaacgtgaacgccggcaagtccaccaccaatatcatgatcacgaccatcatcatcgtgattatcgtgatcctgctgtccctgatcgccgtgggcctgctgctttattgataatag

SEQ ID NO: 8 - protein, 510 aa, synthetic construct
MELLILKANAITTILTAVTFCFASGQNITEEFYQSTCSAVSKGYLGALRTGWYHSVITIELSNIKENKCNGTDAKVKLIKQELDKYKNAVTDLQLLMQSTPATGSGSAICSGVAVCKVLHLEGEVNKIKSALLSTNKAVVSLSNGVSVLTFKVLDLKNYIDKQLLPIVNKQSCSIPNIETVIEFQQKNNRLLEITREFSVNAGVTTPVSTYMLTNSELLSLINDMPITNDQKKLMSNNVQIVRQQSYSIMCIIKEEVLAYVVQLPLYGVIDTPCWKLHTSPLCTTNTKEGSNICLTRTDRGWYCDNAGSVSFFPQAETCKVQSNRVFCDTMNSRTLPSEVNLCNVDIFNPKYDCKIMTSKTDVSSSVITSLGAIVSCYGKTKCTASNKNRGIIKTFSNGCDYVSNKGVDTVSVGNTLYCVNKQEGQSLYVKGEPIINFYDPLVFPSSEFDASISQVNEKINQSLAFIRKSDELLHNVNAGKSTTNIMITTIIIVIIVILLSLIAVGLLLY

SEQ ID NO: 9 - RNA, 1841 nt, synthetic construct
  source 1..1841: mol_type = other RNA
agcggctcggccattttgtcccagtcagtccggaggctgcggctgcagaagtaccgcctgcggagtaactgcaaaggccaccatggaactgctgatcctgaaggccaacgccatcaccaccatcctgaccgccgtgaccttctgttttgccagcggccagaacatcaccgaggaattctaccagagcacctgtagcgccgtgtccaagggatatctgggcgcccttagaaccggctggtaccacagcgtgatcaccatcgagctgagcaacatcaaagaaaacaagtgcaacggcaccgacgccaaagtgaagctgatcaagcaagagctggacaagtacaagaatgccgtgaccgacctgcagctgctgatgcagtctacaccagccacaggctctggcagcgccatttgttctggtgtcgccgtgtgcaaagtgctgcacctggaaggcgaagtgaacaagatcaagagcgccctgctgagcaccaacaaggccgtggtgtctctgagcaatggcgtgtccgtgctgaccttcaaggtgctggacctgaagaactacatcgacaaacagctgctgcccatcgtcaacaagcagtcctgcagcatccccaacatcgagacagtgatcgagttccagcagaagaacaaccggctgctggaaatcacccgcgagttctctgtgaatgccggcgtgaccacacctgtgtccacctacatgctgaccaacagcgagctgctgagcctgatcaacgacatgcccatcaccaacgaccagaaaaagctgatgagcaacaacgtgcagatcgtgcggcagcagagctacagcatcatgtgcattatcaaagaagaggtgctggcctacgtggtgcagctgcctctgtatggcgtgatcgataccccttgctggaagctgcacacaagccctctgtgcaccaccaacaccaaagagggcagcaacatctgcctgaccagaaccgacagaggctggtactgcgataatgccggcagcgtctcattcttcccacaagccgagacatgcaaggtgcagagcaaccgggtgttctgcgacaccatgaatagcagaaccctgccttccgaagtgaatctgtgcaacgtggacatcttcaaccctaagtacgactgcaagatcatgaccagcaagaccgacgtgtccagcagtgtgatcacctcactgggcgccatcgtgtcctgttacggcaagaccaagtgcaccgccagcaacaagaaccggggcatcatcaagaccttcagcaacggctgcgactacgtgtccaacaaaggcgtggacaccgtgtctgtgggcaacaccctgtactgcgtgaacaaacaagagggccagtctctgtacgtgaagggcgagcccatcatcaacttctacgaccctctggtgttccccagcagcgagttcgatgccagcatcagccaagtgaacgagaagatcaatcagagcctggccttcatcagaaagtccgatgagctgctgcacaacgtgaacgccggcaagtccaccaccaatatcatgatcacgaccatcatcatcgtgattatcgtgatcctgctgtccctgatcgccgtgggcctgctgctttattgataataggctggagcctcggtggccatgcttcttgccccttgggcctccccccagcccctcctccccttcctgcacccgtacccccgtggtctttgaataaagtctgagtgggcggcaaaaaaaaaaaaaaaaaaaaaaaaaaaaaaaaaaaaaaaaaaaaaaaaaaaaaaaaaaaaaaaaaaaaaaaaaaaaaaaaaaaaaaaaaaaaaaaaaaaaaaaaaaaaaa

SEQ ID NO: 10 - DNA, 1841 bp, synthetic construct
  source 1..1841: mol_type = other DNA
agcggctcggccattttgtcccagtcagtccggaggctgcggctgcagaagtaccgcctgcggagtaactgcaaaggccaccatggaactgctgatcctgaaggccaacgccatcaccaccatcctgaccgccgtgaccttctgttttgccagcggccagaacatcaccgaggaattctaccagagcacctgtagcgccgtgtccaagggatatctgggcgcccttagaaccggctggtacaccagcgtgatcaccatcgagctgagcaacatcaaagaaaacaagtgcaacggcaccgacgccaaagtgaagctgatcaagcaagagctggacaagtacaagaatgccgtgaccgacctgcagctgctgatgcagtctacaccagccacaggctctggcagcgccatttgttctggtgtcgccgtgtgcaaagtgctgcacctggaaggcgaagtgaacaagatcaagagcgccctgctgagcaccaacaaggccgtggtgtctctgagcaatggcgtgtccgtgctgaccttcaaggtgctggacctgaagaactacatcgacaaacagctgctgcccatcgtcaacaagcagtcctgcagcatccccaacatcgagacagtgatcgagttccagcagaagaacaaccggctgctggaaatcacccgcgagttctctgtgaatgccggcgtgaccacacctgtgtccacctacatgctgaccaacagcgagctgctgagcctgatcaacgacatgcccatcaccaacgaccagaaaaagctgatgagcaacaacgtgcagatcgtgcggcagcagagctacagcatcatgtgcattatcaaagaagagatcctggcctacgtggtgcagctgcctctgtatggcgtgatcgataccccttgctggaagctgcacacaagccctctgtgcaccaccaacaccaaagagggcagcaacatctgcctgaccagaaccgacagaggctggtactgcgataatgccggcagcgtctcattcttcccacaagccgagacatgcaaggtgcagagcaaccgggtgttctgcgacaccatgaatagcagaaccctgccttccgaagtgaatctgtgcaacgtggacatcttcaaccctaagtacgactgcaagatcatgaccagcaagaccgacgtgtccagcagtgtgatcacctcactgggcgccatcgtgtcctgttacggcaagaccaagtgcaccgccagcaacaagaaccggggcatcatcaagaccttcagcaacggctgcgactacgtgtccaacaaaggcgtggacaccgtgtctgtgggcaacaccctgtactgcgtgaacaaacaagagggccagtctctgtacgtgaagggcgagcccatcatcaacttctacgaccctctggtgttccccagcagcgagttcgatgccagcatcagccaagtgaacgagaagatcaatcagagcctggccttcatcagaaagtccgatgagctgctgcacaacgtgaacgccggcaagtccaccaccaatatcatgatcacgaccatcatcatcgtgattatcgtgatcctgctgtccctgatcgccgtgggcctgctgctttattgataataggctggagcctcggtggccatgcttcttgccccttgggcctccccccagcccctcctccccttcctgcacccgtacccccgtggtctttgaataaagtctgagtgggcggcaaaaaaaaaaaaaaaaaaaaaaaaaaaaaaaaaaaaaaaaaaaaaaaaaaaaaaaaaaaaaaaaaaaaaaaaaaaaaaaaaaaaaaaaaaaaaaaaaaaaaaaaaaaaaa

SEQ ID NO: 11 - DNA, 1539 bp, synthetic construct
  source 1..1539: mol_type = other DNA
atggaactgctgatcctgaaggccaacgccatcaccaccatcctgaccgccgtgaccttctgttttgccagcggccagaacatcaccgaggaattctaccagagcacctgtagcgccgtgtccaagggatatctgggcgcccttagaaccggctggtacaccagcgtgatcaccatcgagctgagcaacatcaaagaaaacaagtgcaacggcaccgacgccaaagtgaagctgatcaagcaagagctggacaagtacaagaatgccgtgaccgacctgcagctgctgatgcagtctacaccagccacaggctctggcagcgccatttgttctggtgtcgccgtgtgcaaagtgctgcacctggaaggcgaagtgaacaagatcaagagcgccctgctgagcaccaacaaggccgtggtgtctctgagcaatggcgtgtccgtgctgaccttcaaggtgctggacctgaagaactacatcgacaaacagctgctgcccatcgtcaacaagcagtcctgcagcatccccaacatcgagacagtgatcgagttccagcagaagaacaaccggctgctggaaatcacccgcgagttctctgtgaatgccggcgtgaccacacctgtgtccacctacatgctgaccaacagcgagctgctgagcctgatcaacgacatgcccatcaccaacgaccagaaaaagctgatgagcaacaacgtgcagatcgtgcggcagcagagctacagcatcatgtgcattatcaaagaagagatcctggcctacgtggtgcagctgcctctgtatggcgtgatcgataccccttgctggaagctgcacacaagccctctgtgcaccaccaacaccaaagagggcagcaacatctgcctgaccagaaccgacagaggctggtactgcgataatgccggcagcgtctcattcttcccacaagccgagacatgcaaggtgcagagcaaccgggtgttctgcgacaccatgaatagcagaaccctgccttccgaagtgaatctgtgcaacgtggacatcttcaaccctaagtacgactgcaagatcatgaccagcaagaccgacgtgtccagcagtgtgatcacctcactgggcgccatcgtgtcctgttacggcaagaccaagtgcaccgccagcaacaagaaccggggcatcatcaagaccttcagcaacggctgcgactacgtgtccaacaaaggcgtggacaccgtgtctgtgggcaacaccctgtactgcgtgaacaaacaagagggccagtctctgtacgtgaagggcgagcccatcatcaacttctacgaccctctggtgttccccagcagcgagttcgatgccagcatcagccaagtgaacgagaagatcaatcagagcctggccttcatcagaaagtccgatgagctgctgcacaacgtgaacgccggcaagtccaccaccaatatcatgatcacgaccatcatcatcgtgattatcgtgatcctgctgtccctgatcgccgtgggcctgctgctttattgataatag

SEQ ID NO: 12 - protein, 510 aa, synthetic construct
MELLILKANAITTILTAVTFCFASGQNITEEFYQSTCSAVSKGYLGALRTGWYTSVITIELSNIKENKCNGTDAKVKLIKQELDKYKNAVTDLQLLMQSTPATGSGSAICSGVAVCKVLHLEGEVNKIKSALLSTNKAVVSLSNGVSVLTFKVLDLKNYIDKQLLPIVNKQSCSIPNIETVIEFQQKNNRLLEITREFSVNAGVTTPVSTYMLTNSELLSLINDMPITNDQKKLMSNNVQIVRQQSYSIMCIIKEEILAYVVQLPLYGVIDTPCWKLHTSPLCTTNTKEGSNICLTRTDRGWYCDNAGSVSFFPQAETCKVQSNRVFCDTMNSRTLPSEVNLCNVDIFNPKYDCKIMTSKTDVSSSVITSLGAIVSCYGKTKCTASNKNRGIIKTFSNGCDYVSNKGVDTVSVGNTLYCVNKQEGQSLYVKGEPIINFYDPLVFPSSEFDASISQVNEKINQSLAFIRKSDELLHNVNAGKSTTNIMITTIIIVIIVILLSLIAVGLLLY

SEQ ID NO: 13 - RNA, 1841 nt, synthetic construct
  source 1..1841: mol_type = other RNA
agcggctcggccattttgtcccagtcagtccggaggctgcggctgcagaagtaccgcctgcggagtaactgcaaaggccaccatggaactgctgatcctgaaggccaacgccatcaccaccatcctgaccgccgtgaccttctgttttgccagcggccagaacatcaccgaggaattctaccagagcacctgtagcgccgtgtccaagggatatctgggcgcccttagaaccggctggtacaccagcgtgatcaccatcgagctgagcaacatcaaagaaaacaagtgcaacggcaccgacgccaaagtgaagctgatcaagcaagagctggacaagtacaagaatgccgtgaccgacctgcagctgctgatgcagtctacaccagccacaggctctggcagcgccatttgttctggtgtcgccgtgtgcaaagtgctgcacctggaaggcgaagtgaacaagatcaagagcgccctgctgagcaccaacaaggccgtggtgtctctgagcaatggcgtgtccgtgctgaccttcaaggtgctggacctgaagaactacatcgacaaacagctgctgcccatcgtcaacaagcagtcctgcagcatccccaacatcgagacagtgatcgagttccagcagaagaacaaccggctgctggaaatcacccgcgagttctctgtgaatgccggcgtgaccacacctgtgtccacctacatgctgaccaacagcgagctgctgagcctgatcaacgacatgcccatcaccaacgaccagaaaaagctgatgagcaacaacgtgcagatcgtgcggcagcagagctacagcatcatgtgcattatcaaagaagagatcctggcctacgtggtgcagctgcctctgtatggcgtgatcgataccccttgctggaagctgcacacaagccctctgtgcaccaccaacaccaaagagggcagcaacatctgcctgaccagaaccgacagaggctggtactgcgataatgccggcagcgtctcattcttcccacaagccgagacatgcaaggtgcagagcaaccgggtgttctgcgacaccatgaatagcagaaccctgccttccgaagtgaatctgtgcaacgtggacatcttcaaccctaagtacgactgcaagatcatgaccagcaagaccgacgtgtccagcagtgtgatcacctcactgggcgccatcgtgtcctgttacggcaagaccaagtgcaccgccagcaacaagaaccggggcatcatcaagaccttcagcaacggctgcgactacgtgtccaacaaaggcgtggacaccgtgtctgtgggcaacaccctgtactgcgtgaacaaacaagagggccagtctctgtacgtgaagggcgagcccatcatcaacttctacgaccctctggtgttccccagcagcgagttcgatgccagcatcagccaagtgaacgagaagatcaatcagagcctggccttcatcagaaagtccgatgagctgctgcacaacgtgaacgccggcaagtccaccaccaatatcatgatcacgaccatcatcatcgtgattatcgtgatcctgctgtccctgatcgccgtgggcctgctgctttattgataataggctggagcctcggtggccatgcttcttgccccttgggcctccccccagcccctcctccccttcctgcacccgtacccccgtggtctttgaataaagtctgagtgggcggcaaaaaaaaaaaaaaaaaaaaaaaaaaaaaaaaaaaaaaaaaaaaaaaaaaaaaaaaaaaaaaaaaaaaaaaaaaaaaaaaaaaaaaaaaaaaaaaaaaaaaaaaaaaaaa

SEQ ID NO: 14 - DNA, 1841 bp, synthetic construct
  source 1..1841: mol_type = other DNA
agcggctcggccattttgtcccagtcagtccggaggctgcggctgcagaagtaccgcctgcggagtaactgcaaaggccaccatggaactgctgatcctgaaggccaacgccatcaccaccatcctgaccgccgtgaccttctgttttgccagcggccagaacatcaccgaggaattctaccagagcacctgtagcgccgtgtccaagggatatctgggcgcccttagaaccggctggtacaccagcgtgatcaccatcgagctgagcaacatcaaagaaaacaagtgcaacggcaccgacgccaaagtgaagctgatcaagcaagagctggacaagtacaagaatgccgtgaccgacctgcagctgctgatgcagtctacaccagccacaggctctggcagcgccatttgttctggtgtcgccgtgtgcaaagtgctgcacctggaaggcgaagtgaacaagatcaagagcgccctgctgagcaccaacaaggccgtggtgtctctgagcaatggcgtgtccgtgctgaccatcaaggtgctggacctgaagaactacatcgacaaacagctgctgcccatcgtcaacaagcagtcctgccccatcagcaacatcgagacagtgatcgagttccagcagaagaacaaccggctgctggaaatcacccgcgagttctctgtgaatgccggcgtgaccacacctgtgtccacctacatgctgaccaacagcgagctgctgagcctgatcaacgacatgcccatcaccaacgaccagaaaaagctgatgagcaacaacgtgcagatcgtgcggcagcagagctacagcatcatgtgcattatcaaagaagaggtgctggcctacgtggtgcagctgcctctgtatggcgtgatcgataccccttgctggaagctgcacacaagccctctgtgcaccaccaacaccaaagagggcagcaacatctgcctgaccagaaccgacagaggctggtactgcgataatgccggcagcgtctcattcttcccacaagccgagacatgcaaggtgcagagcaaccgggtgttctgcgacaccatgaatagcagaaccctgccttccgaagtgaatctgtgcaacgtggacatcttcaaccctaagtacgactgcaagatcatgaccagcaagaccgacgtgtccagcagtgtgatcacctcactgggcgccatcgtgtcctgttacggcaagaccaagtgcaccgccagcaacaagaaccggggcatcatcaagaccttcagcaacggctgcgactacgtgtccaacaaaggcgtggacaccgtgtctgtgggcaacaccctgtactgcgtgaacaaacaagagggccagtctctgtacgtgaagggcgagcccatcatcaacttctacgaccctctggtgttccccagcagcgagttcgatgccagcatcagccaagtgaacgagaagatcaatcagagcctggccttcatcagaaagtccgatgagctgctgcacaacgtgaacgccggcaagtccaccaccaatatcatgatcacgaccatcatcatcgtgattatcgtgatcctgctgtccctgatcgccgtgggcctgctgctttattgataataggctggagcctcggtggccatgcttcttgccccttgggcctccccccagcccctcctccccttcctgcacccgtacccccgtggtctttgaataaagtctgagtgggcggcaaaaaaaaaaaaaaaaaaaaaaaaaaaaaaaaaaaaaaaaaaaaaaaaaaaaaaaaaaaaaaaaaaaaaaaaaaaaaaaaaaaaaaaaaaaaaaaaaaaaaaaaaaaaaa

SEQ ID NO: 15 - DNA, 1539 bp, synthetic construct
  source 1..1539: mol_type = other DNA
atggaactgctgatcctgaaggccaacgccatcaccaccatcctgaccgccgtgaccttctgttttgccagcggccagaacatcaccgaggaattctaccagagcacctgtagcgccgtgtccaagggatatctgggcgcccttagaaccggctggtacaccagcgtgatcaccatcgagctgagcaacatcaaagaaaacaagtgcaacggcaccgacgccaaagtgaagctgatcaagcaagagctggacaagtacaagaatgccgtgaccgacctgcagctgctgatgcagtctacaccagccacaggctctggcagcgccatttgttctggtgtcgccgtgtgcaaagtgctgcacctggaaggcgaagtgaacaagatcaagagcgccctgctgagcaccaacaaggccgtggtgtctctgagcaatggcgtgtccgtgctgaccatcaaggtgctggacctgaagaactacatcgacaaacagctgctgcccatcgtcaacaagcagtcctgccccatcagcaacatcgagacagtgatcgagttccagcagaagaacaaccggctgctggaaatcacccgcgagttctctgtgaatgccggcgtgaccacacctgtgtccacctacatgctgaccaacagcgagctgctgagcctgatcaacgacatgcccatcaccaacgaccagaaaaagctgatgagcaacaacgtgcagatcgtgcggcagcagagctacagcatcatgtgcattatcaaagaagaggtgctggcctacgtggtgcagctgcctctgtatggcgtgatcgataccccttgctggaagctgcacacaagccctctgtgcaccaccaacaccaaagagggcagcaacatctgcctgaccagaaccgacagaggctggtactgcgataatgccggcagcgtctcattcttcccacaagccgagacatgcaaggtgcagagcaaccgggtgttctgcgacaccatgaatagcagaaccctgccttccgaagtgaatctgtgcaacgtggacatcttcaaccctaagtacgactgcaagatcatgaccagcaagaccgacgtgtccagcagtgtgatcacctcactgggcgccatcgtgtcctgttacggcaagaccaagtgcaccgccagcaacaagaaccggggcatcatcaagaccttcagcaacggctgcgactacgtgtccaacaaaggcgtggacaccgtgtctgtgggcaacaccctgtactgcgtgaacaaacaagagggccagtctctgtacgtgaagggcgagcccatcatcaacttctacgaccctctggtgttccccagcagcgagttcgatgccagcatcagccaagtgaacgagaagatcaatcagagcctggccttcatcagaaagtccgatgagctgctgcacaacgtgaacgccggcaagtccaccaccaatatcatgatcacgaccatcatcatcgtgattatcgtgatcctgctgtccctgatcgccgtgggcctgctgctttattgataatag

SEQ ID NO: 16 - protein, 510 aa, synthetic construct
MELLILKANAITTILTAVTFCFASGQNITEEFYQSTCSAVSKGYLGALRTGWYTSVITIELSNIKENKCNGTDAKVKLIKQELDKYKNAVTDLQLLMQSTPATGSGSAICSGVAVCKVLHLEGEVNKIKSALLSTNKAVVSLSNGVSVLTIKVLDLKNYIDKQLLPIVNKQSCPISNIETVIEFQQKNNRLLEITREFSVNAGVTTPVSTYMLTNSELLSLINDMPITNDQKKLMSNNVQIVRQQSYSIMCIIKEEVLAYVVQLPLYGVIDTPCWKLHTSPLCTTNTKEGSNICLTRTDRGWYCDNAGSVSFFPQAETCKVQSNRVFCDTMNSRTLPSEVNLCNVDIFNPKYDCKIMTSKTDVSSSVITSLGAIVSCYGKTKCTASNKNRGIIKTFSNGCDYVSNKGVDTVSVGNTLYCVNKQEGQSLYVKGEPIINFYDPLVFPSSEFDASISQVNEKINQSLAFIRKSDELLHNVNAGKSTTNIMITTIIIVIIVILLSLIAVGLLLY

SEQ ID NO: 17 - RNA, 1841 nt, synthetic construct
  source 1..1841: mol_type = other RNA
agcggctcggccattttgtcccagtcagtccggaggctgcggctgcagaagtaccgcctgcggagtaactgcaaaggccaccatggaactgctgatcctgaaggccaacgccatcaccaccatcctgaccgccgtgaccttctgttttgccagcggccagaacatcaccgaggaattctaccagagcacctgtagcgccgtgtccaagggatatctgggcgcccttagaaccggctggtacaccagcgtgatcaccatcgagctgagcaacatcaaagaaaacaagtgcaacggcaccgacgccaaagtgaagctgatcaagcaagagctggacaagtacaagaatgccgtgaccgacctgcagctgctgatgcagtctacaccagccacaggctctggcagcgccatttgttctggtgtcgccgtgtgcaaagtgctgcacctggaaggcgaagtgaacaagatcaagagcgccctgctgagcaccaacaaggccgtggtgtctctgagcaatggcgtgtccgtgctgaccatcaaggtgctggacctgaagaactacatcgacaaacagctgctgcccatcgtcaacaagcagtcctgccccatcagcaacatcgagacagtgatcgagttccagcagaagaacaaccggctgctggaaatcacccgcgagttctctgtgaatgccggcgtgaccacacctgtgtccacctacatgctgaccaacagcgagctgctgagcctgatcaacgacatgcccatcaccaacgaccagaaaaagctgatgagcaacaacgtgcagatcgtgcggcagcagagctacagcatcatgtgcattatcaaagaagaggtgctggcctacgtggtgcagctgcctctgtatggcgtgatcgataccccttgctggaagctgcacacaagccctctgtgcaccaccaacaccaaagagggcagcaacatctgcctgaccagaaccgacagaggctggtactgcgataatgccggcagcgtctcattcttcccacaagccgagacatgcaaggtgcagagcaaccgggtgttctgcgacaccatgaatagcagaaccctgccttccgaagtgaatctgtgcaacgtggacatcttcaaccctaagtacgactgcaagatcatgaccagcaagaccgacgtgtccagcagtgtgatcacctcactgggcgccatcgtgtcctgttacggcaagaccaagtgcaccgccagcaacaagaaccggggcatcatcaagaccttcagcaacggctgcgactacgtgtccaacaaaggcgtggacaccgtgtctgtgggcaacaccctgtactgcgtgaacaaacaagagggccagtctctgtacgtgaagggcgagcccatcatcaacttctacgaccctctggtgttccccagcagcgagttcgatgccagcatcagccaagtgaacgagaagatcaatcagagcctggccttcatcagaaagtccgatgagctgctgcacaacgtgaacgccggcaagtccaccaccaatatcatgatcacgaccatcatcatcgtgattatcgtgatcctgctgtccctgatcgccgtgggcctgctgctttattgataataggctggagcctcggtggccatgcttcttgccccttgggcctccccccagcccctcctccccttcctgcacccgtacccccgtggtctttgaataaagtctgagtgggcggcaaaaaaaaaaaaaaaaaaaaaaaaaaaaaaaaaaaaaaaaaaaaaaaaaaaaaaaaaaaaaaaaaaaaaaaaaaaaaaaaaaaaaaaaaaaaaaaaaaaaaaaaaaaaaa

SEQ ID NO: 18 - DNA, 1841 bp, synthetic construct
  source 1..1841: mol_type = other DNA
agcggctcggccattttgtcccagtcagtccggaggctgcggctgcagaagtaccgcctgcggagtaactgcaaaggccaccatggaactgctgatcctgaaggccaacgccatcaccaccatcctgaccgccgtgaccttctgttttgccagcggccagaacatcaccgaggaattctaccagagcacctgtagcgccgtgtccaagggatatctgggcgcccttagaaccggctggtacaccagcgtgatcaccatcgagctgagcaacatcaaagaaaacaagtgcaacggcaccgacgccaaagtgaagctgatcaagcaagagctggacaagtacaagaatgccgtgaccgacctgcagctgctgatgcagtctacaccagccacaggctctggcagcgccatttgttctggtgtcgccgtgtgcaaagtgctgcacctggaaggcgaagtgaacaagatcaagagcgccctgctgagcaccaacaaggccgtggtgtctctgagcaatggcgtgtccgtgctgaccatcaaggtgctggacctgaagaactacatcgacaaacagctgctgcccatcgtcaacaagcagtcctgcagcatcagccccatcgagacagtgatcgagttccagcagaagaacaaccggctgctggaaatcacccgcgagttctctgtgaatgccggcgtgaccacacctgtgtccacctacatgctgaccaacagcgagctgctgagcctgatcaacgacatgcccatcaccaacgaccagaaaaagctgatgagcaacaacgtgcagatcgtgcggcagcagagctacagcatcatgtgcattatcaaagaagaggtgctggcctacgtggtgcagctgcctctgtatggcgtgatcgataccccttgctggaagctgcacacaagccctctgtgcaccaccaacaccaaagagggcagcaacatctgcctgaccagaaccgacagaggctggtactgcgataatgccggcagcgtctcattcttcccacaagccgagacatgcaaggtgcagagcaaccgggtgttctgcgacaccatgaatagcagaaccctgccttccgaagtgaatctgtgcaacgtggacatcttcaaccctaagtacgactgcaagatcatgaccagcaagaccgacgtgtccagcagtgtgatcacctcactgggcgccatcgtgtcctgttacggcaagaccaagtgcaccgccagcaacaagaaccggggcatcatcaagaccttcagcaacggctgcgactacgtgtccaacaaaggcgtggacaccgtgtctgtgggcaacaccctgtactgcgtgaacaaacaagagggccagtctctgtacgtgaagggcgagcccatcatcaacttctacgaccctctggtgttccccagcagcgagttcgatgccagcatcagccaagtgaacgagaagatcaatcagagcctggccttcatcagaaagtccgatgagctgctgcacaacgtgaacgccggcaagtccaccaccaatatcatgatcacgaccatcatcatcgtgattatcgtgatcctgctgtccctgatcgccgtgggcctgctgctttattgataataggctggagcctcggtggccatgcttcttgccccttgggcctccccccagcccctcctccccttcctgcacccgtacccccgtggtctttgaataaagtctgagtgggcggcaaaaaaaaaaaaaaaaaaaaaaaaaaaaaaaaaaaaaaaaaaaaaaaaaaaaaaaaaaaaaaaaaaaaaaaaaaaaaaaaaaaaaaaaaaaaaaaaaaaaaaaaaaaaaa

SEQ ID NO: 19 - DNA, 1539 bp, synthetic construct
  source 1..1539: mol_type = other DNA
atggaactgctgatcctgaaggccaacgccatcaccaccatcctgaccgccgtgaccttctgttttgccagcggccagaacatcaccgaggaattctaccagagcacctgtagcgccgtgtccaagggatatctgggcgcccttagaaccggctggtacaccagcgtgatcaccatcgagctgagcaacatcaaagaaaacaagtgcaacggcaccgacgccaaagtgaagctgatcaagcaagagctggacaagtacaagaatgccgtgaccgacctgcagctgctgatgcagtctacaccagccacaggctctggcagcgccatttgttctggtgtcgccgtgtgcaaagtgctgcacctggaaggcgaagtgaacaagatcaagagcgccctgctgagcaccaacaaggccgtggtgtctctgagcaatggcgtgtccgtgctgaccatcaaggtgctggacctgaagaactacatcgacaaacagctgctgcccatcgtcaacaagcagtcctgcagcatcagccccatcgagacagtgatcgagttccagcagaagaacaaccggctgctggaaatcacccgcgagttctctgtgaatgccggcgtgaccacacctgtgtccacctacatgctgaccaacagcgagctgctgagcctgatcaacgacatgcccatcaccaacgaccagaaaaagctgatgagcaacaacgtgcagatcgtgcggcagcagagctacagcatcatgtgcattatcaaagaagaggtgctggcctacgtggtgcagctgcctctgtatggcgtgatcgataccccttgctggaagctgcacacaagccctctgtgcaccaccaacaccaaagagggcagcaacatctgcctgaccagaaccgacagaggctggtactgcgataatgccggcagcgtctcattcttcccacaagccgagacatgcaaggtgcagagcaaccgggtgttctgcgacaccatgaatagcagaaccctgccttccgaagtgaatctgtgcaacgtggacatcttcaaccctaagtacgactgcaagatcatgaccagcaagaccgacgtgtccagcagtgtgatcacctcactgggcgccatcgtgtcctgttacggcaagaccaagtgcaccgccagcaacaagaaccggggcatcatcaagaccttcagcaacggctgcgactacgtgtccaacaaaggcgtggacaccgtgtctgtgggcaacaccctgtactgcgtgaacaaacaagagggccagtctctgtacgtgaagggcgagcccatcatcaacttctacgaccctctggtgttccccagcagcgagttcgatgccagcatcagccaagtgaacgagaagatcaatcagagcctggccttcatcagaaagtccgatgagctgctgcacaacgtgaacgccggcaagtccaccaccaatatcatgatcacgaccatcatcatcgtgattatcgtgatcctgctgtccctgatcgccgtgggcctgctgctttattgataatag

SEQ ID NO: 20 - protein, 510 aa, synthetic construct
MELLILKANAITTILTAVTFCFASGQNITEEFYQSTCSAVSKGYLGALRTGWYTSVITIELSNIKENKCNGTDAKVKLIKQELDKYKNAVTDLQLLMQSTPATGSGSAICSGVAVCKVLHLEGEVNKIKSALLSTNKAVVSLSNGVSVLTIKVLDLKNYIDKQLLPIVNKQSCSISPIETVIEFQQKNNRLLEITREFSVNAGVTTPVSTYMLTNSELLSLINDMPITNDQKKLMSNNVQIVRQQSYSIMCIIKEEVLAYVVQLPLYGVIDTPCWKLHTSPLCTTNTKEGSNICLTRTDRGWYCDNAGSVSFFPQAETCKVQSNRVFCDTMNSRTLPSEVNLCNVDIFNPKYDCKIMTSKTDVSSSVITSLGAIVSCYGKTKCTASNKNRGIIKTFSNGCDYVSNKGVDTVSVGNTLYCVNKQEGQSLYVKGEPIINFYDPLVFPSSEFDASISQVNEKINQSLAFIRKSDELLHNVNAGKSTTNIMITTIIIVIIVILLSLIAVGLLLY

SEQ ID NO: 21 - RNA, 1841 nt, synthetic construct
  source 1..1841: mol_type = other RNA
agcggctcggccattttgtcccagtcagtccggaggctgcggctgcagaagtaccgcctgcggagtaactgcaaaggccaccatggaactgctgatcctgaaggccaacgccatcaccaccatcctgaccgccgtgaccttctgttttgccagcggccagaacatcaccgaggaattctaccagagcacctgtagcgccgtgtccaagggatatctgggcgcccttagaaccggctggtacaccagcgtgatcaccatcgagctgagcaacatcaaagaaaacaagtgcaacggcaccgacgccaaagtgaagctgatcaagcaagagctggacaagtacaagaatgccgtgaccgacctgcagctgctgatgcagtctacaccagccacaggctctggcagcgccatttgttctggtgtcgccgtgtgcaaagtgctgcacctggaaggcgaagtgaacaagatcaagagcgccctgctgagcaccaacaaggccgtggtgtctctgagcaatggcgtgtccgtgctgaccatcaaggtgctggacctgaagaactacatcgacaaacagctgctgcccatcgtcaacaagcagtcctgcagcatcagccccatcgagacagtgatcgagttccagcagaagaacaaccggctgctggaaatcacccgcgagttctctgtgaatgccggcgtgaccacacctgtgtccacctacatgctgaccaacagcgagctgctgagcctgatcaacgacatgcccatcaccaacgaccagaaaaagctgatgagcaacaacgtgcagatcgtgcggcagcagagctacagcatcatgtgcattatcaaagaagaggtgctggcctacgtggtgcagctgcctctgtatggcgtgatcgataccccttgctggaagctgcacacaagccctctgtgcaccaccaacaccaaagagggcagcaacatctgcctgaccagaaccgacagaggctggtactgcgataatgccggcagcgtctcattcttcccacaagccgagacatgcaaggtgcagagcaaccgggtgttctgcgacaccatgaatagcagaaccctgccttccgaagtgaatctgtgcaacgtggacatcttcaaccctaagtacgactgcaagatcatgaccagcaagaccgacgtgtccagcagtgtgatcacctcactgggcgccatcgtgtcctgttacggcaagaccaagtgcaccgccagcaacaagaaccggggcatcatcaagaccttcagcaacggctgcgactacgtgtccaacaaaggcgtggacaccgtgtctgtgggcaacaccctgtactgcgtgaacaaacaagagggccagtctctgtacgtgaagggcgagcccatcatcaacttctacgaccctctggtgttccccagcagcgagttcgatgccagcatcagccaagtgaacgagaagatcaatcagagcctggccttcatcagaaagtccgatgagctgctgcacaacgtgaacgccggcaagtccaccaccaatatcatgatcacgaccatcatcatcgtgattatcgtgatcctgctgtccctgatcgccgtgggcctgctgctttattgataataggctggagcctcggtggccatgcttcttgccccttgggcctccccccagcccctcctccccttcctgcacccgtacccccgtggtctttgaataaagtctgagtgggcggcaaaaaaaaaaaaaaaaaaaaaaaaaaaaaaaaaaaaaaaaaaaaaaaaaaaaaaaaaaaaaaaaaaaaaaaaaaaaaaaaaaaaaaaaaaaaaaaaaaaaaaaaaaaaaa

SEQ ID NO: 22 - DNA, 1841 bp, synthetic construct
  source 1..1841: mol_type = other DNA
agcggctcggccattttgtcccagtcagtccggaggctgcggctgcagaagtaccgcctgcggagtaactgcaaaggccaccatggaactgctgatcctgaaggccaacgccatcaccaccatcctgaccgccgtgaccttctgttttgccagcggccagaacatcaccgaggaattctaccagagcacctgtagcgccgtgtccaagggatatctgggcgcccttagaaccggctggtacacctgcgtgatcaccatcgagctgagcaacatcaaagaaaacaagtgcaacggcaccgacgccaaagtgaagctgatcaagcaagagctggacaagtacaagaatgccgtgaccgacctgcagctgctgatgcagtctacaccagccacaggctctggcagcgccattgcttctggtgtcgccgtgtctaaagtgctgcacctggaaggcgaagtgaacaagatcaagagcgccctgctgagcaccaacaaggccgtggtgtctctgagcaatggcgtgtccgtgtgcaccatcaaggtgctggacctgaagaactacatcgacaaacagctgctgcccatcgtcaacaagcagtcctgcagcatccccaacatcgagacagtgatcgagttccagcagaagaacaaccggctgctggaaatcacccgcgagttctctgtgaatgccggcgtgaccacacctgtgtccacctacatgctgaccaacagcgagctgctgagcctgatcaacgacatgcccatcaccaacgaccagaaaaagctgatgagcaacaacgtgcagatcgtgcggcagcagagctacagcatcatgagcattatcaaagaagaggtgctggcctacgtggtgcagctgcctctgtatggcgtgatcgataccccttgctggaagctgcacacaagccctctgtgcaccaccaacaccaaagagggcagcaacatctgcctgaccagaaccgacagaggctggtactgcgataatgccggcagcgtctcattcttcccacaagccgagacatgcaaggtgcagagcaaccgggtgttctgcgacaccatgaatagcagaaccctgccttccgaagtgaatctgtgcaacgtggacatcttcaaccctaagtacgactgcaagatcatgaccagcaagaccgacgtgtccagcagtgtgatcacctcactgggcgccatcgtgtcctgttacggcaagaccaagtgcaccgccagcaacaagaaccggggcatcatcaagaccttcagcaacggctgcgactacgtgtccaacaaaggcgtggacaccgtgtctgtgggcaacaccctgtactacgtgaacaaacaagagggccagtctctgtacgtgaagggcgagcccatcatcaacttctacgaccctctggtgttccccagcagcgagttcgatgccagcatcagccaagtgaacgagaagatcaatcagagcctggccttcatcagaaagtccgatgagctgctgcacaacgtgaacgccggcaagtccaccaccaatatcatgatcacgaccatcatcatcgtgattatcgtgatcctgctgtccctgatcgccgtgggcctgctgctttattgataataggctggagcctcggtggccatgcttcttgccccttgggcctccccccagcccctcctccccttcctgcacccgtacccccgtggtctttgaataaagtctgagtgggcggcaaaaaaaaaaaaaaaaaaaaaaaaaaaaaaaaaaaaaaaaaaaaaaaaaaaaaaaaaaaaaaaaaaaaaaaaaaaaaaaaaaaaaaaaaaaaaaaaaaaaaaaaaaaaaa

SEQ ID NO: 23 - DNA, 1539 bp, synthetic construct
  source 1..1539: mol_type = other DNA
atggaactgctgatcctgaaggccaacgccatcaccaccatcctgaccgccgtgaccttctgttttgccagcggccagaacatcaccgaggaattctaccagagcacctgtagcgccgtgtccaagggatatctgggcgcccttagaaccggctggtacacctgcgtgatcaccatcgagctgagcaacatcaaagaaaacaagtgcaacggcaccgacgccaaagtgaagctgatcaagcaagagctggacaagtacaagaatgccgtgaccgacctgcagctgctgatgcagtctacaccagccacaggctctggcagcgccattgcttctggtgtcgccgtgtctaaagtgctgcacctggaaggcgaagtgaacaagatcaagagcgccctgctgagcaccaacaaggccgtggtgtctctgagcaatggcgtgtccgtgtgcaccatcaaggtgctggacctgaagaactacatcgacaaacagctgctgcccatcgtcaacaagcagtcctgcagcatccccaacatcgagacagtgatcgagttccagcagaagaacaaccggctgctggaaatcacccgcgagttctctgtgaatgccggcgtgaccacacctgtgtccacctacatgctgaccaacagcgagctgctgagcctgatcaacgacatgcccatcaccaacgaccagaaaaagctgatgagcaacaacgtgcagatcgtgcggcagcagagctacagcatcatgagcattatcaaagaagaggtgctggcctacgtggtgcagctgcctctgtatggcgtgatcgataccccttgctggaagctgcacacaagccctctgtgcaccaccaacaccaaagagggcagcaacatctgcctgaccagaaccgacagaggctggtactgcgataatgccggcagcgtctcattcttcccacaagccgagacatgcaaggtgcagagcaaccgggtgttctgcgacaccatgaatagcagaaccctgccttccgaagtgaatctgtgcaacgtggacatcttcaaccctaagtacgactgcaagatcatgaccagcaagaccgacgtgtccagcagtgtgatcacctcactgggcgccatcgtgtcctgttacggcaagaccaagtgcaccgccagcaacaagaaccggggcatcatcaagaccttcagcaacggctgcgactacgtgtccaacaaaggcgtggacaccgtgtctgtgggcaacaccctgtactacgtgaacaaacaagagggccagtctctgtacgtgaagggcgagcccatcatcaacttctacgaccctctggtgttccccagcagcgagttcgatgccagcatcagccaagtgaacgagaagatcaatcagagcctggccttcatcagaaagtccgatgagctgctgcacaacgtgaacgccggcaagtccaccaccaatatcatgatcacgaccatcatcatcgtgattatcgtgatcctgctgtccctgatcgccgtgggcctgctgctttattgataatag

SEQ ID NO: 24 - protein, 510 aa, synthetic construct
MELLILKANAITTILTAVTFCFASGQNITEEFYQSTCSAVSKGYLGALRTGWYTCVITIELSNIKENKCNGTDAKVKLIKQELDKYKNAVTDLQLLMQSTPATGSGSAIASGVAVSKVLHLEGEVNKIKSALLSTNKAVVSLSNGVSVCTIKVLDLKNYIDKQLLPIVNKQSCSIPNIETVIEFQQKNNRLLEITREFSVNAGVTTPVSTYMLTNSELLSLINDMPITNDQKKLMSNNVQIVRQQSYSIMSIIKEEVLAYVVQLPLYGVIDTPCWKLHTSPLCTTNTKEGSNICLTRTDRGWYCDNAGSVSFFPQAETCKVQSNRVFCDTMNSRTLPSEVNLCNVDIFNPKYDCKIMTSKTDVSSSVITSLGAIVSCYGKTKCTASNKNRGIIKTFSNGCDYVSNKGVDTVSVGNTLYYVNKQEGQSLYVKGEPIINFYDPLVFPSSEFDASISQVNEKINQSLAFIRKSDELLHNVNAGKSTTNIMITTIIIVIIVILLSLIAVGLLLY

SEQ ID NO: 25 - RNA, 1841 nt, synthetic construct
  source 1..1841: mol_type = other RNA
agcggctcggccattttgtcccagtcagtccggaggctgcggctgcagaagtaccgcctgcggagtaactgcaaaggccaccatggaactgctgatcctgaaggccaacgccatcaccaccatcctgaccgccgtgaccttctgttttgccagcggccagaacatcaccgaggaattctaccagagcacctgtagcgccgtgtccaagggatatctgggcgcccttagaaccggctggtacacctgcgtgatcaccatcgagctgagcaacatcaaagaaaacaagtgcaacggcaccgacgccaaagtgaagctgatcaagcaagagctggacaagtacaagaatgccgtgaccgacctgcagctgctgatgcagtctacaccagccacaggctctggcagcgccattgcttctggtgtcgccgtgtctaaagtgctgcacctggaaggcgaagtgaacaagatcaagagcgccctgctgagcaccaacaaggccgtggtgtctctgagcaatggcgtgtccgtgtgcaccatcaaggtgctggacctgaagaactacatcgacaaacagctgctgcccatcgtcaacaagcagtcctgcagcatccccaacatcgagacagtgatcgagttccagcagaagaacaaccggctgctggaaatcacccgcgagttctctgtgaatgccggcgtgaccacacctgtgtccacctacatgctgaccaacagcgagctgctgagcctgatcaacgacatgcccatcaccaacgaccagaaaaagctgatgagcaacaacgtgcagatcgtgcggcagcagagctacagcatcatgagcattatcaaagaagaggtgctggcctacgtggtgcagctgcctctgtatggcgtgatcgataccccttgctggaagctgcacacaagccctctgtgcaccaccaacaccaaagagggcagcaacatctgcctgaccagaaccgacagaggctggtactgcgataatgccggcagcgtctcattcttcccacaagccgagacatgcaaggtgcagagcaaccgggtgttctgcgacaccatgaatagcagaaccctgccttccgaagtgaatctgtgcaacgtggacatcttcaaccctaagtacgactgcaagatcatgaccagcaagaccgacgtgtccagcagtgtgatcacctcactgggcgccatcgtgtcctgttacggcaagaccaagtgcaccgccagcaacaagaaccggggcatcatcaagaccttcagcaacggctgcgactacgtgtccaacaaaggcgtggacaccgtgtctgtgggcaacaccctgtactacgtgaacaaacaagagggccagtctctgtacgtgaagggcgagcccatcatcaacttctacgaccctctggtgttccccagcagcgagttcgatgccagcatcagccaagtgaacgagaagatcaatcagagcctggccttcatcagaaagtccgatgagctgctgcacaacgtgaacgccggcaagtccaccaccaatatcatgatcacgaccatcatcatcgtgattatcgtgatcctgctgtccctgatcgccgtgggcctgctgctttattgataataggctggagcctcggtggccatgcttcttgccccttgggcctccccccagcccctcctccccttcctgcacccgtacccccgtggtctttgaataaagtctgagtgggcggcaaaaaaaaaaaaaaaaaaaaaaaaaaaaaaaaaaaaaaaaaaaaaaaaaaaaaaaaaaaaaaaaaaaaaaaaaaaaaaaaaaaaaaaaaaaaaaaaaaaaaaaaaaaaaa

SEQ ID NO: 26 - DNA, 1841 bp, synthetic construct
  source 1..1841: mol_type = other DNA
agcggctcggccattttgtcccagtcagtccggaggctgcggctgcagaagtaccgcctgcggagtaactgcaaaggccaccatggaactgctgatcctgaaggccaacgccatcaccaccatcctgaccgccgtgaccttctgttttgccagcggccagaacatcaccgaggaattctactgcagcacctgtagcgccgtgtccaagggatatctgggcgcccttagaaccggctggtacaccagcgtgatcctgatcgagctgagcaacatcaaagaaaacaagtgcaacggcaccgacgccaaagtgaagctgatcaagcaagagctggacaagtacaagaatgccgtgaccgacctgcagctgctgatgcagtctacaccagccacaggctctggcagcgccattgcttctggtgtcgccgtgtctaaagtgctgcacctggaaggcgaagtgaacaagatcaagagcgccctgctgagcaccaacaaggccgtggtgtctctgagcaatggcgtgtccgtgctgaccttcaaggtgctggacctgaagaactacatcgacaaacagctgctgcccatcgtcaacaagcagtcctgcagcatccccaacatcgagacagtgatcgagttccagcagaagaacaaccggctgctggaaatcacccgcgagttctctgtgaatgccggcgtgaccacacctgtgtccacctacatgctgaccaacagcgagctgctgagcctgatcaacgacatgcccatcaccaacgaccagaaaaagctgatgagcaacaacgtgcagatcgtgcggcagcagagctacagcatcatgagcattatcaaagaagaggtgctggcctacgtggtgcagctgcctctgtatggcgtgatcgataccccttgctggaagctgcacacaagccctctgtgcaccaccaacaccaaagagggcagcaacatctgcctgaccagaaccgacagaggctggtactgcgataatgccggcagcgtctcattcttcccacaagccgagacatgcaaggtgcagagcaaccgggtgttctgcgacaccatgaatagcagaaccctgccttccgaagtgaatctgtgcaacgtggacatcttcaaccctaagtacgactgcaagatcatgaccagcaagaccgacgtgtccagcagtgtgatcacctcactgggcgccatcgtgtcctgttacggcaagaccaagtgcaccgccagcaacaagaaccggggcatcatcaagaccttcagcaacggctgcgactacgtgtccaacaaaggcgtggacaccgtgtctgtgggcaacaccctgtactacgtgaacaaacaagagggccagtctctgtacgtgaagtgcgagcccatcatcaacttctacgaccctctggtgttccccagcagcgagttcgatgccagcatcagccaagtgaacgagaagatcaatcagagcctggccttcatcagaaagtccgatgagctgctgcacaacgtgaacgccggcaagtccaccaccaatatcatgatcacgaccatcatcatcgtgattatcgtgatcctgctgtccctgatcgccgtgggcctgctgctttattgataataggctggagcctcggtggccatgcttcttgccccttgggcctccccccagcccctcctccccttcctgcacccgtacccccgtggtctttgaataaagtctgagtgggcggcaaaaaaaaaaaaaaaaaaaaaaaaaaaaaaaaaaaaaaaaaaaaaaaaaaaaaaaaaaaaaaaaaaaaaaaaaaaaaaaaaaaaaaaaaaaaaaaaaaaaaaaaaaaaaa

SEQ ID NO: 27 - DNA, 1539 bp, synthetic construct
  source 1..1539: mol_type = other DNA
atggaactgctgatcctgaaggccaacgccatcaccaccatcctgaccgccgtgaccttctgttttgccagcggccagaacatcaccgaggaattctactgcagcacctgtagcgccgtgtccaagggatatctgggcgcccttagaaccggctggtacaccagcgtgatcctgatcgagctgagcaacatcaaagaaaacaagtgcaacggcaccgacgccaaagtgaagctgatcaagcaagagctggacaagtacaagaatgccgtgaccgacctgcagctgctgatgcagtctacaccagccacaggctctggcagcgccattgcttctggtgtcgccgtgtctaaagtgctgcacctggaaggcgaagtgaacaagatcaagagcgccctgctgagcaccaacaaggccgtggtgtctctgagcaatggcgtgtccgtgctgaccttcaaggtgctggacctgaagaactacatcgacaaacagctgctgcccatcgtcaacaagcagtcctgcagcatccccaacatcgagacagtgatcgagttccagcagaagaacaaccggctgctggaaatcacccgcgagttctctgtgaatgccggcgtgaccacacctgtgtccacctacatgctgaccaacagcgagctgctgagcctgatcaacgacatgcccatcaccaacgaccagaaaaagctgatgagcaacaacgtgcagatcgtgcggcagcagagctacagcatcatgagcattatcaaagaagaggtgctggcctacgtggtgcagctgcctctgtatggcgtgatcgataccccttgctggaagctgcacacaagccctctgtgcaccaccaacaccaaagagggcagcaacatctgcctgaccagaaccgacagaggctggtactgcgataatgccggcagcgtctcattcttcccacaagccgagacatgcaaggtgcagagcaaccgggtgttctgcgacaccatgaatagcagaaccctgccttccgaagtgaatctgtgcaacgtggacatcttcaaccctaagtacgactgcaagatcatgaccagcaagaccgacgtgtccagcagtgtgatcacctcactgggcgccatcgtgtcctgttacggcaagaccaagtgcaccgccagcaacaagaaccggggcatcatcaagaccttcagcaacggctgcgactacgtgtccaacaaaggcgtggacaccgtgtctgtgggcaacaccctgtactacgtgaacaaacaagagggccagtctctgtacgtgaagtgcgagcccatcatcaacttctacgaccctctggtgttccccagcagcgagttcgatgccagcatcagccaagtgaacgagaagatcaatcagagcctggccttcatcagaaagtccgatgagctgctgcacaacgtgaacgccggcaagtccaccaccaatatcatgatcacgaccatcatcatcgtgattatcgtgatcctgctgtccctgatcgccgtgggcctgctgctttattgataatag

SEQ ID NO: 28 - protein, 510 aa, synthetic construct
MELLILKANAITTILTAVTFCFASGQNITEEFYCSTCSAVSKGYLGALRTGWYTSVILIELSNIKENKCNGTDAKVKLIKQELDKYKNAVTDLQLLMQSTPATGSGSAIASGVAVSKVLHLEGEVNKIKSALLSTNKAVVSLSNGVSVLTFKVLDLKNYIDKQLLPIVNKQSCSIPNIETVIEFQQKNNRLLEITREFSVNAGVTTPVSTYMLTNSELLSLINDMPITNDQKKLMSNNVQIVRQQSYSIMSIIKEEVLAYVVQLPLYGVIDTPCWKLHTSPLCTTNTKEGSNICLTRTDRGWYCDNAGSVSFFPQAETCKVQSNRVFCDTMNSRTLPSEVNLCNVDIFNPKYDCKIMTSKTDVSSSVITSLGAIVSCYGKTKCTASNKNRGIIKTFSNGCDYVSNKGVDTVSVGNTLYYVNKQEGQSLYVKCEPIINFYDPLVFPSSEFDASISQVNEKINQSLAFIRKSDELLHNVNAGKSTTNIMITTIIIVIIVILLSLIAVGLLLY

SEQ ID NO: 29 - RNA, 1841 nt, synthetic construct
  source 1..1841: mol_type = other RNA
agcggctcggccattttgtcccagtcagtccggaggctgcggctgcagaagtaccgcctgcggagtaactgcaaaggccaccatggaactgctgatcctgaaggccaacgccatcaccaccatcctgaccgccgtgaccttctgttttgccagcggccagaacatcaccgaggaattctactgcagcacctgtagcgccgtgtccaagggatatctgggcgcccttagaaccggctggtacaccagcgtgatcctgatcgagctgagcaacatcaaagaaaacaagtgcaacggcaccgacgccaaagtgaagctgatcaagcaagagctggacaagtacaagaatgccgtgaccgacctgcagctgctgatgcagtctacaccagccacaggctctggcagcgccattgcttctggtgtcgccgtgtctaaagtgctgcacctggaaggcgaagtgaacaagatcaagagcgccctgctgagcaccaacaaggccgtggtgtctctgagcaatggcgtgtccgtgctgaccttcaaggtgctggacctgaagaactacatcgacaaacagctgctgcccatcgtcaacaagcagtcctgcagcatccccaacatcgagacagtgatcgagttccagcagaagaacaaccggctgctggaaatcacccgcgagttctctgtgaatgccggcgtgaccacacctgtgtccacctacatgctgaccaacagcgagctgctgagcctgatcaacgacatgcccatcaccaacgaccagaaaaagctgatgagcaacaacgtgcagatcgtgcggcagcagagctacagcatcatgagcattatcaaagaagaggtgctggcctacgtggtgcagctgcctctgtatggcgtgatcgataccccttgctggaagctgcacacaagccctctgtgcaccaccaacaccaaagagggcagcaacatctgcctgaccagaaccgacagaggctggtactgcgataatgccggcagcgtctcattcttcccacaagccgagacatgcaaggtgcagagcaaccgggtgttctgcgacaccatgaatagcagaaccctgccttccgaagtgaatctgtgcaacgtggacatcttcaaccctaagtacgactgcaagatcatgaccagcaagaccgacgtgtccagcagtgtgatcacctcactgggcgccatcgtgtcctgttacggcaagaccaagtgcaccgccagcaacaagaaccggggcatcatcaagaccttcagcaacggctgcgactacgtgtccaacaaaggcgtggacaccgtgtctgtgggcaacaccctgtactacgtgaacaaacaagagggccagtctctgtacgtgaagtgcgagcccatcatcaacttctacgaccctctggtgttccccagcagcgagttcgatgccagcatcagccaagtgaacgagaagatcaatcagagcctggccttcatcagaaagtccgatgagctgctgcacaacgtgaacgccggcaagtccaccaccaatatcatgatcacgaccatcatcatcgtgattatcgtgatcctgctgtccctgatcgccgtgggcctgctgctttattgataataggctggagcctcggtggccatgcttcttgccccttgggcctccccccagcccctcctccccttcctgcacccgtacccccgtggtctttgaataaagtctgagtgggcggcaaaaaaaaaaaaaaaaaaaaaaaaaaaaaaaaaaaaaaaaaaaaaaaaaaaaaaaaaaaaaaaaaaaaaaaaaaaaaaaaaaaaaaaaaaaaaaaaaaaaaaaaaaaaaa

SEQ ID NO: 30 - DNA, 1841 bp, synthetic construct
  source 1..1841: mol_type = other DNA
agcggctcggccattttgtcccagtcagtccggaggctgcggctgcagaagtaccgcctgcggagtaactgcaaaggccaccatggaactgctgatcctgaaggccaacgccatcaccaccatcctgaccgccgtgaccttctgttttgccagcggccagaacatcaccgaggaattctaccagagcacctgtagcgccgtgtccaagggatatctgggcgcccttagaaccggctggtacacctgcgtgatcctgatcgagctgagcaacatcaaagaaaacaagtgcaacggcaccgacgccaaagtgaagctgatcaagcaagagctggacaagtacaagaatgccgtgaccgacctgcagctgctgatgcagtctacaccagccacaggctctggcagcgccattgcttctggtgtcgccgtgtctaaagtgctgcacctggaaggcgaagtgaacaagatcaagagcgccctgctgagcaccaacaaggccgtggtgtctctgagcaatggcgtgtccgtgtgcaccttcaaggtgctggacctgaagaactacatcgacaaacagctgctgcccatcgtcaacaagcagtcctgcagcatccccaacatcgagacagtgatcgagttccagcagaagaacaaccggctgctggaaatcacccgcgagttctctgtgaatgccggcgtgaccacacctgtgtccacctacatgctgaccaacagcgagctgctgagcctgatcaacgacatgcccatcaccaacgaccagaaaaagctgatgagcaacaacgtgcagatcgtgcggcagcagagctacagcatcatgagcattatcaaagaagaggtgctggcctacgtggtgcagctgcctctgtatggcgtgatcgataccccttgctggaagctgcacacaagccctctgtgcaccaccaacaccaaagagggcagcaacatctgcctgaccagaaccgacagaggctggtactgcgataatgccggcagcgtctcattcttcccacaagccgagacatgcaaggtgcagagcaaccgggtgttctgcgacaccatgaatagcagaaccctgccttccgaagtgaatctgtgcaacgtggacatcttcaaccctaagtacgactgcaagatcatgaccagcaagaccgacgtgtccagcagtgtgatcacctcactgggcgccatcgtgtcctgttacggcaagaccaagtgcaccgccagcaacaagaaccggggcatcatcaagaccttcagcaacggctgcgactacgtgtccaacaaaggcgtggacaccgtgtctgtgggcaacaccctgtactacgtgaacaaacaagagggccagtctctgtacgtgaagggcgagcccatcatcaacttctacgaccctctggtgttccccagcagcgagttcgatgccagcatcagccaagtgaacgagaagatcaatcagagcctggccttcatcagaaagtccgatgagctgctgcacaacgtgaacgccggcaagtccaccaccaatatcatgatcacgaccatcatcatcgtgattatcgtgatcctgctgtccctgatcgccgtgggcctgctgctttattgataataggctggagcctcggtggccatgcttcttgccccttgggcctccccccagcccctcctccccttcctgcacccgtacccccgtggtctttgaataaagtctgagtgggcggcaaaaaaaaaaaaaaaaaaaaaaaaaaaaaaaaaaaaaaaaaaaaaaaaaaaaaaaaaaaaaaaaaaaaaaaaaaaaaaaaaaaaaaaaaaaaaaaaaaaaaaaaaaaaaa

SEQ ID NO: 31 - DNA, 1539 bp, synthetic construct
  source 1..1539: mol_type = other DNA
atggaactgctgatcctgaaggccaacgccatcaccaccatcctgaccgccgtgaccttctgttttgccagcggccagaacatcaccgaggaattctaccagagcacctgtagcgccgtgtccaagggatatctgggcgcccttagaaccggctggtacacctgcgtgatcctgatcgagctgagcaacatcaaagaaaacaagtgcaacggcaccgacgccaaagtgaagctgatcaagcaagagctggacaagtacaagaatgccgtgaccgacctgcagctgctgatgcagtctacaccagccacaggctctggcagcgccattgcttctggtgtcgccgtgtctaaagtgctgcacctggaaggcgaagtgaacaagatcaagagcgccctgctgagcaccaacaaggccgtggtgtctctgagcaatggcgtgtccgtgtgcaccttcaaggtgctggacctgaagaactacatcgacaaacagctgctgcccatcgtcaacaagcagtcctgcagcatccccaacatcgagacagtgatcgagttccagcagaagaacaaccggctgctggaaatcacccgcgagttctctgtgaatgccggcgtgaccacacctgtgtccacctacatgctgaccaacagcgagctgctgagcctgatcaacgacatgcccatcaccaacgaccagaaaaagctgatgagcaacaacgtgcagatcgtgcggcagcagagctacagcatcatgagcattatcaaagaagaggtgctggcctacgtggtgcagctgcctctgtatggcgtgatcgataccccttgctggaagctgcacacaagccctctgtgcaccaccaacaccaaagagggcagcaacatctgcctgaccagaaccgacagaggctggtactgcgataatgccggcagcgtctcattcttcccacaagccgagacatgcaaggtgcagagcaaccgggtgttctgcgacaccatgaatagcagaaccctgccttccgaagtgaatctgtgcaacgtggacatcttcaaccctaagtacgactgcaagatcatgaccagcaagaccgacgtgtccagcagtgtgatcacctcactgggcgccatcgtgtcctgttacggcaagaccaagtgcaccgccagcaacaagaaccggggcatcatcaagaccttcagcaacggctgcgactacgtgtccaacaaaggcgtggacaccgtgtctgtgggcaacaccctgtactacgtgaacaaacaagagggccagtctctgtacgtgaagggcgagcccatcatcaacttctacgaccctctggtgttccccagcagcgagttcgatgccagcatcagccaagtgaacgagaagatcaatcagagcctggccttcatcagaaagtccgatgagctgctgcacaacgtgaacgccggcaagtccaccaccaatatcatgatcacgaccatcatcatcgtgattatcgtgatcctgctgtccctgatcgccgtgggcctgctgctttattgataatag

SEQ ID NO: 32 - protein, 510 aa, synthetic construct
MELLILKANAITTILTAVTFCFASGQNITEEFYQSTCSAVSKGYLGALRTGWYTCVILIELSNIKENKCNGTDAKVKLIKQELDKYKNAVTDLQLLMQSTPATGSGSAIASGVAVSKVLHLEGEVNKIKSALLSTNKAVVSLSNGVSVCTFKVLDLKNYIDKQLLPIVNKQSCSIPNIETVIEFQQKNNRLLEITREFSVNAGVTTPVSTYMLTNSELLSLINDMPITNDQKKLMSNNVQIVRQQSYSIMSIIKEEVLAYVVQLPLYGVIDTPCWKLHTSPLCTTNTKEGSNICLTRTDRGWYCDNAGSVSFFPQAETCKVQSNRVFCDTMNSRTLPSEVNLCNVDIFNPKYDCKIMTSKTDVSSSVITSLGAIVSCYGKTKCTASNKNRGIIKTFSNGCDYVSNKGVDTVSVGNTLYYVNKQEGQSLYVKGEPIINFYDPLVFPSSEFDASISQVNEKINQSLAFIRKSDELLHNVNAGKSTTNIMITTIIIVIIVILLSLIAVGLLLY

SEQ ID NO: 33 - RNA, 1841 nt, synthetic construct
  source 1..1841: mol_type = other RNA
agcggctcggccattttgtcccagtcagtccggaggctgcggctgcagaagtaccgcctgcggagtaactgcaaaggccaccatggaactgctgatcctgaaggccaacgccatcaccaccatcctgaccgccgtgaccttctgttttgccagcggccagaacatcaccgaggaattctaccagagcacctgtagcgccgtgtccaagggatatctgggcgcccttagaaccggctggtacacctgcgtgatcctgatcgagctgagcaacatcaaagaaaacaagtgcaacggcaccgacgccaaagtgaagctgatcaagcaagagctggacaagtacaagaatgccgtgaccgacctgcagctgctgatgcagtctacaccagccacaggctctggcagcgccattgcttctggtgtcgccgtgtctaaagtgctgcacctggaaggcgaagtgaacaagatcaagagcgccctgctgagcaccaacaaggccgtggtgtctctgagcaatggcgtgtccgtgtgcaccttcaaggtgctggacctgaagaactacatcgacaaacagctgctgcccatcgtcaacaagcagtcctgcagcatccccaacatcgagacagtgatcgagttccagcagaagaacaaccggctgctggaaatcacccgcgagttctctgtgaatgccggcgtgaccacacctgtgtccacctacatgctgaccaacagcgagctgctgagcctgatcaacgacatgcccatcaccaacgaccagaaaaagctgatgagcaacaacgtgcagatcgtgcggcagcagagctacagcatcatgagcattatcaaagaagaggtgctggcctacgtggtgcagctgcctctgtatggcgtgatcgataccccttgctggaagctgcacacaagccctctgtgcaccaccaacaccaaagagggcagcaacatctgcctgaccagaaccgacagaggctggtactgcgataatgccggcagcgtctcattcttcccacaagccgagacatgcaaggtgcagagcaaccgggtgttctgcgacaccatgaatagcagaaccctgccttccgaagtgaatctgtgcaacgtggacatcttcaaccctaagtacgactgcaagatcatgaccagcaagaccgacgtgtccagcagtgtgatcacctcactgggcgccatcgtgtcctgttacggcaagaccaagtgcaccgccagcaacaagaaccggggcatcatcaagaccttcagcaacggctgcgactacgtgtccaacaaaggcgtggacaccgtgtctgtgggcaacaccctgtactacgtgaacaaacaagagggccagtctctgtacgtgaagggcgagcccatcatcaacttctacgaccctctggtgttccccagcagcgagttcgatgccagcatcagccaagtgaacgagaagatcaatcagagcctggccttcatcagaaagtccgatgagctgctgcacaacgtgaacgccggcaagtccaccaccaatatcatgatcacgaccatcatcatcgtgattatcgtgatcctgctgtccctgatcgccgtgggcctgctgctttattgataataggctggagcctcggtggccatgcttcttgccccttgggcctccccccagcccctcctccccttcctgcacccgtacccccgtggtctttgaataaagtctgagtgggcggcaaaaaaaaaaaaaaaaaaaaaaaaaaaaaaaaaaaaaaaaaaaaaaaaaaaaaaaaaaaaaaaaaaaaaaaaaaaaaaaaaaaaaaaaaaaaaaaaaaaaaaaaaaaaaa

SEQ ID NO: 34 - DNA, 1841 bp, synthetic construct
  source 1..1841: mol_type = other DNA
agcggctcggccattttgtcccagtcagtccggaggctgcggctgcagaagtaccgcctgcggagtaactgcaaaggccaccatggaactgctgatcctgaaggccaacgccatcaccaccatcctgaccgccgtgaccttctgttttgccagcggccagaacatcaccgaggaattctactgcagcacctgtagcgccgtgtccaagggatatctgggcgcccttagaaccggctggtacaccagcgtgatcaccatcgagctgagcaacatcaaagaaaacaagtgcaacggcaccgacgccaaagtgaagctgatcaagcaagagctggacaagtacaagaatgccgtgaccgacctgcagctgctgatgcagtctacaccagccacaggctctggcagcgccattgcttctggtgtcgccgtgtctaaagtgctgcacctggaaggcgaagtgaacaagatcaagagcgccctgctgagcaccaacaaggccgtggtgtctctgagcaatggcgtgtccgtgctgaccttcaaggtgctggacctgaagaactacatcgacaaacagctgctgcccatcgtcaacaagcagtcctgcagcatccccaacatcgagatcgtgatcgagttccagcagaagaacaaccggctgctggaaatcacccgcgagttctctgtgaatgccggcgtgaccacacctgtgtccacctacatgctgaccaacagcgagctgctgagcctgatcaacgacatgcccatcaccaacgaccagaaaaagctgatgagcaacaacgtgcagatcgtgcggcagcagagctacagcatcatgagcattatcaaagaagaggtgctggcctacgtggtgcagctgcctctgtatggcgtgatcgataccccttgctggaagctgcacacaagccctctgtgcaccaccaacaccaaagagggcagcaacatctgcctgaccagaaccgacagaggctggtactgcgataatgccggcagcgtctcattcttcccacaagccgagacatgcaaggtgcagagcaaccgggtgttctgcgacaccatgaatagcagaaccctgccttccgaagtgaatctgtgcaacgtggacatcttcaaccctaagtacgactgcaagatcatgaccagcaagaccgacgtgtccagcagtgtgatcacctcactgggcgccatcgtgtcctgttacggcaagaccaagtgcaccgccagcaacaagaaccggggcatcatcaagaccttcagcaacggctgcgactacgtgtccaacaaaggcgtggacaccgtgtctgtgggcaacaccctgtactacgtgaacaaacaagagggccagtctctgtacgtgaagtgcgagcccatcatcaacttctacgaccctctggtgttccccagcagcgagttcgatgccagcatcagccaagtgaacgagaagatcaatcagagcctggccttcatcagaaagtccgatgagctgctgcacaacgtgaacgccggcaagtccaccaccaatatcatgatcacgaccatcatcatcgtgattatcgtgatcctgctgtccctgatcgccgtgggcctgctgctttattgataataggctggagcctcggtggccatgcttcttgccccttgggcctccccccagcccctcctccccttcctgcacccgtacccccgtggtctttgaataaagtctgagtgggcggcaaaaaaaaaaaaaaaaaaaaaaaaaaaaaaaaaaaaaaaaaaaaaaaaaaaaaaaaaaaaaaaaaaaaaaaaaaaaaaaaaaaaaaaaaaaaaaaaaaaaaaaaaaaaaa

SEQ ID NO: 35 - DNA, 1539 bp, synthetic construct
  source 1..1539: mol_type = other DNA
atggaactgctgatcctgaaggccaacgccatcaccaccatcctgaccgccgtgaccttctgttttgccagcggccagaacatcaccgaggaattctactgcagcacctgtagcgccgtgtccaagggatatctgggcgcccttagaaccggctggtacaccagcgtgatcaccatcgagctgagcaacatcaaagaaaacaagtgcaacggcaccgacgccaaagtgaagctgatcaagcaagagctggacaagtacaagaatgccgtgaccgacctgcagctgctgatgcagtctacaccagccacaggctctggcagcgccattgcttctggtgtcgccgtgtctaaagtgctgcacctggaaggcgaagtgaacaagatcaagagcgccctgctgagcaccaacaaggccgtggtgtctctgagcaatggcgtgtccgtgctgaccttcaaggtgctggacctgaagaactacatcgacaaacagctgctgcccatcgtcaacaagcagtcctgcagcatccccaacatcgagatcgtgatcgagttccagcagaagaacaaccggctgctggaaatcacccgcgagttctctgtgaatgccggcgtgaccacacctgtgtccacctacatgctgaccaacagcgagctgctgagcctgatcaacgacatgcccatcaccaacgaccagaaaaagctgatgagcaacaacgtgcagatcgtgcggcagcagagctacagcatcatgagcattatcaaagaagaggtgctggcctacgtggtgcagctgcctctgtatggcgtgatcgataccccttgctggaagctgcacacaagccctctgtgcaccaccaacaccaaagagggcagcaacatctgcctgaccagaaccgacagaggctggtactgcgataatgccggcagcgtctcattcttcccacaagccgagacatgcaaggtgcagagcaaccgggtgttctgcgacaccatgaatagcagaaccctgccttccgaagtgaatctgtgcaacgtggacatcttcaaccctaagtacgactgcaagatcatgaccagcaagaccgacgtgtccagcagtgtgatcacctcactgggcgccatcgtgtcctgttacggcaagaccaagtgcaccgccagcaacaagaaccggggcatcatcaagaccttcagcaacggctgcgactacgtgtccaacaaaggcgtggacaccgtgtctgtgggcaacaccctgtactacgtgaacaaacaagagggccagtctctgtacgtgaagtgcgagcccatcatcaacttctacgaccctctggtgttccccagcagcgagttcgatgccagcatcagccaagtgaacgagaagatcaatcagagcctggccttcatcagaaagtccgatgagctgctgcacaacgtgaacgccggcaagtccaccaccaatatcatgatcacgaccatcatcatcgtgattatcgtgatcctgctgtccctgatcgccgtgggcctgctgctttattgataatag

SEQ ID NO: 36 - protein, 510 aa, synthetic construct
MELLILKANAITTILTAVTFCFASGQNITEEFYCSTCSAVSKGYLGALRTGWYTSVITIELSNIKENKCNGTDAKVKLIKQELDKYKNAVTDLQLLMQSTPATGSGSAIASGVAVSKVLHLEGEVNKIKSALLSTNKAVVSLSNGVSVLTFKVLDLKNYIDKQLLPIVNKQSCSIPNIEIVIEFQQKNNRLLEITREFSVNAGVTTPVSTYMLTNSELLSLINDMPITNDQKKLMSNNVQIVRQQSYSIMSIIKEEVLAYVVQLPLYGVIDTPCWKLHTSPLCTTNTKEGSNICLTRTDRGWYCDNAGSVSFFPQAETCKVQSNRVFCDTMNSRTLPSEVNLCNVDIFNPKYDCKIMTSKTDVSSSVITSLGAIVSCYGKTKCTASNKNRGIIKTFSNGCDYVSNKGVDTVSVGNTLYYVNKQEGQSLYVKCEPIINFYDPLVFPSSEFDASISQVNEKINQSLAFIRKSDELLHNVNAGKSTTNIMITTIIIVIIVILLSLIAVGLLLY

SEQ ID NO: 37 - RNA, 1841 nt, synthetic construct
  source 1..1841: mol_type = other RNA
agcggctcggccattttgtcccagtcagtccggaggctgcggctgcagaagtaccgcctgcggagtaactgcaaaggccaccatggaactgctgatcctgaaggccaacgccatcaccaccatcctgaccgccgtgaccttctgttttgccagcggccagaacatcaccgaggaattctactgcagcacctgtagcgccgtgtccaagggatatctgggcgcccttagaaccggctggtacaccagcgtgatcaccatcgagctgagcaacatcaaagaaaacaagtgcaacggcaccgacgccaaagtgaagctgatcaagcaagagctggacaagtacaagaatgccgtgaccgacctgcagctgctgatgcagtctacaccagccacaggctctggcagcgccattgcttctggtgtcgccgtgtctaaagtgctgcacctggaaggcgaagtgaacaagatcaagagcgccctgctgagcaccaacaaggccgtggtgtctctgagcaatggcgtgtccgtgctgaccttcaaggtgctggacctgaagaactacatcgacaaacagctgctgcccatcgtcaacaagcagtcctgcagcatccccaacatcgagatcgtgatcgagttccagcagaagaacaaccggctgctggaaatcacccgcgagttctctgtgaatgccggcgtgaccacacctgtgtccacctacatgctgaccaacagcgagctgctgagcctgatcaacgacatgcccatcaccaacgaccagaaaaagctgatgagcaacaacgtgcagatcgtgcggcagcagagctacagcatcatgagcattatcaaagaagaggtgctggcctacgtggtgcagctgcctctgtatggcgtgatcgataccccttgctggaagctgcacacaagccctctgtgcaccaccaacaccaaagagggcagcaacatctgcctgaccagaaccgacagaggctggtactgcgataatgccggcagcgtctcattcttcccacaagccgagacatgcaaggtgcagagcaaccgggtgttctgcgacaccatgaatagcagaaccctgccttccgaagtgaatctgtgcaacgtggacatcttcaaccctaagtacgactgcaagatcatgaccagcaagaccgacgtgtccagcagtgtgatcacctcactgggcgccatcgtgtcctgttacggcaagaccaagtgcaccgccagcaacaagaaccggggcatcatcaagaccttcagcaacggctgcgactacgtgtccaacaaaggcgtggacaccgtgtctgtgggcaacaccctgtactacgtgaacaaacaagagggccagtctctgtacgtgaagtgcgagcccatcatcaacttctacgaccctctggtgttccccagcagcgagttcgatgccagcatcagccaagtgaacgagaagatcaatcagagcctggccttcatcagaaagtccgatgagctgctgcacaacgtgaacgccggcaagtccaccaccaatatcatgatcacgaccatcatcatcgtgattatcgtgatcctgctgtccctgatcgccgtgggcctgctgctttattgataataggctggagcctcggtggccatgcttcttgccccttgggcctccccccagcccctcctccccttcctgcacccgtacccccgtggtctttgaataaagtctgagtgggcggcaaaaaaaaaaaaaaaaaaaaaaaaaaaaaaaaaaaaaaaaaaaaaaaaaaaaaaaaaaaaaaaaaaaaaaaaaaaaaaaaaaaaaaaaaaaaaaaaaaaaaaaaaaaaaa

SEQ ID NO: 38 - DNA, 1841 bp, synthetic construct
  source 1..1841: mol_type = other DNA
agcggctcggccattttgtcccagtcagtccggaggctgcggctgcagaagtaccgcctgcggagtaactgcaaaggccaccatggaactgctgatcctgaaggccaacgccatcaccaccatcctgaccgccgtgaccttctgttttgccagcggccagaacatcaccgaggaattctaccagagcacctgtagcgccgtgtccaagggatatctgggcgcccttagaaccggctggtacacctgcgtgatcaccatcgagctgagcaacatcaaagaaaacaagtgcaacggcaccgacgccaaagtgaagctgatcaagcaagagctggacaagtacaagaatgccgtgaccgacctgcagctgctgatgcagtctacaccagccacaggctctggcagcgccattgcttctggtgtcgccgtgtctaaagtgctgcacctggaaggcgaagtgaacaagatcaagagcgccctgctgagcaccaacaaggccgtggtgtctctgagcaatggcgtgtccgtgtgcaccttcaaggtgctggacctgaagaactacatcgacaaacagctgctgcccatcgtcaacaagcagtcctgcagcatccccaacatcgagatcgtgatcgagttccagcagaagaacaaccggctgctggaaatcacccgcgagttctctgtgaatgccggcgtgaccacacctgtgtccacctacatgctgaccaacagcgagctgctgagcctgatcaacgacatgcccatcaccaacgaccagaaaaagctgatgagcaacaacgtgcagatcgtgcggcagcagagctacagcatcatgagcattatcaaagaagaggtgctggcctacgtggtgcagctgcctctgtatggcgtgatcgataccccttgctggaagctgcacacaagccctctgtgcaccaccaacaccaaagagggcagcaacatctgcctgaccagaaccgacagaggctggtactgcgataatgccggcagcgtctcattcttcccacaagccgagacatgcaaggtgcagagcaaccgggtgttctgcgacaccatgaatagcagaaccctgccttccgaagtgaatctgtgcaacgtggacatcttcaaccctaagtacgactgcaagatcatgaccagcaagaccgacgtgtccagcagtgtgatcacctcactgggcgccatcgtgtcctgttacggcaagaccaagtgcaccgccagcaacaagaaccggggcatcatcaagaccttcagcaacggctgcgactacgtgtccaacaaaggcgtggacaccgtgtctgtgggcaacaccctgtactacgtgaacaaacaagagggccagtctctgtacgtgaagggcgagcccatcatcaacttctacgaccctctggtgttccccagcagcgagttcgatgccagcatcagccaagtgaacgagaagatcaatcagagcctggccttcatcagaaagtccgatgagctgctgcacaacgtgaacgccggcaagtccaccaccaatatcatgatcacgaccatcatcatcgtgattatcgtgatcctgctgtccctgatcgccgtgggcctgctgctttattgataataggctggagcctcggtggccatgcttcttgccccttgggcctccccccagcccctcctccccttcctgcacccgtacccccgtggtctttgaataaagtctgagtgggcggcaaaaaaaaaaaaaaaaaaaaaaaaaaaaaaaaaaaaaaaaaaaaaaaaaaaaaaaaaaaaaaaaaaaaaaaaaaaaaaaaaaaaaaaaaaaaaaaaaaaaaaaaaaaaaa

SEQ ID NO: 39 - DNA, 1539 bp, synthetic construct
  source 1..1539: mol_type = other DNA
atggaactgctgatcctgaaggccaacgccatcaccaccatcctgaccgccgtgaccttctgttttgccagcggccagaacatcaccgaggaattctaccagagcacctgtagcgccgtgtccaagggatatctgggcgcccttagaaccggctggtacacctgcgtgatcaccatcgagctgagcaacatcaaagaaaacaagtgcaacggcaccgacgccaaagtgaagctgatcaagcaagagctggacaagtacaagaatgccgtgaccgacctgcagctgctgatgcagtctacaccagccacaggctctggcagcgccattgcttctggtgtcgccgtgtctaaagtgctgcacctggaaggcgaagtgaacaagatcaagagcgccctgctgagcaccaacaaggccgtggtgtctctgagcaatggcgtgtccgtgtgcaccttcaaggtgctggacctgaagaactacatcgacaaacagctgctgcccatcgtcaacaagcagtcctgcagcatccccaacatcgagatcgtgatcgagttccagcagaagaacaaccggctgctggaaatcacccgcgagttctctgtgaatgccggcgtgaccacacctgtgtccacctacatgctgaccaacagcgagctgctgagcctgatcaacgacatgcccatcaccaacgaccagaaaaagctgatgagcaacaacgtgcagatcgtgcggcagcagagctacagcatcatgagcattatcaaagaagaggtgctggcctacgtggtgcagctgcctctgtatggcgtgatcgataccccttgctggaagctgcacacaagccctctgtgcaccaccaacaccaaagagggcagcaacatctgcctgaccagaaccgacagaggctggtactgcgataatgccggcagcgtctcattcttcccacaagccgagacatgcaaggtgcagagcaaccgggtgttctgcgacaccatgaatagcagaaccctgccttccgaagtgaatctgtgcaacgtggacatcttcaaccctaagtacgactgcaagatcatgaccagcaagaccgacgtgtccagcagtgtgatcacctcactgggcgccatcgtgtcctgttacggcaagaccaagtgcaccgccagcaacaagaaccggggcatcatcaagaccttcagcaacggctgcgactacgtgtccaacaaaggcgtggacaccgtgtctgtgggcaacaccctgtactacgtgaacaaacaagagggccagtctctgtacgtgaagggcgagcccatcatcaacttctacgaccctctggtgttccccagcagcgagttcgatgccagcatcagccaagtgaacgagaagatcaatcagagcctggccttcatcagaaagtccgatgagctgctgcacaacgtgaacgccggcaagtccaccaccaatatcatgatcacgaccatcatcatcgtgattatcgtgatcctgctgtccctgatcgccgtgggcctgctgctttattgataatag

SEQ ID NO: 40 - protein, 510 aa, synthetic construct
MELLILKANAITTILTAVTFCFASGQNITEEFYQSTCSAVSKGYLGALRTGWYTCVITIELSNIKENKCNGTDAKVKLIKQELDKYKNAVTDLQLLMQSTPATGSGSAIASGVAVSKVLHLEGEVNKIKSALLSTNKAVVSLSNGVSVCTFKVLDLKNYIDKQLLPIVNKQSCSIPNIEIVIEFQQKNNRLLEITREFSVNAGVTTPVSTYMLTNSELLSLINDMPITNDQKKLMSNNVQIVRQQSYSIMSIIKEEVLAYVVQLPLYGVIDTPCWKLHTSPLCTTNTKEGSNICLTRTDRGWYCDNAGSVSFFPQAETCKVQSNRVFCDTMNSRTLPSEVNLCNVDIFNPKYDCKIMTSKTDVSSSVITSLGAIVSCYGKTKCTASNKNRGIIKTFSNGCDYVSNKGVDTVSVGNTLYYVNKQEGQSLYVKGEPIINFYDPLVFPSSEFDASISQVNEKINQSLAFIRKSDELLHNVNAGKSTTNIMITTIIIVIIVILLSLIAVGLLLY

SEQ ID NO: 41 - RNA, 1841 nt, synthetic construct
  source 1..1841: mol_type = other RNA
agcggctcggccattttgtcccagtcagtccggaggctgcggctgcagaagtaccgcctgcggagtaactgcaaaggccaccatggaactgctgatcctgaaggccaacgccatcaccaccatcctgaccgccgtgaccttctgttttgccagcggccagaacatcaccgaggaattctaccagagcacctgtagcgccgtgtccaagggatatctgggcgcccttagaaccggctggtacacctgcgtgatcaccatcgagctgagcaacatcaaagaaaacaagtgcaacggcaccgacgccaaagtgaagctgatcaagcaagagctggacaagtacaagaatgccgtgaccgacctgcagctgctgatgcagtctacaccagccacaggctctggcagcgccattgcttctggtgtcgccgtgtctaaagtgctgcacctggaaggcgaagtgaacaagatcaagagcgccctgctgagcaccaacaaggccgtggtgtctctgagcaatggcgtgtccgtgtgcaccttcaaggtgctggacctgaagaactacatcgacaaacagctgctgcccatcgtcaacaagcagtcctgcagcatccccaacatcgagatcgtgatcgagttccagcagaagaacaaccggctgctggaaatcacccgcgagttctctgtgaatgccggcgtgaccacacctgtgtccacctacatgctgaccaacagcgagctgctgagcctgatcaacgacatgcccatcaccaacgaccagaaaaagctgatgagcaacaacgtgcagatcgtgcggcagcagagctacagcatcatgagcattatcaaagaagaggtgctggcctacgtggtgcagctgcctctgtatggcgtgatcgataccccttgctggaagctgcacacaagccctctgtgcaccaccaacaccaaagagggcagcaacatctgcctgaccagaaccgacagaggctggtactgcgataatgccggcagcgtctcattcttcccacaagccgagacatgcaaggtgcagagcaaccgggtgttctgcgacaccatgaatagcagaaccctgccttccgaagtgaatctgtgcaacgtggacatcttcaaccctaagtacgactgcaagatcatgaccagcaagaccgacgtgtccagcagtgtgatcacctcactgggcgccatcgtgtcctgttacggcaagaccaagtgcaccgccagcaacaagaaccggggcatcatcaagaccttcagcaacggctgcgactacgtgtccaacaaaggcgtggacaccgtgtctgtgggcaacaccctgtactacgtgaacaaacaagagggccagtctctgtacgtgaagggcgagcccatcatcaacttctacgaccctctggtgttccccagcagcgagttcgatgccagcatcagccaagtgaacgagaagatcaatcagagcctggccttcatcagaaagtccgatgagctgctgcacaacgtgaacgccggcaagtccaccaccaatatcatgatcacgaccatcatcatcgtgattatcgtgatcctgctgtccctgatcgccgtgggcctgctgctttattgataataggctggagcctcggtggccatgcttcttgccccttgggcctccccccagcccctcctccccttcctgcacccgtacccccgtggtctttgaataaagtctgagtgggcggcaaaaaaaaaaaaaaaaaaaaaaaaaaaaaaaaaaaaaaaaaaaaaaaaaaaaaaaaaaaaaaaaaaaaaaaaaaaaaaaaaaaaaaaaaaaaaaaaaaaaaaaaaaaaaa

SEQ ID NO: 42 - DNA, 1841 bp, synthetic construct
  source 1..1841: mol_type = other DNA
agcggctcggccattttgtcccagtcagtccggaggctgcggctgcagaagtaccgcctgcggagtaactgcaaaggccaccatggaactgctgatcctgaaggccaacgccatcaccaccatcctgaccgccgtgaccttctgttttgccagcggccagaacatcaccgaggaattctaccagagcacctgtagcgccgtgtccaagggatatctgggcgcccttagaaccggctggtacaccagcgtgatcaccatcgagctgagcaacatcaaagaaaacaagtgcaacggcaccgacgccaaagtgaagctgatcaagcaagagctggacaagtacaagaatgccgtgaccgacctgcagctgctgatgcagtctacaccagcctgcggctctggcagcgcctgcgcttctggtgtcgccgtgtctaaagtgctgcacctggaaggcgaagtgaacaagatcaagagcgccctgctgagcaccaacaaggccgtggtgtctctgagcaatggcgtgtccgtgctgaccttcaaggtgctggacctgaagaactacatcgacaaacagctgctgcccatcgtcaacaagcagtcctgcagcatccccaacatcgagacagtgatcgagttccagcagaagaacaaccggctgctggaaatcacccgcgagttctctgtgaatgccggcgtgaccacacctgtgtccacctacatgctgaccaacagcgagctgctgagcctgatcaacgacatgcccatcaccaacgaccagaaaaagctgatgagcaacaacgtgcagatcgtgcggcagcagagctacagcatcatgagcattatcaaagaagaggtgctggcctacgtggtgcagctgcctctgtatggcgtgatcgataccccttgctggaagctgcacacaagccctctgtgcaccaccaacaccaaagagggcagcaacatctgcctgaccagaaccgacagaggctggtactgcgataatgccggcagcgtctcattcttcccacaagccgagacatgcaaggtgcagagcaaccgggtgttctgcgacaccatgaatagcagaaccctgccttccgaagtgaatctgtgcaacgtggacatcttcaaccctaagtacgactgcaagatcatgaccagcaagaccgacgtgtccagcagtgtgatcacctcactgggcgccatcgtgtcctgttacggcaagaccaagtgcaccgccagcaacaagaaccggggcatcatcaagaccttcagcaacggctgcgactacgtgtccaacaaaggcgtggacaccgtgtctgtgggcaacaccctgtactgcgtgaacaaacaagagggccagtctctgtacgtgaagggcgagcccatcatcaacttctacgaccctctggtgttccccagcagcgagttcgatgccagcatcagccaagtgaacgagaagatcaatcagagcctggccttcatcagaaagtccgatgagctgctgcacaacgtgaacgccggcaagtccaccaccaatatcatgatcacgaccatcatcatcgtgattatcgtgatcctgctgtccctgatcgccgtgggcctgctgctttattgataataggctggagcctcggtggccatgcttcttgccccttgggcctccccccagcccctcctccccttcctgcacccgtacccccgtggtctttgaataaagtctgagtgggcggcaaaaaaaaaaaaaaaaaaaaaaaaaaaaaaaaaaaaaaaaaaaaaaaaaaaaaaaaaaaaaaaaaaaaaaaaaaaaaaaaaaaaaaaaaaaaaaaaaaaaaaaaaaaaaa

SEQ ID NO: 43 - DNA, 1539 bp, synthetic construct
  source 1..1539: mol_type = other DNA
atggaactgctgatcctgaaggccaacgccatcaccaccatcctgaccgccgtgaccttctgttttgccagcggccagaacatcaccgaggaattctaccagagcacctgtagcgccgtgtccaagggatatctgggcgcccttagaaccggctggtacaccagcgtgatcaccatcgagctgagcaacatcaaagaaaacaagtgcaacggcaccgacgccaaagtgaagctgatcaagcaagagctggacaagtacaagaatgccgtgaccgacctgcagctgctgatgcagtctacaccagcctgcggctctggcagcgcctgcgcttctggtgtcgccgtgtctaaagtgctgcacctggaaggcgaagtgaacaagatcaagagcgccctgctgagcaccaacaaggccgtggtgtctctgagcaatggcgtgtccgtgctgaccttcaaggtgctggacctgaagaactacatcgacaaacagctgctgcccatcgtcaacaagcagtcctgcagcatccccaacatcgagacagtgatcgagttccagcagaagaacaaccggctgctggaaatcacccgcgagttctctgtgaatgccggcgtgaccacacctgtgtccacctacatgctgaccaacagcgagctgctgagcctgatcaacgacatgcccatcaccaacgaccagaaaaagctgatgagcaacaacgtgcagatcgtgcggcagcagagctacagcatcatgagcattatcaaagaagaggtgctggcctacgtggtgcagctgcctctgtatggcgtgatcgataccccttgctggaagctgcacacaagccctctgtgcaccaccaacaccaaagagggcagcaacatctgcctgaccagaaccgacagaggctggtactgcgataatgccggcagcgtctcattcttcccacaagccgagacatgcaaggtgcagagcaaccgggtgttctgcgacaccatgaatagcagaaccctgccttccgaagtgaatctgtgcaacgtggacatcttcaaccctaagtacgactgcaagatcatgaccagcaagaccgacgtgtccagcagtgtgatcacctcactgggcgccatcgtgtcctgttacggcaagaccaagtgcaccgccagcaacaagaaccggggcatcatcaagaccttcagcaacggctgcgactacgtgtccaacaaaggcgtggacaccgtgtctgtgggcaacaccctgtactgcgtgaacaaacaagagggccagtctctgtacgtgaagggcgagcccatcatcaacttctacgaccctctggtgttccccagcagcgagttcgatgccagcatcagccaagtgaacgagaagatcaatcagagcctggccttcatcagaaagtccgatgagctgctgcacaacgtgaacgccggcaagtccaccaccaatatcatgatcacgaccatcatcatcgtgattatcgtgatcctgctgtccctgatcgccgtgggcctgctgctttattgataatag

SEQ ID NO: 44 - protein, 510 aa, synthetic construct
MELLILKANAITTILTAVTFCFASGQNITEEFYQSTCSAVSKGYLGALRTGWYTSVITIELSNIKENKCNGTDAKVKLIKQELDKYKNAVTDLQLLMQSTPACGSGSACASGVAVSKVLHLEGEVNKIKSALLSTNKAVVSLSNGVSVLTFKVLDLKNYIDKQLLPIVNKQSCSIPNIETVIEFQQKNNRLLEITREFSVNAGVTTPVSTYMLTNSELLSLINDMPITNDQKKLMSNNVQIVRQQSYSIMSIIKEEVLAYVVQLPLYGVIDTPCWKLHTSPLCTTNTKEGSNICLTRTDRGWYCDNAGSVSFFPQAETCKVQSNRVFCDTMNSRTLPSEVNLCNVDIFNPKYDCKIMTSKTDVSSSVITSLGAIVSCYGKTKCTASNKNRGIIKTFSNGCDYVSNKGVDTVSVGNTLYCVNKQEGQSLYVKGEPIINFYDPLVFPSSEFDASISQVNEKINQSLAFIRKSDELLHNVNAGKSTTNIMITTIIIVIIVILLSLIAVGLLLY

SEQ ID NO: 45 - RNA, 1841 nt, synthetic construct
  source 1..1841: mol_type = other RNA
agcggctcggccattttgtcccagtcagtccggaggctgcggctgcagaagtaccgcctgcggagtaactgcaaaggccaccatggaactgctgatcctgaaggccaacgccatcaccaccatcctgaccgccgtgaccttctgttttgccagcggccagaacatcaccgaggaattctaccagagcacctgtagcgccgtgtccaagggatatctgggcgcccttagaaccggctggtacaccagcgtgatcaccatcgagctgagcaacatcaaagaaaacaagtgcaacggcaccgacgccaaagtgaagctgatcaagcaagagctggacaagtacaagaatgccgtgaccgacctgcagctgctgatgcagtctacaccagcctgcggctctggcagcgcctgcgcttctggtgtcgccgtgtctaaagtgctgcacctggaaggcgaagtgaacaagatcaagagcgccctgctgagcaccaacaaggccgtggtgtctctgagcaatggcgtgtccgtgctgaccttcaaggtgctggacctgaagaactacatcgacaaacagctgctgcccatcgtcaacaagcagtcctgcagcatccccaacatcgagacagtgatcgagttccagcagaagaacaaccggctgctggaaatcacccgcgagttctctgtgaatgccggcgtgaccacacctgtgtccacctacatgctgaccaacagcgagctgctgagcctgatcaacgacatgcccatcaccaacgaccagaaaaagctgatgagcaacaacgtgcagatcgtgcggcagcagagctacagcatcatgagcattatcaaagaagaggtgctggcctacgtggtgcagctgcctctgtatggcgtgatcgataccccttgctggaagctgcacacaagccctctgtgcaccaccaacaccaaagagggcagcaacatctgcctgaccagaaccgacagaggctggtactgcgataatgccggcagcgtctcattcttcccacaagccgagacatgcaaggtgcagagcaaccgggtgttctgcgacaccatgaatagcagaaccctgccttccgaagtgaatctgtgcaacgtggacatcttcaaccctaagtacgactgcaagatcatgaccagcaagaccgacgtgtccagcagtgtgatcacctcactgggcgccatcgtgtcctgttacggcaagaccaagtgcaccgccagcaacaagaaccggggcatcatcaagaccttcagcaacggctgcgactacgtgtccaacaaaggcgtggacaccgtgtctgtgggcaacaccctgtactgcgtgaacaaacaagagggccagtctctgtacgtgaagggcgagcccatcatcaacttctacgaccctctggtgttccccagcagcgagttcgatgccagcatcagccaagtgaacgagaagatcaatcagagcctggccttcatcagaaagtccgatgagctgctgcacaacgtgaacgccggcaagtccaccaccaatatcatgatcacgaccatcatcatcgtgattatcgtgatcctgctgtccctgatcgccgtgggcctgctgctttattgataataggctggagcctcggtggccatgcttcttgccccttgggcctccccccagcccctcctccccttcctgcacccgtacccccgtggtctttgaataaagtctgagtgggcggcaaaaaaaaaaaaaaaaaaaaaaaaaaaaaaaaaaaaaaaaaaaaaaaaaaaaaaaaaaaaaaaaaaaaaaaaaaaaaaaaaaaaaaaaaaaaaaaaaaaaaaaaaaaaaa

SEQ ID NO: 46 - DNA, 1841 bp, synthetic construct
  source 1..1841: mol_type = other DNA
agcggctcggccattttgtcccagtcagtccggaggctgcggctgcagaagtaccgcctgcggagtaactgcaaaggccaccatggaactgctgatcctgaaggccaacgccatcaccaccatcctgaccgccgtgaccttctgttttgccagcggccagaacatcaccgaggaattctactgcagcacctgtagcgccgtgtccaagggatatctgggcgcccttagaaccggctggtacaccagcgtgatcaccatcgagctgagcaacatcaaagaaaacaagtgcaacggcaccgacgccaaagtgaagctgatcaagcaagagctggacaagtacaagaatgccgtgaccgacctgcagctgctgatgcagtctacaccagccacaggctctggcagcgccatttgttctggtgtcgccgtgtctaaagtgctgcacctggaaggcgaagtgaacaagatcaagagcgccctgctgagcaccaacaaggccgtggtgtctctgagcaatggcgtgtccgtgctgaccatcaaggtgctggacctgaagaactacatcgacaaacagctgctgcccatcgtcaacaagcagtcctgcagcatccccaacatcgagacagtgatcgagttccagcagaagaacaaccggctgctggaaatcacccgcgagttctctgtgaatgccggcgtgaccacacctgtgtccacctacatgctgaccaacagcgagctgctgagcctgatcaacgacatgcccatcaccaacgaccagaaaaagctgatgagcaacaacgtgcagatcgtgcggcagcagagctacagcatcatgagcattatcaaagaagaggtgctggcctacgtggtgcagctgcctctgtatggcgtgatcgataccccttgctggaagctgcacacaagccctctgtgcaccaccaacaccaaagagggcagcaacatctgcctgaccagaaccgacagaggctggtactgcgataatgccggcagcgtctcattcttcccacaagccgagacatgcaaggtgcagagcaaccgggtgttctgcgacaccatgaatagcagaaccctgccttccgaagtgaatctgtgcaacgtggacatcttcaaccctaagtacgactgcaagatcatgaccagcaagaccgacgtgtccagcagtgtgatcacctcactgggcgccatcgtgtcctgttacggcaagaccaagtgcaccgccagcaacaagaaccggggcatcatcaagaccttcagcaacggctgcgactacgtgtccaacaaaggcgtggacaccgtgtctgtgggcaacaccctgtactgcgtgaacaaacaagagggccagtctctgtacgtgaagtgcgagcccatcatcaacttctacgaccctctggtgttccccagcagcgagttcgatgccagcatcagccaagtgaacgagaagatcaatcagagcctggccttcatcagaaagtccgatgagctgctgcacaacgtgaacgccggcaagtccaccaccaatatcatgatcacgaccatcatcatcgtgattatcgtgatcctgctgtccctgatcgccgtgggcctgctgctttattgataataggctggagcctcggtggccatgcttcttgccccttgggcctccccccagcccctcctccccttcctgcacccgtacccccgtggtctttgaataaagtctgagtgggcggcaaaaaaaaaaaaaaaaaaaaaaaaaaaaaaaaaaaaaaaaaaaaaaaaaaaaaaaaaaaaaaaaaaaaaaaaaaaaaaaaaaaaaaaaaaaaaaaaaaaaaaaaaaaaaa

SEQ ID NO: 47 - DNA, 1539 bp, synthetic construct
  source 1..1539: mol_type = other DNA
atggaactgctgatcctgaaggccaacgccatcaccaccatcctgaccgccgtgaccttctgttttgccagcggccagaacatcaccgaggaattctactgcagcacctgtagcgccgtgtccaagggatatctgggcgcccttagaaccggctggtacaccagcgtgatcaccatcgagctgagcaacatcaaagaaaacaagtgcaacggcaccgacgccaaagtgaagctgatcaagcaagagctggacaagtacaagaatgccgtgaccgacctgcagctgctgatgcagtctacaccagccacaggctctggcagcgccatttgttctggtgtcgccgtgtctaaagtgctgcacctggaaggcgaagtgaacaagatcaagagcgccctgctgagcaccaacaaggccgtggtgtctctgagcaatggcgtgtccgtgctgaccatcaaggtgctggacctgaagaactacatcgacaaacagctgctgcccatcgtcaacaagcagtcctgcagcatccccaacatcgagacagtgatcgagttccagcagaagaacaaccggctgctggaaatcacccgcgagttctctgtgaatgccggcgtgaccacacctgtgtccacctacatgctgaccaacagcgagctgctgagcctgatcaacgacatgcccatcaccaacgaccagaaaaagctgatgagcaacaacgtgcagatcgtgcggcagcagagctacagcatcatgagcattatcaaagaagaggtgctggcctacgtggtgcagctgcctctgtatggcgtgatcgataccccttgctggaagctgcacacaagccctctgtgcaccaccaacaccaaagagggcagcaacatctgcctgaccagaaccgacagaggctggtactgcgataatgccggcagcgtctcattcttcccacaagccgagacatgcaaggtgcagagcaaccgggtgttctgcgacaccatgaatagcagaaccctgccttccgaagtgaatctgtgcaacgtggacatcttcaaccctaagtacgactgcaagatcatgaccagcaagaccgacgtgtccagcagtgtgatcacctcactgggcgccatcgtgtcctgttacggcaagaccaagtgcaccgccagcaacaagaaccggggcatcatcaagaccttcagcaacggctgcgactacgtgtccaacaaaggcgtggacaccgtgtctgtgggcaacaccctgtactgcgtgaacaaacaagagggccagtctctgtacgtgaagtgcgagcccatcatcaacttctacgaccctctggtgttccccagcagcgagttcgatgccagcatcagccaagtgaacgagaagatcaatcagagcctggccttcatcagaaagtccgatgagctgctgcacaacgtgaacgccggcaagtccaccaccaatatcatgatcacgaccatcatcatcgtgattatcgtgatcctgctgtccctgatcgccgtgggcctgctgctttattgataatag

SEQ ID NO: 48 - protein, 510 aa, synthetic construct
MELLILKANAITTILTAVTFCFASGQNITEEFYCSTCSAVSKGYLGALRTGWYTSVITIELSNIKENKCNGTDAKVKLIKQELDKYKNAVTDLQLLMQSTPATGSGSAICSGVAVSKVLHLEGEVNKIKSALLSTNKAVVSLSNGVSVLTIKVLDLKNYIDKQLLPIVNKQSCSIPNIETVIEFQQKNNRLLEITREFSVNAGVTTPVSTYMLTNSELLSLINDMPITNDQKKLMSNNVQIVRQQSYSIMSIIKEEVLAYVVQLPLYGVIDTPCWKLHTSPLCTTNTKEGSNICLTRTDRGWYCDNAGSVSFFPQAETCKVQSNRVFCDTMNSRTLPSEVNLCNVDIFNPKYDCKIMTSKTDVSSSVITSLGAIVSCYGKTKCTASNKNRGIIKTFSNGCDYVSNKGVDTVSVGNTLYCVNKQEGQSLYVKCEPIINFYDPLVFPSSEFDASISQVNEKINQSLAFIRKSDELLHNVNAGKSTTNIMITTIIIVIIVILLSLIAVGLLLY

SEQ ID NO: 49 - RNA, 1841 nt, synthetic construct
  source 1..1841: mol_type = other RNA
agcggctcggccattttgtcccagtcagtccggaggctgcggctgcagaagtaccgcctgcggagtaactgcaaaggccaccatggaactgctgatcctgaaggccaacgccatcaccaccatcctgaccgccgtgaccttctgttttgccagcggccagaacatcaccgaggaattctactgcagcacctgtagcgccgtgtccaagggatatctgggcgcccttagaaccggctggtacaccagcgtgatcaccatcgagctgagcaacatcaaagaaaacaagtgcaacggcaccgacgccaaagtgaagctgatcaagcaagagctggacaagtacaagaatgccgtgaccgacctgcagctgctgatgcagtctacaccagccacaggctctggcagcgccatttgttctggtgtcgccgtgtctaaagtgctgcacctggaaggcgaagtgaacaagatcaagagcgccctgctgagcaccaacaaggccgtggtgtctctgagcaatggcgtgtccgtgctgaccatcaaggtgctggacctgaagaactacatcgacaaacagctgctgcccatcgtcaacaagcagtcctgcagcatccccaacatcgagacagtgatcgagttccagcagaagaacaaccggctgctggaaatcacccgcgagttctctgtgaatgccggcgtgaccacacctgtgtccacctacatgctgaccaacagcgagctgctgagcctgatcaacgacatgcccatcaccaacgaccagaaaaagctgatgagcaacaacgtgcagatcgtgcggcagcagagctacagcatcatgagcattatcaaagaagaggtgctggcctacgtggtgcagctgcctctgtatggcgtgatcgataccccttgctggaagctgcacacaagccctctgtgcaccaccaacaccaaagagggcagcaacatctgcctgaccagaaccgacagaggctggtactgcgataatgccggcagcgtctcattcttcccacaagccgagacatgcaaggtgcagagcaaccgggtgttctgcgacaccatgaatagcagaaccctgccttccgaagtgaatctgtgcaacgtggacatcttcaaccctaagtacgactgcaagatcatgaccagcaagaccgacgtgtccagcagtgtgatcacctcactgggcgccatcgtgtcctgttacggcaagaccaagtgcaccgccagcaacaagaaccggggcatcatcaagaccttcagcaacggctgcgactacgtgtccaacaaaggcgtggacaccgtgtctgtgggcaacaccctgtactgcgtgaacaaacaagagggccagtctctgtacgtgaagtgcgagcccatcatcaacttctacgaccctctggtgttccccagcagcgagttcgatgccagcatcagccaagtgaacgagaagatcaatcagagcctggccttcatcagaaagtccgatgagctgctgcacaacgtgaacgccggcaagtccaccaccaatatcatgatcacgaccatcatcatcgtgattatcgtgatcctgctgtccctgatcgccgtgggcctgctgctttattgataataggctggagcctcggtggccatgcttcttgccccttgggcctccccccagcccctcctccccttcctgcacccgtacccccgtggtctttgaataaagtctgagtgggcggcaaaaaaaaaaaaaaaaaaaaaaaaaaaaaaaaaaaaaaaaaaaaaaaaaaaaaaaaaaaaaaaaaaaaaaaaaaaaaaaaaaaaaaaaaaaaaaaaaaaaaaaaaaaaaa

SEQ ID NO: 50 - DNA, 1841 bp, synthetic construct
  source 1..1841: mol_type = other DNA
agcggctcggccattttgtcccagtcagtccggaggctgcggctgcagaagtaccgcctgcggagtaactgcaaaggccaccatggaactgctgatcctgaaggccaacgccatcaccaccatcctgaccgccgtgaccttctgttttgccagcggccagaacatcaccgaggaattctaccagagcacctgtagcgccgtgtccaagggatatctgggcgcccttagaaccggctggtacacctgcgtgatcaccatcgagctgagcaacatcaaagaaaacaagtgcaacggcaccgacgccaaagtgaagctgatcaagcaagagctggacaagtacaagaatgccgtgaccgacctgcagctgctgatgcagtctacaccagccacaggctctggcagcgccatttgttctggtgtcgccgtgtctaaagtgctgcacctggaaggcgaagtgaacaagatcaagagcgccctgctgagcaccaacaaggccgtggtgtctctgagcaatggcgtgtccgtgtgcaccatcaaggtgctggacctgaagaactacatcgacaaacagctgctgcccatcgtcaacaagcagtcctgcagcatccccaacatcgagacagtgatcgagttccagcagaagaacaaccggctgctggaaatcacccgcgagttctctgtgaatgccggcgtgaccacacctgtgtccacctacatgctgaccaacagcgagctgctgagcctgatcaacgacatgcccatcaccaacgaccagaaaaagctgatgagcaacaacgtgcagatcgtgcggcagcagagctacagcatcatgagcattatcaaagaagaggtgctggcctacgtggtgcagctgcctctgtatggcgtgatcgataccccttgctggaagctgcacacaagccctctgtgcaccaccaacaccaaagagggcagcaacatctgcctgaccagaaccgacagaggctggtactgcgataatgccggcagcgtctcattcttcccacaagccgagacatgcaaggtgcagagcaaccgggtgttctgcgacaccatgaatagcagaaccctgccttccgaagtgaatctgtgcaacgtggacatcttcaaccctaagtacgactgcaagatcatgaccagcaagaccgacgtgtccagcagtgtgatcacctcactgggcgccatcgtgtcctgttacggcaagaccaagtgcaccgccagcaacaagaaccggggcatcatcaagaccttcagcaacggctgcgactacgtgtccaacaaaggcgtggacaccgtgtctgtgggcaacaccctgtactgcgtgaacaaacaagagggccagtctctgtacgtgaagggcgagcccatcatcaacttctacgaccctctggtgttccccagcagcgagttcgatgccagcatcagccaagtgaacgagaagatcaatcagagcctggccttcatcagaaagtccgatgagctgctgcacaacgtgaacgccggcaagtccaccaccaatatcatgatcacgaccatcatcatcgtgattatcgtgatcctgctgtccctgatcgccgtgggcctgctgctttattgataataggctggagcctcggtggccatgcttcttgccccttgggcctccccccagcccctcctccccttcctgcacccgtacccccgtggtctttgaataaagtctgagtgggcggcaaaaaaaaaaaaaaaaaaaaaaaaaaaaaaaaaaaaaaaaaaaaaaaaaaaaaaaaaaaaaaaaaaaaaaaaaaaaaaaaaaaaaaaaaaaaaaaaaaaaaaaaaaaaaa

SEQ ID NO: 51 - DNA, 1539 bp, synthetic construct
  source 1..1539: mol_type = other DNA
atggaactgctgatcctgaaggccaacgccatcaccaccatcctgaccgccgtgaccttctgttttgccagcggccagaacatcaccgaggaattctaccagagcacctgtagcgccgtgtccaagggatatctgggcgcccttagaaccggctggtacacctgcgtgatcaccatcgagctgagcaacatcaaagaaaacaagtgcaacggcaccgacgccaaagtgaagctgatcaagcaagagctggacaagtacaagaatgccgtgaccgacctgcagctgctgatgcagtctacaccagccacaggctctggcagcgccatttgttctggtgtcgccgtgtctaaagtgctgcacctggaaggcgaagtgaacaagatcaagagcgccctgctgagcaccaacaaggccgtggtgtctctgagcaatggcgtgtccgtgtgcaccatcaaggtgctggacctgaagaactacatcgacaaacagctgctgcccatcgtcaacaagcagtcctgcagcatccccaacatcgagacagtgatcgagttccagcagaagaacaaccggctgctggaaatcacccgcgagttctctgtgaatgccggcgtgaccacacctgtgtccacctacatgctgaccaacagcgagctgctgagcctgatcaacgacatgcccatcaccaacgaccagaaaaagctgatgagcaacaacgtgcagatcgtgcggcagcagagctacagcatcatgagcattatcaaagaagaggtgctggcctacgtggtgcagctgcctctgtatggcgtgatcgataccccttgctggaagctgcacacaagccctctgtgcaccaccaacaccaaagagggcagcaacatctgcctgaccagaaccgacagaggctggtactgcgataatgccggcagcgtctcattcttcccacaagccgagacatgcaaggtgcagagcaaccgggtgttctgcgacaccatgaatagcagaaccctgccttccgaagtgaatctgtgcaacgtggacatcttcaaccctaagtacgactgcaagatcatgaccagcaagaccgacgtgtccagcagtgtgatcacctcactgggcgccatcgtgtcctgttacggcaagaccaagtgcaccgccagcaacaagaaccggggcatcatcaagaccttcagcaacggctgcgactacgtgtccaacaaaggcgtggacaccgtgtctgtgggcaacaccctgtactgcgtgaacaaacaagagggccagtctctgtacgtgaagggcgagcccatcatcaacttctacgaccctctggtgttccccagcagcgagttcgatgccagcatcagccaagtgaacgagaagatcaatcagagcctggccttcatcagaaagtccgatgagctgctgcacaacgtgaacgccggcaagtccaccaccaatatcatgatcacgaccatcatcatcgtgattatcgtgatcctgctgtccctgatcgccgtgggcctgctgctttattgataatag

SEQ ID NO: 52 - protein, 510 aa, synthetic construct
MELLILKANAITTILTAVTFCFASGQNITEEFYQSTCSAVSKGYLGALRTGWYTCVITIELSNIKENKCNGTDAKVKLIKQELDKYKNAVTDLQLLMQSTPATGSGSAICSGVAVSKVLHLEGEVNKIKSALLSTNKAVVSLSNGVSVCTIKVLDLKNYIDKQLLPIVNKQSCSIPNIETVIEFQQKNNRLLEITREFSVNAGVTTPVSTYMLTNSELLSLINDMPITNDQKKLMSNNVQIVRQQSYSIMSIIKEEVLAYVVQLPLYGVIDTPCWKLHTSPLCTTNTKEGSNICLTRTDRGWYCDNAGSVSFFPQAETCKVQSNRVFCDTMNSRTLPSEVNLCNVDIFNPKYDCKIMTSKTDVSSSVITSLGAIVSCYGKTKCTASNKNRGIIKTFSNGCDYVSNKGVDTVSVGNTLYCVNKQEGQSLYVKGEPIINFYDPLVFPSSEFDASISQVNEKINQSLAFIRKSDELLHNVNAGKSTTNIMITTIIIVIIVILLSLIAVGLLLY

SEQ ID NO: 53 - RNA, 1841 nt, synthetic construct
  source 1..1841: mol_type = other RNA
agcggctcggccattttgtcccagtcagtccggaggctgcggctgcagaagtaccgcctgcggagtaactgcaaaggccaccatggaactgctgatcctgaaggccaacgccatcaccaccatcctgaccgccgtgaccttctgttttgccagcggccagaacatcaccgaggaattctaccagagcacctgtagcgccgtgtccaagggatatctgggcgcccttagaaccggctggtacacctgcgtgatcaccatcgagctgagcaacatcaaagaaaacaagtgcaacggcaccgacgccaaagtgaagctgatcaagcaagagctggacaagtacaagaatgccgtgaccgacctgcagctgctgatgcagtctacaccagccacaggctctggcagcgccatttgttctggtgtcgccgtgtctaaagtgctgcacctggaaggcgaagtgaacaagatcaagagcgccctgctgagcaccaacaaggccgtggtgtctctgagcaatggcgtgtccgtgtgcaccatcaaggtgctggacctgaagaactacatcgacaaacagctgctgcccatcgtcaacaagcagtcctgcagcatccccaacatcgagacagtgatcgagttccagcagaagaacaaccggctgctggaaatcacccgcgagttctctgtgaatgccggcgtgaccacacctgtgtccacctacatgctgaccaacagcgagctgctgagcctgatcaacgacatgcccatcaccaacgaccagaaaaagctgatgagcaacaacgtgcagatcgtgcggcagcagagctacagcatcatgagcattatcaaagaagaggtgctggcctacgtggtgcagctgcctctgtatggcgtgatcgataccccttgctggaagctgcacacaagccctctgtgcaccaccaacaccaaagagggcagcaacatctgcctgaccagaaccgacagaggctggtactgcgataatgccggcagcgtctcattcttcccacaagccgagacatgcaaggtgcagagcaaccgggtgttctgcgacaccatgaatagcagaaccctgccttccgaagtgaatctgtgcaacgtggacatcttcaaccctaagtacgactgcaagatcatgaccagcaagaccgacgtgtccagcagtgtgatcacctcactgggcgccatcgtgtcctgttacggcaagaccaagtgcaccgccagcaacaagaaccggggcatcatcaagaccttcagcaacggctgcgactacgtgtccaacaaaggcgtggacaccgtgtctgtgggcaacaccctgtactgcgtgaacaaacaagagggccagtctctgtacgtgaagggcgagcccatcatcaacttctacgaccctctggtgttccccagcagcgagttcgatgccagcatcagccaagtgaacgagaagatcaatcagagcctggccttcatcagaaagtccgatgagctgctgcacaacgtgaacgccggcaagtccaccaccaatatcatgatcacgaccatcatcatcgtgattatcgtgatcctgctgtccctgatcgccgtgggcctgctgctttattgataataggctggagcctcggtggccatgcttcttgccccttgggcctccccccagcccctcctccccttcctgcacccgtacccccgtggtctttgaataaagtctgagtgggcggcaaaaaaaaaaaaaaaaaaaaaaaaaaaaaaaaaaaaaaaaaaaaaaaaaaaaaaaaaaaaaaaaaaaaaaaaaaaaaaaaaaaaaaaaaaaaaaaaaaaaaaaaaaaaaa

SEQ ID NO: 54 - DNA, 1841 bp, synthetic construct
  source 1..1841: mol_type = other DNA
agcggctcggccattttgtcccagtcagtccggaggctgcggctgcagaagtaccgcctgcggagtaactgcaaaggccaccatggaactgctgatcctgaaggccaacgccatcaccaccatcctgaccgccgtgaccttctgttttgccagcggccagaacatcaccgaggaattctactgcagcacctgtagcgccgtgtccaagggatatctgggcgcccttagaaccggctggtacaccagcgtgatcctgatcgagctgagcaacatcaaagaaaacaagtgcaacggcaccgacgccaaagtgaagctgatcaagcaagagctggacaagtacaagaatgccgtgaccgacctgcagctgctgatgcagtctacaccagccacaggctctggcagcgccatttgttctggtgtcgccgtgtctaaagtgctgcacctggaaggcgaagtgaacaagatcaagagcgccctgctgagcaccaacaaggccgtggtgtctctgagcaatggcgtgtccgtgctgaccttcaaggtgctggacctgaagaactacatcgacaaacagctgctgcccatcgtcaacaagcagtcctgcagcatccccaacatcgagacagtgatcgagttccagcagaagaacaaccggctgctggaaatcacccgcgagttctctgtgaatgccggcgtgaccacacctgtgtccacctacatgctgaccaacagcgagctgctgagcctgatcaacgacatgcccatcaccaacgaccagaaaaagctgatgagcaacaacgtgcagatcgtgcggcagcagagctacagcatcatgagcattatcaaagaagaggtgctggcctacgtggtgcagctgcctctgtatggcgtgatcgataccccttgctggaagctgcacacaagccctctgtgcaccaccaacaccaaagagggcagcaacatctgcctgaccagaaccgacagaggctggtactgcgataatgccggcagcgtctcattcttcccacaagccgagacatgcaaggtgcagagcaaccgggtgttctgcgacaccatgaatagcagaaccctgccttccgaagtgaatctgtgcaacgtggacatcttcaaccctaagtacgactgcaagatcatgaccagcaagaccgacgtgtccagcagtgtgatcacctcactgggcgccatcgtgtcctgttacggcaagaccaagtgcaccgccagcaacaagaaccggggcatcatcaagaccttcagcaacggctgcgactacgtgtccaacaaaggcgtggacaccgtgtctgtgggcaacaccctgtactgcgtgaacaaacaagagggccagtctctgtacgtgaagtgcgagcccatcatcaacttctacgaccctctggtgttccccagcagcgagttcgatgccagcatcagccaagtgaacgagaagatcaatcagagcctggccttcatcagaaagtccgatgagctgctgcacaacgtgaacgccggcaagtccaccaccaatatcatgatcacgaccatcatcatcgtgattatcgtgatcctgctgtccctgatcgccgtgggcctgctgctttattgataataggctggagcctcggtggccatgcttcttgccccttgggcctccccccagcccctcctccccttcctgcacccgtacccccgtggtctttgaataaagtctgagtgggcggcaaaaaaaaaaaaaaaaaaaaaaaaaaaaaaaaaaaaaaaaaaaaaaaaaaaaaaaaaaaaaaaaaaaaaaaaaaaaaaaaaaaaaaaaaaaaaaaaaaaaaaaaaaaaaa

SEQ ID NO: 55 - DNA, 1539 bp, synthetic construct
  source 1..1539: mol_type = other DNA
atggaactgctgatcctgaaggccaacgccatcaccaccatcctgaccgccgtgaccttctgttttgccagcggccagaacatcaccgaggaattctactgcagcacctgtagcgccgtgtccaagggatatctgggcgcccttagaaccggctggtacaccagcgtgatcctgatcgagctgagcaacatcaaagaaaacaagtgcaacggcaccgacgccaaagtgaagctgatcaagcaagagctggacaagtacaagaatgccgtgaccgacctgcagctgctgatgcagtctacaccagccacaggctctggcagcgccatttgttctggtgtcgccgtgtctaaagtgctgcacctggaaggcgaagtgaacaagatcaagagcgccctgctgagcaccaacaaggccgtggtgtctctgagcaatggcgtgtccgtgctgaccttcaaggtgctggacctgaagaactacatcgacaaacagctgctgcccatcgtcaacaagcagtcctgcagcatccccaacatcgagacagtgatcgagttccagcagaagaacaaccggctgctggaaatcacccgcgagttctctgtgaatgccggcgtgaccacacctgtgtccacctacatgctgaccaacagcgagctgctgagcctgatcaacgacatgcccatcaccaacgaccagaaaaagctgatgagcaacaacgtgcagatcgtgcggcagcagagctacagcatcatgagcattatcaaagaagaggtgctggcctacgtggtgcagctgcctctgtatggcgtgatcgataccccttgctggaagctgcacacaagccctctgtgcaccaccaacaccaaagagggcagcaacatctgcctgaccagaaccgacagaggctggtactgcgataatgccggcagcgtctcattcttcccacaagccgagacatgcaaggtgcagagcaaccgggtgttctgcgacaccatgaatagcagaaccctgccttccgaagtgaatctgtgcaacgtggacatcttcaaccctaagtacgactgcaagatcatgaccagcaagaccgacgtgtccagcagtgtgatcacctcactgggcgccatcgtgtcctgttacggcaagaccaagtgcaccgccagcaacaagaaccggggcatcatcaagaccttcagcaacggctgcgactacgtgtccaacaaaggcgtggacaccgtgtctgtgggcaacaccctgtactgcgtgaacaaacaagagggccagtctctgtacgtgaagtgcgagcccatcatcaacttctacgaccctctggtgttccccagcagcgagttcgatgccagcatcagccaagtgaacgagaagatcaatcagagcctggccttcatcagaaagtccgatgagctgctgcacaacgtgaacgccggcaagtccaccaccaatatcatgatcacgaccatcatcatcgtgattatcgtgatcctgctgtccctgatcgccgtgggcctgctgctttattgataatag

SEQ ID NO: 56 - protein, 510 aa, synthetic construct
MELLILKANAITTILTAVTFCFASGQNITEEFYCSTCSAVSKGYLGALRTGWYTSVILIELSNIKENKCNGTDAKVKLIKQELDKYKNAVTDLQLLMQSTPATGSGSAICSGVAVSKVLHLEGEVNKIKSALLSTNKAVVSLSNGVSVLTFKVLDLKNYIDKQLLPIVNKQSCSIPNIETVIEFQQKNNRLLEITREFSVNAGVTTPVSTYMLTNSELLSLINDMPITNDQKKLMSNNVQIVRQQSYSIMSIIKEEVLAYVVQLPLYGVIDTPCWKLHTSPLCTTNTKEGSNICLTRTDRGWYCDNAGSVSFFPQAETCKVQSNRVFCDTMNSRTLPSEVNLCNVDIFNPKYDCKIMTSKTDVSSSVITSLGAIVSCYGKTKCTASNKNRGIIKTFSNGCDYVSNKGVDTVSVGNTLYCVNKQEGQSLYVKCEPIINFYDPLVFPSSEFDASISQVNEKINQSLAFIRKSDELLHNVNAGKSTTNIMITTIIIVIIVILLSLIAVGLLLY

SEQ ID NO: 57 - RNA, 1841 nt, synthetic construct
  source 1..1841: mol_type = other RNA
agcggctcggccattttgtcccagtcagtccggaggctgcggctgcagaagtaccgcctgcggagtaactgcaaaggccaccatggaactgctgatcctgaaggccaacgccatcaccaccatcctgaccgccgtgaccttctgttttgccagcggccagaacatcaccgaggaattctactgcagcacctgtagcgccgtgtccaagggatatctgggcgcccttagaaccggctggtacaccagcgtgatcctgatcgagctgagcaacatcaaagaaaacaagtgcaacggcaccgacgccaaagtgaagctgatcaagcaagagctggacaagtacaagaatgccgtgaccgacctgcagctgctgatgcagtctacaccagccacaggctctggcagcgccatttgttctggtgtcgccgtgtctaaagtgctgcacctggaaggcgaagtgaacaagatcaagagcgccctgctgagcaccaacaaggccgtggtgtctctgagcaatggcgtgtccgtgctgaccttcaaggtgctggacctgaagaactacatcgacaaacagctgctgcccatcgtcaacaagcagtcctgcagcatccccaacatcgagacagtgatcgagttccagcagaagaacaaccggctgctggaaatcacccgcgagttctctgtgaatgccggcgtgaccacacctgtgtccacctacatgctgaccaacagcgagctgctgagcctgatcaacgacatgcccatcaccaacgaccagaaaaagctgatgagcaacaacgtgcagatcgtgcggcagcagagctacagcatcatgagcattatcaaagaagaggtgctggcctacgtggtgcagctgcctctgtatggcgtgatcgataccccttgctggaagctgcacacaagccctctgtgcaccaccaacaccaaagagggcagcaacatctgcctgaccagaaccgacagaggctggtactgcgataatgccggcagcgtctcattcttcccacaagccgagacatgcaaggtgcagagcaaccgggtgttctgcgacaccatgaatagcagaaccctgccttccgaagtgaatctgtgcaacgtggacatcttcaaccctaagtacgactgcaagatcatgaccagcaagaccgacgtgtccagcagtgtgatcacctcactgggcgccatcgtgtcctgttacggcaagaccaagtgcaccgccagcaacaagaaccggggcatcatcaagaccttcagcaacggctgcgactacgtgtccaacaaaggcgtggacaccgtgtctgtgggcaacaccctgtactgcgtgaacaaacaagagggccagtctctgtacgtgaagtgcgagcccatcatcaacttctacgaccctctggtgttccccagcagcgagttcgatgccagcatcagccaagtgaacgagaagatcaatcagagcctggccttcatcagaaagtccgatgagctgctgcacaacgtgaacgccggcaagtccaccaccaatatcatgatcacgaccatcatcatcgtgattatcgtgatcctgctgtccctgatcgccgtgggcctgctgctttattgataataggctggagcctcggtggccatgcttcttgccccttgggcctccccccagcccctcctccccttcctgcacccgtacccccgtggtctttgaataaagtctgagtgggcggcaaaaaaaaaaaaaaaaaaaaaaaaaaaaaaaaaaaaaaaaaaaaaaaaaaaaaaaaaaaaaaaaaaaaaaaaaaaaaaaaaaaaaaaaaaaaaaaaaaaaaaaaaaaaaa

SEQ ID NO: 58 - DNA, 1841 bp, synthetic construct
  source 1..1841: mol_type = other DNA
agcggctcggccattttgtcccagtcagtccggaggctgcggctgcagaagtaccgcctgcggagtaactgcaaaggccaccatggaactgctgatcctgaaggccaacgccatcaccaccatcctgaccgccgtgaccttctgttttgccagcggccagaacatcaccgaggaattctaccagagcacctgtagcgccgtgtccaagggatatctgggcgcccttagaaccggctggtacacctgcgtgatcctgatcgagctgagcaacatcaaagaaaacaagtgcaacggcaccgacgccaaagtgaagctgatcaagcaagagctggacaagtacaagaatgccgtgaccgacctgcagctgctgatgcagtctacaccagccacaggctctggcagcgccatttgttctggtgtcgccgtgtctaaagtgctgcacctggaaggcgaagtgaacaagatcaagagcgccctgctgagcaccaacaaggccgtggtgtctctgagcaatggcgtgtccgtgtgcaccttcaaggtgctggacctgaagaactacatcgacaaacagctgctgcccatcgtcaacaagcagtcctgcagcatccccaacatcgagacagtgatcgagttccagcagaagaacaaccggctgctggaaatcacccgcgagttctctgtgaatgccggcgtgaccacacctgtgtccacctacatgctgaccaacagcgagctgctgagcctgatcaacgacatgcccatcaccaacgaccagaaaaagctgatgagcaacaacgtgcagatcgtgcggcagcagagctacagcatcatgagcattatcaaagaagaggtgctggcctacgtggtgcagctgcctctgtatggcgtgatcgataccccttgctggaagctgcacacaagccctctgtgcaccaccaacaccaaagagggcagcaacatctgcctgaccagaaccgacagaggctggtactgcgataatgccggcagcgtctcattcttcccacaagccgagacatgcaaggtgcagagcaaccgggtgttctgcgacaccatgaatagcagaaccctgccttccgaagtgaatctgtgcaacgtggacatcttcaaccctaagtacgactgcaagatcatgaccagcaagaccgacgtgtccagcagtgtgatcacctcactgggcgccatcgtgtcctgttacggcaagaccaagtgcaccgccagcaacaagaaccggggcatcatcaagaccttcagcaacggctgcgactacgtgtccaacaaaggcgtggacaccgtgtctgtgggcaacaccctgtactgcgtgaacaaacaagagggccagtctctgtacgtgaagggcgagcccatcatcaacttctacgaccctctggtgttccccagcagcgagttcgatgccagcatcagccaagtgaacgagaagatcaatcagagcctggccttcatcagaaagtccgatgagctgctgcacaacgtgaacgccggcaagtccaccaccaatatcatgatcacgaccatcatcatcgtgattatcgtgatcctgctgtccctgatcgccgtgggcctgctgctttattgataataggctggagcctcggtggccatgcttcttgccccttgggcctccccccagcccctcctccccttcctgcacccgtacccccgtggtctttgaataaagtctgagtgggcggcaaaaaaaaaaaaaaaaaaaaaaaaaaaaaaaaaaaaaaaaaaaaaaaaaaaaaaaaaaaaaaaaaaaaaaaaaaaaaaaaaaaaaaaaaaaaaaaaaaaaaaaaaaaaaa

SEQ ID NO: 59 - DNA, 1539 bp, synthetic construct
  source 1..1539: mol_type = other DNA
atggaactgctgatcctgaaggccaacgccatcaccaccatcctgaccgccgtgaccttctgttttgccagcggccagaacatcaccgaggaattctaccagagcacctgtagcgccgtgtccaagggatatctgggcgcccttagaaccggctggtacacctgcgtgatcctgatcgagctgagcaacatcaaagaaaacaagtgcaacggcaccgacgccaaagtgaagctgatcaagcaagagctggacaagtacaagaatgccgtgaccgacctgcagctgctgatgcagtctacaccagccacaggctctggcagcgccatttgttctggtgtcgccgtgtctaaagtgctgcacctggaaggcgaagtgaacaagatcaagagcgccctgctgagcaccaacaaggccgtggtgtctctgagcaatggcgtgtccgtgtgcaccttcaaggtgctggacctgaagaactacatcgacaaacagctgctgcccatcgtcaacaagcagtcctgcagcatccccaacatcgagacagtgatcgagttccagcagaagaacaaccggctgctggaaatcacccgcgagttctctgtgaatgccggcgtgaccacacctgtgtccacctacatgctgaccaacagcgagctgctgagcctgatcaacgacatgcccatcaccaacgaccagaaaaagctgatgagcaacaacgtgcagatcgtgcggcagcagagctacagcatcatgagcattatcaaagaagaggtgctggcctacgtggtgcagctgcctctgtatggcgtgatcgataccccttgctggaagctgcacacaagccctctgtgcaccaccaacaccaaagagggcagcaacatctgcctgaccagaaccgacagaggctggtactgcgataatgccggcagcgtctcattcttcccacaagccgagacatgcaaggtgcagagcaaccgggtgttctgcgacaccatgaatagcagaaccctgccttccgaagtgaatctgtgcaacgtggacatcttcaaccctaagtacgactgcaagatcatgaccagcaagaccgacgtgtccagcagtgtgatcacctcactgggcgccatcgtgtcctgttacggcaagaccaagtgcaccgccagcaacaagaaccggggcatcatcaagaccttcagcaacggctgcgactacgtgtccaacaaaggcgtggacaccgtgtctgtgggcaacaccctgtactgcgtgaacaaacaagagggccagtctctgtacgtgaagggcgagcccatcatcaacttctacgaccctctggtgttccccagcagcgagttcgatgccagcatcagccaagtgaacgagaagatcaatcagagcctggccttcatcagaaagtccgatgagctgctgcacaacgtgaacgccggcaagtccaccaccaatatcatgatcacgaccatcatcatcgtgattatcgtgatcctgctgtccctgatcgccgtgggcctgctgctttattgataatag

SEQ ID NO: 60 - protein, 510 aa, synthetic construct
MELLILKANAITTILTAVTFCFASGQNITEEFYQSTCSAVSKGYLGALRTGWYTCVILIELSNIKENKCNGTDAKVKLIKQELDKYKNAVTDLQLLMQSTPATGSGSAICSGVAVSKVLHLEGEVNKIKSALLSTNKAVVSLSNGVSVCTFKVLDLKNYIDKQLLPIVNKQSCSIPNIETVIEFQQKNNRLLEITREFSVNAGVTTPVSTYMLTNSELLSLINDMPITNDQKKLMSNNVQIVRQQSYSIMSIIKEEVLAYVVQLPLYGVIDTPCWKLHTSPLCTTNTKEGSNICLTRTDRGWYCDNAGSVSFFPQAETCKVQSNRVFCDTMNSRTLPSEVNLCNVDIFNPKYDCKIMTSKTDVSSSVITSLGAIVSCYGKTKCTASNKNRGIIKTFSNGCDYVSNKGVDTVSVGNTLYCVNKQEGQSLYVKGEPIINFYDPLVFPSSEFDASISQVNEKINQSLAFIRKSDELLHNVNAGKSTTNIMITTIIIVIIVILLSLIAVGLLLY

SEQ ID NO: 61 - RNA, 1841 nt, synthetic construct
  source 1..1841: mol_type = other RNA
agcggctcggccattttgtcccagtcagtccggaggctgcggctgcagaagtaccgcctgcggagtaactgcaaaggccaccatggaactgctgatcctgaaggccaacgccatcaccaccatcctgaccgccgtgaccttctgttttgccagcggccagaacatcaccgaggaattctaccagagcacctgtagcgccgtgtccaagggatatctgggcgcccttagaaccggctggtacacctgcgtgatcctgatcgagctgagcaacatcaaagaaaacaagtgcaacggcaccgacgccaaagtgaagctgatcaagcaagagctggacaagtacaagaatgccgtgaccgacctgcagctgctgatgcagtctacaccagccacaggctctggcagcgccatttgttctggtgtcgccgtgtctaaagtgctgcacctggaaggcgaagtgaacaagatcaagagcgccctgctgagcaccaacaaggccgtggtgtctctgagcaatggcgtgtccgtgtgcaccttcaaggtgctggacctgaagaactacatcgacaaacagctgctgcccatcgtcaacaagcagtcctgcagcatccccaacatcgagacagtgatcgagttccagcagaagaacaaccggctgctggaaatcacccgcgagttctctgtgaatgccggcgtgaccacacctgtgtccacctacatgctgaccaacagcgagctgctgagcctgatcaacgacatgcccatcaccaacgaccagaaaaagctgatgagcaacaacgtgcagatcgtgcggcagcagagctacagcatcatgagcattatcaaagaagaggtgctggcctacgtggtgcagctgcctctgtatggcgtgatcgataccccttgctggaagctgcacacaagccctctgtgcaccaccaacaccaaagagggcagcaacatctgcctgaccagaaccgacagaggctggtactgcgataatgccggcagcgtctcattcttcccacaagccgagacatgcaaggtgcagagcaaccgggtgttctgcgacaccatgaatagcagaaccctgccttccgaagtgaatctgtgcaacgtggacatcttcaaccctaagtacgactgcaagatcatgaccagcaagaccgacgtgtccagcagtgtgatcacctcactgggcgccatcgtgtcctgttacggcaagaccaagtgcaccgccagcaacaagaaccggggcatcatcaagaccttcagcaacggctgcgactacgtgtccaacaaaggcgtggacaccgtgtctgtgggcaacaccctgtactgcgtgaacaaacaagagggccagtctctgtacgtgaagggcgagcccatcatcaacttctacgaccctctggtgttccccagcagcgagttcgatgccagcatcagccaagtgaacgagaagatcaatcagagcctggccttcatcagaaagtccgatgagctgctgcacaacgtgaacgccggcaagtccaccaccaatatcatgatcacgaccatcatcatcgtgattatcgtgatcctgctgtccctgatcgccgtgggcctgctgctttattgataataggctggagcctcggtggccatgcttcttgccccttgggcctccccccagcccctcctccccttcctgcacccgtacccccgtggtctttgaataaagtctgagtgggcggcaaaaaaaaaaaaaaaaaaaaaaaaaaaaaaaaaaaaaaaaaaaaaaaaaaaaaaaaaaaaaaaaaaaaaaaaaaaaaaaaaaaaaaaaaaaaaaaaaaaaaaaaaaaaaa

SEQ ID NO: 62 - DNA, 1841 bp, synthetic construct
  source 1..1841: mol_type = other DNA
agcggctcggccattttgtcccagtcagtccggaggctgcggctgcagaagtaccgcctgcggagtaactgcaaaggccaccatggaactgctgatcctgaaggccaacgccatcaccaccatcctgaccgccgtgaccttctgttttgccagcggccagaacatcaccgaggaattctactgcagcacctgtagcgccgtgtccaagggatatctgggcgcccttagaaccggctggtacaccagcgtgatcaccatcgagctgagcaacatcaaagaaaacaagtgcaacggcaccgacgccaaagtgaagctgatcaagcaagagctggacaagtacaagaatgccgtgaccgacctgcagctgctgatgcagtctacaccagccacaggctctggcagcgccatttgttctggtgtcgccgtgtctaaagtgctgcacctggaaggcgaagtgaacaagatcaagagcgccctgctgagcaccaacaaggccgtggtgtctctgagcaatggcgtgtccgtgctgaccttcaaggtgctggacctgaagaactacatcgacaaacagctgctgcccatcgtcaacaagcagtcctgcagcatccccaacatcgagatcgtgatcgagttccagcagaagaacaaccggctgctggaaatcacccgcgagttctctgtgaatgccggcgtgaccacacctgtgtccacctacatgctgaccaacagcgagctgctgagcctgatcaacgacatgcccatcaccaacgaccagaaaaagctgatgagcaacaacgtgcagatcgtgcggcagcagagctacagcatcatgagcattatcaaagaagaggtgctggcctacgtggtgcagctgcctctgtatggcgtgatcgataccccttgctggaagctgcacacaagccctctgtgcaccaccaacaccaaagagggcagcaacatctgcctgaccagaaccgacagaggctggtactgcgataatgccggcagcgtctcattcttcccacaagccgagacatgcaaggtgcagagcaaccgggtgttctgcgacaccatgaatagcagaaccctgccttccgaagtgaatctgtgcaacgtggacatcttcaaccctaagtacgactgcaagatcatgaccagcaagaccgacgtgtccagcagtgtgatcacctcactgggcgccatcgtgtcctgttacggcaagaccaagtgcaccgccagcaacaagaaccggggcatcatcaagaccttcagcaacggctgcgactacgtgtccaacaaaggcgtggacaccgtgtctgtgggcaacaccctgtactgcgtgaacaaacaagagggccagtctctgtacgtgaagtgcgagcccatcatcaacttctacgaccctctggtgttccccagcagcgagttcgatgccagcatcagccaagtgaacgagaagatcaatcagagcctggccttcatcagaaagtccgatgagctgctgcacaacgtgaacgccggcaagtccaccaccaatatcatgatcacgaccatcatcatcgtgattatcgtgatcctgctgtccctgatcgccgtgggcctgctgctttattgataataggctggagcctcggtggccatgcttcttgccccttgggcctccccccagcccctcctccccttcctgcacccgtacccccgtggtctttgaataaagtctgagtgggcggcaaaaaaaaaaaaaaaaaaaaaaaaaaaaaaaaaaaaaaaaaaaaaaaaaaaaaaaaaaaaaaaaaaaaaaaaaaaaaaaaaaaaaaaaaaaaaaaaaaaaaaaaaaaaaa

SEQ ID NO: 63 - DNA, 1539 bp, synthetic construct
  source 1..1539: mol_type = other DNA
atggaactgctgatcctgaaggccaacgccatcaccaccatcctgaccgccgtgaccttctgttttgccagcggccagaacatcaccgaggaattctactgcagcacctgtagcgccgtgtccaagggatatctgggcgcccttagaaccggctggtacaccagcgtgatcaccatcgagctgagcaacatcaaagaaaacaagtgcaacggcaccgacgccaaagtgaagctgatcaagcaagagctggacaagtacaagaatgccgtgaccgacctgcagctgctgatgcagtctacaccagccacaggctctggcagcgccatttgttctggtgtcgccgtgtctaaagtgctgcacctggaaggcgaagtgaacaagatcaagagcgccctgctgagcaccaacaaggccgtggtgtctctgagcaatggcgtgtccgtgctgaccttcaaggtgctggacctgaagaactacatcgacaaacagctgctgcccatcgtcaacaagcagtcctgcagcatccccaacatcgagatcgtgatcgagttccagcagaagaacaaccggctgctggaaatcacccgcgagttctctgtgaatgccggcgtgaccacacctgtgtccacctacatgctgaccaacagcgagctgctgagcctgatcaacgacatgcccatcaccaacgaccagaaaaagctgatgagcaacaacgtgcagatcgtgcggcagcagagctacagcatcatgagcattatcaaagaagaggtgctggcctacgtggtgcagctgcctctgtatggcgtgatcgataccccttgctggaagctgcacacaagccctctgtgcaccaccaacaccaaagagggcagcaacatctgcctgaccagaaccgacagaggctggtactgcgataatgccggcagcgtctcattcttcccacaagccgagacatgcaaggtgcagagcaaccgggtgttctgcgacaccatgaatagcagaaccctgccttccgaagtgaatctgtgcaacgtggacatcttcaaccctaagtacgactgcaagatcatgaccagcaagaccgacgtgtccagcagtgtgatcacctcactgggcgccatcgtgtcctgttacggcaagaccaagtgcaccgccagcaacaagaaccggggcatcatcaagaccttcagcaacggctgcgactacgtgtccaacaaaggcgtggacaccgtgtctgtgggcaacaccctgtactgcgtgaacaaacaagagggccagtctctgtacgtgaagtgcgagcccatcatcaacttctacgaccctctggtgttccccagcagcgagttcgatgccagcatcagccaagtgaacgagaagatcaatcagagcctggccttcatcagaaagtccgatgagctgctgcacaacgtgaacgccggcaagtccaccaccaatatcatgatcacgaccatcatcatcgtgattatcgtgatcctgctgtccctgatcgccgtgggcctgctgctttattgataatag

SEQ ID NO: 64 - protein, 510 aa, synthetic construct
MELLILKANAITTILTAVTFCFASGQNITEEFYCSTCSAVSKGYLGALRTGWYTSVITIELSNIKENKCNGTDAKVKLIKQELDKYKNAVTDLQLLMQSTPATGSGSAICSGVAVSKVLHLEGEVNKIKSALLSTNKAVVSLSNGVSVLTFKVLDLKNYIDKQLLPIVNKQSCSIPNIEIVIEFQQKNNRLLEITREFSVNAGVTTPVSTYMLTNSELLSLINDMPITNDQKKLMSNNVQIVRQQSYSIMSIIKEEVLAYVVQLPLYGVIDTPCWKLHTSPLCTTNTKEGSNICLTRTDRGWYCDNAGSVSFFPQAETCKVQSNRVFCDTMNSRTLPSEVNLCNVDIFNPKYDCKIMTSKTDVSSSVITSLGAIVSCYGKTKCTASNKNRGIIKTFSNGCDYVSNKGVDTVSVGNTLYCVNKQEGQSLYVKCEPIINFYDPLVFPSSEFDASISQVNEKINQSLAFIRKSDELLHNVNAGKSTTNIMITTIIIVIIVILLSLIAVGLLLY

SEQ ID NO: 65 - RNA, 1841 nt, synthetic construct
  source 1..1841: mol_type = other RNA
agcggctcggccattttgtcccagtcagtccggaggctgcggctgcagaagtaccgcctgcggagtaactgcaaaggccaccatggaactgctgatcctgaaggccaacgccatcaccaccatcctgaccgccgtgaccttctgttttgccagcggccagaacatcaccgaggaattctactgcagcacctgtagcgccgtgtccaagggatatctgggcgcccttagaaccggctggtacaccagcgtgatcaccatcgagctgagcaacatcaaagaaaacaagtgcaacggcaccgacgccaaagtgaagctgatcaagcaagagctggacaagtacaagaatgccgtgaccgacctgcagctgctgatgcagtctacaccagccacaggctctggcagcgccatttgttctggtgtcgccgtgtctaaagtgctgcacctggaaggcgaagtgaacaagatcaagagcgccctgctgagcaccaacaaggccgtggtgtctctgagcaatggcgtgtccgtgctgaccttcaaggtgctggacctgaagaactacatcgacaaacagctgctgcccatcgtcaacaagcagtcctgcagcatccccaacatcgagatcgtgatcgagttccagcagaagaacaaccggctgctggaaatcacccgcgagttctctgtgaatgccggcgtgaccacacctgtgtccacctacatgctgaccaacagcgagctgctgagcctgatcaacgacatgcccatcaccaacgaccagaaaaagctgatgagcaacaacgtgcagatcgtgcggcagcagagctacagcatcatgagcattatcaaagaagaggtgctggcctacgtggtgcagctgcctctgtatggcgtgatcgataccccttgctggaagctgcacacaagccctctgtgcaccaccaacaccaaagagggcagcaacatctgcctgaccagaaccgacagaggctggtactgcgataatgccggcagcgtctcattcttcccacaagccgagacatgcaaggtgcagagcaaccgggtgttctgcgacaccatgaatagcagaaccctgccttccgaagtgaatctgtgcaacgtggacatcttcaaccctaagtacgactgcaagatcatgaccagcaagaccgacgtgtccagcagtgtgatcacctcactgggcgccatcgtgtcctgttacggcaagaccaagtgcaccgccagcaacaagaaccggggcatcatcaagaccttcagcaacggctgcgactacgtgtccaacaaaggcgtggacaccgtgtctgtgggcaacaccctgtactgcgtgaacaaacaagagggccagtctctgtacgtgaagtgcgagcccatcatcaacttctacgaccctctggtgttccccagcagcgagttcgatgccagcatcagccaagtgaacgagaagatcaatcagagcctggccttcatcagaaagtccgatgagctgctgcacaacgtgaacgccggcaagtccaccaccaatatcatgatcacgaccatcatcatcgtgattatcgtgatcctgctgtccctgatcgccgtgggcctgctgctttattgataataggctggagcctcggtggccatgcttcttgccccttgggcctccccccagcccctcctccccttcctgcacccgtacccccgtggtctttgaataaagtctgagtgggcggcaaaaaaaaaaaaaaaaaaaaaaaaaaaaaaaaaaaaaaaaaaaaaaaaaaaaaaaaaaaaaaaaaaaaaaaaaaaaaaaaaaaaaaaaaaaaaaaaaaaaaaaaaaaaaa

SEQ ID NO: 66 - DNA, 1841 bp, synthetic construct
  source 1..1841: mol_type = other DNA
agcggctcggccattttgtcccagtcagtccggaggctgcggctgcagaagtaccgcctgcggagtaactgcaaaggccaccatggaactgctgatcctgaaggccaacgccatcaccaccatcctgaccgccgtgaccttctgttttgccagcggccagaacatcaccgaggaattctaccagagcacctgtagcgccgtgtccaagggatatctgggcgcccttagaaccggctggtacacctgcgtgatcaccatcgagctgagcaacatcaaagaaaacaagtgcaacggcaccgacgccaaagtgaagctgatcaagcaagagctggacaagtacaagaatgccgtgaccgacctgcagctgctgatgcagtctacaccagccacaggctctggcagcgccatttgttctggtgtcgccgtgtctaaagtgctgcacctggaaggcgaagtgaacaagatcaagagcgccctgctgagcaccaacaaggccgtggtgtctctgagcaatggcgtgtccgtgtgcaccttcaaggtgctggacctgaagaactacatcgacaaacagctgctgcccatcgtcaacaagcagtcctgcagcatccccaacatcgagatcgtgatcgagttccagcagaagaacaaccggctgctggaaatcacccgcgagttctctgtgaatgccggcgtgaccacacctgtgtccacctacatgctgaccaacagcgagctgctgagcctgatcaacgacatgcccatcaccaacgaccagaaaaagctgatgagcaacaacgtgcagatcgtgcggcagcagagctacagcatcatgagcattatcaaagaagaggtgctggcctacgtggtgcagctgcctctgtatggcgtgatcgataccccttgctggaagctgcacacaagccctctgtgcaccaccaacaccaaagagggcagcaacatctgcctgaccagaaccgacagaggctggtactgcgataatgccggcagcgtctcattcttcccacaagccgagacatgcaaggtgcagagcaaccgggtgttctgcgacaccatgaatagcagaaccctgccttccgaagtgaatctgtgcaacgtggacatcttcaaccctaagtacgactgcaagatcatgaccagcaagaccgacgtgtccagcagtgtgatcacctcactgggcgccatcgtgtcctgttacggcaagaccaagtgcaccgccagcaacaagaaccggggcatcatcaagaccttcagcaacggctgcgactacgtgtccaacaaaggcgtggacaccgtgtctgtgggcaacaccctgtactgcgtgaacaaacaagagggccagtctctgtacgtgaagggcgagcccatcatcaacttctacgaccctctggtgttccccagcagcgagttcgatgccagcatcagccaagtgaacgagaagatcaatcagagcctggccttcatcagaaagtccgatgagctgctgcacaacgtgaacgccggcaagtccaccaccaatatcatgatcacgaccatcatcatcgtgattatcgtgatcctgctgtccctgatcgccgtgggcctgctgctttattgataataggctggagcctcggtggccatgcttcttgccccttgggcctccccccagcccctcctccccttcctgcacccgtacccccgtggtctttgaataaagtctgagtgggcggcaaaaaaaaaaaaaaaaaaaaaaaaaaaaaaaaaaaaaaaaaaaaaaaaaaaaaaaaaaaaaaaaaaaaaaaaaaaaaaaaaaaaaaaaaaaaaaaaaaaaaaaaaaaaaa

SEQ ID NO: 67 - DNA, 1539 bp, synthetic construct
  source 1..1539: mol_type = other DNA
atggaactgctgatcctgaaggccaacgccatcaccaccatcctgaccgccgtgaccttctgttttgccagcggccagaacatcaccgaggaattctaccagagcacctgtagcgccgtgtccaagggatatctgggcgcccttagaaccggctggtacacctgcgtgatcaccatcgagctgagcaacatcaaagaaaacaagtgcaacggcaccgacgccaaagtgaagctgatcaagcaagagctggacaagtacaagaatgccgtgaccgacctgcagctgctgatgcagtctacaccagccacaggctctggcagcgccatttgttctggtgtcgccgtgtctaaagtgctgcacctggaaggcgaagtgaacaagatcaagagcgccctgctgagcaccaacaaggccgtggtgtctctgagcaatggcgtgtccgtgtgcaccttcaaggtgctggacctgaagaactacatcgacaaacagctgctgcccatcgtcaacaagcagtcctgcagcatccccaacatcgagatcgtgatcgagttccagcagaagaacaaccggctgctggaaatcacccgcgagttctctgtgaatgccggcgtgaccacacctgtgtccacctacatgctgaccaacagcgagctgctgagcctgatcaacgacatgcccatcaccaacgaccagaaaaagctgatgagcaacaacgtgcagatcgtgcggcagcagagctacagcatcatgagcattatcaaagaagaggtgctggcctacgtggtgcagctgcctctgtatggcgtgatcgataccccttgctggaagctgcacacaagccctctgtgcaccaccaacaccaaagagggcagcaacatctgcctgaccagaaccgacagaggctggtactgcgataatgccggcagcgtctcattcttcccacaagccgagacatgcaaggtgcagagcaaccgggtgttctgcgacaccatgaatagcagaaccctgccttccgaagtgaatctgtgcaacgtggacatcttcaaccctaagtacgactgcaagatcatgaccagcaagaccgacgtgtccagcagtgtgatcacctcactgggcgccatcgtgtcctgttacggcaagaccaagtgcaccgccagcaacaagaaccggggcatcatcaagaccttcagcaacggctgcgactacgtgtccaacaaaggcgtggacaccgtgtctgtgggcaacaccctgtactgcgtgaacaaacaagagggccagtctctgtacgtgaagggcgagcccatcatcaacttctacgaccctctggtgttccccagcagcgagttcgatgccagcatcagccaagtgaacgagaagatcaatcagagcctggccttcatcagaaagtccgatgagctgctgcacaacgtgaacgccggcaagtccaccaccaatatcatgatcacgaccatcatcatcgtgattatcgtgatcctgctgtccctgatcgccgtgggcctgctgctttattgataatag

SEQ ID NO: 68 - protein, 510 aa, synthetic construct
MELLILKANAITTILTAVTFCFASGQNITEEFYQSTCSAVSKGYLGALRTGWYTCVITIELSNIKENKCNGTDAKVKLIKQELDKYKNAVTDLQLLMQSTPATGSGSAICSGVAVSKVLHLEGEVNKIKSALLSTNKAVVSLSNGVSVCTFKVLDLKNYIDKQLLPIVNKQSCSIPNIEIVIEFQQKNNRLLEITREFSVNAGVTTPVSTYMLTNSELLSLINDMPITNDQKKLMSNNVQIVRQQSYSIMSIIKEEVLAYVVQLPLYGVIDTPCWKLHTSPLCTTNTKEGSNICLTRTDRGWYCDNAGSVSFFPQAETCKVQSNRVFCDTMNSRTLPSEVNLCNVDIFNPKYDCKIMTSKTDVSSSVITSLGAIVSCYGKTKCTASNKNRGIIKTFSNGCDYVSNKGVDTVSVGNTLYCVNKQEGQSLYVKGEPIINFYDPLVFPSSEFDASISQVNEKINQSLAFIRKSDELLHNVNAGKSTTNIMITTIIIVIIVILLSLIAVGLLLY

SEQ ID NO: 69 - RNA, 1841 nt, synthetic construct
  source 1..1841: mol_type = other RNA
agcggctcggccattttgtcccagtcagtccggaggctgcggctgcagaagtaccgcctgcggagtaactgcaaaggccaccatggaactgctgatcctgaaggccaacgccatcaccaccatcctgaccgccgtgaccttctgttttgccagcggccagaacatcaccgaggaattctaccagagcacctgtagcgccgtgtccaagggatatctgggcgcccttagaaccggctggtacacctgcgtgatcaccatcgagctgagcaacatcaaagaaaacaagtgcaacggcaccgacgccaaagtgaagctgatcaagcaagagctggacaagtacaagaatgccgtgaccgacctgcagctgctgatgcagtctacaccagccacaggctctggcagcgccatttgttctggtgtcgccgtgtctaaagtgctgcacctggaaggcgaagtgaacaagatcaagagcgccctgctgagcaccaacaaggccgtggtgtctctgagcaatggcgtgtccgtgtgcaccttcaaggtgctggacctgaagaactacatcgacaaacagctgctgcccatcgtcaacaagcagtcctgcagcatccccaacatcgagatcgtgatcgagttccagcagaagaacaaccggctgctggaaatcacccgcgagttctctgtgaatgccggcgtgaccacacctgtgtccacctacatgctgaccaacagcgagctgctgagcctgatcaacgacatgcccatcaccaacgaccagaaaaagctgatgagcaacaacgtgcagatcgtgcggcagcagagctacagcatcatgagcattatcaaagaagaggtgctggcctacgtggtgcagctgcctctgtatggcgtgatcgataccccttgctggaagctgcacacaagccctctgtgcaccaccaacaccaaagagggcagcaacatctgcctgaccagaaccgacagaggctggtactgcgataatgccggcagcgtctcattcttcccacaagccgagacatgcaaggtgcagagcaaccgggtgttctgcgacaccatgaatagcagaaccctgccttccgaagtgaatctgtgcaacgtggacatcttcaaccctaagtacgactgcaagatcatgaccagcaagaccgacgtgtccagcagtgtgatcacctcactgggcgccatcgtgtcctgttacggcaagaccaagtgcaccgccagcaacaagaaccggggcatcatcaagaccttcagcaacggctgcgactacgtgtccaacaaaggcgtggacaccgtgtctgtgggcaacaccctgtactgcgtgaacaaacaagagggccagtctctgtacgtgaagggcgagcccatcatcaacttctacgaccctctggtgttccccagcagcgagttcgatgccagcatcagccaagtgaacgagaagatcaatcagagcctggccttcatcagaaagtccgatgagctgctgcacaacgtgaacgccggcaagtccaccaccaatatcatgatcacgaccatcatcatcgtgattatcgtgatcctgctgtccctgatcgccgtgggcctgctgctttattgataataggctggagcctcggtggccatgcttcttgccccttgggcctccccccagcccctcctccccttcctgcacccgtacccccgtggtctttgaataaagtctgagtgggcggcaaaaaaaaaaaaaaaaaaaaaaaaaaaaaaaaaaaaaaaaaaaaaaaaaaaaaaaaaaaaaaaaaaaaaaaaaaaaaaaaaaaaaaaaaaaaaaaaaaaaaaaaaaaaaa

SEQ ID NO: 70 - DNA, 1844 bp, synthetic construct
  source 1..1844: mol_type = other DNA
agcggctcggccattttgtcccagtcagtccggaggctgcggctgcagaagtaccgcctgcggagtaactgcaaaggccaccatggaactgctgatcctgaaggccaacgccatcaccaccatcctgaccgccgtgaccttctgttttgccagcggccagaacatcaccgaggaattctaccagagcacctgtagcgccgtgtccaagggatatctgggcgcccttagaaccggctggtacaccagcgtgatcaccatcgagctgagcaacatcaaagaaaacaagtgcaacggcaccgacgccaaagtgaagctgatcaagcaagagctggacaagtacaagaatgccgtgaccgacctgcagctgctgatgcagtctacaccagcctgcggctctggcagcgcctgcgcttctggtgtcgccgtgtctaaagtgctgcacctggaaggcgaagtgaacaagatcaagagcgccctgctgagcaccaacaaggccgtggtgtctctgagcggctgcggcgtgtccgtgctgaccttcaaggtgctggacctgaagaactacatcgacaaacagctgctgcccatcgtcaacaagcagtcctgcagcatccccaacatcgagacagtgatcgagttccagcagaagaacaaccggctgctggaaatcacccgcgagttctctgtgaatgccggcgtgaccacacctgtgtccacctacatgctgaccaacagcgagctgctgagcctgatcaacgacatgcccatcaccaacgaccagaaaaagctgatgagcaacaacgtgcagatcgtgcggcagcagagctacagcatcatgagcattatcaaagaagaggtgctggcctacgtggtgcagctgcctctgtatggcgtgatcgataccccttgctggaagctgcacacaagccctctgtgcaccaccaacaccaaagagggcagcaacatctgcctgaccagaaccgacagaggctggtactgcgataatgccggcagcgtctcattcttcccacaagccgagacatgcaaggtgcagagcaaccgggtgttctgcgacaccatgaatagcagaaccctgccttccgaagtgaatctgtgcaacgtggacatcttcaaccctaagtacgactgcaagatcatgaccagcaagaccgacgtgtccagcagtgtgatcacctcactgggcgccatcgtgtcctgttacggcaagaccaagtgcaccgccagcaacaagtgccggggcatcatcaagaccttcagcaacggctgcgactacgtgtccaacaaaggcgtggacaccgtgtctgtgggcaacaccctgtactacgtgaacaaacaagagggccagtctctgtacgtgaagggcgagcccatcatcaacttctacgaccctctggtgttccccagcagcgagttcgatgccagcatcagccaagtgaacgagaagatcaatcagagcctggccttcatcagaaagtccgatgagctgctgcacaacgtgaacgccggcaagtccaccaccaatatcatgatcacgaccatcatcatcgtgattatcgtgatcctgctgtccctgatcgccgtgggcctgctgctttattgataataggctggagcctcggtggccatgcttcttgccccttgggcctccccccagcccctcctccccttcctgcacccgtacccccgtggtctttgaataaagtctgagtgggcggcaaaaaaaaaaaaaaaaaaaaaaaaaaaaaaaaaaaaaaaaaaaaaaaaaaaaaaaaaaaaaaaaaaaaaaaaaaaaaaaaaaaaaaaaaaaaaaaaaaaaaaaaaaaaaa

SEQ ID NO: 71 - DNA, 1542 bp, synthetic construct
  source 1..1542: mol_type = other DNA
atggaactgctgatcctgaaggccaacgccatcaccaccatcctgaccgccgtgaccttctgttttgccagcggccagaacatcaccgaggaattctaccagagcacctgtagcgccgtgtccaagggatatctgggcgcccttagaaccggctggtacaccagcgtgatcaccatcgagctgagcaacatcaaagaaaacaagtgcaacggcaccgacgccaaagtgaagctgatcaagcaagagctggacaagtacaagaatgccgtgaccgacctgcagctgctgatgcagtctacaccagcctgcggctctggcagcgcctgcgcttctggtgtcgccgtgtctaaagtgctgcacctggaaggcgaagtgaacaagatcaagagcgccctgctgagcaccaacaaggccgtggtgtctctgagcggctgcggcgtgtccgtgctgaccttcaaggtgctggacctgaagaactacatcgacaaacagctgctgcccatcgtcaacaagcagtcctgcagcatccccaacatcgagacagtgatcgagttccagcagaagaacaaccggctgctggaaatcacccgcgagttctctgtgaatgccggcgtgaccacacctgtgtccacctacatgctgaccaacagcgagctgctgagcctgatcaacgacatgcccatcaccaacgaccagaaaaagctgatgagcaacaacgtgcagatcgtgcggcagcagagctacagcatcatgagcattatcaaagaagaggtgctggcctacgtggtgcagctgcctctgtatggcgtgatcgataccccttgctggaagctgcacacaagccctctgtgcaccaccaacaccaaagagggcagcaacatctgcctgaccagaaccgacagaggctggtactgcgataatgccggcagcgtctcattcttcccacaagccgagacatgcaaggtgcagagcaaccgggtgttctgcgacaccatgaatagcagaaccctgccttccgaagtgaatctgtgcaacgtggacatcttcaaccctaagtacgactgcaagatcatgaccagcaagaccgacgtgtccagcagtgtgatcacctcactgggcgccatcgtgtcctgttacggcaagaccaagtgcaccgccagcaacaagtgccggggcatcatcaagaccttcagcaacggctgcgactacgtgtccaacaaaggcgtggacaccgtgtctgtgggcaacaccctgtactacgtgaacaaacaagagggccagtctctgtacgtgaagggcgagcccatcatcaacttctacgaccctctggtgttccccagcagcgagttcgatgccagcatcagccaagtgaacgagaagatcaatcagagcctggccttcatcagaaagtccgatgagctgctgcacaacgtgaacgccggcaagtccaccaccaatatcatgatcacgaccatcatcatcgtgattatcgtgatcctgctgtccctgatcgccgtgggcctgctgctttattgataatag

SEQ ID NO: 72 - protein, 511 aa, synthetic construct
MELLILKANAITTILTAVTFCFASGQNITEEFYQSTCSAVSKGYLGALRTGWYTSVITIELSNIKENKCNGTDAKVKLIKQELDKYKNAVTDLQLLMQSTPACGSGSACASGVAVSKVLHLEGEVNKIKSALLSTNKAVVSLSGCGVSVLTFKVLDLKNYIDKQLLPIVNKQSCSIPNIETVIEFQQKNNRLLEITREFSVNAGVTTPVSTYMLTNSELLSLINDMPITNDQKKLMSNNVQIVRQQSYSIMSIIKEEVLAYVVQLPLYGVIDTPCWKLHTSPLCTTNTKEGSNICLTRTDRGWYCDNAGSVSFFPQAETCKVQSNRVFCDTMNSRTLPSEVNLCNVDIFNPKYDCKIMTSKTDVSSSVITSLGAIVSCYGKTKCTASNKCRGIIKTFSNGCDYVSNKGVDTVSVGNTLYYVNKQEGQSLYVKGEPIINFYDPLVFPSSEFDASISQVNEKINQSLAFIRKSDELLHNVNAGKSTTNIMITTIIIVIIVILLSLIAVGLLLY

SEQ ID NO: 73 - RNA, 1844 nt, synthetic construct
  source 1..1844: mol_type = other RNA
agcggctcggccattttgtcccagtcagtccggaggctgcggctgcagaagtaccgcctgcggagtaactgcaaaggccaccatggaactgctgatcctgaaggccaacgccatcaccaccatcctgaccgccgtgaccttctgttttgccagcggccagaacatcaccgaggaattctaccagagcacctgtagcgccgtgtccaagggatatctgggcgcccttagaaccggctggtacaccagcgtgatcaccatcgagctgagcaacatcaaagaaaacaagtgcaacggcaccgacgccaaagtgaagctgatcaagcaagagctggacaagtacaagaatgccgtgaccgacctgcagctgctgatgcagtctacaccagcctgcggctctggcagcgcctgcgcttctggtgtcgccgtgtctaaagtgctgcacctggaaggcgaagtgaacaagatcaagagcgccctgctgagcaccaacaaggccgtggtgtctctgagcggctgcggcgtgtccgtgctgaccttcaaggtgctggacctgaagaactacatcgacaaacagctgctgcccatcgtcaacaagcagtcctgcagcatccccaacatcgagacagtgatcgagttccagcagaagaacaaccggctgctggaaatcacccgcgagttctctgtgaatgccggcgtgaccacacctgtgtccacctacatgctgaccaacagcgagctgctgagcctgatcaacgacatgcccatcaccaacgaccagaaaaagctgatgagcaacaacgtgcagatcgtgcggcagcagagctacagcatcatgagcattatcaaagaagaggtgctggcctacgtggtgcagctgcctctgtatggcgtgatcgataccccttgctggaagctgcacacaagccctctgtgcaccaccaacaccaaagagggcagcaacatctgcctgaccagaaccgacagaggctggtactgcgataatgccggcagcgtctcattcttcccacaagccgagacatgcaaggtgcagagcaaccgggtgttctgcgacaccatgaatagcagaaccctgccttccgaagtgaatctgtgcaacgtggacatcttcaaccctaagtacgactgcaagatcatgaccagcaagaccgacgtgtccagcagtgtgatcacctcactgggcgccatcgtgtcctgttacggcaagaccaagtgcaccgccagcaacaagtgccggggcatcatcaagaccttcagcaacggctgcgactacgtgtccaacaaaggcgtggacaccgtgtctgtgggcaacaccctgtactacgtgaacaaacaagagggccagtctctgtacgtgaagggcgagcccatcatcaacttctacgaccctctggtgttccccagcagcgagttcgatgccagcatcagccaagtgaacgagaagatcaatcagagcctggccttcatcagaaagtccgatgagctgctgcacaacgtgaacgccggcaagtccaccaccaatatcatgatcacgaccatcatcatcgtgattatcgtgatcctgctgtccctgatcgccgtgggcctgctgctttattgataataggctggagcctcggtggccatgcttcttgccccttgggcctccccccagcccctcctccccttcctgcacccgtacccccgtggtctttgaataaagtctgagtgggcggcaaaaaaaaaaaaaaaaaaaaaaaaaaaaaaaaaaaaaaaaaaaaaaaaaaaaaaaaaaaaaaaaaaaaaaaaaaaaaaaaaaaaaaaaaaaaaaaaaaaaaaaaaaaaaa

SEQ ID NO: 74 - DNA, 1841 bp, synthetic construct
  source 1..1841: mol_type = other DNA
agcggctcggccattttgtcccagtcagtccggaggctgcggctgcagaagtaccgcctgcggagtaactgcaaaggccaccatggaactgctgatcctgaaggccaacgccatcaccaccatcctgaccgccgtgaccttctgttttgccagcggccagaacatctgcgaggaattctaccagagcacctgtagcgccgtgtccaagggatatctgggcgcccttagaaccggctggtacaccagcgtgatcaccatcgagctgagcaacatcaaagaaaacaagtgcaacggcaccgacgccaaagtgaagctgatcaagcaagagctggacaagtacaagaatgccgtgaccgacctgcagctgctgatgcagtctacaccagccacaggctctggcagcgccattgcctctggtgtcgccgtgtctaaagtgctgcacctggaaggcgaagtgaacaagatcaagagcgccctgctgagcaccaacaaggccgtggtgtctctgagcaatggcgtgtccgtgctgaccttcaaggtgctggacctgaagaactacatcgacaaacagctgctgcccatcctgaacaagcagtcctgcagcatccccaacatcgagacagtgatcgagttccagcagaagaacaaccggctgctggaaatcacccgcgagttctctgtgaatgccggcgtgaccacacctgtgtccacctacatgctgaccaacagcgagctgctgagcctgatcaacgacatgcccatcaccaacgaccagaaaaagctgatgagcaacaacgtgcagatcgtgcggcagcagagctacagcatcatgagcattatcaaagaagaggtgctggcctacgtggtgcagctgcctctgtatggcgtgatcgataccccttgctggaagctgcacacaagccctctgtgcaccaccaacaccaaagagggcagcaacatctgcctgaccagaaccgacagaggctggtactgcgataatgccggcagcgtctcattcttcccacaagccgagacatgcaaggtgcagagcaaccgggtgttctgcgacaccatgaatagcagaaccctgccttccgaagtgaatctgtgcaacgtggacatcttcaaccctaagtacgactgcaagatcatgaccagcaagaccgacgtgtccagcagtgtgatcacctcactgggcgccatcgtgtcctgttacggcaagaccaagtgcaccgccagcaacaagaaccggggcatcatcaagaccttcagcaacggctgcgactacgtgtccaacaaaggcgtggacaccgtgtctgtgggcaacaccctgtactacgtgaacaaacaagagggctgctctctgtacgtgaagggcgagcccatcatcaacttctacgaccctctggtgttccccagcgacgagttcgatgccagcatcagccaagtgaacgagaagatcaatcagagcctggccttcatcagaaagtccgatgagctgctgcacaacgtgaacgccggcaagtccaccaccaatatcatgatcacgaccatcatcatcgtgattatcgtgatcctgctgtccctgatcgccgtgggcctgctgctttattgataataggctggagcctcggtggccatgcttcttgccccttgggcctccccccagcccctcctccccttcctgcacccgtacccccgtggtctttgaataaagtctgagtgggcggcaaaaaaaaaaaaaaaaaaaaaaaaaaaaaaaaaaaaaaaaaaaaaaaaaaaaaaaaaaaaaaaaaaaaaaaaaaaaaaaaaaaaaaaaaaaaaaaaaaaaaaaaaaaaaa

SEQ ID NO: 75 - DNA, 1539 bp, synthetic construct
  source 1..1539: mol_type = other DNA
atggaactgctgatcctgaaggccaacgccatcaccaccatcctgaccgccgtgaccttctgttttgccagcggccagaacatctgcgaggaattctaccagagcacctgtagcgccgtgtccaagggatatctgggcgcccttagaaccggctggtacaccagcgtgatcaccatcgagctgagcaacatcaaagaaaacaagtgcaacggcaccgacgccaaagtgaagctgatcaagcaagagctggacaagtacaagaatgccgtgaccgacctgcagctgctgatgcagtctacaccagccacaggctctggcagcgccattgcctctggtgtcgccgtgtctaaagtgctgcacctggaaggcgaagtgaacaagatcaagagcgccctgctgagcaccaacaaggccgtggtgtctctgagcaatggcgtgtccgtgctgaccttcaaggtgctggacctgaagaactacatcgacaaacagctgctgcccatcctgaacaagcagtcctgcagcatccccaacatcgagacagtgatcgagttccagcagaagaacaaccggctgctggaaatcacccgcgagttctctgtgaatgccggcgtgaccacacctgtgtccacctacatgctgaccaacagcgagctgctgagcctgatcaacgacatgcccatcaccaacgaccagaaaaagctgatgagcaacaacgtgcagatcgtgcggcagcagagctacagcatcatgagcattatcaaagaagaggtgctggcctacgtggtgcagctgcctctgtatggcgtgatcgataccccttgctggaagctgcacacaagccctctgtgcaccaccaacaccaaagagggcagcaacatctgcctgaccagaaccgacagaggctggtactgcgataatgccggcagcgtctcattcttcccacaagccgagacatgcaaggtgcagagcaaccgggtgttctgcgacaccatgaatagcagaaccctgccttccgaagtgaatctgtgcaacgtggacatcttcaaccctaagtacgactgcaagatcatgaccagcaagaccgacgtgtccagcagtgtgatcacctcactgggcgccatcgtgtcctgttacggcaagaccaagtgcaccgccagcaacaagaaccggggcatcatcaagaccttcagcaacggctgcgactacgtgtccaacaaaggcgtggacaccgtgtctgtgggcaacaccctgtactacgtgaacaaacaagagggctgctctctgtacgtgaagggcgagcccatcatcaacttctacgaccctctggtgttccccagcgacgagttcgatgccagcatcagccaagtgaacgagaagatcaatcagagcctggccttcatcagaaagtccgatgagctgctgcacaacgtgaacgccggcaagtccaccaccaatatcatgatcacgaccatcatcatcgtgattatcgtgatcctgctgtccctgatcgccgtgggcctgctgctttattgataatag

SEQ ID NO: 76 - protein, 510 aa, synthetic construct
MELLILKANAITTILTAVTFCFASGQNICEEFYQSTCSAVSKGYLGALRTGWYTSVITIELSNIKENKCNGTDAKVKLIKQELDKYKNAVTDLQLLMQSTPATGSGSAIASGVAVSKVLHLEGEVNKIKSALLSTNKAVVSLSNGVSVLTFKVLDLKNYIDKQLLPILNKQSCSIPNIETVIEFQQKNNRLLEITREFSVNAGVTTPVSTYMLTNSELLSLINDMPITNDQKKLMSNNVQIVRQQSYSIMSIIKEEVLAYVVQLPLYGVIDTPCWKLHTSPLCTTNTKEGSNICLTRTDRGWYCDNAGSVSFFPQAETCKVQSNRVFCDTMNSRTLPSEVNLCNVDIFNPKYDCKIMTSKTDVSSSVITSLGAIVSCYGKTKCTASNKNRGIIKTFSNGCDYVSNKGVDTVSVGNTLYYVNKQEGCSLYVKGEPIINFYDPLVFPSDEFDASISQVNEKINQSLAFIRKSDELLHNVNAGKSTTNIMITTIIIVIIVILLSLIAVGLLLY

SEQ ID NO: 77 - RNA, 1841 nt, synthetic construct
  source 1..1841: mol_type = other RNA
agcggctcggccattttgtcccagtcagtccggaggctgcggctgcagaagtaccgcctgcggagtaactgcaaaggccaccatggaactgctgatcctgaaggccaacgccatcaccaccatcctgaccgccgtgaccttctgttttgccagcggccagaacatctgcgaggaattctaccagagcacctgtagcgccgtgtccaagggatatctgggcgcccttagaaccggctggtacaccagcgtgatcaccatcgagctgagcaacatcaaagaaaacaagtgcaacggcaccgacgccaaagtgaagctgatcaagcaagagctggacaagtacaagaatgccgtgaccgacctgcagctgctgatgcagtctacaccagccacaggctctggcagcgccattgcctctggtgtcgccgtgtctaaagtgctgcacctggaaggcgaagtgaacaagatcaagagcgccctgctgagcaccaacaaggccgtggtgtctctgagcaatggcgtgtccgtgctgaccttcaaggtgctggacctgaagaactacatcgacaaacagctgctgcccatcctgaacaagcagtcctgcagcatccccaacatcgagacagtgatcgagttccagcagaagaacaaccggctgctggaaatcacccgcgagttctctgtgaatgccggcgtgaccacacctgtgtccacctacatgctgaccaacagcgagctgctgagcctgatcaacgacatgcccatcaccaacgaccagaaaaagctgatgagcaacaacgtgcagatcgtgcggcagcagagctacagcatcatgagcattatcaaagaagaggtgctggcctacgtggtgcagctgcctctgtatggcgtgatcgataccccttgctggaagctgcacacaagccctctgtgcaccaccaacaccaaagagggcagcaacatctgcctgaccagaaccgacagaggctggtactgcgataatgccggcagcgtctcattcttcccacaagccgagacatgcaaggtgcagagcaaccgggtgttctgcgacaccatgaatagcagaaccctgccttccgaagtgaatctgtgcaacgtggacatcttcaaccctaagtacgactgcaagatcatgaccagcaagaccgacgtgtccagcagtgtgatcacctcactgggcgccatcgtgtcctgttacggcaagaccaagtgcaccgccagcaacaagaaccggggcatcatcaagaccttcagcaacggctgcgactacgtgtccaacaaaggcgtggacaccgtgtctgtgggcaacaccctgtactacgtgaacaaacaagagggctgctctctgtacgtgaagggcgagcccatcatcaacttctacgaccctctggtgttccccagcgacgagttcgatgccagcatcagccaagtgaacgagaagatcaatcagagcctggccttcatcagaaagtccgatgagctgctgcacaacgtgaacgccggcaagtccaccaccaatatcatgatcacgaccatcatcatcgtgattatcgtgatcctgctgtccctgatcgccgtgggcctgctgctttattgataataggctggagcctcggtggccatgcttcttgccccttgggcctccccccagcccctcctccccttcctgcacccgtacccccgtggtctttgaataaagtctgagtgggcggcaaaaaaaaaaaaaaaaaaaaaaaaaaaaaaaaaaaaaaaaaaaaaaaaaaaaaaaaaaaaaaaaaaaaaaaaaaaaaaaaaaaaaaaaaaaaaaaaaaaaaaaaaaaaaa

SEQ ID NO: 78 - DNA, 1841 bp, synthetic construct
  source 1..1841: mol_type = other DNA
agcggctcggccattttgtcccagtcagtccggaggctgcggctgcagaagtaccgcctgcggagtaactgcaaaggccaccatggaactgctgatcctgaaggccaacgccatcaccaccatcctgaccgccgtgaccttctgttttgccagcggccagaacatcaccgagtgcttctaccagagcacctgtagcgccgtgtccaagggatatctgggcgcccttagaaccggctggtacaccagcgtgatcaccatcgagctgagcaacatcaaagaaaacaagtgcaacggcaccgacgccaaagtgaagctgatcaagcaagagctggacaagtacaagaatgccgtgaccgacctgcagctgctgatgcagtctacaccagccacaggctctggcagcgccattgcctctggtgtcgccgtgtctaaagtgctgcacctggaaggcgaagtgaacaagatcaagagcgccctgctgagcaccaacaaggccgtggtgtctctgagcaatggcgtgtccgtgctgaccttcaaggtgctggacctgaagaactacatcgacaaacagctgctgcccatcctgaacaagcagtcctgcagcatccccaacatcgagacagtgatcgagttccagcagaagaacaaccggctgctggaaatcacccgcgagttctctgtgaatgccggcgtgaccacacctgtgtccacctacatgctgaccaacagcgagctgctgagcctgatcaacgacatgcccatcaccaacgaccagaaaaagctgatgagcaacaacgtgcagatcgtgcggcagcagagctacagcatcatgagcattatcaaagaagaggtgctggcctacgtggtgcagctgcctctgtatggcgtgatcgataccccttgctggaagctgcacacaagccctctgtgcaccaccaacaccaaagagggcagcaacatctgcctgaccagaaccgacagaggctggtactgcgataatgccggcagcgtctcattcttcccacaagccgagacatgcaaggtgcagagcaaccgggtgttctgcgacaccatgaatagcagaaccctgccttccgaagtgaatctgtgcaacgtggacatcttcaaccctaagtacgactgcaagatcatgaccagcaagaccgacgtgtccagcagtgtgatcacctcactgggcgccatcgtgtcctgttacggcaagaccaagtgcaccgccagcaacaagaaccggggcatcatcaagaccttcagcaacggctgcgactacgtgtccaacaaaggcgtggacaccgtgtctgtgggcaacaccctgtactacgtgaacaaacaagagggccagtcttgctacgtgaagggcgagcccatcatcaacttctacgaccctctggtgttccccagcgacgagttcgatgccagcatcagccaagtgaacgagaagatcaatcagagcctggccttcatcagaaagtccgatgagctgctgcacaacgtgaacgccggcaagtccaccaccaatatcatgatcacgaccatcatcatcgtgattatcgtgatcctgctgtccctgatcgccgtgggcctgctgctttattgataataggctggagcctcggtggccatgcttcttgccccttgggcctccccccagcccctcctccccttcctgcacccgtacccccgtggtctttgaataaagtctgagtgggcggcaaaaaaaaaaaaaaaaaaaaaaaaaaaaaaaaaaaaaaaaaaaaaaaaaaaaaaaaaaaaaaaaaaaaaaaaaaaaaaaaaaaaaaaaaaaaaaaaaaaaaaaaaaaaaa

SEQ ID NO: 79 - DNA, 1539 bp, synthetic construct
  source 1..1539: mol_type = other DNA
atggaactgctgatcctgaaggccaacgccatcaccaccatcctgaccgccgtgaccttctgttttgccagcggccagaacatcaccgagtgcttctaccagagcacctgtagcgccgtgtccaagggatatctgggcgcccttagaaccggctggtacaccagcgtgatcaccatcgagctgagcaacatcaaagaaaacaagtgcaacggcaccgacgccaaagtgaagctgatcaagcaagagctggacaagtacaagaatgccgtgaccgacctgcagctgctgatgcagtctacaccagccacaggctctggcagcgccattgcctctggtgtcgccgtgtctaaagtgctgcacctggaaggcgaagtgaacaagatcaagagcgccctgctgagcaccaacaaggccgtggtgtctctgagcaatggcgtgtccgtgctgaccttcaaggtgctggacctgaagaactacatcgacaaacagctgctgcccatcctgaacaagcagtcctgcagcatccccaacatcgagacagtgatcgagttccagcagaagaacaaccggctgctggaaatcacccgcgagttctctgtgaatgccggcgtgaccacacctgtgtccacctacatgctgaccaacagcgagctgctgagcctgatcaacgacatgcccatcaccaacgaccagaaaaagctgatgagcaacaacgtgcagatcgtgcggcagcagagctacagcatcatgagcattatcaaagaagaggtgctggcctacgtggtgcagctgcctctgtatggcgtgatcgataccccttgctggaagctgcacacaagccctctgtgcaccaccaacaccaaagagggcagcaacatctgcctgaccagaaccgacagaggctggtactgcgataatgccggcagcgtctcattcttcccacaagccgagacatgcaaggtgcagagcaaccgggtgttctgcgacaccatgaatagcagaaccctgccttccgaagtgaatctgtgcaacgtggacatcttcaaccctaagtacgactgcaagatcatgaccagcaagaccgacgtgtccagcagtgtgatcacctcactgggcgccatcgtgtcctgttacggcaagaccaagtgcaccgccagcaacaagaaccggggcatcatcaagaccttcagcaacggctgcgactacgtgtccaacaaaggcgtggacaccgtgtctgtgggcaacaccctgtactacgtgaacaaacaagagggccagtcttgctacgtgaagggcgagcccatcatcaacttctacgaccctctggtgttccccagcgacgagttcgatgccagcatcagccaagtgaacgagaagatcaatcagagcctggccttcatcagaaagtccgatgagctgctgcacaacgtgaacgccggcaagtccaccaccaatatcatgatcacgaccatcatcatcgtgattatcgtgatcctgctgtccctgatcgccgtgggcctgctgctttattgataatag

SEQ ID NO: 80 - protein, 510 aa, synthetic construct
MELLILKANAITTILTAVTFCFASGQNITECFYQSTCSAVSKGYLGALRTGWYTSVITIELSNIKENKCNGTDAKVKLIKQELDKYKNAVTDLQLLMQSTPATGSGSAIASGVAVSKVLHLEGEVNKIKSALLSTNKAVVSLSNGVSVLTFKVLDLKNYIDKQLLPILNKQSCSIPNIETVIEFQQKNNRLLEITREFSVNAGVTTPVSTYMLTNSELLSLINDMPITNDQKKLMSNNVQIVRQQSYSIMSIIKEEVLAYVVQLPLYGVIDTPCWKLHTSPLCTTNTKEGSNICLTRTDRGWYCDNAGSVSFFPQAETCKVQSNRVFCDTMNSRTLPSEVNLCNVDIFNPKYDCKIMTSKTDVSSSVITSLGAIVSCYGKTKCTASNKNRGIIKTFSNGCDYVSNKGVDTVSVGNTLYYVNKQEGQSCYVKGEPIINFYDPLVFPSDEFDASISQVNEKINQSLAFIRKSDELLHNVNAGKSTTNIMITTIIIVIIVILLSLIAVGLLLY

SEQ ID NO: 81 - RNA, 1841 nt, synthetic construct
  source 1..1841: mol_type = other RNA
agcggctcggccattttgtcccagtcagtccggaggctgcggctgcagaagtaccgcctgcggagtaactgcaaaggccaccatggaactgctgatcctgaaggccaacgccatcaccaccatcctgaccgccgtgaccttctgttttgccagcggccagaacatcaccgagtgcttctaccagagcacctgtagcgccgtgtccaagggatatctgggcgcccttagaaccggctggtacaccagcgtgatcaccatcgagctgagcaacatcaaagaaaacaagtgcaacggcaccgacgccaaagtgaagctgatcaagcaagagctggacaagtacaagaatgccgtgaccgacctgcagctgctgatgcagtctacaccagccacaggctctggcagcgccattgcctctggtgtcgccgtgtctaaagtgctgcacctggaaggcgaagtgaacaagatcaagagcgccctgctgagcaccaacaaggccgtggtgtctctgagcaatggcgtgtccgtgctgaccttcaaggtgctggacctgaagaactacatcgacaaacagctgctgcccatcctgaacaagcagtcctgcagcatccccaacatcgagacagtgatcgagttccagcagaagaacaaccggctgctggaaatcacccgcgagttctctgtgaatgccggcgtgaccacacctgtgtccacctacatgctgaccaacagcgagctgctgagcctgatcaacgacatgcccatcaccaacgaccagaaaaagctgatgagcaacaacgtgcagatcgtgcggcagcagagctacagcatcatgagcattatcaaagaagaggtgctggcctacgtggtgcagctgcctctgtatggcgtgatcgataccccttgctggaagctgcacacaagccctctgtgcaccaccaacaccaaagagggcagcaacatctgcctgaccagaaccgacagaggctggtactgcgataatgccggcagcgtctcattcttcccacaagccgagacatgcaaggtgcagagcaaccgggtgttctgcgacaccatgaatagcagaaccctgccttccgaagtgaatctgtgcaacgtggacatcttcaaccctaagtacgactgcaagatcatgaccagcaagaccgacgtgtccagcagtgtgatcacctcactgggcgccatcgtgtcctgttacggcaagaccaagtgcaccgccagcaacaagaaccggggcatcatcaagaccttcagcaacggctgcgactacgtgtccaacaaaggcgtggacaccgtgtctgtgggcaacaccctgtactacgtgaacaaacaagagggccagtcttgctacgtgaagggcgagcccatcatcaacttctacgaccctctggtgttccccagcgacgagttcgatgccagcatcagccaagtgaacgagaagatcaatcagagcctggccttcatcagaaagtccgatgagctgctgcacaacgtgaacgccggcaagtccaccaccaatatcatgatcacgaccatcatcatcgtgattatcgtgatcctgctgtccctgatcgccgtgggcctgctgctttattgataataggctggagcctcggtggccatgcttcttgccccttgggcctccccccagcccctcctccccttcctgcacccgtacccccgtggtctttgaataaagtctgagtgggcggcaaaaaaaaaaaaaaaaaaaaaaaaaaaaaaaaaaaaaaaaaaaaaaaaaaaaaaaaaaaaaaaaaaaaaaaaaaaaaaaaaaaaaaaaaaaaaaaaaaaaaaaaaaaaaa

SEQ ID NO: 82 - DNA, 1841 bp, synthetic construct
  source 1..1841: mol_type = other DNA
agcggctcggccattttgtcccagtcagtccggaggctgcggctgcagaagtaccgcctgcggagtaactgcaaaggccaccatggaactgctgatcctgaaggccaacgccatcaccaccatcctgaccgccgtgaccttctgttttgccagcggccagaacatcaccgaggaatgctaccagagcacctgtagcgccgtgtccaagggatatctgggcgcccttagaaccggctggtacaccagcgtgatcaccatcgagctgagcaacatcaaagaaaacaagtgcaacggcaccgacgccaaagtgaagctgatcaagcaagagctggacaagtacaagaatgccgtgaccgacctgcagctgctgatgcagtctacaccagccacaggctctggcagcgccattgcctctggtgtcgccgtgtctaaagtgctgcacctggaaggcgaagtgaacaagatcaagagcgccctgctgagcaccaacaaggccgtggtgtctctgagcaatggcgtgtccgtgctgaccttcaaggtgctggacctgaagaactacatcgacaaacagctgctgcccatcctgaacaagcagtcctgcagcatccccaacatcgagacagtgatcgagttccagcagaagaacaaccggctgctggaaatcacccgcgagttctctgtgaatgccggcgtgaccacacctgtgtccacctacatgctgaccaacagcgagctgctgagcctgatcaacgacatgcccatcaccaacgaccagaaaaagctgatgagcaacaacgtgcagatcgtgcggcagcagagctacagcatcatgagcattatcaaagaagaggtgctggcctacgtggtgcagctgcctctgtatggcgtgatcgataccccttgctggaagctgcacacaagccctctgtgcaccaccaacaccaaagagggcagcaacatctgcctgaccagaaccgacagaggctggtactgcgataatgccggcagcgtctcattcttcccacaagccgagacatgcaaggtgcagagcaaccgggtgttctgcgacaccatgaatagcagaaccctgccttccgaagtgaatctgtgcaacgtggacatcttcaaccctaagtacgactgcaagatcatgaccagcaagaccgacgtgtccagcagtgtgatcacctcactgggcgccatcgtgtcctgttacggcaagaccaagtgcaccgccagcaacaagaaccggggcatcatcaagaccttcagcaacggctgcgactacgtgtccaacaaaggcgtggacaccgtgtctgtgggcaacaccctgtactacgtgaacaaacaagagggccagtctctgtgcgtgaagggcgagcccatcatcaacttctacgaccctctggtgttccccagcgacgagttcgatgccagcatcagccaagtgaacgagaagatcaatcagagcctggccttcatcagaaagtccgatgagctgctgcacaacgtgaacgccggcaagtccaccaccaatatcatgatcacgaccatcatcatcgtgattatcgtgatcctgctgtccctgatcgccgtgggcctgctgctttattgataataggctggagcctcggtggccatgcttcttgccccttgggcctccccccagcccctcctccccttcctgcacccgtacccccgtggtctttgaataaagtctgagtgggcggcaaaaaaaaaaaaaaaaaaaaaaaaaaaaaaaaaaaaaaaaaaaaaaaaaaaaaaaaaaaaaaaaaaaaaaaaaaaaaaaaaaaaaaaaaaaaaaaaaaaaaaaaaaaaaa

SEQ ID NO: 83 - DNA, 1539 bp, synthetic construct
  source 1..1539: mol_type = other DNA
atggaactgctgatcctgaaggccaacgccatcaccaccatcctgaccgccgtgaccttctgttttgccagcggccagaacatcaccgaggaatgctaccagagcacctgtagcgccgtgtccaagggatatctgggcgcccttagaaccggctggtacaccagcgtgatcaccatcgagctgagcaacatcaaagaaaacaagtgcaacggcaccgacgccaaagtgaagctgatcaagcaagagctggacaagtacaagaatgccgtgaccgacctgcagctgctgatgcagtctacaccagccacaggctctggcagcgccattgcctctggtgtcgccgtgtctaaagtgctgcacctggaaggcgaagtgaacaagatcaagagcgccctgctgagcaccaacaaggccgtggtgtctctgagcaatggcgtgtccgtgctgaccttcaaggtgctggacctgaagaactacatcgacaaacagctgctgcccatcctgaacaagcagtcctgcagcatccccaacatcgagacagtgatcgagttccagcagaagaacaaccggctgctggaaatcacccgcgagttctctgtgaatgccggcgtgaccacacctgtgtccacctacatgctgaccaacagcgagctgctgagcctgatcaacgacatgcccatcaccaacgaccagaaaaagctgatgagcaacaacgtgcagatcgtgcggcagcagagctacagcatcatgagcattatcaaagaagaggtgctggcctacgtggtgcagctgcctctgtatggcgtgatcgataccccttgctggaagctgcacacaagccctctgtgcaccaccaacaccaaagagggcagcaacatctgcctgaccagaaccgacagaggctggtactgcgataatgccggcagcgtctcattcttcccacaagccgagacatgcaaggtgcagagcaaccgggtgttctgcgacaccatgaatagcagaaccctgccttccgaagtgaatctgtgcaacgtggacatcttcaaccctaagtacgactgcaagatcatgaccagcaagaccgacgtgtccagcagtgtgatcacctcactgggcgccatcgtgtcctgttacggcaagaccaagtgcaccgccagcaacaagaaccggggcatcatcaagaccttcagcaacggctgcgactacgtgtccaacaaaggcgtggacaccgtgtctgtgggcaacaccctgtactacgtgaacaaacaagagggccagtctctgtgcgtgaagggcgagcccatcatcaacttctacgaccctctggtgttccccagcgacgagttcgatgccagcatcagccaagtgaacgagaagatcaatcagagcctggccttcatcagaaagtccgatgagctgctgcacaacgtgaacgccggcaagtccaccaccaatatcatgatcacgaccatcatcatcgtgattatcgtgatcctgctgtccctgatcgccgtgggcctgctgctttattgataatag

SEQ ID NO: 84 - protein, 510 aa, synthetic construct
MELLILKANAITTILTAVTFCFASGQNITEECYQSTCSAVSKGYLGALRTGWYTSVITIELSNIKENKCNGTDAKVKLIKQELDKYKNAVTDLQLLMQSTPATGSGSAIASGVAVSKVLHLEGEVNKIKSALLSTNKAVVSLSNGVSVLTFKVLDLKNYIDKQLLPILNKQSCSIPNIETVIEFQQKNNRLLEITREFSVNAGVTTPVSTYMLTNSELLSLINDMPITNDQKKLMSNNVQIVRQQSYSIMSIIKEEVLAYVVQLPLYGVIDTPCWKLHTSPLCTTNTKEGSNICLTRTDRGWYCDNAGSVSFFPQAETCKVQSNRVFCDTMNSRTLPSEVNLCNVDIFNPKYDCKIMTSKTDVSSSVITSLGAIVSCYGKTKCTASNKNRGIIKTFSNGCDYVSNKGVDTVSVGNTLYYVNKQEGQSLCVKGEPIINFYDPLVFPSDEFDASISQVNEKINQSLAFIRKSDELLHNVNAGKSTTNIMITTIIIVIIVILLSLIAVGLLLY

SEQ ID NO: 85 - RNA, 1841 nt, synthetic construct
  source 1..1841: mol_type = other RNA
agcggctcggccattttgtcccagtcagtccggaggctgcggctgcagaagtaccgcctgcggagtaactgcaaaggccaccatggaactgctgatcctgaaggccaacgccatcaccaccatcctgaccgccgtgaccttctgttttgccagcggccagaacatcaccgaggaatgctaccagagcacctgtagcgccgtgtccaagggatatctgggcgcccttagaaccggctggtacaccagcgtgatcaccatcgagctgagcaacatcaaagaaaacaagtgcaacggcaccgacgccaaagtgaagctgatcaagcaagagctggacaagtacaagaatgccgtgaccgacctgcagctgctgatgcagtctacaccagccacaggctctggcagcgccattgcctctggtgtcgccgtgtctaaagtgctgcacctggaaggcgaagtgaacaagatcaagagcgccctgctgagcaccaacaaggccgtggtgtctctgagcaatggcgtgtccgtgctgaccttcaaggtgctggacctgaagaactacatcgacaaacagctgctgcccatcctgaacaagcagtcctgcagcatccccaacatcgagacagtgatcgagttccagcagaagaacaaccggctgctggaaatcacccgcgagttctctgtgaatgccggcgtgaccacacctgtgtccacctacatgctgaccaacagcgagctgctgagcctgatcaacgacatgcccatcaccaacgaccagaaaaagctgatgagcaacaacgtgcagatcgtgcggcagcagagctacagcatcatgagcattatcaaagaagaggtgctggcctacgtggtgcagctgcctctgtatggcgtgatcgataccccttgctggaagctgcacacaagccctctgtgcaccaccaacaccaaagagggcagcaacatctgcctgaccagaaccgacagaggctggtactgcgataatgccggcagcgtctcattcttcccacaagccgagacatgcaaggtgcagagcaaccgggtgttctgcgacaccatgaatagcagaaccctgccttccgaagtgaatctgtgcaacgtggacatcttcaaccctaagtacgactgcaagatcatgaccagcaagaccgacgtgtccagcagtgtgatcacctcactgggcgccatcgtgtcctgttacggcaagaccaagtgcaccgccagcaacaagaaccggggcatcatcaagaccttcagcaacggctgcgactacgtgtccaacaaaggcgtggacaccgtgtctgtgggcaacaccctgtactacgtgaacaaacaagagggccagtctctgtgcgtgaagggcgagcccatcatcaacttctacgaccctctggtgttccccagcgacgagttcgatgccagcatcagccaagtgaacgagaagatcaatcagagcctggccttcatcagaaagtccgatgagctgctgcacaacgtgaacgccggcaagtccaccaccaatatcatgatcacgaccatcatcatcgtgattatcgtgatcctgctgtccctgatcgccgtgggcctgctgctttattgataataggctggagcctcggtggccatgcttcttgccccttgggcctccccccagcccctcctccccttcctgcacccgtacccccgtggtctttgaataaagtctgagtgggcggcaaaaaaaaaaaaaaaaaaaaaaaaaaaaaaaaaaaaaaaaaaaaaaaaaaaaaaaaaaaaaaaaaaaaaaaaaaaaaaaaaaaaaaaaaaaaaaaaaaaaaaaaaaaaaa

SEQ ID NO: 86 - DNA, 1841 bp, synthetic construct
  source 1..1841: mol_type = other DNA
agcggctcggccattttgtcccagtcagtccggaggctgcggctgcagaagtaccgcctgcggagtaactgcaaaggccaccatggaactgctgatcctgaaggccaacgccatcaccaccatcctgaccgccgtgaccttctgttttgccagcggccagaacatcaccgaggaattctactgcagcacctgtagcgccgtgtccaagggatatctgggcgcccttagaaccggctggtacaccagcgtgatcaccatcgagctgagcaacatcaaagaaaacaagtgcaacggcaccgacgccaaagtgaagctgatcaagcaagagctggacaagtacaagaatgccgtgaccgacctgcagctgctgatgcagtctacaccagccacaggctctggcagcgccattgcctctggtgtcgccgtgtctaaagtgctgcacctggaaggcgaagtgaacaagatcaagagcgccctgctgagcaccaacaaggccgtggtgtctctgagcaatggcgtgtccgtgctgaccttcaaggtgctggacctgaagaactacatcgacaaacagctgctgcccatcctgaacaagcagtcctgcagcatccccaacatcgagacagtgatcgagttccagcagaagaacaaccggctgctggaaatcacccgcgagttctctgtgaatgccggcgtgaccacacctgtgtccacctacatgctgaccaacagcgagctgctgagcctgatcaacgacatgcccatcaccaacgaccagaaaaagctgatgagcaacaacgtgcagatcgtgcggcagcagagctacagcatcatgagcattatcaaagaagaggtgctggcctacgtggtgcagctgcctctgtatggcgtgatcgataccccttgctggaagctgcacacaagccctctgtgcaccaccaacaccaaagagggcagcaacatctgcctgaccagaaccgacagaggctggtactgcgataatgccggcagcgtctcattcttcccacaagccgagacatgcaaggtgcagagcaaccgggtgttctgcgacaccatgaatagcagaaccctgccttccgaagtgaatctgtgcaacgtggacatcttcaaccctaagtacgactgcaagatcatgaccagcaagaccgacgtgtccagcagtgtgatcacctcactgggcgccatcgtgtcctgttacggcaagaccaagtgcaccgccagcaacaagaaccggggcatcatcaagaccttcagcaacggctgcgactacgtgtccaacaaaggcgtggacaccgtgtctgtgggcaacaccctgtactacgtgaacaaacaagagggccagtctctgtacgtgtgcggcgagcccatcatcaacttctacgaccctctggtgttccccagcgacgagttcgatgccagcatcagccaagtgaacgagaagatcaatcagagcctggccttcatcagaaagtccgatgagctgctgcacaacgtgaacgccggcaagtccaccaccaatatcatgatcacgaccatcatcatcgtgattatcgtgatcctgctgtccctgatcgccgtgggcctgctgctttattgataataggctggagcctcggtggccatgcttcttgccccttgggcctccccccagcccctcctccccttcctgcacccgtacccccgtggtctttgaataaagtctgagtgggcggcaaaaaaaaaaaaaaaaaaaaaaaaaaaaaaaaaaaaaaaaaaaaaaaaaaaaaaaaaaaaaaaaaaaaaaaaaaaaaaaaaaaaaaaaaaaaaaaaaaaaaaaaaaaaaa

SEQ ID NO: 87 - DNA, 1539 bp, synthetic construct
  source 1..1539: mol_type = other DNA
atggaactgctgatcctgaaggccaacgccatcaccaccatcctgaccgccgtgaccttctgttttgccagcggccagaacatcaccgaggaattctactgcagcacctgtagcgccgtgtccaagggatatctgggcgcccttagaaccggctggtacaccagcgtgatcaccatcgagctgagcaacatcaaagaaaacaagtgcaacggcaccgacgccaaagtgaagctgatcaagcaagagctggacaagtacaagaatgccgtgaccgacctgcagctgctgatgcagtctacaccagccacaggctctggcagcgccattgcctctggtgtcgccgtgtctaaagtgctgcacctggaaggcgaagtgaacaagatcaagagcgccctgctgagcaccaacaaggccgtggtgtctctgagcaatggcgtgtccgtgctgaccttcaaggtgctggacctgaagaactacatcgacaaacagctgctgcccatcctgaacaagcagtcctgcagcatccccaacatcgagacagtgatcgagttccagcagaagaacaaccggctgctggaaatcacccgcgagttctctgtgaatgccggcgtgaccacacctgtgtccacctacatgctgaccaacagcgagctgctgagcctgatcaacgacatgcccatcaccaacgaccagaaaaagctgatgagcaacaacgtgcagatcgtgcggcagcagagctacagcatcatgagcattatcaaagaagaggtgctggcctacgtggtgcagctgcctctgtatggcgtgatcgataccccttgctggaagctgcacacaagccctctgtgcaccaccaacaccaaagagggcagcaacatctgcctgaccagaaccgacagaggctggtactgcgataatgccggcagcgtctcattcttcccacaagccgagacatgcaaggtgcagagcaaccgggtgttctgcgacaccatgaatagcagaaccctgccttccgaagtgaatctgtgcaacgtggacatcttcaaccctaagtacgactgcaagatcatgaccagcaagaccgacgtgtccagcagtgtgatcacctcactgggcgccatcgtgtcctgttacggcaagaccaagtgcaccgccagcaacaagaaccggggcatcatcaagaccttcagcaacggctgcgactacgtgtccaacaaaggcgtggacaccgtgtctgtgggcaacaccctgtactacgtgaacaaacaagagggccagtctctgtacgtgtgcggcgagcccatcatcaacttctacgaccctctggtgttccccagcgacgagttcgatgccagcatcagccaagtgaacgagaagatcaatcagagcctggccttcatcagaaagtccgatgagctgctgcacaacgtgaacgccggcaagtccaccaccaatatcatgatcacgaccatcatcatcgtgattatcgtgatcctgctgtccctgatcgccgtgggcctgctgctttattgataatag

SEQ ID NO: 88 - protein, 510 aa, synthetic construct
MELLILKANAITTILTAVTFCFASGQNITEEFYCSTCSAVSKGYLGALRTGWYTSVITIELSNIKENKCNGTDAKVKLIKQELDKYKNAVTDLQLLMQSTPATGSGSAIASGVAVSKVLHLEGEVNKIKSALLSTNKAVVSLSNGVSVLTFKVLDLKNYIDKQLLPILNKQSCSIPNIETVIEFQQKNNRLLEITREFSVNAGVTTPVSTYMLTNSELLSLINDMPITNDQKKLMSNNVQIVRQQSYSIMSIIKEEVLAYVVQLPLYGVIDTPCWKLHTSPLCTTNTKEGSNICLTRTDRGWYCDNAGSVSFFPQAETCKVQSNRVFCDTMNSRTLPSEVNLCNVDIFNPKYDCKIMTSKTDVSSSVITSLGAIVSCYGKTKCTASNKNRGIIKTFSNGCDYVSNKGVDTVSVGNTLYYVNKQEGQSLYVCGEPIINFYDPLVFPSDEFDASISQVNEKINQSLAFIRKSDELLHNVNAGKSTTNIMITTIIIVIIVILLSLIAVGLLLY

SEQ ID NO: 89 - RNA, 1841 nt, synthetic construct
  source 1..1841: mol_type = other RNA
agcggctcggccattttgtcccagtcagtccggaggctgcggctgcagaagtaccgcctgcggagtaactgcaaaggccaccatggaactgctgatcctgaaggccaacgccatcaccaccatcctgaccgccgtgaccttctgttttgccagcggccagaacatcaccgaggaattctactgcagcacctgtagcgccgtgtccaagggatatctgggcgcccttagaaccggctggtacaccagcgtgatcaccatcgagctgagcaacatcaaagaaaacaagtgcaacggcaccgacgccaaagtgaagctgatcaagcaagagctggacaagtacaagaatgccgtgaccgacctgcagctgctgatgcagtctacaccagccacaggctctggcagcgccattgcctctggtgtcgccgtgtctaaagtgctgcacctggaaggcgaagtgaacaagatcaagagcgccctgctgagcaccaacaaggccgtggtgtctctgagcaatggcgtgtccgtgctgaccttcaaggtgctggacctgaagaactacatcgacaaacagctgctgcccatcctgaacaagcagtcctgcagcatccccaacatcgagacagtgatcgagttccagcagaagaacaaccggctgctggaaatcacccgcgagttctctgtgaatgccggcgtgaccacacctgtgtccacctacatgctgaccaacagcgagctgctgagcctgatcaacgacatgcccatcaccaacgaccagaaaaagctgatgagcaacaacgtgcagatcgtgcggcagcagagctacagcatcatgagcattatcaaagaagaggtgctggcctacgtggtgcagctgcctctgtatggcgtgatcgataccccttgctggaagctgcacacaagccctctgtgcaccaccaacaccaaagagggcagcaacatctgcctgaccagaaccgacagaggctggtactgcgataatgccggcagcgtctcattcttcccacaagccgagacatgcaaggtgcagagcaaccgggtgttctgcgacaccatgaatagcagaaccctgccttccgaagtgaatctgtgcaacgtggacatcttcaaccctaagtacgactgcaagatcatgaccagcaagaccgacgtgtccagcagtgtgatcacctcactgggcgccatcgtgtcctgttacggcaagaccaagtgcaccgccagcaacaagaaccggggcatcatcaagaccttcagcaacggctgcgactacgtgtccaacaaaggcgtggacaccgtgtctgtgggcaacaccctgtactacgtgaacaaacaagagggccagtctctgtacgtgtgcggcgagcccatcatcaacttctacgaccctctggtgttccccagcgacgagttcgatgccagcatcagccaagtgaacgagaagatcaatcagagcctggccttcatcagaaagtccgatgagctgctgcacaacgtgaacgccggcaagtccaccaccaatatcatgatcacgaccatcatcatcgtgattatcgtgatcctgctgtccctgatcgccgtgggcctgctgctttattgataataggctggagcctcggtggccatgcttcttgccccttgggcctccccccagcccctcctccccttcctgcacccgtacccccgtggtctttgaataaagtctgagtgggcggcaaaaaaaaaaaaaaaaaaaaaaaaaaaaaaaaaaaaaaaaaaaaaaaaaaaaaaaaaaaaaaaaaaaaaaaaaaaaaaaaaaaaaaaaaaaaaaaaaaaaaaaaaaaaaa

SEQ ID NO: 90 - DNA, 1841 bp, synthetic construct
  source 1..1841: mol_type = other DNA
agcggctcggccattttgtcccagtcagtccggaggctgcggctgcagaagtaccgcctgcggagtaactgcaaaggccaccatggaactgctgatcctgaaggccaacgccatcaccaccatcctgaccgccgtgaccttctgttttgccagcggccagaacatcaccgaggaattctaccagagctgctgtagcgccgtgtccaagggatatctgggcgcccttagaaccggctggtacaccagcgtgatcaccatcgagctgagcaacatcaaagaaaacaagtgcaacggcaccgacgccaaagtgaagctgatcaagcaagagctggacaagtacaagaatgccgtgaccgacctgcagctgctgatgcagtctacaccagccacaggctctggcagcgccattgcctctggtgtcgccgtgtctaaagtgctgcacctggaaggcgaagtgaacaagatcaagagcgccctgctgagcaccaacaaggccgtggtgtctctgagcaatggcgtgtccgtgctgaccttcaaggtgctggacctgaagaactacatcgacaaacagctgctgcccatcctgaacaagcagtcctgcagcatccccaacatcgagacagtgatcgagttccagcagaagaacaaccggctgctggaaatcacccgcgagttctctgtgaatgccggcgtgaccacacctgtgtccacctacatgctgaccaacagcgagctgctgagcctgatcaacgacatgcccatcaccaacgaccagaaaaagctgatgagcaacaacgtgcagatcgtgcggcagcagagctacagcatcatgagcattatcaaagaagaggtgctggcctacgtggtgcagctgcctctgtatggcgtgatcgataccccttgctggaagctgcacacaagccctctgtgcaccaccaacaccaaagagggcagcaacatctgcctgaccagaaccgacagaggctggtactgcgataatgccggcagcgtctcattcttcccacaagccgagacatgcaaggtgcagagcaaccgggtgttctgcgacaccatgaatagcagaaccctgccttccgaagtgaatctgtgcaacgtggacatcttcaaccctaagtacgactgcaagatcatgaccagcaagaccgacgtgtccagcagtgtgatcacctcactgggcgccatcgtgtcctgttacggcaagaccaagtgcaccgccagcaacaagaaccggggcatcatcaagaccttcagcaacggctgcgactacgtgtccaacaaaggcgtggacaccgtgtctgtgggcaacaccctgtactacgtgaacaaacaagagggccagtctctgtacgtgaagtgcgagcccatcatcaacttctacgaccctctggtgttccccagcgacgagttcgatgccagcatcagccaagtgaacgagaagatcaatcagagcctggccttcatcagaaagtccgatgagctgctgcacaacgtgaacgccggcaagtccaccaccaatatcatgatcacgaccatcatcatcgtgattatcgtgatcctgctgtccctgatcgccgtgggcctgctgctttattgataataggctggagcctcggtggccatgcttcttgccccttgggcctccccccagcccctcctccccttcctgcacccgtacccccgtggtctttgaataaagtctgagtgggcggcaaaaaaaaaaaaaaaaaaaaaaaaaaaaaaaaaaaaaaaaaaaaaaaaaaaaaaaaaaaaaaaaaaaaaaaaaaaaaaaaaaaaaaaaaaaaaaaaaaaaaaaaaaaaaa

SEQ ID NO: 91 - DNA, 1539 bp, synthetic construct
  source 1..1539: mol_type = other DNA
atggaactgctgatcctgaaggccaacgccatcaccaccatcctgaccgccgtgaccttctgttttgccagcggccagaacatcaccgaggaattctaccagagctgctgtagcgccgtgtccaagggatatctgggcgcccttagaaccggctggtacaccagcgtgatcaccatcgagctgagcaacatcaaagaaaacaagtgcaacggcaccgacgccaaagtgaagctgatcaagcaagagctggacaagtacaagaatgccgtgaccgacctgcagctgctgatgcagtctacaccagccacaggctctggcagcgccattgcctctggtgtcgccgtgtctaaagtgctgcacctggaaggcgaagtgaacaagatcaagagcgccctgctgagcaccaacaaggccgtggtgtctctgagcaatggcgtgtccgtgctgaccttcaaggtgctggacctgaagaactacatcgacaaacagctgctgcccatcctgaacaagcagtcctgcagcatccccaacatcgagacagtgatcgagttccagcagaagaacaaccggctgctggaaatcacccgcgagttctctgtgaatgccggcgtgaccacacctgtgtccacctacatgctgaccaacagcgagctgctgagcctgatcaacgacatgcccatcaccaacgaccagaaaaagctgatgagcaacaacgtgcagatcgtgcggcagcagagctacagcatcatgagcattatcaaagaagaggtgctggcctacgtggtgcagctgcctctgtatggcgtgatcgataccccttgctggaagctgcacacaagccctctgtgcaccaccaacaccaaagagggcagcaacatctgcctgaccagaaccgacagaggctggtactgcgataatgccggcagcgtctcattcttcccacaagccgagacatgcaaggtgcagagcaaccgggtgttctgcgacaccatgaatagcagaaccctgccttccgaagtgaatctgtgcaacgtggacatcttcaaccctaagtacgactgcaagatcatgaccagcaagaccgacgtgtccagcagtgtgatcacctcactgggcgccatcgtgtcctgttacggcaagaccaagtgcaccgccagcaacaagaaccggggcatcatcaagaccttcagcaacggctgcgactacgtgtccaacaaaggcgtggacaccgtgtctgtgggcaacaccctgtactacgtgaacaaacaagagggccagtctctgtacgtgaagtgcgagcccatcatcaacttctacgaccctctggtgttccccagcgacgagttcgatgccagcatcagccaagtgaacgagaagatcaatcagagcctggccttcatcagaaagtccgatgagctgctgcacaacgtgaacgccggcaagtccaccaccaatatcatgatcacgaccatcatcatcgtgattatcgtgatcctgctgtccctgatcgccgtgggcctgctgctttattgataatag

SEQ ID NO: 92 - protein, 510 aa, synthetic construct
MELLILKANAITTILTAVTFCFASGQNITEEFYQSCCSAVSKGYLGALRTGWYTSVITIELSNIKENKCNGTDAKVKLIKQELDKYKNAVTDLQLLMQSTPATGSGSAIASGVAVSKVLHLEGEVNKIKSALLSTNKAVVSLSNGVSVLTFKVLDLKNYIDKQLLPILNKQSCSIPNIETVIEFQQKNNRLLEITREFSVNAGVTTPVSTYMLTNSELLSLINDMPITNDQKKLMSNNVQIVRQQSYSIMSIIKEEVLAYVVQLPLYGVIDTPCWKLHTSPLCTTNTKEGSNICLTRTDRGWYCDNAGSVSFFPQAETCKVQSNRVFCDTMNSRTLPSEVNLCNVDIFNPKYDCKIMTSKTDVSSSVITSLGAIVSCYGKTKCTASNKNRGIIKTFSNGCDYVSNKGVDTVSVGNTLYYVNKQEGQSLYVKCEPIINFYDPLVFPSDEFDASISQVNEKINQSLAFIRKSDELLHNVNAGKSTTNIMITTIIIVIIVILLSLIAVGLLLY

SEQ ID NO: 93 - RNA, 1841 nt, synthetic construct
  source 1..1841: mol_type = other RNA
agcggctcggccattttgtcccagtcagtccggaggctgcggctgcagaagtaccgcctgcggagtaactgcaaaggccaccatggaactgctgatcctgaaggccaacgccatcaccaccatcctgaccgccgtgaccttctgttttgccagcggccagaacatcaccgaggaattctaccagagctgctgtagcgccgtgtccaagggatatctgggcgcccttagaaccggctggtacaccagcgtgatcaccatcgagctgagcaacatcaaagaaaacaagtgcaacggcaccgacgccaaagtgaagctgatcaagcaagagctggacaagtacaagaatgccgtgaccgacctgcagctgctgatgcagtctacaccagccacaggctctggcagcgccattgcctctggtgtcgccgtgtctaaagtgctgcacctggaaggcgaagtgaacaagatcaagagcgccctgctgagcaccaacaaggccgtggtgtctctgagcaatggcgtgtccgtgctgaccttcaaggtgctggacctgaagaactacatcgacaaacagctgctgcccatcctgaacaagcagtcctgcagcatccccaacatcgagacagtgatcgagttccagcagaagaacaaccggctgctggaaatcacccgcgagttctctgtgaatgccggcgtgaccacacctgtgtccacctacatgctgaccaacagcgagctgctgagcctgatcaacgacatgcccatcaccaacgaccagaaaaagctgatgagcaacaacgtgcagatcgtgcggcagcagagctacagcatcatgagcattatcaaagaagaggtgctggcctacgtggtgcagctgcctctgtatggcgtgatcgataccccttgctggaagctgcacacaagccctctgtgcaccaccaacaccaaagagggcagcaacatctgcctgaccagaaccgacagaggctggtactgcgataatgccggcagcgtctcattcttcccacaagccgagacatgcaaggtgcagagcaaccgggtgttctgcgacaccatgaatagcagaaccctgccttccgaagtgaatctgtgcaacgtggacatcttcaaccctaagtacgactgcaagatcatgaccagcaagaccgacgtgtccagcagtgtgatcacctcactgggcgccatcgtgtcctgttacggcaagaccaagtgcaccgccagcaacaagaaccggggcatcatcaagaccttcagcaacggctgcgactacgtgtccaacaaaggcgtggacaccgtgtctgtgggcaacaccctgtactacgtgaacaaacaagagggccagtctctgtacgtgaagtgcgagcccatcatcaacttctacgaccctctggtgttccccagcgacgagttcgatgccagcatcagccaagtgaacgagaagatcaatcagagcctggccttcatcagaaagtccgatgagctgctgcacaacgtgaacgccggcaagtccaccaccaatatcatgatcacgaccatcatcatcgtgattatcgtgatcctgctgtccctgatcgccgtgggcctgctgctttattgataataggctggagcctcggtggccatgcttcttgccccttgggcctccccccagcccctcctccccttcctgcacccgtacccccgtggtctttgaataaagtctgagtgggcggcaaaaaaaaaaaaaaaaaaaaaaaaaaaaaaaaaaaaaaaaaaaaaaaaaaaaaaaaaaaaaaaaaaaaaaaaaaaaaaaaaaaaaaaaaaaaaaaaaaaaaaaaaaaaaa

SEQ ID NO: 94 - DNA, 1841 bp, synthetic construct
  source 1..1841: mol_type = other DNA
agcggctcggccattttgtcccagtcagtccggaggctgcggctgcagaagtaccgcctgcggagtaactgcaaaggccaccatggaactgctgatcctgaaggccaacgccatcaccaccatcctgaccgccgtgaccttctgttttgccagcggctgcaacatcaccgaggaattctaccagagcacctgtagcgccgtgtccaagggatatctgggcgcccttagaaccggctggtacaccagcgtgatcaccatcgagctgagcaacatcaaagaaaacaagtgcaacggcaccgacgccaaagtgaagctgatcaagcaagagctggacaagtacaagaatgccgtgaccgacctgcagctgctgatgcagtctacaccagccacaggctctggcagcgccattgcctctggtgtcgccgtgtctaaagtgctgcacctggaaggcgaagtgaacaagatcaagagcgccctgctgagcaccaacaaggccgtggtgtctctgagcaatggcgtgtccgtgctgaccttcaaggtgctggacctgaagaactacatcgacaaacagctgctgcccatcctgaacaagcagtcctgcagcatccccaacatcgagacagtgatcgagttccagcagaagaacaaccggctgctggaaatcacccgcgagttctctgtgaatgccggcgtgaccacacctgtgtccacctacatgctgaccaacagcgagctgctgagcctgatcaacgacatgcccatcaccaacgaccagaaaaagctgatgagcaacaacgtgcagatcgtgcggcagcagagctacagcatcatgagcattatcaaagaagaggtgctggcctacgtggtgcagctgcctctgtatggcgtgatcgataccccttgctggaagctgcacacaagccctctgtgcaccaccaacaccaaagagggcagcaacatctgcctgaccagaaccgacagaggctggtactgcgataatgccggcagcgtctcattcttcccacaagccgagacatgcaaggtgcagagcaaccgggtgttctgcgacaccatgaatagcagaaccctgccttccgaagtgaatctgtgcaacgtggacatcttcaaccctaagtacgactgcaagatcatgaccagcaagaccgacgtgtccagcagtgtgatcacctcactgggcgccatcgtgtcctgttacggcaagaccaagtgcaccgccagcaacaagaaccggggcatcatcaagaccttcagcaacggctgcgactacgtgtccaacaaaggcgtggacaccgtgtctgtgggcaacaccctgtactacgtgaactgccaagagggccagtctctgtacgtgaagggcgagcccatcatcaacttctacgaccctctggtgttccccagcgacgagttcgatgccagcatcagccaagtgaacgagaagatcaatcagagcctggccttcatcagaaagtccgatgagctgctgcacaacgtgaacgccggcaagtccaccaccaatatcatgatcacgaccatcatcatcgtgattatcgtgatcctgctgtccctgatcgccgtgggcctgctgctttattgataataggctggagcctcggtggccatgcttcttgccccttgggcctccccccagcccctcctccccttcctgcacccgtacccccgtggtctttgaataaagtctgagtgggcggcaaaaaaaaaaaaaaaaaaaaaaaaaaaaaaaaaaaaaaaaaaaaaaaaaaaaaaaaaaaaaaaaaaaaaaaaaaaaaaaaaaaaaaaaaaaaaaaaaaaaaaaaaaaaaa

SEQ ID NO: 95 - DNA, 1539 bp, synthetic construct
  source 1..1539: mol_type = other DNA
atggaactgctgatcctgaaggccaacgccatcaccaccatcctgaccgccgtgaccttctgttttgccagcggctgcaacatcaccgaggaattctaccagagcacctgtagcgccgtgtccaagggatatctgggcgcccttagaaccggctggtacaccagcgtgatcaccatcgagctgagcaacatcaaagaaaacaagtgcaacggcaccgacgccaaagtgaagctgatcaagcaagagctggacaagtacaagaatgccgtgaccgacctgcagctgctgatgcagtctacaccagccacaggctctggcagcgccattgcctctggtgtcgccgtgtctaaagtgctgcacctggaaggcgaagtgaacaagatcaagagcgccctgctgagcaccaacaaggccgtggtgtctctgagcaatggcgtgtccgtgctgaccttcaaggtgctggacctgaagaactacatcgacaaacagctgctgcccatcctgaacaagcagtcctgcagcatccccaacatcgagacagtgatcgagttccagcagaagaacaaccggctgctggaaatcacccgcgagttctctgtgaatgccggcgtgaccacacctgtgtccacctacatgctgaccaacagcgagctgctgagcctgatcaacgacatgcccatcaccaacgaccagaaaaagctgatgagcaacaacgtgcagatcgtgcggcagcagagctacagcatcatgagcattatcaaagaagaggtgctggcctacgtggtgcagctgcctctgtatggcgtgatcgataccccttgctggaagctgcacacaagccctctgtgcaccaccaacaccaaagagggcagcaacatctgcctgaccagaaccgacagaggctggtactgcgataatgccggcagcgtctcattcttcccacaagccgagacatgcaaggtgcagagcaaccgggtgttctgcgacaccatgaatagcagaaccctgccttccgaagtgaatctgtgcaacgtggacatcttcaaccctaagtacgactgcaagatcatgaccagcaagaccgacgtgtccagcagtgtgatcacctcactgggcgccatcgtgtcctgttacggcaagaccaagtgcaccgccagcaacaagaaccggggcatcatcaagaccttcagcaacggctgcgactacgtgtccaacaaaggcgtggacaccgtgtctgtgggcaacaccctgtactacgtgaactgccaagagggccagtctctgtacgtgaagggcgagcccatcatcaacttctacgaccctctggtgttccccagcgacgagttcgatgccagcatcagccaagtgaacgagaagatcaatcagagcctggccttcatcagaaagtccgatgagctgctgcacaacgtgaacgccggcaagtccaccaccaatatcatgatcacgaccatcatcatcgtgattatcgtgatcctgctgtccctgatcgccgtgggcctgctgctttattgataatag

SEQ ID NO: 96 - protein, 510 aa, synthetic construct
MELLILKANAITTILTAVTFCFASGCNITEEFYQSTCSAVSKGYLGALRTGWYTSVITIELSNIKENKCNGTDAKVKLIKQELDKYKNAVTDLQLLMQSTPATGSGSAIASGVAVSKVLHLEGEVNKIKSALLSTNKAVVSLSNGVSVLTFKVLDLKNYIDKQLLPILNKQSCSIPNIETVIEFQQKNNRLLEITREFSVNAGVTTPVSTYMLTNSELLSLINDMPITNDQKKLMSNNVQIVRQQSYSIMSIIKEEVLAYVVQLPLYGVIDTPCWKLHTSPLCTTNTKEGSNICLTRTDRGWYCDNAGSVSFFPQAETCKVQSNRVFCDTMNSRTLPSEVNLCNVDIFNPKYDCKIMTSKTDVSSSVITSLGAIVSCYGKTKCTASNKNRGIIKTFSNGCDYVSNKGVDTVSVGNTLYYVNCQEGQSLYVKGEPIINFYDPLVFPSDEFDASISQVNEKINQSLAFIRKSDELLHNVNAGKSTTNIMITTIIIVIIVILLSLIAVGLLLY

SEQ ID NO: 97 - RNA, 1841 nt, synthetic construct
  source 1..1841: mol_type = other RNA
agcggctcggccattttgtcccagtcagtccggaggctgcggctgcagaagtaccgcctgcggagtaactgcaaaggccaccatggaactgctgatcctgaaggccaacgccatcaccaccatcctgaccgccgtgaccttctgttttgccagcggctgcaacatcaccgaggaattctaccagagcacctgtagcgccgtgtccaagggatatctgggcgcccttagaaccggctggtacaccagcgtgatcaccatcgagctgagcaacatcaaagaaaacaagtgcaacggcaccgacgccaaagtgaagctgatcaagcaagagctggacaagtacaagaatgccgtgaccgacctgcagctgctgatgcagtctacaccagccacaggctctggcagcgccattgcctctggtgtcgccgtgtctaaagtgctgcacctggaaggcgaagtgaacaagatcaagagcgccctgctgagcaccaacaaggccgtggtgtctctgagcaatggcgtgtccgtgctgaccttcaaggtgctggacctgaagaactacatcgacaaacagctgctgcccatcctgaacaagcagtcctgcagcatccccaacatcgagacagtgatcgagttccagcagaagaacaaccggctgctggaaatcacccgcgagttctctgtgaatgccggcgtgaccacacctgtgtccacctacatgctgaccaacagcgagctgctgagcctgatcaacgacatgcccatcaccaacgaccagaaaaagctgatgagcaacaacgtgcagatcgtgcggcagcagagctacagcatcatgagcattatcaaagaagaggtgctggcctacgtggtgcagctgcctctgtatggcgtgatcgataccccttgctggaagctgcacacaagccctctgtgcaccaccaacaccaaagagggcagcaacatctgcctgaccagaaccgacagaggctggtactgcgataatgccggcagcgtctcattcttcccacaagccgagacatgcaaggtgcagagcaaccgggtgttctgcgacaccatgaatagcagaaccctgccttccgaagtgaatctgtgcaacgtggacatcttcaaccctaagtacgactgcaagatcatgaccagcaagaccgacgtgtccagcagtgtgatcacctcactgggcgccatcgtgtcctgttacggcaagaccaagtgcaccgccagcaacaagaaccggggcatcatcaagaccttcagcaacggctgcgactacgtgtccaacaaaggcgtggacaccgtgtctgtgggcaacaccctgtactacgtgaactgccaagagggccagtctctgtacgtgaagggcgagcccatcatcaacttctacgaccctctggtgttccccagcgacgagttcgatgccagcatcagccaagtgaacgagaagatcaatcagagcctggccttcatcagaaagtccgatgagctgctgcacaacgtgaacgccggcaagtccaccaccaatatcatgatcacgaccatcatcatcgtgattatcgtgatcctgctgtccctgatcgccgtgggcctgctgctttattgataataggctggagcctcggtggccatgcttcttgccccttgggcctccccccagcccctcctccccttcctgcacccgtacccccgtggtctttgaataaagtctgagtgggcggcaaaaaaaaaaaaaaaaaaaaaaaaaaaaaaaaaaaaaaaaaaaaaaaaaaaaaaaaaaaaaaaaaaaaaaaaaaaaaaaaaaaaaaaaaaaaaaaaaaaaaaaaaaaaaa

SEQ ID NO: 98 - DNA, 1841 bp, synthetic construct
  source 1..1841: mol_type = other DNA
agcggctcggccattttgtcccagtcagtccggaggctgcggctgcagaagtaccgcctgcggagtaactgcaaaggccaccatggaactgctgatcctgaaggccaacgccatcaccaccatcctgaccgccgtgaccttctgttttgccagcggccagtgcatcaccgaggaattctaccagagcacctgtagcgccgtgtccaagggatatctgggcgcccttagaaccggctggtacaccagcgtgatcaccatcgagctgagcaacatcaaagaaaacaagtgcaacggcaccgacgccaaagtgaagctgatcaagcaagagctggacaagtacaagaatgccgtgaccgacctgcagctgctgatgcagtctacaccagccacaggctctggcagcgccattgcctctggtgtcgccgtgtctaaagtgctgcacctggaaggcgaagtgaacaagatcaagagcgccctgctgagcaccaacaaggccgtggtgtctctgagcaatggcgtgtccgtgctgaccttcaaggtgctggacctgaagaactacatcgacaaacagctgctgcccatcctgaacaagcagtcctgcagcatccccaacatcgagacagtgatcgagttccagcagaagaacaaccggctgctggaaatcacccgcgagttctctgtgaatgccggcgtgaccacacctgtgtccacctacatgctgaccaacagcgagctgctgagcctgatcaacgacatgcccatcaccaacgaccagaaaaagctgatgagcaacaacgtgcagatcgtgcggcagcagagctacagcatcatgagcattatcaaagaagaggtgctggcctacgtggtgcagctgcctctgtatggcgtgatcgataccccttgctggaagctgcacacaagccctctgtgcaccaccaacaccaaagagggcagcaacatctgcctgaccagaaccgacagaggctggtactgcgataatgccggcagcgtctcattcttcccacaagccgagacatgcaaggtgcagagcaaccgggtgttctgcgacaccatgaatagcagaaccctgccttccgaagtgaatctgtgcaacgtggacatcttcaaccctaagtacgactgcaagatcatgaccagcaagaccgacgtgtccagcagtgtgatcacctcactgggcgccatcgtgtcctgttacggcaagaccaagtgcaccgccagcaacaagaaccggggcatcatcaagaccttcagcaacggctgcgactacgtgtccaacaaaggcgtggacaccgtgtctgtgggcaacaccctgtactacgtgaacaaatgcgagggccagtctctgtacgtgaagggcgagcccatcatcaacttctacgaccctctggtgttccccagcgacgagttcgatgccagcatcagccaagtgaacgagaagatcaatcagagcctggccttcatcagaaagtccgatgagctgctgcacaacgtgaacgccggcaagtccaccaccaatatcatgatcacgaccatcatcatcgtgattatcgtgatcctgctgtccctgatcgccgtgggcctgctgctttattgataataggctggagcctcggtggccatgcttcttgccccttgggcctccccccagcccctcctccccttcctgcacccgtacccccgtggtctttgaataaagtctgagtgggcggcaaaaaaaaaaaaaaaaaaaaaaaaaaaaaaaaaaaaaaaaaaaaaaaaaaaaaaaaaaaaaaaaaaaaaaaaaaaaaaaaaaaaaaaaaaaaaaaaaaaaaaaaaaaaaa

SEQ ID NO: 99 - DNA, 1539 bp, synthetic construct
  source 1..1539: mol_type = other DNA
atggaactgctgatcctgaaggccaacgccatcaccaccatcctgaccgccgtgaccttctgttttgccagcggccagtgcatcaccgaggaattctaccagagcacctgtagcgccgtgtccaagggatatctgggcgcccttagaaccggctggtacaccagcgtgatcaccatcgagctgagcaacatcaaagaaaacaagtgcaacggcaccgacgccaaagtgaagctgatcaagcaagagctggacaagtacaagaatgccgtgaccgacctgcagctgctgatgcagtctacaccagccacaggctctggcagcgccattgcctctggtgtcgccgtgtctaaagtgctgcacctggaaggcgaagtgaacaagatcaagagcgccctgctgagcaccaacaaggccgtggtgtctctgagcaatggcgtgtccgtgctgaccttcaaggtgctggacctgaagaactacatcgacaaacagctgctgcccatcctgaacaagcagtcctgcagcatccccaacatcgagacagtgatcgagttccagcagaagaacaaccggctgctggaaatcacccgcgagttctctgtgaatgccggcgtgaccacacctgtgtccacctacatgctgaccaacagcgagctgctgagcctgatcaacgacatgcccatcaccaacgaccagaaaaagctgatgagcaacaacgtgcagatcgtgcggcagcagagctacagcatcatgagcattatcaaagaagaggtgctggcctacgtggtgcagctgcctctgtatggcgtgatcgataccccttgctggaagctgcacacaagccctctgtgcaccaccaacaccaaagagggcagcaacatctgcctgaccagaaccgacagaggctggtactgcgataatgccggcagcgtctcattcttcccacaagccgagacatgcaaggtgcagagcaaccgggtgttctgcgacaccatgaatagcagaaccctgccttccgaagtgaatctgtgcaacgtggacatcttcaaccctaagtacgactgcaagatcatgaccagcaagaccgacgtgtccagcagtgtgatcacctcactgggcgccatcgtgtcctgttacggcaagaccaagtgcaccgccagcaacaagaaccggggcatcatcaagaccttcagcaacggctgcgactacgtgtccaacaaaggcgtggacaccgtgtctgtgggcaacaccctgtactacgtgaacaaatgcgagggccagtctctgtacgtgaagggcgagcccatcatcaacttctacgaccctctggtgttccccagcgacgagttcgatgccagcatcagccaagtgaacgagaagatcaatcagagcctggccttcatcagaaagtccgatgagctgctgcacaacgtgaacgccggcaagtccaccaccaatatcatgatcacgaccatcatcatcgtgattatcgtgatcctgctgtccctgatcgccgtgggcctgctgctttattgataatag

SEQ ID NO: 100 - protein, 510 aa, synthetic construct
MELLILKANAITTILTAVTFCFASGQCITEEFYQSTCSAVSKGYLGALRTGWYTSVITIELSNIKENKCNGTDAKVKLIKQELDKYKNAVTDLQLLMQSTPATGSGSAIASGVAVSKVLHLEGEVNKIKSALLSTNKAVVSLSNGVSVLTFKVLDLKNYIDKQLLPILNKQSCSIPNIETVIEFQQKNNRLLEITREFSVNAGVTTPVSTYMLTNSELLSLINDMPITNDQKKLMSNNVQIVRQQSYSIMSIIKEEVLAYVVQLPLYGVIDTPCWKLHTSPLCTTNTKEGSNICLTRTDRGWYCDNAGSVSFFPQAETCKVQSNRVFCDTMNSRTLPSEVNLCNVDIFNPKYDCKIMTSKTDVSSSVITSLGAIVSCYGKTKCTASNKNRGIIKTFSNGCDYVSNKGVDTVSVGNTLYYVNKCEGQSLYVKGEPIINFYDPLVFPSDEFDASISQVNEKINQSLAFIRKSDELLHNVNAGKSTTNIMITTIIIVIIVILLSLIAVGLLLY

SEQ ID NO: 101 - RNA, 1841 nt, synthetic construct
  source 1..1841: mol_type = other RNA
agcggctcggccattttgtcccagtcagtccggaggctgcggctgcagaagtaccgcctgcggagtaactgcaaaggccaccatggaactgctgatcctgaaggccaacgccatcaccaccatcctgaccgccgtgaccttctgttttgccagcggccagtgcatcaccgaggaattctaccagagcacctgtagcgccgtgtccaagggatatctgggcgcccttagaaccggctggtacaccagcgtgatcaccatcgagctgagcaacatcaaagaaaacaagtgcaacggcaccgacgccaaagtgaagctgatcaagcaagagctggacaagtacaagaatgccgtgaccgacctgcagctgctgatgcagtctacaccagccacaggctctggcagcgccattgcctctggtgtcgccgtgtctaaagtgctgcacctggaaggcgaagtgaacaagatcaagagcgccctgctgagcaccaacaaggccgtggtgtctctgagcaatggcgtgtccgtgctgaccttcaaggtgctggacctgaagaactacatcgacaaacagctgctgcccatcctgaacaagcagtcctgcagcatccccaacatcgagacagtgatcgagttccagcagaagaacaaccggctgctggaaatcacccgcgagttctctgtgaatgccggcgtgaccacacctgtgtccacctacatgctgaccaacagcgagctgctgagcctgatcaacgacatgcccatcaccaacgaccagaaaaagctgatgagcaacaacgtgcagatcgtgcggcagcagagctacagcatcatgagcattatcaaagaagaggtgctggcctacgtggtgcagctgcctctgtatggcgtgatcgataccccttgctggaagctgcacacaagccctctgtgcaccaccaacaccaaagagggcagcaacatctgcctgaccagaaccgacagaggctggtactgcgataatgccggcagcgtctcattcttcccacaagccgagacatgcaaggtgcagagcaaccgggtgttctgcgacaccatgaatagcagaaccctgccttccgaagtgaatctgtgcaacgtggacatcttcaaccctaagtacgactgcaagatcatgaccagcaagaccgacgtgtccagcagtgtgatcacctcactgggcgccatcgtgtcctgttacggcaagaccaagtgcaccgccagcaacaagaaccggggcatcatcaagaccttcagcaacggctgcgactacgtgtccaacaaaggcgtggacaccgtgtctgtgggcaacaccctgtactacgtgaacaaatgcgagggccagtctctgtacgtgaagggcgagcccatcatcaacttctacgaccctctggtgttccccagcgacgagttcgatgccagcatcagccaagtgaacgagaagatcaatcagagcctggccttcatcagaaagtccgatgagctgctgcacaacgtgaacgccggcaagtccaccaccaatatcatgatcacgaccatcatcatcgtgattatcgtgatcctgctgtccctgatcgccgtgggcctgctgctttattgataataggctggagcctcggtggccatgcttcttgccccttgggcctccccccagcccctcctccccttcctgcacccgtacccccgtggtctttgaataaagtctgagtgggcggcaaaaaaaaaaaaaaaaaaaaaaaaaaaaaaaaaaaaaaaaaaaaaaaaaaaaaaaaaaaaaaaaaaaaaaaaaaaaaaaaaaaaaaaaaaaaaaaaaaaaaaaaaaaaaa

SEQ ID NO: 102 - DNA, 1841 bp, synthetic construct
  source 1..1841: mol_type = other DNA
agcggctcggccattttgtcccagtcagtccggaggctgcggctgcagaagtaccgcctgcggagtaactgcaaaggccaccatggaactgctgatcctgaaggccaacgccatcaccaccatcctgaccgccgtgaccttctgttttgccagcggccagaacatcaccgaggaattctaccagagcacctgtagcgccgtgtccaagggatatctgggcgcccttagaaccggctggtacacctgcgtgatcaccatcgagctgagcaacatcaaagaaaacaagtgcaacggcaccgacgccaaagtgaagctgatcaagcaagagctggacaagtacaagaatgccgtgaccgacctgcagctgctgatgcagtctacaccagccacaggctctggcagcgccattgcctctggtgtcgcctgctctaaagtgctgcacctggaaggcgaagtgaacaagatcaagagcgccctgctgagcaccaacaaggccgtggtgtctctgagcaatggcgtgtccgtgctgaccttcaaggtgctggacctgaagaactacatcgacaaacagctgctgcccatcctgaacaagcagtcctgcagcatccccaacatcgagacagtgatcgagttccagcagaagaacaaccggctgctggaaatcacccgcgagttctctgtgaatgccggcgtgaccacacctgtgtccacctacatgctgaccaacagcgagctgctgagcctgatcaacgacatgcccatcaccaacgaccagaaaaagctgatgagcaacaacgtgcagatcgtgcggcagcagagctacagcatcatgagcattatcaaagaagaggtgctggcctacgtggtgcagctgcctctgtatggcgtgatcgataccccttgctggaagctgcacacaagccctctgtgcaccaccaacaccaaagagggcagcaacatctgcctgaccagaaccgacagaggctggtactgcgataatgccggcagcgtctcattcttcccacaagccgagacatgcaaggtgcagagcaaccgggtgttctgcgacaccatgaatagcagaaccctgccttccgaagtgaatctgtgcaacgtggacatcttcaaccctaagtacgactgcaagatcatgaccagcaagaccgacgtgtccagcagtgtgatcacctcactgggcgccatcgtgtcctgttacggcaagaccaagtgcaccgccagcaacaagaaccggggcatcatcaagaccttcagcaacggctgcgactacgtgtccaacaaaggcgtggacaccgtgtctgtgggcaacaccctgtactacgtgaacaaacaagagggccagtctctgtacgtgaagggcgagcccatcatcaacttctacgaccctctggtgttccccagcgacgagttcgatgccagcatcagccaagtgaacgagaagatcaatcagagcctggccttcatcagaaagtccgatgagctgctgcacaacgtgaacgccggcaagtccaccaccaatatcatgatcacgaccatcatcatcgtgattatcgtgatcctgctgtccctgatcgccgtgggcctgctgctttattgataataggctggagcctcggtggccatgcttcttgccccttgggcctccccccagcccctcctccccttcctgcacccgtacccccgtggtctttgaataaagtctgagtgggcggcaaaaaaaaaaaaaaaaaaaaaaaaaaaaaaaaaaaaaaaaaaaaaaaaaaaaaaaaaaaaaaaaaaaaaaaaaaaaaaaaaaaaaaaaaaaaaaaaaaaaaaaaaaaaaa

SEQ ID NO: 103 - DNA, 1539 bp, synthetic construct
  source 1..1539: mol_type = other DNA
atggaactgctgatcctgaaggccaacgccatcaccaccatcctgaccgccgtgaccttctgttttgccagcggccagaacatcaccgaggaattctaccagagcacctgtagcgccgtgtccaagggatatctgggcgcccttagaaccggctggtacacctgcgtgatcaccatcgagctgagcaacatcaaagaaaacaagtgcaacggcaccgacgccaaagtgaagctgatcaagcaagagctggacaagtacaagaatgccgtgaccgacctgcagctgctgatgcagtctacaccagccacaggctctggcagcgccattgcctctggtgtcgcctgctctaaagtgctgcacctggaaggcgaagtgaacaagatcaagagcgccctgctgagcaccaacaaggccgtggtgtctctgagcaatggcgtgtccgtgctgaccttcaaggtgctggacctgaagaactacatcgacaaacagctgctgcccatcctgaacaagcagtcctgcagcatccccaacatcgagacagtgatcgagttccagcagaagaacaaccggctgctggaaatcacccgcgagttctctgtgaatgccggcgtgaccacacctgtgtccacctacatgctgaccaacagcgagctgctgagcctgatcaacgacatgcccatcaccaacgaccagaaaaagctgatgagcaacaacgtgcagatcgtgcggcagcagagctacagcatcatgagcattatcaaagaagaggtgctggcctacgtggtgcagctgcctctgtatggcgtgatcgataccccttgctggaagctgcacacaagccctctgtgcaccaccaacaccaaagagggcagcaacatctgcctgaccagaaccgacagaggctggtactgcgataatgccggcagcgtctcattcttcccacaagccgagacatgcaaggtgcagagcaaccgggtgttctgcgacaccatgaatagcagaaccctgccttccgaagtgaatctgtgcaacgtggacatcttcaaccctaagtacgactgcaagatcatgaccagcaagaccgacgtgtccagcagtgtgatcacctcactgggcgccatcgtgtcctgttacggcaagaccaagtgcaccgccagcaacaagaaccggggcatcatcaagaccttcagcaacggctgcgactacgtgtccaacaaaggcgtggacaccgtgtctgtgggcaacaccctgtactacgtgaacaaacaagagggccagtctctgtacgtgaagggcgagcccatcatcaacttctacgaccctctggtgttccccagcgacgagttcgatgccagcatcagccaagtgaacgagaagatcaatcagagcctggccttcatcagaaagtccgatgagctgctgcacaacgtgaacgccggcaagtccaccaccaatatcatgatcacgaccatcatcatcgtgattatcgtgatcctgctgtccctgatcgccgtgggcctgctgctttattgataatag

SEQ ID NO: 104 - protein, 510 aa, synthetic construct
MELLILKANAITTILTAVTFCFASGQNITEEFYQSTCSAVSKGYLGALRTGWYTCVITIELSNIKENKCNGTDAKVKLIKQELDKYKNAVTDLQLLMQSTPATGSGSAIASGVACSKVLHLEGEVNKIKSALLSTNKAVVSLSNGVSVLTFKVLDLKNYIDKQLLPILNKQSCSIPNIETVIEFQQKNNRLLEITREFSVNAGVTTPVSTYMLTNSELLSLINDMPITNDQKKLMSNNVQIVRQQSYSIMSIIKEEVLAYVVQLPLYGVIDTPCWKLHTSPLCTTNTKEGSNICLTRTDRGWYCDNAGSVSFFPQAETCKVQSNRVFCDTMNSRTLPSEVNLCNVDIFNPKYDCKIMTSKTDVSSSVITSLGAIVSCYGKTKCTASNKNRGIIKTFSNGCDYVSNKGVDTVSVGNTLYYVNKQEGQSLYVKGEPIINFYDPLVFPSDEFDASISQVNEKINQSLAFIRKSDELLHNVNAGKSTTNIMITTIIIVIIVILLSLIAVGLLLY

SEQ ID NO: 105 - RNA, 1841 nt, synthetic construct
  source 1..1841: mol_type = other RNA
agcggctcggccattttgtcccagtcagtccggaggctgcggctgcagaagtaccgcctgcggagtaactgcaaaggccaccatggaactgctgatcctgaaggccaacgccatcaccaccatcctgaccgccgtgaccttctgttttgccagcggccagaacatcaccgaggaattctaccagagcacctgtagcgccgtgtccaagggatatctgggcgcccttagaaccggctggtacacctgcgtgatcaccatcgagctgagcaacatcaaagaaaacaagtgcaacggcaccgacgccaaagtgaagctgatcaagcaagagctggacaagtacaagaatgccgtgaccgacctgcagctgctgatgcagtctacaccagccacaggctctggcagcgccattgcctctggtgtcgcctgctctaaagtgctgcacctggaaggcgaagtgaacaagatcaagagcgccctgctgagcaccaacaaggccgtggtgtctctgagcaatggcgtgtccgtgctgaccttcaaggtgctggacctgaagaactacatcgacaaacagctgctgcccatcctgaacaagcagtcctgcagcatccccaacatcgagacagtgatcgagttccagcagaagaacaaccggctgctggaaatcacccgcgagttctctgtgaatgccggcgtgaccacacctgtgtccacctacatgctgaccaacagcgagctgctgagcctgatcaacgacatgcccatcaccaacgaccagaaaaagctgatgagcaacaacgtgcagatcgtgcggcagcagagctacagcatcatgagcattatcaaagaagaggtgctggcctacgtggtgcagctgcctctgtatggcgtgatcgataccccttgctggaagctgcacacaagccctctgtgcaccaccaacaccaaagagggcagcaacatctgcctgaccagaaccgacagaggctggtactgcgataatgccggcagcgtctcattcttcccacaagccgagacatgcaaggtgcagagcaaccgggtgttctgcgacaccatgaatagcagaaccctgccttccgaagtgaatctgtgcaacgtggacatcttcaaccctaagtacgactgcaagatcatgaccagcaagaccgacgtgtccagcagtgtgatcacctcactgggcgccatcgtgtcctgttacggcaagaccaagtgcaccgccagcaacaagaaccggggcatcatcaagaccttcagcaacggctgcgactacgtgtccaacaaaggcgtggacaccgtgtctgtgggcaacaccctgtactacgtgaacaaacaagagggccagtctctgtacgtgaagggcgagcccatcatcaacttctacgaccctctggtgttccccagcgacgagttcgatgccagcatcagccaagtgaacgagaagatcaatcagagcctggccttcatcagaaagtccgatgagctgctgcacaacgtgaacgccggcaagtccaccaccaatatcatgatcacgaccatcatcatcgtgattatcgtgatcctgctgtccctgatcgccgtgggcctgctgctttattgataataggctggagcctcggtggccatgcttcttgccccttgggcctccccccagcccctcctccccttcctgcacccgtacccccgtggtctttgaataaagtctgagtgggcggcaaaaaaaaaaaaaaaaaaaaaaaaaaaaaaaaaaaaaaaaaaaaaaaaaaaaaaaaaaaaaaaaaaaaaaaaaaaaaaaaaaaaaaaaaaaaaaaaaaaaaaaaaaaaaa

SEQ ID NO: 106 - DNA, 1841 bp, synthetic construct
  source 1..1841: mol_type = other DNA
agcggctcggccattttgtcccagtcagtccggaggctgcggctgcagaagtaccgcctgcggagtaactgcaaaggccaccatggaactgctgatcctgaaggccaacgccatcaccaccatcctgaccgccgtgaccttctgttttgccagcggccagaacatcaccgaggaattctaccagagcacctgtagcgccgtgtccaagggatatctgggcgcccttagaaccggctggtgcaccagcgtgatcaccatcgagctgagcaacatcaaagaaaacaagtgcaacggcaccgacgccaaagtgaagctgatcaagcaagagctggacaagtacaagaatgccgtgaccgacctgcagctgctgatgcagtctacaccagccacaggctctggcagcgccattgcctctggtgtctgcgtgtctaaagtgctgcacctggaaggcgaagtgaacaagatcaagagcgccctgctgagcaccaacaaggccgtggtgtctctgagcaatggcgtgtccgtgctgaccttcaaggtgctggacctgaagaactacatcgacaaacagctgctgcccatcctgaacaagcagtcctgcagcatccccaacatcgagacagtgatcgagttccagcagaagaacaaccggctgctggaaatcacccgcgagttctctgtgaatgccggcgtgaccacacctgtgtccacctacatgctgaccaacagcgagctgctgagcctgatcaacgacatgcccatcaccaacgaccagaaaaagctgatgagcaacaacgtgcagatcgtgcggcagcagagctacagcatcatgagcattatcaaagaagaggtgctggcctacgtggtgcagctgcctctgtatggcgtgatcgataccccttgctggaagctgcacacaagccctctgtgcaccaccaacaccaaagagggcagcaacatctgcctgaccagaaccgacagaggctggtactgcgataatgccggcagcgtctcattcttcccacaagccgagacatgcaaggtgcagagcaaccgggtgttctgcgacaccatgaatagcagaaccctgccttccgaagtgaatctgtgcaacgtggacatcttcaaccctaagtacgactgcaagatcatgaccagcaagaccgacgtgtccagcagtgtgatcacctcactgggcgccatcgtgtcctgttacggcaagaccaagtgcaccgccagcaacaagaaccggggcatcatcaagaccttcagcaacggctgcgactacgtgtccaacaaaggcgtggacaccgtgtctgtgggcaacaccctgtactacgtgaacaaacaagagggccagtctctgtacgtgaagggcgagcccatcatcaacttctacgaccctctggtgttccccagcgacgagttcgatgccagcatcagccaagtgaacgagaagatcaatcagagcctggccttcatcagaaagtccgatgagctgctgcacaacgtgaacgccggcaagtccaccaccaatatcatgatcacgaccatcatcatcgtgattatcgtgatcctgctgtccctgatcgccgtgggcctgctgctttattgataataggctggagcctcggtggccatgcttcttgccccttgggcctccccccagcccctcctccccttcctgcacccgtacccccgtggtctttgaataaagtctgagtgggcggcaaaaaaaaaaaaaaaaaaaaaaaaaaaaaaaaaaaaaaaaaaaaaaaaaaaaaaaaaaaaaaaaaaaaaaaaaaaaaaaaaaaaaaaaaaaaaaaaaaaaaaaaaaaaaa

SEQ ID NO: 107 - DNA, 1539 bp, synthetic construct
  source 1..1539: mol_type = other DNA
atggaactgctgatcctgaaggccaacgccatcaccaccatcctgaccgccgtgaccttctgttttgccagcggccagaacatcaccgaggaattctaccagagcacctgtagcgccgtgtccaagggatatctgggcgcccttagaaccggctggtgcaccagcgtgatcaccatcgagctgagcaacatcaaagaaaacaagtgcaacggcaccgacgccaaagtgaagctgatcaagcaagagctggacaagtacaagaatgccgtgaccgacctgcagctgctgatgcagtctacaccagccacaggctctggcagcgccattgcctctggtgtctgcgtgtctaaagtgctgcacctggaaggcgaagtgaacaagatcaagagcgccctgctgagcaccaacaaggccgtggtgtctctgagcaatggcgtgtccgtgctgaccttcaaggtgctggacctgaagaactacatcgacaaacagctgctgcccatcctgaacaagcagtcctgcagcatccccaacatcgagacagtgatcgagttccagcagaagaacaaccggctgctggaaatcacccgcgagttctctgtgaatgccggcgtgaccacacctgtgtccacctacatgctgaccaacagcgagctgctgagcctgatcaacgacatgcccatcaccaacgaccagaaaaagctgatgagcaacaacgtgcagatcgtgcggcagcagagctacagcatcatgagcattatcaaagaagaggtgctggcctacgtggtgcagctgcctctgtatggcgtgatcgataccccttgctggaagctgcacacaagccctctgtgcaccaccaacaccaaagagggcagcaacatctgcctgaccagaaccgacagaggctggtactgcgataatgccggcagcgtctcattcttcccacaagccgagacatgcaaggtgcagagcaaccgggtgttctgcgacaccatgaatagcagaaccctgccttccgaagtgaatctgtgcaacgtggacatcttcaaccctaagtacgactgcaagatcatgaccagcaagaccgacgtgtccagcagtgtgatcacctcactgggcgccatcgtgtcctgttacggcaagaccaagtgcaccgccagcaacaagaaccggggcatcatcaagaccttcagcaacggctgcgactacgtgtccaacaaaggcgtggacaccgtgtctgtgggcaacaccctgtactacgtgaacaaacaagagggccagtctctgtacgtgaagggcgagcccatcatcaacttctacgaccctctggtgttccccagcgacgagttcgatgccagcatcagccaagtgaacgagaagatcaatcagagcctggccttcatcagaaagtccgatgagctgctgcacaacgtgaacgccggcaagtccaccaccaatatcatgatcacgaccatcatcatcgtgattatcgtgatcctgctgtccctgatcgccgtgggcctgctgctttattgataatag

SEQ ID NO: 108 - protein, 510 aa, synthetic construct
MELLILKANAITTILTAVTFCFASGQNITEEFYQSTCSAVSKGYLGALRTGWCTSVITIELSNIKENKCNGTDAKVKLIKQELDKYKNAVTDLQLLMQSTPATGSGSAIASGVCVSKVLHLEGEVNKIKSALLSTNKAVVSLSNGVSVLTFKVLDLKNYIDKQLLPILNKQSCSIPNIETVIEFQQKNNRLLEITREFSVNAGVTTPVSTYMLTNSELLSLINDMPITNDQKKLMSNNVQIVRQQSYSIMSIIKEEVLAYVVQLPLYGVIDTPCWKLHTSPLCTTNTKEGSNICLTRTDRGWYCDNAGSVSFFPQAETCKVQSNRVFCDTMNSRTLPSEVNLCNVDIFNPKYDCKIMTSKTDVSSSVITSLGAIVSCYGKTKCTASNKNRGIIKTFSNGCDYVSNKGVDTVSVGNTLYYVNKQEGQSLYVKGEPIINFYDPLVFPSDEFDASISQVNEKINQSLAFIRKSDELLHNVNAGKSTTNIMITTIIIVIIVILLSLIAVGLLLY

SEQ ID NO: 109 - RNA, 1841 nt, synthetic construct
  source 1..1841: mol_type = other RNA
agcggctcggccattttgtcccagtcagtccggaggctgcggctgcagaagtaccgcctgcggagtaactgcaaaggccaccatggaactgctgatcctgaaggccaacgccatcaccaccatcctgaccgccgtgaccttctgttttgccagcggccagaacatcaccgaggaattctaccagagcacctgtagcgccgtgtccaagggatatctgggcgcccttagaaccggctggtgcaccagcgtgatcaccatcgagctgagcaacatcaaagaaaacaagtgcaacggcaccgacgccaaagtgaagctgatcaagcaagagctggacaagtacaagaatgccgtgaccgacctgcagctgctgatgcagtctacaccagccacaggctctggcagcgccattgcctctggtgtctgcgtgtctaaagtgctgcacctggaaggcgaagtgaacaagatcaagagcgccctgctgagcaccaacaaggccgtggtgtctctgagcaatggcgtgtccgtgctgaccttcaaggtgctggacctgaagaactacatcgacaaacagctgctgcccatcctgaacaagcagtcctgcagcatccccaacatcgagacagtgatcgagttccagcagaagaacaaccggctgctggaaatcacccgcgagttctctgtgaatgccggcgtgaccacacctgtgtccacctacatgctgaccaacagcgagctgctgagcctgatcaacgacatgcccatcaccaacgaccagaaaaagctgatgagcaacaacgtgcagatcgtgcggcagcagagctacagcatcatgagcattatcaaagaagaggtgctggcctacgtggtgcagctgcctctgtatggcgtgatcgataccccttgctggaagctgcacacaagccctctgtgcaccaccaacaccaaagagggcagcaacatctgcctgaccagaaccgacagaggctggtactgcgataatgccggcagcgtctcattcttcccacaagccgagacatgcaaggtgcagagcaaccgggtgttctgcgacaccatgaatagcagaaccctgccttccgaagtgaatctgtgcaacgtggacatcttcaaccctaagtacgactgcaagatcatgaccagcaagaccgacgtgtccagcagtgtgatcacctcactgggcgccatcgtgtcctgttacggcaagaccaagtgcaccgccagcaacaagaaccggggcatcatcaagaccttcagcaacggctgcgactacgtgtccaacaaaggcgtggacaccgtgtctgtgggcaacaccctgtactacgtgaacaaacaagagggccagtctctgtacgtgaagggcgagcccatcatcaacttctacgaccctctggtgttccccagcgacgagttcgatgccagcatcagccaagtgaacgagaagatcaatcagagcctggccttcatcagaaagtccgatgagctgctgcacaacgtgaacgccggcaagtccaccaccaatatcatgatcacgaccatcatcatcgtgattatcgtgatcctgctgtccctgatcgccgtgggcctgctgctttattgataataggctggagcctcggtggccatgcttcttgccccttgggcctccccccagcccctcctccccttcctgcacccgtacccccgtggtctttgaataaagtctgagtgggcggcaaaaaaaaaaaaaaaaaaaaaaaaaaaaaaaaaaaaaaaaaaaaaaaaaaaaaaaaaaaaaaaaaaaaaaaaaaaaaaaaaaaaaaaaaaaaaaaaaaaaaaaaaaaaaa

SEQ ID NO: 110 - DNA, 1841 bp, synthetic construct
  source 1..1841: mol_type = other DNA
agcggctcggccattttgtcccagtcagtccggaggctgcggctgcagaagtaccgcctgcggagtaactgcaaaggccaccatggaactgctgatcctgaaggccaacgccatcaccaccatcctgaccgccgtgaccttctgttttgccagcggccagaacatcaccgaggaattctaccagagcacctgtagcgccgtgtccaagggatatctgggcgcccttagaaccggctggtacacctgcgtgatcaccatcgagctgagcaacatcaaagaaaacaagtgcaacggcaccgacgccaaagtgaagctgatcaagcaagagctggacaagtacaagaatgccgtgaccgacctgcagctgctgatgcagtctacaccagccacaggctctggcagcgccattgcctctggtgtcgccgtgtctaaagtgctgcacctggaaggcgaagtgaacaagatcaagagcgccctgctgagcaccaacaaggccgtggtgtctctgagcaatggcgtgtgcgtgctgaccttcaaggtgctggacctgaagaactacatcgacaaacagctgctgcccatcctgaacaagcagtcctgcagcatccccaacatcgagacagtgatcgagttccagcagaagaacaaccggctgctggaaatcacccgcgagttctctgtgaatgccggcgtgaccacacctgtgtccacctacatgctgaccaacagcgagctgctgagcctgatcaacgacatgcccatcaccaacgaccagaaaaagctgatgagcaacaacgtgcagatcgtgcggcagcagagctacagcatcatgagcattatcaaagaagaggtgctggcctacgtggtgcagctgcctctgtatggcgtgatcgataccccttgctggaagctgcacacaagccctctgtgcaccaccaacaccaaagagggcagcaacatctgcctgaccagaaccgacagaggctggtactgcgataatgccggcagcgtctcattcttcccacaagccgagacatgcaaggtgcagagcaaccgggtgttctgcgacaccatgaatagcagaaccctgccttccgaagtgaatctgtgcaacgtggacatcttcaaccctaagtacgactgcaagatcatgaccagcaagaccgacgtgtccagcagtgtgatcacctcactgggcgccatcgtgtcctgttacggcaagaccaagtgcaccgccagcaacaagaaccggggcatcatcaagaccttcagcaacggctgcgactacgtgtccaacaaaggcgtggacaccgtgtctgtgggcaacaccctgtactacgtgaacaaacaagagggccagtctctgtacgtgaagggcgagcccatcatcaacttctacgaccctctggtgttccccagcgacgagttcgatgccagcatcagccaagtgaacgagaagatcaatcagagcctggccttcatcagaaagtccgatgagctgctgcacaacgtgaacgccggcaagtccaccaccaatatcatgatcacgaccatcatcatcgtgattatcgtgatcctgctgtccctgatcgccgtgggcctgctgctttattgataataggctggagcctcggtggccatgcttcttgccccttgggcctccccccagcccctcctccccttcctgcacccgtacccccgtggtctttgaataaagtctgagtgggcggcaaaaaaaaaaaaaaaaaaaaaaaaaaaaaaaaaaaaaaaaaaaaaaaaaaaaaaaaaaaaaaaaaaaaaaaaaaaaaaaaaaaaaaaaaaaaaaaaaaaaaaaaaaaaaa

SEQ ID NO: 111 - DNA, 1539 bp, synthetic construct
  source 1..1539: mol_type = other DNA
atggaactgctgatcctgaaggccaacgccatcaccaccatcctgaccgccgtgaccttctgttttgccagcggccagaacatcaccgaggaattctaccagagcacctgtagcgccgtgtccaagggatatctgggcgcccttagaaccggctggtacacctgcgtgatcaccatcgagctgagcaacatcaaagaaaacaagtgcaacggcaccgacgccaaagtgaagctgatcaagcaagagctggacaagtacaagaatgccgtgaccgacctgcagctgctgatgcagtctacaccagccacaggctctggcagcgccattgcctctggtgtcgccgtgtctaaagtgctgcacctggaaggcgaagtgaacaagatcaagagcgccctgctgagcaccaacaaggccgtggtgtctctgagcaatggcgtgtgcgtgctgaccttcaaggtgctggacctgaagaactacatcgacaaacagctgctgcccatcctgaacaagcagtcctgcagcatccccaacatcgagacagtgatcgagttccagcagaagaacaaccggctgctggaaatcacccgcgagttctctgtgaatgccggcgtgaccacacctgtgtccacctacatgctgaccaacagcgagctgctgagcctgatcaacgacatgcccatcaccaacgaccagaaaaagctgatgagcaacaacgtgcagatcgtgcggcagcagagctacagcatcatgagcattatcaaagaagaggtgctggcctacgtggtgcagctgcctctgtatggcgtgatcgataccccttgctggaagctgcacacaagccctctgtgcaccaccaacaccaaagagggcagcaacatctgcctgaccagaaccgacagaggctggtactgcgataatgccggcagcgtctcattcttcccacaagccgagacatgcaaggtgcagagcaaccgggtgttctgcgacaccatgaatagcagaaccctgccttccgaagtgaatctgtgcaacgtggacatcttcaaccctaagtacgactgcaagatcatgaccagcaagaccgacgtgtccagcagtgtgatcacctcactgggcgccatcgtgtcctgttacggcaagaccaagtgcaccgccagcaacaagaaccggggcatcatcaagaccttcagcaacggctgcgactacgtgtccaacaaaggcgtggacaccgtgtctgtgggcaacaccctgtactacgtgaacaaacaagagggccagtctctgtacgtgaagggcgagcccatcatcaacttctacgaccctctggtgttccccagcgacgagttcgatgccagcatcagccaagtgaacgagaagatcaatcagagcctggccttcatcagaaagtccgatgagctgctgcacaacgtgaacgccggcaagtccaccaccaatatcatgatcacgaccatcatcatcgtgattatcgtgatcctgctgtccctgatcgccgtgggcctgctgctttattgataatag

SEQ ID NO: 112 - protein, 510 aa, synthetic construct
MELLILKANAITTILTAVTFCFASGQNITEEFYQSTCSAVSKGYLGALRTGWYTCVITIELSNIKENKCNGTDAKVKLIKQELDKYKNAVTDLQLLMQSTPATGSGSAIASGVAVSKVLHLEGEVNKIKSALLSTNKAVVSLSNGVCVLTFKVLDLKNYIDKQLLPILNKQSCSIPNIETVIEFQQKNNRLLEITREFSVNAGVTTPVSTYMLTNSELLSLINDMPITNDQKKLMSNNVQIVRQQSYSIMSIIKEEVLAYVVQLPLYGVIDTPCWKLHTSPLCTTNTKEGSNICLTRTDRGWYCDNAGSVSFFPQAETCKVQSNRVFCDTMNSRTLPSEVNLCNVDIFNPKYDCKIMTSKTDVSSSVITSLGAIVSCYGKTKCTASNKNRGIIKTFSNGCDYVSNKGVDTVSVGNTLYYVNKQEGQSLYVKGEPIINFYDPLVFPSDEFDASISQVNEKINQSLAFIRKSDELLHNVNAGKSTTNIMITTIIIVIIVILLSLIAVGLLLY

SEQ ID NO: 113 - RNA, 1841 nt, synthetic construct
  source 1..1841: mol_type = other RNA
agcggctcggccattttgtcccagtcagtccggaggctgcggctgcagaagtaccgcctgcggagtaactgcaaaggccaccatggaactgctgatcctgaaggccaacgccatcaccaccatcctgaccgccgtgaccttctgttttgccagcggccagaacatcaccgaggaattctaccagagcacctgtagcgccgtgtccaagggatatctgggcgcccttagaaccggctggtacacctgcgtgatcaccatcgagctgagcaacatcaaagaaaacaagtgcaacggcaccgacgccaaagtgaagctgatcaagcaagagctggacaagtacaagaatgccgtgaccgacctgcagctgctgatgcagtctacaccagccacaggctctggcagcgccattgcctctggtgtcgccgtgtctaaagtgctgcacctggaaggcgaagtgaacaagatcaagagcgccctgctgagcaccaacaaggccgtggtgtctctgagcaatggcgtgtgcgtgctgaccttcaaggtgctggacctgaagaactacatcgacaaacagctgctgcccatcctgaacaagcagtcctgcagcatccccaacatcgagacagtgatcgagttccagcagaagaacaaccggctgctggaaatcacccgcgagttctctgtgaatgccggcgtgaccacacctgtgtccacctacatgctgaccaacagcgagctgctgagcctgatcaacgacatgcccatcaccaacgaccagaaaaagctgatgagcaacaacgtgcagatcgtgcggcagcagagctacagcatcatgagcattatcaaagaagaggtgctggcctacgtggtgcagctgcctctgtatggcgtgatcgataccccttgctggaagctgcacacaagccctctgtgcaccaccaacaccaaagagggcagcaacatctgcctgaccagaaccgacagaggctggtactgcgataatgccggcagcgtctcattcttcccacaagccgagacatgcaaggtgcagagcaaccgggtgttctgcgacaccatgaatagcagaaccctgccttccgaagtgaatctgtgcaacgtggacatcttcaaccctaagtacgactgcaagatcatgaccagcaagaccgacgtgtccagcagtgtgatcacctcactgggcgccatcgtgtcctgttacggcaagaccaagtgcaccgccagcaacaagaaccggggcatcatcaagaccttcagcaacggctgcgactacgtgtccaacaaaggcgtggacaccgtgtctgtgggcaacaccctgtactacgtgaacaaacaagagggccagtctctgtacgtgaagggcgagcccatcatcaacttctacgaccctctggtgttccccagcgacgagttcgatgccagcatcagccaagtgaacgagaagatcaatcagagcctggccttcatcagaaagtccgatgagctgctgcacaacgtgaacgccggcaagtccaccaccaatatcatgatcacgaccatcatcatcgtgattatcgtgatcctgctgtccctgatcgccgtgggcctgctgctttattgataataggctggagcctcggtggccatgcttcttgccccttgggcctccccccagcccctcctccccttcctgcacccgtacccccgtggtctttgaataaagtctgagtgggcggcaaaaaaaaaaaaaaaaaaaaaaaaaaaaaaaaaaaaaaaaaaaaaaaaaaaaaaaaaaaaaaaaaaaaaaaaaaaaaaaaaaaaaaaaaaaaaaaaaaaaaaaaaaaaaa

SEQ ID NO: 114 - DNA, 1841 bp, synthetic construct
  source 1..1841: mol_type = other DNA
agcggctcggccattttgtcccagtcagtccggaggctgcggctgcagaagtaccgcctgcggagtaactgcaaaggccaccatggaactgctgatcctgaaggccaacgccatcaccaccatcctgaccgccgtgaccttctgttttgccagcggccagaacatcaccgaggaattctaccagagcacctgtagcgccgtgtccaagggatatctgggcgcccttagaaccggctggtactgcagcgtgatcaccatcgagctgagcaacatcaaagaaaacaagtgcaacggcaccgacgccaaagtgaagctgatcaagcaagagctggacaagtacaagaatgccgtgaccgacctgcagctgctgatgcagtctacaccagccacaggctctggcagcgccattgcctctggttgcgccgtgtctaaagtgctgcacctggaaggcgaagtgaacaagatcaagagcgccctgctgagcaccaacaaggccgtggtgtctctgagcaatggcgtgtccgtgctgaccttcaaggtgctggacctgaagaactacatcgacaaacagctgctgcccatcctgaacaagcagtcctgcagcatccccaacatcgagacagtgatcgagttccagcagaagaacaaccggctgctggaaatcacccgcgagttctctgtgaatgccggcgtgaccacacctgtgtccacctacatgctgaccaacagcgagctgctgagcctgatcaacgacatgcccatcaccaacgaccagaaaaagctgatgagcaacaacgtgcagatcgtgcggcagcagagctacagcatcatgagcattatcaaagaagaggtgctggcctacgtggtgcagctgcctctgtatggcgtgatcgataccccttgctggaagctgcacacaagccctctgtgcaccaccaacaccaaagagggcagcaacatctgcctgaccagaaccgacagaggctggtactgcgataatgccggcagcgtctcattcttcccacaagccgagacatgcaaggtgcagagcaaccgggtgttctgcgacaccatgaatagcagaaccctgccttccgaagtgaatctgtgcaacgtggacatcttcaaccctaagtacgactgcaagatcatgaccagcaagaccgacgtgtccagcagtgtgatcacctcactgggcgccatcgtgtcctgttacggcaagaccaagtgcaccgccagcaacaagaaccggggcatcatcaagaccttcagcaacggctgcgactacgtgtccaacaaaggcgtggacaccgtgtctgtgggcaacaccctgtactacgtgaacaaacaagagggccagtctctgtacgtgaagggcgagcccatcatcaacttctacgaccctctggtgttccccagcgacgagttcgatgccagcatcagccaagtgaacgagaagatcaatcagagcctggccttcatcagaaagtccgatgagctgctgcacaacgtgaacgccggcaagtccaccaccaatatcatgatcacgaccatcatcatcgtgattatcgtgatcctgctgtccctgatcgccgtgggcctgctgctttattgataataggctggagcctcggtggccatgcttcttgccccttgggcctccccccagcccctcctccccttcctgcacccgtacccccgtggtctttgaataaagtctgagtgggcggcaaaaaaaaaaaaaaaaaaaaaaaaaaaaaaaaaaaaaaaaaaaaaaaaaaaaaaaaaaaaaaaaaaaaaaaaaaaaaaaaaaaaaaaaaaaaaaaaaaaaaaaaaaaaaa

SEQ ID NO: 115 - DNA, 1539 bp, synthetic construct
  source 1..1539: mol_type = other DNA
atggaactgctgatcctgaaggccaacgccatcaccaccatcctgaccgccgtgaccttctgttttgccagcggccagaacatcaccgaggaattctaccagagcacctgtagcgccgtgtccaagggatatctgggcgcccttagaaccggctggtactgcagcgtgatcaccatcgagctgagcaacatcaaagaaaacaagtgcaacggcaccgacgccaaagtgaagctgatcaagcaagagctggacaagtacaagaatgccgtgaccgacctgcagctgctgatgcagtctacaccagccacaggctctggcagcgccattgcctctggttgcgccgtgtctaaagtgctgcacctggaaggcgaagtgaacaagatcaagagcgccctgctgagcaccaacaaggccgtggtgtctctgagcaatggcgtgtccgtgctgaccttcaaggtgctggacctgaagaactacatcgacaaacagctgctgcccatcctgaacaagcagtcctgcagcatccccaacatcgagacagtgatcgagttccagcagaagaacaaccggctgctggaaatcacccgcgagttctctgtgaatgccggcgtgaccacacctgtgtccacctacatgctgaccaacagcgagctgctgagcctgatcaacgacatgcccatcaccaacgaccagaaaaagctgatgagcaacaacgtgcagatcgtgcggcagcagagctacagcatcatgagcattatcaaagaagaggtgctggcctacgtggtgcagctgcctctgtatggcgtgatcgataccccttgctggaagctgcacacaagccctctgtgcaccaccaacaccaaagagggcagcaacatctgcctgaccagaaccgacagaggctggtactgcgataatgccggcagcgtctcattcttcccacaagccgagacatgcaaggtgcagagcaaccgggtgttctgcgacaccatgaatagcagaaccctgccttccgaagtgaatctgtgcaacgtggacatcttcaaccctaagtacgactgcaagatcatgaccagcaagaccgacgtgtccagcagtgtgatcacctcactgggcgccatcgtgtcctgttacggcaagaccaagtgcaccgccagcaacaagaaccggggcatcatcaagaccttcagcaacggctgcgactacgtgtccaacaaaggcgtggacaccgtgtctgtgggcaacaccctgtactacgtgaacaaacaagagggccagtctctgtacgtgaagggcgagcccatcatcaacttctacgaccctctggtgttccccagcgacgagttcgatgccagcatcagccaagtgaacgagaagatcaatcagagcctggccttcatcagaaagtccgatgagctgctgcacaacgtgaacgccggcaagtccaccaccaatatcatgatcacgaccatcatcatcgtgattatcgtgatcctgctgtccctgatcgccgtgggcctgctgctttattgataatag

SEQ ID NO: 116 - protein, 510 aa, synthetic construct
MELLILKANAITTILTAVTFCFASGQNITEEFYQSTCSAVSKGYLGALRTGWYCSVITIELSNIKENKCNGTDAKVKLIKQELDKYKNAVTDLQLLMQSTPATGSGSAIASGCAVSKVLHLEGEVNKIKSALLSTNKAVVSLSNGVSVLTFKVLDLKNYIDKQLLPILNKQSCSIPNIETVIEFQQKNNRLLEITREFSVNAGVTTPVSTYMLTNSELLSLINDMPITNDQKKLMSNNVQIVRQQSYSIMSIIKEEVLAYVVQLPLYGVIDTPCWKLHTSPLCTTNTKEGSNICLTRTDRGWYCDNAGSVSFFPQAETCKVQSNRVFCDTMNSRTLPSEVNLCNVDIFNPKYDCKIMTSKTDVSSSVITSLGAIVSCYGKTKCTASNKNRGIIKTFSNGCDYVSNKGVDTVSVGNTLYYVNKQEGQSLYVKGEPIINFYDPLVFPSDEFDASISQVNEKINQSLAFIRKSDELLHNVNAGKSTTNIMITTIIIVIIVILLSLIAVGLLLY

SEQ ID NO: 117 - RNA, 1841 nt, synthetic construct
  source 1..1841: mol_type = other RNA
agcggctcggccattttgtcccagtcagtccggaggctgcggctgcagaagtaccgcctgcggagtaactgcaaaggccaccatggaactgctgatcctgaaggccaacgccatcaccaccatcctgaccgccgtgaccttctgttttgccagcggccagaacatcaccgaggaattctaccagagcacctgtagcgccgtgtccaagggatatctgggcgcccttagaaccggctggtactgcagcgtgatcaccatcgagctgagcaacatcaaagaaaacaagtgcaacggcaccgacgccaaagtgaagctgatcaagcaagagctggacaagtacaagaatgccgtgaccgacctgcagctgctgatgcagtctacaccagccacaggctctggcagcgccattgcctctggttgcgccgtgtctaaagtgctgcacctggaaggcgaagtgaacaagatcaagagcgccctgctgagcaccaacaaggccgtggtgtctctgagcaatggcgtgtccgtgctgaccttcaaggtgctggacctgaagaactacatcgacaaacagctgctgcccatcctgaacaagcagtcctgcagcatccccaacatcgagacagtgatcgagttccagcagaagaacaaccggctgctggaaatcacccgcgagttctctgtgaatgccggcgtgaccacacctgtgtccacctacatgctgaccaacagcgagctgctgagcctgatcaacgacatgcccatcaccaacgaccagaaaaagctgatgagcaacaacgtgcagatcgtgcggcagcagagctacagcatcatgagcattatcaaagaagaggtgctggcctacgtggtgcagctgcctctgtatggcgtgatcgataccccttgctggaagctgcacacaagccctctgtgcaccaccaacaccaaagagggcagcaacatctgcctgaccagaaccgacagaggctggtactgcgataatgccggcagcgtctcattcttcccacaagccgagacatgcaaggtgcagagcaaccgggtgttctgcgacaccatgaatagcagaaccctgccttccgaagtgaatctgtgcaacgtggacatcttcaaccctaagtacgactgcaagatcatgaccagcaagaccgacgtgtccagcagtgtgatcacctcactgggcgccatcgtgtcctgttacggcaagaccaagtgcaccgccagcaacaagaaccggggcatcatcaagaccttcagcaacggctgcgactacgtgtccaacaaaggcgtggacaccgtgtctgtgggcaacaccctgtactacgtgaacaaacaagagggccagtctctgtacgtgaagggcgagcccatcatcaacttctacgaccctctggtgttccccagcgacgagttcgatgccagcatcagccaagtgaacgagaagatcaatcagagcctggccttcatcagaaagtccgatgagctgctgcacaacgtgaacgccggcaagtccaccaccaatatcatgatcacgaccatcatcatcgtgattatcgtgatcctgctgtccctgatcgccgtgggcctgctgctttattgataataggctggagcctcggtggccatgcttcttgccccttgggcctccccccagcccctcctccccttcctgcacccgtacccccgtggtctttgaataaagtctgagtgggcggcaaaaaaaaaaaaaaaaaaaaaaaaaaaaaaaaaaaaaaaaaaaaaaaaaaaaaaaaaaaaaaaaaaaaaaaaaaaaaaaaaaaaaaaaaaaaaaaaaaaaaaaaaaaaaa

SEQ ID NO: 118 - DNA, 1841 bp, synthetic construct
  source 1..1841: mol_type = other DNA
agcggctcggccattttgtcccagtcagtccggaggctgcggctgcagaagtaccgcctgcggagtaactgcaaaggccaccatggaactgctgatcctgaaggccaacgccatcaccaccatcctgaccgccgtgaccttctgttttgccagcggccagaacatcaccgaggaattctaccagagcacctgtagcgccgtgtccaagggatatctgggcgcccttagaaccggctggtactgcagcgtgatcaccatcgagctgagcaacatcaaagaaaacaagtgcaacggcaccgacgccaaagtgaagctgatcaagcaagagctggacaagtacaagaatgccgtgaccgacctgcagctgctgatgcagtctacaccagccacaggctctggcagcgccattgcctctggtgtctgcgtgtctaaagtgctgcacctggaaggcgaagtgaacaagatcaagagcgccctgctgagcaccaacaaggccgtggtgtctctgagcaatggcgtgtccgtgctgaccttcaaggtgctggacctgaagaactacatcgacaaacagctgctgcccatcctgaacaagcagtcctgcagcatccccaacatcgagacagtgatcgagttccagcagaagaacaaccggctgctggaaatcacccgcgagttctctgtgaatgccggcgtgaccacacctgtgtccacctacatgctgaccaacagcgagctgctgagcctgatcaacgacatgcccatcaccaacgaccagaaaaagctgatgagcaacaacgtgcagatcgtgcggcagcagagctacagcatcatgagcattatcaaagaagaggtgctggcctacgtggtgcagctgcctctgtatggcgtgatcgataccccttgctggaagctgcacacaagccctctgtgcaccaccaacaccaaagagggcagcaacatctgcctgaccagaaccgacagaggctggtactgcgataatgccggcagcgtctcattcttcccacaagccgagacatgcaaggtgcagagcaaccgggtgttctgcgacaccatgaatagcagaaccctgccttccgaagtgaatctgtgcaacgtggacatcttcaaccctaagtacgactgcaagatcatgaccagcaagaccgacgtgtccagcagtgtgatcacctcactgggcgccatcgtgtcctgttacggcaagaccaagtgcaccgccagcaacaagaaccggggcatcatcaagaccttcagcaacggctgcgactacgtgtccaacaaaggcgtggacaccgtgtctgtgggcaacaccctgtactacgtgaacaaacaagagggccagtctctgtacgtgaagggcgagcccatcatcaacttctacgaccctctggtgttccccagcgacgagttcgatgccagcatcagccaagtgaacgagaagatcaatcagagcctggccttcatcagaaagtccgatgagctgctgcacaacgtgaacgccggcaagtccaccaccaatatcatgatcacgaccatcatcatcgtgattatcgtgatcctgctgtccctgatcgccgtgggcctgctgctttattgataataggctggagcctcggtggccatgcttcttgccccttgggcctccccccagcccctcctccccttcctgcacccgtacccccgtggtctttgaataaagtctgagtgggcggcaaaaaaaaaaaaaaaaaaaaaaaaaaaaaaaaaaaaaaaaaaaaaaaaaaaaaaaaaaaaaaaaaaaaaaaaaaaaaaaaaaaaaaaaaaaaaaaaaaaaaaaaaaaaaa

SEQ ID NO: 119 - DNA, 1539 bp, synthetic construct
  source 1..1539: mol_type = other DNA
atggaactgctgatcctgaaggccaacgccatcaccaccatcctgaccgccgtgaccttctgttttgccagcggccagaacatcaccgaggaattctaccagagcacctgtagcgccgtgtccaagggatatctgggcgcccttagaaccggctggtactgcagcgtgatcaccatcgagctgagcaacatcaaagaaaacaagtgcaacggcaccgacgccaaagtgaagctgatcaagcaagagctggacaagtacaagaatgccgtgaccgacctgcagctgctgatgcagtctacaccagccacaggctctggcagcgccattgcctctggtgtctgcgtgtctaaagtgctgcacctggaaggcgaagtgaacaagatcaagagcgccctgctgagcaccaacaaggccgtggtgtctctgagcaatggcgtgtccgtgctgaccttcaaggtgctggacctgaagaactacatcgacaaacagctgctgcccatcctgaacaagcagtcctgcagcatccccaacatcgagacagtgatcgagttccagcagaagaacaaccggctgctggaaatcacccgcgagttctctgtgaatgccggcgtgaccacacctgtgtccacctacatgctgaccaacagcgagctgctgagcctgatcaacgacatgcccatcaccaacgaccagaaaaagctgatgagcaacaacgtgcagatcgtgcggcagcagagctacagcatcatgagcattatcaaagaagaggtgctggcctacgtggtgcagctgcctctgtatggcgtgatcgataccccttgctggaagctgcacacaagccctctgtgcaccaccaacaccaaagagggcagcaacatctgcctgaccagaaccgacagaggctggtactgcgataatgccggcagcgtctcattcttcccacaagccgagacatgcaaggtgcagagcaaccgggtgttctgcgacaccatgaatagcagaaccctgccttccgaagtgaatctgtgcaacgtggacatcttcaaccctaagtacgactgcaagatcatgaccagcaagaccgacgtgtccagcagtgtgatcacctcactgggcgccatcgtgtcctgttacggcaagaccaagtgcaccgccagcaacaagaaccggggcatcatcaagaccttcagcaacggctgcgactacgtgtccaacaaaggcgtggacaccgtgtctgtgggcaacaccctgtactacgtgaacaaacaagagggccagtctctgtacgtgaagggcgagcccatcatcaacttctacgaccctctggtgttccccagcgacgagttcgatgccagcatcagccaagtgaacgagaagatcaatcagagcctggccttcatcagaaagtccgatgagctgctgcacaacgtgaacgccggcaagtccaccaccaatatcatgatcacgaccatcatcatcgtgattatcgtgatcctgctgtccctgatcgccgtgggcctgctgctttattgataatag

SEQ ID NO: 120 - protein, 510 aa, synthetic construct
MELLILKANAITTILTAVTFCFASGQNITEEFYQSTCSAVSKGYLGALRTGWYCSVITIELSNIKENKCNGTDAKVKLIKQELDKYKNAVTDLQLLMQSTPATGSGSAIASGVCVSKVLHLEGEVNKIKSALLSTNKAVVSLSNGVSVLTFKVLDLKNYIDKQLLPILNKQSCSIPNIETVIEFQQKNNRLLEITREFSVNAGVTTPVSTYMLTNSELLSLINDMPITNDQKKLMSNNVQIVRQQSYSIMSIIKEEVLAYVVQLPLYGVIDTPCWKLHTSPLCTTNTKEGSNICLTRTDRGWYCDNAGSVSFFPQAETCKVQSNRVFCDTMNSRTLPSEVNLCNVDIFNPKYDCKIMTSKTDVSSSVITSLGAIVSCYGKTKCTASNKNRGIIKTFSNGCDYVSNKGVDTVSVGNTLYYVNKQEGQSLYVKGEPIINFYDPLVFPSDEFDASISQVNEKINQSLAFIRKSDELLHNVNAGKSTTNIMITTIIIVIIVILLSLIAVGLLLY

SEQ ID NO: 121 - RNA, 1841 nt, synthetic construct
  source 1..1841: mol_type = other RNA
agcggctcggccattttgtcccagtcagtccggaggctgcggctgcagaagtaccgcctgcggagtaactgcaaaggccaccatggaactgctgatcctgaaggccaacgccatcaccaccatcctgaccgccgtgaccttctgttttgccagcggccagaacatcaccgaggaattctaccagagcacctgtagcgccgtgtccaagggatatctgggcgcccttagaaccggctggtactgcagcgtgatcaccatcgagctgagcaacatcaaagaaaacaagtgcaacggcaccgacgccaaagtgaagctgatcaagcaagagctggacaagtacaagaatgccgtgaccgacctgcagctgctgatgcagtctacaccagccacaggctctggcagcgccattgcctctggtgtctgcgtgtctaaagtgctgcacctggaaggcgaagtgaacaagatcaagagcgccctgctgagcaccaacaaggccgtggtgtctctgagcaatggcgtgtccgtgctgaccttcaaggtgctggacctgaagaactacatcgacaaacagctgctgcccatcctgaacaagcagtcctgcagcatccccaacatcgagacagtgatcgagttccagcagaagaacaaccggctgctggaaatcacccgcgagttctctgtgaatgccggcgtgaccacacctgtgtccacctacatgctgaccaacagcgagctgctgagcctgatcaacgacatgcccatcaccaacgaccagaaaaagctgatgagcaacaacgtgcagatcgtgcggcagcagagctacagcatcatgagcattatcaaagaagaggtgctggcctacgtggtgcagctgcctctgtatggcgtgatcgataccccttgctggaagctgcacacaagccctctgtgcaccaccaacaccaaagagggcagcaacatctgcctgaccagaaccgacagaggctggtactgcgataatgccggcagcgtctcattcttcccacaagccgagacatgcaaggtgcagagcaaccgggtgttctgcgacaccatgaatagcagaaccctgccttccgaagtgaatctgtgcaacgtggacatcttcaaccctaagtacgactgcaagatcatgaccagcaagaccgacgtgtccagcagtgtgatcacctcactgggcgccatcgtgtcctgttacggcaagaccaagtgcaccgccagcaacaagaaccggggcatcatcaagaccttcagcaacggctgcgactacgtgtccaacaaaggcgtggacaccgtgtctgtgggcaacaccctgtactacgtgaacaaacaagagggccagtctctgtacgtgaagggcgagcccatcatcaacttctacgaccctctggtgttccccagcgacgagttcgatgccagcatcagccaagtgaacgagaagatcaatcagagcctggccttcatcagaaagtccgatgagctgctgcacaacgtgaacgccggcaagtccaccaccaatatcatgatcacgaccatcatcatcgtgattatcgtgatcctgctgtccctgatcgccgtgggcctgctgctttattgataataggctggagcctcggtggccatgcttcttgccccttgggcctccccccagcccctcctccccttcctgcacccgtacccccgtggtctttgaataaagtctgagtgggcggcaaaaaaaaaaaaaaaaaaaaaaaaaaaaaaaaaaaaaaaaaaaaaaaaaaaaaaaaaaaaaaaaaaaaaaaaaaaaaaaaaaaaaaaaaaaaaaaaaaaaaaaaaaaaaa

SEQ ID NO: 122 - DNA, 1841 bp, synthetic construct
  source 1..1841: mol_type = other DNA
agcggctcggccattttgtcccagtcagtccggaggctgcggctgcagaagtaccgcctgcggagtaactgcaaaggccaccatggaactgctgatcctgaaggccaacgccatcaccaccatcctgaccgccgtgaccttctgttttgccagcggccagaacatcaccgaggaattctaccagagcacctgtagcgccgtgtgcaagggatatctgggcgcccttagaaccggctggtacaccagcgtgatcaccatcgagctgagcaacatcaaagaaaacaagtgcaacggcaccgacgccaaagtgaagctgatcaagcaagagctggacaagtacaagaatgccgtgaccgacctgcagctgctgatgcagtctacaccagccacaggctctggcagcgccattgcctctggtgtcgccgtgtctaaagtgctgcacctggaaggcgaagtgaacaagatcaagagcgccctgctgagcaccaacaaggccgtggtgtctctgagcaatggcgtgtccgtgctgaccttcaaggtgctggacctgaagaactacatcgacaaacagctgctgcccatcctgaacaagcagtcctgcagcatccccaacatcgagacagtgatcgagttccagcagaagaacaaccggctgctggaaatcacccgcgagttctctgtgaatgccggcgtgaccacacctgtgtccacctacatgctgaccaacagcgagctgctgagcctgatcaacgacatgcccatcaccaacgaccagaaaaagctgatgagcaacaacgtgcagatcgtgcggcagcagagctacagcatcatgagcattatcaaagaagaggtgctggcctacgtggtgcagctgcctctgtatggcgtgatcgataccccttgctggaagctgcacacatgccctctgtgcaccaccaacaccaaagagggcagcaacatctgcctgaccagaaccgacagaggctggtactgcgataatgccggcagcgtctcattcttcccacaagccgagacatgcaaggtgcagagcaaccgggtgttctgcgacaccatgaatagcagaaccctgccttccgaagtgaatctgtgcaacgtggacatcttcaaccctaagtacgactgcaagatcatgaccagcaagaccgacgtgtccagcagtgtgatcacctcactgggcgccatcgtgtcctgttacggcaagaccaagtgcaccgccagcaacaagaaccggggcatcatcaagaccttcagcaacggctgcgactacgtgtccaacaaaggcgtggacaccgtgtctgtgggcaacaccctgtactacgtgaacaaacaagagggccagtctctgtacgtgaagggcgagcccatcatcaacttctacgaccctctggtgttccccagcgacgagttcgatgccagcatcagccaagtgaacgagaagatcaatcagagcctggccttcatcagaaagtccgatgagctgctgcacaacgtgaacgccggcaagtccaccaccaatatcatgatcacgaccatcatcatcgtgattatcgtgatcctgctgtccctgatcgccgtgggcctgctgctttattgataataggctggagcctcggtggccatgcttcttgccccttgggcctccccccagcccctcctccccttcctgcacccgtacccccgtggtctttgaataaagtctgagtgggcggcaaaaaaaaaaaaaaaaaaaaaaaaaaaaaaaaaaaaaaaaaaaaaaaaaaaaaaaaaaaaaaaaaaaaaaaaaaaaaaaaaaaaaaaaaaaaaaaaaaaaaaaaaaaaaa

SEQ ID NO: 123 - DNA, 1539 bp, synthetic construct
  source 1..1539: mol_type = other DNA
atggaactgctgatcctgaaggccaacgccatcaccaccatcctgaccgccgtgaccttctgttttgccagcggccagaacatcaccgaggaattctaccagagcacctgtagcgccgtgtgcaagggatatctgggcgcccttagaaccggctggtacaccagcgtgatcaccatcgagctgagcaacatcaaagaaaacaagtgcaacggcaccgacgccaaagtgaagctgatcaagcaagagctggacaagtacaagaatgccgtgaccgacctgcagctgctgatgcagtctacaccagccacaggctctggcagcgccattgcctctggtgtcgccgtgtctaaagtgctgcacctggaaggcgaagtgaacaagatcaagagcgccctgctgagcaccaacaaggccgtggtgtctctgagcaatggcgtgtccgtgctgaccttcaaggtgctggacctgaagaactacatcgacaaacagctgctgcccatcctgaacaagcagtcctgcagcatccccaacatcgagacagtgatcgagttccagcagaagaacaaccggctgctggaaatcacccgcgagttctctgtgaatgccggcgtgaccacacctgtgtccacctacatgctgaccaacagcgagctgctgagcctgatcaacgacatgcccatcaccaacgaccagaaaaagctgatgagcaacaacgtgcagatcgtgcggcagcagagctacagcatcatgagcattatcaaagaagaggtgctggcctacgtggtgcagctgcctctgtatggcgtgatcgataccccttgctggaagctgcacacatgccctctgtgcaccaccaacaccaaagagggcagcaacatctgcctgaccagaaccgacagaggctggtactgcgataatgccggcagcgtctcattcttcccacaagccgagacatgcaaggtgcagagcaaccgggtgttctgcgacaccatgaatagcagaaccctgccttccgaagtgaatctgtgcaacgtggacatcttcaaccctaagtacgactgcaagatcatgaccagcaagaccgacgtgtccagcagtgtgatcacctcactgggcgccatcgtgtcctgttacggcaagaccaagtgcaccgccagcaacaagaaccggggcatcatcaagaccttcagcaacggctgcgactacgtgtccaacaaaggcgtggacaccgtgtctgtgggcaacaccctgtactacgtgaacaaacaagagggccagtctctgtacgtgaagggcgagcccatcatcaacttctacgaccctctggtgttccccagcgacgagttcgatgccagcatcagccaagtgaacgagaagatcaatcagagcctggccttcatcagaaagtccgatgagctgctgcacaacgtgaacgccggcaagtccaccaccaatatcatgatcacgaccatcatcatcgtgattatcgtgatcctgctgtccctgatcgccgtgggcctgctgctttattgataatag

SEQ ID NO: 124 - protein, 510 aa, synthetic construct
MELLILKANAITTILTAVTFCFASGQNITEEFYQSTCSAVCKGYLGALRTGWYTSVITIELSNIKENKCNGTDAKVKLIKQELDKYKNAVTDLQLLMQSTPATGSGSAIASGVAVSKVLHLEGEVNKIKSALLSTNKAVVSLSNGVSVLTFKVLDLKNYIDKQLLPILNKQSCSIPNIETVIEFQQKNNRLLEITREFSVNAGVTTPVSTYMLTNSELLSLINDMPITNDQKKLMSNNVQIVRQQSYSIMSIIKEEVLAYVVQLPLYGVIDTPCWKLHTCPLCTTNTKEGSNICLTRTDRGWYCDNAGSVSFFPQAETCKVQSNRVFCDTMNSRTLPSEVNLCNVDIFNPKYDCKIMTSKTDVSSSVITSLGAIVSCYGKTKCTASNKNRGIIKTFSNGCDYVSNKGVDTVSVGNTLYYVNKQEGQSLYVKGEPIINFYDPLVFPSDEFDASISQVNEKINQSLAFIRKSDELLHNVNAGKSTTNIMITTIIIVIIVILLSLIAVGLLLY

SEQ ID NO: 125 - RNA, 1841 nt, synthetic construct
  source 1..1841: mol_type = other RNA
agcggctcggccattttgtcccagtcagtccggaggctgcggctgcagaagtaccgcctgcggagtaactgcaaaggccaccatggaactgctgatcctgaaggccaacgccatcaccaccatcctgaccgccgtgaccttctgttttgccagcggccagaacatcaccgaggaattctaccagagcacctgtagcgccgtgtgcaagggatatctgggcgcccttagaaccggctggtacaccagcgtgatcaccatcgagctgagcaacatcaaagaaaacaagtgcaacggcaccgacgccaaagtgaagctgatcaagcaagagctggacaagtacaagaatgccgtgaccgacctgcagctgctgatgcagtctacaccagccacaggctctggcagcgccattgcctctggtgtcgccgtgtctaaagtgctgcacctggaaggcgaagtgaacaagatcaagagcgccctgctgagcaccaacaaggccgtggtgtctctgagcaatggcgtgtccgtgctgaccttcaaggtgctggacctgaagaactacatcgacaaacagctgctgcccatcctgaacaagcagtcctgcagcatccccaacatcgagacagtgatcgagttccagcagaagaacaaccggctgctggaaatcacccgcgagttctctgtgaatgccggcgtgaccacacctgtgtccacctacatgctgaccaacagcgagctgctgagcctgatcaacgacatgcccatcaccaacgaccagaaaaagctgatgagcaacaacgtgcagatcgtgcggcagcagagctacagcatcatgagcattatcaaagaagaggtgctggcctacgtggtgcagctgcctctgtatggcgtgatcgataccccttgctggaagctgcacacatgccctctgtgcaccaccaacaccaaagagggcagcaacatctgcctgaccagaaccgacagaggctggtactgcgataatgccggcagcgtctcattcttcccacaagccgagacatgcaaggtgcagagcaaccgggtgttctgcgacaccatgaatagcagaaccctgccttccgaagtgaatctgtgcaacgtggacatcttcaaccctaagtacgactgcaagatcatgaccagcaagaccgacgtgtccagcagtgtgatcacctcactgggcgccatcgtgtcctgttacggcaagaccaagtgcaccgccagcaacaagaaccggggcatcatcaagaccttcagcaacggctgcgactacgtgtccaacaaaggcgtggacaccgtgtctgtgggcaacaccctgtactacgtgaacaaacaagagggccagtctctgtacgtgaagggcgagcccatcatcaacttctacgaccctctggtgttccccagcgacgagttcgatgccagcatcagccaagtgaacgagaagatcaatcagagcctggccttcatcagaaagtccgatgagctgctgcacaacgtgaacgccggcaagtccaccaccaatatcatgatcacgaccatcatcatcgtgattatcgtgatcctgctgtccctgatcgccgtgggcctgctgctttattgataataggctggagcctcggtggccatgcttcttgccccttgggcctccccccagcccctcctccccttcctgcacccgtacccccgtggtctttgaataaagtctgagtgggcggcaaaaaaaaaaaaaaaaaaaaaaaaaaaaaaaaaaaaaaaaaaaaaaaaaaaaaaaaaaaaaaaaaaaaaaaaaaaaaaaaaaaaaaaaaaaaaaaaaaaaaaaaaaaaaa

SEQ ID NO: 126 - DNA, 1841 bp, synthetic construct
  source 1..1841: mol_type = other DNA
agcggctcggccattttgtcccagtcagtccggaggctgcggctgcagaagtaccgcctgcggagtaactgcaaaggccaccatggaactgctgatcctgaaggccaacgccatcaccaccatcctgaccgccgtgaccttctgttttgccagcggccagaacatcaccgaggaattctaccagagcacctgtagcgccgtgtccaagggatgcctgggcgcccttagaaccggctggtacaccagcgtgatcaccatcgagctgagcaacatcaaagaaaacaagtgcaacggcaccgacgccaaagtgaagctgatcaagcaagagctggacaagtacaagaatgccgtgaccgacctgcagctgctgatgcagtctacaccagccacaggctctggcagcgccattgcctctggtgtcgccgtgtctaaagtgctgcacctggaaggcgaagtgaacaagatcaagagcgccctgctgagcaccaacaaggccgtggtgtctctgagcaatggcgtgtccgtgctgaccttcaaggtgctggacctgaagaactacatcgacaaacagctgctgcccatcctgaacaagcagtcctgcagcatccccaacatcgagacagtgatcgagttccagcagaagaacaaccggctgctggaaatcacccgcgagttctctgtgaatgccggcgtgaccacacctgtgtccacctacatgctgaccaacagcgagctgctgagcctgatcaacgacatgcccatcaccaacgaccagaaaaagctgatgagcaacaacgtgcagatcgtgcggcagcagagctacagcatcatgagcattatcaaagaagaggtgctggcctacgtggtgcagctgcctctgtatggcgtgatcgataccccttgctggaagctgcacacatgccctctgtgcaccaccaacaccaaagagggcagcaacatctgcctgaccagaaccgacagaggctggtactgcgataatgccggcagcgtctcattcttcccacaagccgagacatgcaaggtgcagagcaaccgggtgttctgcgacaccatgaatagcagaaccctgccttccgaagtgaatctgtgcaacgtggacatcttcaaccctaagtacgactgcaagatcatgaccagcaagaccgacgtgtccagcagtgtgatcacctcactgggcgccatcgtgtcctgttacggcaagaccaagtgcaccgccagcaacaagaaccggggcatcatcaagaccttcagcaacggctgcgactacgtgtccaacaaaggcgtggacaccgtgtctgtgggcaacaccctgtactacgtgaacaaacaagagggccagtctctgtacgtgaagggcgagcccatcatcaacttctacgaccctctggtgttccccagcgacgagttcgatgccagcatcagccaagtgaacgagaagatcaatcagagcctggccttcatcagaaagtccgatgagctgctgcacaacgtgaacgccggcaagtccaccaccaatatcatgatcacgaccatcatcatcgtgattatcgtgatcctgctgtccctgatcgccgtgggcctgctgctttattgataataggctggagcctcggtggccatgcttcttgccccttgggcctccccccagcccctcctccccttcctgcacccgtacccccgtggtctttgaataaagtctgagtgggcggcaaaaaaaaaaaaaaaaaaaaaaaaaaaaaaaaaaaaaaaaaaaaaaaaaaaaaaaaaaaaaaaaaaaaaaaaaaaaaaaaaaaaaaaaaaaaaaaaaaaaaaaaaaaaaa

SEQ ID NO: 127 - DNA, 1539 bp, synthetic construct
  source 1..1539: mol_type = other DNA
atggaactgctgatcctgaaggccaacgccatcaccaccatcctgaccgccgtgaccttctgttttgccagcggccagaacatcaccgaggaattctaccagagcacctgtagcgccgtgtccaagggatgcctgggcgcccttagaaccggctggtacaccagcgtgatcaccatcgagctgagcaacatcaaagaaaacaagtgcaacggcaccgacgccaaagtgaagctgatcaagcaagagctggacaagtacaagaatgccgtgaccgacctgcagctgctgatgcagtctacaccagccacaggctctggcagcgccattgcctctggtgtcgccgtgtctaaagtgctgcacctggaaggcgaagtgaacaagatcaagagcgccctgctgagcaccaacaaggccgtggtgtctctgagcaatggcgtgtccgtgctgaccttcaaggtgctggacctgaagaactacatcgacaaacagctgctgcccatcctgaacaagcagtcctgcagcatccccaacatcgagacagtgatcgagttccagcagaagaacaaccggctgctggaaatcacccgcgagttctctgtgaatgccggcgtgaccacacctgtgtccacctacatgctgaccaacagcgagctgctgagcctgatcaacgacatgcccatcaccaacgaccagaaaaagctgatgagcaacaacgtgcagatcgtgcggcagcagagctacagcatcatgagcattatcaaagaagaggtgctggcctacgtggtgcagctgcctctgtatggcgtgatcgataccccttgctggaagctgcacacatgccctctgtgcaccaccaacaccaaagagggcagcaacatctgcctgaccagaaccgacagaggctggtactgcgataatgccggcagcgtctcattcttcccacaagccgagacatgcaaggtgcagagcaaccgggtgttctgcgacaccatgaatagcagaaccctgccttccgaagtgaatctgtgcaacgtggacatcttcaaccctaagtacgactgcaagatcatgaccagcaagaccgacgtgtccagcagtgtgatcacctcactgggcgccatcgtgtcctgttacggcaagaccaagtgcaccgccagcaacaagaaccggggcatcatcaagaccttcagcaacggctgcgactacgtgtccaacaaaggcgtggacaccgtgtctgtgggcaacaccctgtactacgtgaacaaacaagagggccagtctctgtacgtgaagggcgagcccatcatcaacttctacgaccctctggtgttccccagcgacgagttcgatgccagcatcagccaagtgaacgagaagatcaatcagagcctggccttcatcagaaagtccgatgagctgctgcacaacgtgaacgccggcaagtccaccaccaatatcatgatcacgaccatcatcatcgtgattatcgtgatcctgctgtccctgatcgccgtgggcctgctgctttattgataatag

SEQ ID NO: 128 - protein, 510 aa, synthetic construct
MELLILKANAITTILTAVTFCFASGQNITEEFYQSTCSAVSKGCLGALRTGWYTSVITIELSNIKENKCNGTDAKVKLIKQELDKYKNAVTDLQLLMQSTPATGSGSAIASGVAVSKVLHLEGEVNKIKSALLSTNKAVVSLSNGVSVLTFKVLDLKNYIDKQLLPILNKQSCSIPNIETVIEFQQKNNRLLEITREFSVNAGVTTPVSTYMLTNSELLSLINDMPITNDQKKLMSNNVQIVRQQSYSIMSIIKEEVLAYVVQLPLYGVIDTPCWKLHTCPLCTTNTKEGSNICLTRTDRGWYCDNAGSVSFFPQAETCKVQSNRVFCDTMNSRTLPSEVNLCNVDIFNPKYDCKIMTSKTDVSSSVITSLGAIVSCYGKTKCTASNKNRGIIKTFSNGCDYVSNKGVDTVSVGNTLYYVNKQEGQSLYVKGEPIINFYDPLVFPSDEFDASISQVNEKINQSLAFIRKSDELLHNVNAGKSTTNIMITTIIIVIIVILLSLIAVGLLLY

SEQ ID NO: 129 - RNA, 1841 nt, synthetic construct
  source 1..1841: mol_type = other RNA
agcggctcggccattttgtcccagtcagtccggaggctgcggctgcagaagtaccgcctgcggagtaactgcaaaggccaccatggaactgctgatcctgaaggccaacgccatcaccaccatcctgaccgccgtgaccttctgttttgccagcggccagaacatcaccgaggaattctaccagagcacctgtagcgccgtgtccaagggatgcctgggcgcccttagaaccggctggtacaccagcgtgatcaccatcgagctgagcaacatcaaagaaaacaagtgcaacggcaccgacgccaaagtgaagctgatcaagcaagagctggacaagtacaagaatgccgtgaccgacctgcagctgctgatgcagtctacaccagccacaggctctggcagcgccattgcctctggtgtcgccgtgtctaaagtgctgcacctggaaggcgaagtgaacaagatcaagagcgccctgctgagcaccaacaaggccgtggtgtctctgagcaatggcgtgtccgtgctgaccttcaaggtgctggacctgaagaactacatcgacaaacagctgctgcccatcctgaacaagcagtcctgcagcatccccaacatcgagacagtgatcgagttccagcagaagaacaaccggctgctggaaatcacccgcgagttctctgtgaatgccggcgtgaccacacctgtgtccacctacatgctgaccaacagcgagctgctgagcctgatcaacgacatgcccatcaccaacgaccagaaaaagctgatgagcaacaacgtgcagatcgtgcggcagcagagctacagcatcatgagcattatcaaagaagaggtgctggcctacgtggtgcagctgcctctgtatggcgtgatcgataccccttgctggaagctgcacacatgccctctgtgcaccaccaacaccaaagagggcagcaacatctgcctgaccagaaccgacagaggctggtactgcgataatgccggcagcgtctcattcttcccacaagccgagacatgcaaggtgcagagcaaccgggtgttctgcgacaccatgaatagcagaaccctgccttccgaagtgaatctgtgcaacgtggacatcttcaaccctaagtacgactgcaagatcatgaccagcaagaccgacgtgtccagcagtgtgatcacctcactgggcgccatcgtgtcctgttacggcaagaccaagtgcaccgccagcaacaagaaccggggcatcatcaagaccttcagcaacggctgcgactacgtgtccaacaaaggcgtggacaccgtgtctgtgggcaacaccctgtactacgtgaacaaacaagagggccagtctctgtacgtgaagggcgagcccatcatcaacttctacgaccctctggtgttccccagcgacgagttcgatgccagcatcagccaagtgaacgagaagatcaatcagagcctggccttcatcagaaagtccgatgagctgctgcacaacgtgaacgccggcaagtccaccaccaatatcatgatcacgaccatcatcatcgtgattatcgtgatcctgctgtccctgatcgccgtgggcctgctgctttattgataataggctggagcctcggtggccatgcttcttgccccttgggcctccccccagcccctcctccccttcctgcacccgtacccccgtggtctttgaataaagtctgagtgggcggcaaaaaaaaaaaaaaaaaaaaaaaaaaaaaaaaaaaaaaaaaaaaaaaaaaaaaaaaaaaaaaaaaaaaaaaaaaaaaaaaaaaaaaaaaaaaaaaaaaaaaaaaaaaaaa

SEQ ID NO: 130 - DNA, 1841 bp, synthetic construct
  source 1..1841: mol_type = other DNA
agcggctcggccattttgtcccagtcagtccggaggctgcggctgcagaagtaccgcctgcggagtaactgcaaaggccaccatggaactgctgatcctgaaggccaacgccatcaccaccatcctgaccgccgtgaccttctgttttgccagcggccagaacatcaccgaggaattctaccagagcacctgtagcgccgtgtccaagggatatctgggcgcccttagaaccggctggtacaccagcgtgatcaccatcgagctgagcaacatcaaagaaaacaagtgcaacggcaccgacgccaaagtgaagctgatcaagcaagagctggacaagtacaagaatgccgtgaccgacctgcagctgctgatgcagtcttgcccagccacaggctctggcagcgccattgcctgcggtgtcgccgtgtctaaagtgctgcacctggaaggcgaagtgaacaagatcaagagcgccctgctgagcaccaacaaggccgtggtgtctctgagcaatggcgtgtccgtgctgaccttcaaggtgctggacctgaagaactacatcgacaaacagctgctgcccatcctgaacaagcagtcctgcagcatccccaacatcgagacagtgatcgagttccagcagaagaacaaccggctgctggaaatcacccgcgagttctctgtgaatgccggcgtgaccacacctgtgtccacctacatgctgaccaacagcgagctgctgagcctgatcaacgacatgcccatcaccaacgaccagaaaaagctgatgagcaacaacgtgcagatcgtgcggcagcagagctacagcatcatgagcattatcaaagaagaggtgctggcctacgtggtgcagctgcctctgtatggcgtgatcgataccccttgctggaagctgcacacaagccctctgtgcaccaccaacaccaaagagggcagcaacatctgcctgaccagaaccgacagaggctggtactgcgataatgccggcagcgtctcattcttcccacaagccgagacatgcaaggtgcagagcaaccgggtgttctgcgacaccatgaatagcagaaccctgccttccgaagtgaatctgtgcaacgtggacatcttcaaccctaagtacgactgcaagatcatgaccagcaagaccgacgtgtccagcagtgtgatcacctcactgggcgccatcgtgtcctgttacggcaagaccaagtgcaccgccagcaacaagaaccggggcatcatcaagaccttcagcaacggctgcgactacgtgtccaacaaaggcgtggacaccgtgtctgtgggcaacaccctgtactacgtgaacaaacaagagggccagtctctgtacgtgaagggcgagcccatcatcaacttctacgaccctctggtgttccccagcgacgagttcgatgccagcatcagccaagtgaacgagaagatcaatcagagcctggccttcatcagaaagtccgatgagctgctgcacaacgtgaacgccggcaagtccaccaccaatatcatgatcacgaccatcatcatcgtgattatcgtgatcctgctgtccctgatcgccgtgggcctgctgctttattgataataggctggagcctcggtggccatgcttcttgccccttgggcctccccccagcccctcctccccttcctgcacccgtacccccgtggtctttgaataaagtctgagtgggcggcaaaaaaaaaaaaaaaaaaaaaaaaaaaaaaaaaaaaaaaaaaaaaaaaaaaaaaaaaaaaaaaaaaaaaaaaaaaaaaaaaaaaaaaaaaaaaaaaaaaaaaaaaaaaaa

SEQ ID NO: 131 - DNA, 1539 bp, synthetic construct
  source 1..1539: mol_type = other DNA
atggaactgctgatcctgaaggccaacgccatcaccaccatcctgaccgccgtgaccttctgttttgccagcggccagaacatcaccgaggaattctaccagagcacctgtagcgccgtgtccaagggatatctgggcgcccttagaaccggctggtacaccagcgtgatcaccatcgagctgagcaacatcaaagaaaacaagtgcaacggcaccgacgccaaagtgaagctgatcaagcaagagctggacaagtacaagaatgccgtgaccgacctgcagctgctgatgcagtcttgcccagccacaggctctggcagcgccattgcctgcggtgtcgccgtgtctaaagtgctgcacctggaaggcgaagtgaacaagatcaagagcgccctgctgagcaccaacaaggccgtggtgtctctgagcaatggcgtgtccgtgctgaccttcaaggtgctggacctgaagaactacatcgacaaacagctgctgcccatcctgaacaagcagtcctgcagcatccccaacatcgagacagtgatcgagttccagcagaagaacaaccggctgctggaaatcacccgcgagttctctgtgaatgccggcgtgaccacacctgtgtccacctacatgctgaccaacagcgagctgctgagcctgatcaacgacatgcccatcaccaacgaccagaaaaagctgatgagcaacaacgtgcagatcgtgcggcagcagagctacagcatcatgagcattatcaaagaagaggtgctggcctacgtggtgcagctgcctctgtatggcgtgatcgataccccttgctggaagctgcacacaagccctctgtgcaccaccaacaccaaagagggcagcaacatctgcctgaccagaaccgacagaggctggtactgcgataatgccggcagcgtctcattcttcccacaagccgagacatgcaaggtgcagagcaaccgggtgttctgcgacaccatgaatagcagaaccctgccttccgaagtgaatctgtgcaacgtggacatcttcaaccctaagtacgactgcaagatcatgaccagcaagaccgacgtgtccagcagtgtgatcacctcactgggcgccatcgtgtcctgttacggcaagaccaagtgcaccgccagcaacaagaaccggggcatcatcaagaccttcagcaacggctgcgactacgtgtccaacaaaggcgtggacaccgtgtctgtgggcaacaccctgtactacgtgaacaaacaagagggccagtctctgtacgtgaagggcgagcccatcatcaacttctacgaccctctggtgttccccagcgacgagttcgatgccagcatcagccaagtgaacgagaagatcaatcagagcctggccttcatcagaaagtccgatgagctgctgcacaacgtgaacgccggcaagtccaccaccaatatcatgatcacgaccatcatcatcgtgattatcgtgatcctgctgtccctgatcgccgtgggcctgctgctttattgataatag

SEQ ID NO: 132 - protein, 510 aa, synthetic construct
MELLILKANAITTILTAVTFCFASGQNITEEFYQSTCSAVSKGYLGALRTGWYTSVITIELSNIKENKCNGTDAKVKLIKQELDKYKNAVTDLQLLMQSCPATGSGSAIACGVAVSKVLHLEGEVNKIKSALLSTNKAVVSLSNGVSVLTFKVLDLKNYIDKQLLPILNKQSCSIPNIETVIEFQQKNNRLLEITREFSVNAGVTTPVSTYMLTNSELLSLINDMPITNDQKKLMSNNVQIVRQQSYSIMSIIKEEVLAYVVQLPLYGVIDTPCWKLHTSPLCTTNTKEGSNICLTRTDRGWYCDNAGSVSFFPQAETCKVQSNRVFCDTMNSRTLPSEVNLCNVDIFNPKYDCKIMTSKTDVSSSVITSLGAIVSCYGKTKCTASNKNRGIIKTFSNGCDYVSNKGVDTVSVGNTLYYVNKQEGQSLYVKGEPIINFYDPLVFPSDEFDASISQVNEKINQSLAFIRKSDELLHNVNAGKSTTNIMITTIIIVIIVILLSLIAVGLLLY

SEQ ID NO: 133 - RNA, 1841 nt, synthetic construct
  source 1..1841: mol_type = other RNA
agcggctcggccattttgtcccagtcagtccggaggctgcggctgcagaagtaccgcctgcggagtaactgcaaaggccaccatggaactgctgatcctgaaggccaacgccatcaccaccatcctgaccgccgtgaccttctgttttgccagcggccagaacatcaccgaggaattctaccagagcacctgtagcgccgtgtccaagggatatctgggcgcccttagaaccggctggtacaccagcgtgatcaccatcgagctgagcaacatcaaagaaaacaagtgcaacggcaccgacgccaaagtgaagctgatcaagcaagagctggacaagtacaagaatgccgtgaccgacctgcagctgctgatgcagtcttgcccagccacaggctctggcagcgccattgcctgcggtgtcgccgtgtctaaagtgctgcacctggaaggcgaagtgaacaagatcaagagcgccctgctgagcaccaacaaggccgtggtgtctctgagcaatggcgtgtccgtgctgaccttcaaggtgctggacctgaagaactacatcgacaaacagctgctgcccatcctgaacaagcagtcctgcagcatccccaacatcgagacagtgatcgagttccagcagaagaacaaccggctgctggaaatcacccgcgagttctctgtgaatgccggcgtgaccacacctgtgtccacctacatgctgaccaacagcgagctgctgagcctgatcaacgacatgcccatcaccaacgaccagaaaaagctgatgagcaacaacgtgcagatcgtgcggcagcagagctacagcatcatgagcattatcaaagaagaggtgctggcctacgtggtgcagctgcctctgtatggcgtgatcgataccccttgctggaagctgcacacaagccctctgtgcaccaccaacaccaaagagggcagcaacatctgcctgaccagaaccgacagaggctggtactgcgataatgccggcagcgtctcattcttcccacaagccgagacatgcaaggtgcagagcaaccgggtgttctgcgacaccatgaatagcagaaccctgccttccgaagtgaatctgtgcaacgtggacatcttcaaccctaagtacgactgcaagatcatgaccagcaagaccgacgtgtccagcagtgtgatcacctcactgggcgccatcgtgtcctgttacggcaagaccaagtgcaccgccagcaacaagaaccggggcatcatcaagaccttcagcaacggctgcgactacgtgtccaacaaaggcgtggacaccgtgtctgtgggcaacaccctgtactacgtgaacaaacaagagggccagtctctgtacgtgaagggcgagcccatcatcaacttctacgaccctctggtgttccccagcgacgagttcgatgccagcatcagccaagtgaacgagaagatcaatcagagcctggccttcatcagaaagtccgatgagctgctgcacaacgtgaacgccggcaagtccaccaccaatatcatgatcacgaccatcatcatcgtgattatcgtgatcctgctgtccctgatcgccgtgggcctgctgctttattgataataggctggagcctcggtggccatgcttcttgccccttgggcctccccccagcccctcctccccttcctgcacccgtacccccgtggtctttgaataaagtctgagtgggcggcaaaaaaaaaaaaaaaaaaaaaaaaaaaaaaaaaaaaaaaaaaaaaaaaaaaaaaaaaaaaaaaaaaaaaaaaaaaaaaaaaaaaaaaaaaaaaaaaaaaaaaaaaaaaaa

SEQ ID NO: 134 - DNA, 1841 bp, synthetic construct
  source 1..1841: mol_type = other DNA
agcggctcggccattttgtcccagtcagtccggaggctgcggctgcagaagtaccgcctgcggagtaactgcaaaggccaccatggaactgctgatcctgaaggccaacgccatcaccaccatcctgaccgccgtgaccttctgttttgccagcggccagaacatcaccgaggaattctaccagagcacctgtagcgccgtgtccaagggatatctgggcgcccttagaaccggctggtacaccagcgtgatcaccatcgagctgagcaacatcaaagaaaacaagtgcaacggcaccgacgccaaagtgaagctgatcaagcaagagctggacaagtacaagaatgccgtgaccgacctgcagctgctgatgcagtcttgcccagccacaggctctggcagcgccatttgctctggtgtcgccgtgtctaaagtgctgcacctggaaggcgaagtgaacaagatcaagagcgccctgctgagcaccaacaaggccgtggtgtctctgagcaatggcgtgtccgtgctgaccttcaaggtgctggacctgaagaactacatcgacaaacagctgctgcccatcctgaacaagcagtcctgcagcatccccaacatcgagacagtgatcgagttccagcagaagaacaaccggctgctggaaatcacccgcgagttctctgtgaatgccggcgtgaccacacctgtgtccacctacatgctgaccaacagcgagctgctgagcctgatcaacgacatgcccatcaccaacgaccagaaaaagctgatgagcaacaacgtgcagatcgtgcggcagcagagctacagcatcatgagcattatcaaagaagaggtgctggcctacgtggtgcagctgcctctgtatggcgtgatcgataccccttgctggaagctgcacacaagccctctgtgcaccaccaacaccaaagagggcagcaacatctgcctgaccagaaccgacagaggctggtactgcgataatgccggcagcgtctcattcttcccacaagccgagacatgcaaggtgcagagcaaccgggtgttctgcgacaccatgaatagcagaaccctgccttccgaagtgaatctgtgcaacgtggacatcttcaaccctaagtacgactgcaagatcatgaccagcaagaccgacgtgtccagcagtgtgatcacctcactgggcgccatcgtgtcctgttacggcaagaccaagtgcaccgccagcaacaagaaccggggcatcatcaagaccttcagcaacggctgcgactacgtgtccaacaaaggcgtggacaccgtgtctgtgggcaacaccctgtactacgtgaacaaacaagagggccagtctctgtacgtgaagggcgagcccatcatcaacttctacgaccctctggtgttccccagcgacgagttcgatgccagcatcagccaagtgaacgagaagatcaatcagagcctggccttcatcagaaagtccgatgagctgctgcacaacgtgaacgccggcaagtccaccaccaatatcatgatcacgaccatcatcatcgtgattatcgtgatcctgctgtccctgatcgccgtgggcctgctgctttattgataataggctggagcctcggtggccatgcttcttgccccttgggcctccccccagcccctcctccccttcctgcacccgtacccccgtggtctttgaataaagtctgagtgggcggcaaaaaaaaaaaaaaaaaaaaaaaaaaaaaaaaaaaaaaaaaaaaaaaaaaaaaaaaaaaaaaaaaaaaaaaaaaaaaaaaaaaaaaaaaaaaaaaaaaaaaaaaaaaaaa

SEQ ID NO: 135 - DNA, 1539 bp, synthetic construct
  source 1..1539: mol_type = other DNA
atggaactgctgatcctgaaggccaacgccatcaccaccatcctgaccgccgtgaccttctgttttgccagcggccagaacatcaccgaggaattctaccagagcacctgtagcgccgtgtccaagggatatctgggcgcccttagaaccggctggtacaccagcgtgatcaccatcgagctgagcaacatcaaagaaaacaagtgcaacggcaccgacgccaaagtgaagctgatcaagcaagagctggacaagtacaagaatgccgtgaccgacctgcagctgctgatgcagtcttgcccagccacaggctctggcagcgccatttgctctggtgtcgccgtgtctaaagtgctgcacctggaaggcgaagtgaacaagatcaagagcgccctgctgagcaccaacaaggccgtggtgtctctgagcaatggcgtgtccgtgctgaccttcaaggtgctggacctgaagaactacatcgacaaacagctgctgcccatcctgaacaagcagtcctgcagcatccccaacatcgagacagtgatcgagttccagcagaagaacaaccggctgctggaaatcacccgcgagttctctgtgaatgccggcgtgaccacacctgtgtccacctacatgctgaccaacagcgagctgctgagcctgatcaacgacatgcccatcaccaacgaccagaaaaagctgatgagcaacaacgtgcagatcgtgcggcagcagagctacagcatcatgagcattatcaaagaagaggtgctggcctacgtggtgcagctgcctctgtatggcgtgatcgataccccttgctggaagctgcacacaagccctctgtgcaccaccaacaccaaagagggcagcaacatctgcctgaccagaaccgacagaggctggtactgcgataatgccggcagcgtctcattcttcccacaagccgagacatgcaaggtgcagagcaaccgggtgttctgcgacaccatgaatagcagaaccctgccttccgaagtgaatctgtgcaacgtggacatcttcaaccctaagtacgactgcaagatcatgaccagcaagaccgacgtgtccagcagtgtgatcacctcactgggcgccatcgtgtcctgttacggcaagaccaagtgcaccgccagcaacaagaaccggggcatcatcaagaccttcagcaacggctgcgactacgtgtccaacaaaggcgtggacaccgtgtctgtgggcaacaccctgtactacgtgaacaaacaagagggccagtctctgtacgtgaagggcgagcccatcatcaacttctacgaccctctggtgttccccagcgacgagttcgatgccagcatcagccaagtgaacgagaagatcaatcagagcctggccttcatcagaaagtccgatgagctgctgcacaacgtgaacgccggcaagtccaccaccaatatcatgatcacgaccatcatcatcgtgattatcgtgatcctgctgtccctgatcgccgtgggcctgctgctttattgataatag

SEQ ID NO: 136 - protein, 510 aa, synthetic construct
MELLILKANAITTILTAVTFCFASGQNITEEFYQSTCSAVSKGYLGALRTGWYTSVITIELSNIKENKCNGTDAKVKLIKQELDKYKNAVTDLQLLMQSCPATGSGSAICSGVAVSKVLHLEGEVNKIKSALLSTNKAVVSLSNGVSVLTFKVLDLKNYIDKQLLPILNKQSCSIPNIETVIEFQQKNNRLLEITREFSVNAGVTTPVSTYMLTNSELLSLINDMPITNDQKKLMSNNVQIVRQQSYSIMSIIKEEVLAYVVQLPLYGVIDTPCWKLHTSPLCTTNTKEGSNICLTRTDRGWYCDNAGSVSFFPQAETCKVQSNRVFCDTMNSRTLPSEVNLCNVDIFNPKYDCKIMTSKTDVSSSVITSLGAIVSCYGKTKCTASNKNRGIIKTFSNGCDYVSNKGVDTVSVGNTLYYVNKQEGQSLYVKGEPIINFYDPLVFPSDEFDASISQVNEKINQSLAFIRKSDELLHNVNAGKSTTNIMITTIIIVIIVILLSLIAVGLLLY

SEQ ID NO: 137 - RNA, 1841 nt, synthetic construct
  source 1..1841: mol_type = other RNA
agcggctcggccattttgtcccagtcagtccggaggctgcggctgcagaagtaccgcctgcggagtaactgcaaaggccaccatggaactgctgatcctgaaggccaacgccatcaccaccatcctgaccgccgtgaccttctgttttgccagcggccagaacatcaccgaggaattctaccagagcacctgtagcgccgtgtccaagggatatctgggcgcccttagaaccggctggtacaccagcgtgatcaccatcgagctgagcaacatcaaagaaaacaagtgcaacggcaccgacgccaaagtgaagctgatcaagcaagagctggacaagtacaagaatgccgtgaccgacctgcagctgctgatgcagtcttgcccagccacaggctctggcagcgccatttgctctggtgtcgccgtgtctaaagtgctgcacctggaaggcgaagtgaacaagatcaagagcgccctgctgagcaccaacaaggccgtggtgtctctgagcaatggcgtgtccgtgctgaccttcaaggtgctggacctgaagaactacatcgacaaacagctgctgcccatcctgaacaagcagtcctgcagcatccccaacatcgagacagtgatcgagttccagcagaagaacaaccggctgctggaaatcacccgcgagttctctgtgaatgccggcgtgaccacacctgtgtccacctacatgctgaccaacagcgagctgctgagcctgatcaacgacatgcccatcaccaacgaccagaaaaagctgatgagcaacaacgtgcagatcgtgcggcagcagagctacagcatcatgagcattatcaaagaagaggtgctggcctacgtggtgcagctgcctctgtatggcgtgatcgataccccttgctggaagctgcacacaagccctctgtgcaccaccaacaccaaagagggcagcaacatctgcctgaccagaaccgacagaggctggtactgcgataatgccggcagcgtctcattcttcccacaagccgagacatgcaaggtgcagagcaaccgggtgttctgcgacaccatgaatagcagaaccctgccttccgaagtgaatctgtgcaacgtggacatcttcaaccctaagtacgactgcaagatcatgaccagcaagaccgacgtgtccagcagtgtgatcacctcactgggcgccatcgtgtcctgttacggcaagaccaagtgcaccgccagcaacaagaaccggggcatcatcaagaccttcagcaacggctgcgactacgtgtccaacaaaggcgtggacaccgtgtctgtgggcaacaccctgtactacgtgaacaaacaagagggccagtctctgtacgtgaagggcgagcccatcatcaacttctacgaccctctggtgttccccagcgacgagttcgatgccagcatcagccaagtgaacgagaagatcaatcagagcctggccttcatcagaaagtccgatgagctgctgcacaacgtgaacgccggcaagtccaccaccaatatcatgatcacgaccatcatcatcgtgattatcgtgatcctgctgtccctgatcgccgtgggcctgctgctttattgataataggctggagcctcggtggccatgcttcttgccccttgggcctccccccagcccctcctccccttcctgcacccgtacccccgtggtctttgaataaagtctgagtgggcggcaaaaaaaaaaaaaaaaaaaaaaaaaaaaaaaaaaaaaaaaaaaaaaaaaaaaaaaaaaaaaaaaaaaaaaaaaaaaaaaaaaaaaaaaaaaaaaaaaaaaaaaaaaaaaa

SEQ ID NO: 138 - DNA, 1841 bp, synthetic construct
  source 1..1841: mol_type = other DNA
agcggctcggccattttgtcccagtcagtccggaggctgcggctgcagaagtaccgcctgcggagtaactgcaaaggccaccatggaactgctgatcctgaaggccaacgccatcaccaccatcctgaccgccgtgaccttctgttttgccagcggccagaacatcaccgaggaattctaccagagcacctgtagcgccgtgtccaagggatatctgggcgcccttagaaccggctggtacaccagcgtgatcaccatcgagctgagcaacatcaaagaaaacaagtgcaacggcaccgacgccaaagtgaagctgatcaagcaagagctggacaagtacaagaatgccgtgaccgacctgcagctgctgatgcagtcttgcccagccacaggctctggcagcgccattgcctctggtgtcgccgtgtctaaagtgctgcacctggaaggcgaagtgaacaagatcaagagcgccctgctgagcaccaacaaggccgtggtgtctctgagcaatggcgtgtccgtgctgaccttcaaggtgctggacctgaagaactacatcgacaaacagctgctgcccatcctgaacaagcagtcctgcagcatccccaacatcgagacagtgatcgagttccagcagaagaacaaccggctgctggaaatcacccgcgagttctctgtgaatgccggcgtgaccacacctgtgtccacctacatgctgaccaacagcgagctgctgagcctgatcaacgacatgcccatcaccaacgaccagaaaaagctgatgagcaacaacgtgcagatcgtgcggcagcagagctacagcatcatgagcattatcaaagaagaggtgctggcctactgcgtgcagctgcctctgtatggcgtgatcgataccccttgctggaagctgcacacaagccctctgtgcaccaccaacaccaaagagggcagcaacatctgcctgaccagaaccgacagaggctggtactgcgataatgccggcagcgtctcattcttcccacaagccgagacatgcaaggtgcagagcaaccgggtgttctgcgacaccatgaatagcagaaccctgccttccgaagtgaatctgtgcaacgtggacatcttcaaccctaagtacgactgcaagatcatgaccagcaagaccgacgtgtccagcagtgtgatcacctcactgggcgccatcgtgtcctgttacggcaagaccaagtgcaccgccagcaacaagaaccggggcatcatcaagaccttcagcaacggctgcgactacgtgtccaacaaaggcgtggacaccgtgtctgtgggcaacaccctgtactacgtgaacaaacaagagggccagtctctgtacgtgaagggcgagcccatcatcaacttctacgaccctctggtgttccccagcgacgagttcgatgccagcatcagccaagtgaacgagaagatcaatcagagcctggccttcatcagaaagtccgatgagctgctgcacaacgtgaacgccggcaagtccaccaccaatatcatgatcacgaccatcatcatcgtgattatcgtgatcctgctgtccctgatcgccgtgggcctgctgctttattgataataggctggagcctcggtggccatgcttcttgccccttgggcctccccccagcccctcctccccttcctgcacccgtacccccgtggtctttgaataaagtctgagtgggcggcaaaaaaaaaaaaaaaaaaaaaaaaaaaaaaaaaaaaaaaaaaaaaaaaaaaaaaaaaaaaaaaaaaaaaaaaaaaaaaaaaaaaaaaaaaaaaaaaaaaaaaaaaaaaaa

SEQ ID NO: 139 - DNA, 1539 bp, synthetic construct
  source 1..1539: mol_type = other DNA
atggaactgctgatcctgaaggccaacgccatcaccaccatcctgaccgccgtgaccttctgttttgccagcggccagaacatcaccgaggaattctaccagagcacctgtagcgccgtgtccaagggatatctgggcgcccttagaaccggctggtacaccagcgtgatcaccatcgagctgagcaacatcaaagaaaacaagtgcaacggcaccgacgccaaagtgaagctgatcaagcaagagctggacaagtacaagaatgccgtgaccgacctgcagctgctgatgcagtcttgcccagccacaggctctggcagcgccattgcctctggtgtcgccgtgtctaaagtgctgcacctggaaggcgaagtgaacaagatcaagagcgccctgctgagcaccaacaaggccgtggtgtctctgagcaatggcgtgtccgtgctgaccttcaaggtgctggacctgaagaactacatcgacaaacagctgctgcccatcctgaacaagcagtcctgcagcatccccaacatcgagacagtgatcgagttccagcagaagaacaaccggctgctggaaatcacccgcgagttctctgtgaatgccggcgtgaccacacctgtgtccacctacatgctgaccaacagcgagctgctgagcctgatcaacgacatgcccatcaccaacgaccagaaaaagctgatgagcaacaacgtgcagatcgtgcggcagcagagctacagcatcatgagcattatcaaagaagaggtgctggcctactgcgtgcagctgcctctgtatggcgtgatcgataccccttgctggaagctgcacacaagccctctgtgcaccaccaacaccaaagagggcagcaacatctgcctgaccagaaccgacagaggctggtactgcgataatgccggcagcgtctcattcttcccacaagccgagacatgcaaggtgcagagcaaccgggtgttctgcgacaccatgaatagcagaaccctgccttccgaagtgaatctgtgcaacgtggacatcttcaaccctaagtacgactgcaagatcatgaccagcaagaccgacgtgtccagcagtgtgatcacctcactgggcgccatcgtgtcctgttacggcaagaccaagtgcaccgccagcaacaagaaccggggcatcatcaagaccttcagcaacggctgcgactacgtgtccaacaaaggcgtggacaccgtgtctgtgggcaacaccctgtactacgtgaacaaacaagagggccagtctctgtacgtgaagggcgagcccatcatcaacttctacgaccctctggtgttccccagcgacgagttcgatgccagcatcagccaagtgaacgagaagatcaatcagagcctggccttcatcagaaagtccgatgagctgctgcacaacgtgaacgccggcaagtccaccaccaatatcatgatcacgaccatcatcatcgtgattatcgtgatcctgctgtccctgatcgccgtgggcctgctgctttattgataatag

SEQ ID NO: 140 - protein, 510 aa, synthetic construct
MELLILKANAITTILTAVTFCFASGQNITEEFYQSTCSAVSKGYLGALRTGWYTSVITIELSNIKENKCNGTDAKVKLIKQELDKYKNAVTDLQLLMQSCPATGSGSAIASGVAVSKVLHLEGEVNKIKSALLSTNKAVVSLSNGVSVLTFKVLDLKNYIDKQLLPILNKQSCSIPNIETVIEFQQKNNRLLEITREFSVNAGVTTPVSTYMLTNSELLSLINDMPITNDQKKLMSNNVQIVRQQSYSIMSIIKEEVLAYCVQLPLYGVIDTPCWKLHTSPLCTTNTKEGSNICLTRTDRGWYCDNAGSVSFFPQAETCKVQSNRVFCDTMNSRTLPSEVNLCNVDIFNPKYDCKIMTSKTDVSSSVITSLGAIVSCYGKTKCTASNKNRGIIKTFSNGCDYVSNKGVDTVSVGNTLYYVNKQEGQSLYVKGEPIINFYDPLVFPSDEFDASISQVNEKINQSLAFIRKSDELLHNVNAGKSTTNIMITTIIIVIIVILLSLIAVGLLLY

SEQ ID NO: 141 - RNA, 1841 nt, synthetic construct
  source 1..1841: mol_type = other RNA
agcggctcggccattttgtcccagtcagtccggaggctgcggctgcagaagtaccgcctgcggagtaactgcaaaggccaccatggaactgctgatcctgaaggccaacgccatcaccaccatcctgaccgccgtgaccttctgttttgccagcggccagaacatcaccgaggaattctaccagagcacctgtagcgccgtgtccaagggatatctgggcgcccttagaaccggctggtacaccagcgtgatcaccatcgagctgagcaacatcaaagaaaacaagtgcaacggcaccgacgccaaagtgaagctgatcaagcaagagctggacaagtacaagaatgccgtgaccgacctgcagctgctgatgcagtcttgcccagccacaggctctggcagcgccattgcctctggtgtcgccgtgtctaaagtgctgcacctggaaggcgaagtgaacaagatcaagagcgccctgctgagcaccaacaaggccgtggtgtctctgagcaatggcgtgtccgtgctgaccttcaaggtgctggacctgaagaactacatcgacaaacagctgctgcccatcctgaacaagcagtcctgcagcatccccaacatcgagacagtgatcgagttccagcagaagaacaaccggctgctggaaatcacccgcgagttctctgtgaatgccggcgtgaccacacctgtgtccacctacatgctgaccaacagcgagctgctgagcctgatcaacgacatgcccatcaccaacgaccagaaaaagctgatgagcaacaacgtgcagatcgtgcggcagcagagctacagcatcatgagcattatcaaagaagaggtgctggcctactgcgtgcagctgcctctgtatggcgtgatcgataccccttgctggaagctgcacacaagccctctgtgcaccaccaacaccaaagagggcagcaacatctgcctgaccagaaccgacagaggctggtactgcgataatgccggcagcgtctcattcttcccacaagccgagacatgcaaggtgcagagcaaccgggtgttctgcgacaccatgaatagcagaaccctgccttccgaagtgaatctgtgcaacgtggacatcttcaaccctaagtacgactgcaagatcatgaccagcaagaccgacgtgtccagcagtgtgatcacctcactgggcgccatcgtgtcctgttacggcaagaccaagtgcaccgccagcaacaagaaccggggcatcatcaagaccttcagcaacggctgcgactacgtgtccaacaaaggcgtggacaccgtgtctgtgggcaacaccctgtactacgtgaacaaacaagagggccagtctctgtacgtgaagggcgagcccatcatcaacttctacgaccctctggtgttccccagcgacgagttcgatgccagcatcagccaagtgaacgagaagatcaatcagagcctggccttcatcagaaagtccgatgagctgctgcacaacgtgaacgccggcaagtccaccaccaatatcatgatcacgaccatcatcatcgtgattatcgtgatcctgctgtccctgatcgccgtgggcctgctgctttattgataataggctggagcctcggtggccatgcttcttgccccttgggcctccccccagcccctcctccccttcctgcacccgtacccccgtggtctttgaataaagtctgagtgggcggcaaaaaaaaaaaaaaaaaaaaaaaaaaaaaaaaaaaaaaaaaaaaaaaaaaaaaaaaaaaaaaaaaaaaaaaaaaaaaaaaaaaaaaaaaaaaaaaaaaaaaaaaaaaaaa

SEQ ID NO: 142 - DNA, 1871 bp, synthetic construct
  source 1..1871: mol_type = other DNA
agcggctcggccattttgtcccagtcagtccggaggctgcggctgcagaagtaccgcctgcggagtaactgcaaaggccaccatggaactgctgatcctgaaggccaacgccatcaccaccatcctgaccgccgtgaccttctgttttgccagcggccagaacatcaccgaggaattctaccagagcacctgtagcgccgtgtccaagggatatctgggcgcccttagaaccggctggtacaccagcgtgatcaccatcgagctgagcaacatcaaagaaaacaagtgcaacggcaccgacgccaaagtgaagctgatcaagcaagagctggacaagtacaagaatgccgtgaccgacctgcagctgctgatgcagtctacaccagccacaggctctggctctttctgcggctttctgctcggagtgggcagcgccattgcctctggtgtcgccgtgtctaaagtgctgcacctggaaggcgaagtgaacaagatcaagagcgccctgctgagcaccaacaaggccgtggtgtctctgagcaatggcgtgtccgtgctgaccttcaaggtgctggacctgaagaactacatcgacaaacagctgctgcccatcctgaacaagcagtcctgcagcatccccaacatcgagacagtgatcgagttccagcagaagaacaaccggctgctggaaatcacccgcgagttctctgtgaatgccggcgtgaccacacctgtgtccacctacatgctgaccaacagcgagctgctgagcctgatcaacgacatgcccatcaccaacgaccagaaaaagctgatgagcaacaacgtgcagatcgtgcggcagcagagctacagcatcatgagcattatcaaagaagaggtgctggcctacgtggtgcagctgcctctgtatggcgtgatcgataccccttgctggaagctgcacacaagccctctgtgcaccaccaacaccaaagagggcagcaacatctgcctgaccagatgcgacagaggctggtactgcgataatgccggcagcgtctcattcttcccacaagccgagacatgcaaggtgcagagcaaccgggtgttctgcgacaccatgaatagcagaaccctgccttccgaagtgaatctgtgcaacgtggacatcttcaaccctaagtacgactgcaagatcatgaccagcaagaccgacgtgtccagcagtgtgatcacctcactgggcgccatcgtgtcctgttacggcaagaccaagtgcaccgccagcaacaagaaccggggcatcatcaagaccttcagcaacggctgcgactacgtgtccaacaaaggcgtggacaccgtgtctgtgggcaacaccctgtactacgtgaacaaacaagagggccagtctctgtacgtgaagggcgagcccatcatcaacttctacgaccctctggtgttccccagcgacgagttcgatgccagcatcagccaagtgaacgagaagatcaatcagagcctggccttcatcagaaagtccgatgagctgctgcacaacgtgaacgccggcaagtccaccaccaatatcatgatcacgaccatcatcatcgtgattatcgtgatcctgctgtccctgatcgccgtgggcctgctgctttattgataataggctggagcctcggtggccatgcttcttgccccttgggcctccccccagcccctcctccccttcctgcacccgtacccccgtggtctttgaataaagtctgagtgggcggcaaaaaaaaaaaaaaaaaaaaaaaaaaaaaaaaaaaaaaaaaaaaaaaaaaaaaaaaaaaaaaaaaaaaaaaaaaaaaaaaaaaaaaaaaaaaaaaaaaaaaaaaaaaaaa

SEQ ID NO: 143 - DNA, 1569 bp, synthetic construct
  source 1..1569: mol_type = other DNA
atggaactgctgatcctgaaggccaacgccatcaccaccatcctgaccgccgtgaccttctgttttgccagcggccagaacatcaccgaggaattctaccagagcacctgtagcgccgtgtccaagggatatctgggcgcccttagaaccggctggtacaccagcgtgatcaccatcgagctgagcaacatcaaagaaaacaagtgcaacggcaccgacgccaaagtgaagctgatcaagcaagagctggacaagtacaagaatgccgtgaccgacctgcagctgctgatgcagtctacaccagccacaggctctggctctttctgcggctttctgctcggagtgggcagcgccattgcctctggtgtcgccgtgtctaaagtgctgcacctggaaggcgaagtgaacaagatcaagagcgccctgctgagcaccaacaaggccgtggtgtctctgagcaatggcgtgtccgtgctgaccttcaaggtgctggacctgaagaactacatcgacaaacagctgctgcccatcctgaacaagcagtcctgcagcatccccaacatcgagacagtgatcgagttccagcagaagaacaaccggctgctggaaatcacccgcgagttctctgtgaatgccggcgtgaccacacctgtgtccacctacatgctgaccaacagcgagctgctgagcctgatcaacgacatgcccatcaccaacgaccagaaaaagctgatgagcaacaacgtgcagatcgtgcggcagcagagctacagcatcatgagcattatcaaagaagaggtgctggcctacgtggtgcagctgcctctgtatggcgtgatcgataccccttgctggaagctgcacacaagccctctgtgcaccaccaacaccaaagagggcagcaacatctgcctgaccagatgcgacagaggctggtactgcgataatgccggcagcgtctcattcttcccacaagccgagacatgcaaggtgcagagcaaccgggtgttctgcgacaccatgaatagcagaaccctgccttccgaagtgaatctgtgcaacgtggacatcttcaaccctaagtacgactgcaagatcatgaccagcaagaccgacgtgtccagcagtgtgatcacctcactgggcgccatcgtgtcctgttacggcaagaccaagtgcaccgccagcaacaagaaccggggcatcatcaagaccttcagcaacggctgcgactacgtgtccaacaaaggcgtggacaccgtgtctgtgggcaacaccctgtactacgtgaacaaacaagagggccagtctctgtacgtgaagggcgagcccatcatcaacttctacgaccctctggtgttccccagcgacgagttcgatgccagcatcagccaagtgaacgagaagatcaatcagagcctggccttcatcagaaagtccgatgagctgctgcacaacgtgaacgccggcaagtccaccaccaatatcatgatcacgaccatcatcatcgtgattatcgtgatcctgctgtccctgatcgccgtgggcctgctgctttattgataatag

SEQ ID NO: 144 - protein, 520 aa, synthetic construct
MELLILKANAITTILTAVTFCFASGQNITEEFYQSTCSAVSKGYLGALRTGWYTSVITIELSNIKENKCNGTDAKVKLIKQELDKYKNAVTDLQLLMQSTPATGSGSFCGFLLGVGSAIASGVAVSKVLHLEGEVNKIKSALLSTNKAVVSLSNGVSVLTFKVLDLKNYIDKQLLPILNKQSCSIPNIETVIEFQQKNNRLLEITREFSVNAGVTTPVSTYMLTNSELLSLINDMPITNDQKKLMSNNVQIVRQQSYSIMSIIKEEVLAYVVQLPLYGVIDTPCWKLHTSPLCTTNTKEGSNICLTRCDRGWYCDNAGSVSFFPQAETCKVQSNRVFCDTMNSRTLPSEVNLCNVDIFNPKYDCKIMTSKTDVSSSVITSLGAIVSCYGKTKCTASNKNRGIIKTFSNGCDYVSNKGVDTVSVGNTLYYVNKQEGQSLYVKGEPIINFYDPLVFPSDEFDASISQVNEKINQSLAFIRKSDELLHNVNAGKSTTNIMITTIIIVIIVILLSLIAVGLLLY

SEQ ID NO: 145 - RNA, 1871 nt, synthetic construct
  source 1..1871: mol_type = other RNA
agcggctcggccattttgtcccagtcagtccggaggctgcggctgcagaagtaccgcctgcggagtaactgcaaaggccaccatggaactgctgatcctgaaggccaacgccatcaccaccatcctgaccgccgtgaccttctgttttgccagcggccagaacatcaccgaggaattctaccagagcacctgtagcgccgtgtccaagggatatctgggcgcccttagaaccggctggtacaccagcgtgatcaccatcgagctgagcaacatcaaagaaaacaagtgcaacggcaccgacgccaaagtgaagctgatcaagcaagagctggacaagtacaagaatgccgtgaccgacctgcagctgctgatgcagtctacaccagccacaggctctggctctttctgcggctttctgctcggagtgggcagcgccattgcctctggtgtcgccgtgtctaaagtgctgcacctggaaggcgaagtgaacaagatcaagagcgccctgctgagcaccaacaaggccgtggtgtctctgagcaatggcgtgtccgtgctgaccttcaaggtgctggacctgaagaactacatcgacaaacagctgctgcccatcctgaacaagcagtcctgcagcatccccaacatcgagacagtgatcgagttccagcagaagaacaaccggctgctggaaatcacccgcgagttctctgtgaatgccggcgtgaccacacctgtgtccacctacatgctgaccaacagcgagctgctgagcctgatcaacgacatgcccatcaccaacgaccagaaaaagctgatgagcaacaacgtgcagatcgtgcggcagcagagctacagcatcatgagcattatcaaagaagaggtgctggcctacgtggtgcagctgcctctgtatggcgtgatcgataccccttgctggaagctgcacacaagccctctgtgcaccaccaacaccaaagagggcagcaacatctgcctgaccagatgcgacagaggctggtactgcgataatgccggcagcgtctcattcttcccacaagccgagacatgcaaggtgcagagcaaccgggtgttctgcgacaccatgaatagcagaaccctgccttccgaagtgaatctgtgcaacgtggacatcttcaaccctaagtacgactgcaagatcatgaccagcaagaccgacgtgtccagcagtgtgatcacctcactgggcgccatcgtgtcctgttacggcaagaccaagtgcaccgccagcaacaagaaccggggcatcatcaagaccttcagcaacggctgcgactacgtgtccaacaaaggcgtggacaccgtgtctgtgggcaacaccctgtactacgtgaacaaacaagagggccagtctctgtacgtgaagggcgagcccatcatcaacttctacgaccctctggtgttccccagcgacgagttcgatgccagcatcagccaagtgaacgagaagatcaatcagagcctggccttcatcagaaagtccgatgagctgctgcacaacgtgaacgccggcaagtccaccaccaatatcatgatcacgaccatcatcatcgtgattatcgtgatcctgctgtccctgatcgccgtgggcctgctgctttattgataataggctggagcctcggtggccatgcttcttgccccttgggcctccccccagcccctcctccccttcctgcacccgtacccccgtggtctttgaataaagtctgagtgggcggcaaaaaaaaaaaaaaaaaaaaaaaaaaaaaaaaaaaaaaaaaaaaaaaaaaaaaaaaaaaaaaaaaaaaaaaaaaaaaaaaaaaaaaaaaaaaaaaaaaaaaaaaaaaaaa

SEQ ID NO: 146 - DNA, 1871 bp, synthetic construct
  source 1..1871: mol_type = other DNA
agcggctcggccattttgtcccagtcagtccggaggctgcggctgcagaagtaccgcctgcggagtaactgcaaaggccaccatggaactgctgatcctgaaggccaacgccatcaccaccatcctgaccgccgtgaccttctgttttgccagcggccagaacatcaccgaggaattctaccagagcacctgtagcgccgtgtccaagggatatctgggcgcccttagaaccggctggtacaccagcgtgatcaccatcgagctgagcaacatcaaagaaaacaagtgcaacggcaccgacgccaaagtgaagctgatcaagcaagagctggacaagtacaagaatgccgtgaccgacctgcagctgctgatgcagtctacaccagccacaggctctggctctttcctgtgctttctgctcggagtgggcagcgccattgcctctggtgtcgccgtgtctaaagtgctgcacctggaaggcgaagtgaacaagatcaagagcgccctgctgagcaccaacaaggccgtggtgtctctgagcaatggcgtgtccgtgctgaccttcaaggtgctggacctgaagaactacatcgacaaacagctgctgcccatcctgaacaagcagtcctgcagcatccccaacatcgagacagtgatcgagttccagcagaagaacaaccggctgctggaaatcacccgcgagttctctgtgaatgccggcgtgaccacacctgtgtccacctacatgctgaccaacagcgagctgctgagcctgatcaacgacatgcccatcaccaacgaccagaaaaagctgatgagcaacaacgtgcagatcgtgcggcagcagagctacagcatcatgagcattatcaaagaagaggtgctggcctacgtggtgcagctgcctctgtatggcgtgatcgataccccttgctggaagctgcacacaagccctctgtgcaccaccaacaccaaagagggcagcaacatctgcctgaccagaaccgacagaggctggtactgcgataatgccggcagcgtctcattcttcccatgcgccgagacatgcaaggtgcagagcaaccgggtgttctgcgacaccatgaatagcagaaccctgccttccgaagtgaatctgtgcaacgtggacatcttcaaccctaagtacgactgcaagatcatgaccagcaagaccgacgtgtccagcagtgtgatcacctcactgggcgccatcgtgtcctgttacggcaagaccaagtgcaccgccagcaacaagaaccggggcatcatcaagaccttcagcaacggctgcgactacgtgtccaacaaaggcgtggacaccgtgtctgtgggcaacaccctgtactacgtgaacaaacaagagggccagtctctgtacgtgaagggcgagcccatcatcaacttctacgaccctctggtgttccccagcgacgagttcgatgccagcatcagccaagtgaacgagaagatcaatcagagcctggccttcatcagaaagtccgatgagctgctgcacaacgtgaacgccggcaagtccaccaccaatatcatgatcacgaccatcatcatcgtgattatcgtgatcctgctgtccctgatcgccgtgggcctgctgctttattgataataggctggagcctcggtggccatgcttcttgccccttgggcctccccccagcccctcctccccttcctgcacccgtacccccgtggtctttgaataaagtctgagtgggcggcaaaaaaaaaaaaaaaaaaaaaaaaaaaaaaaaaaaaaaaaaaaaaaaaaaaaaaaaaaaaaaaaaaaaaaaaaaaaaaaaaaaaaaaaaaaaaaaaaaaaaaaaaaaaaa

SEQ ID NO: 147 - DNA, 1569 bp, synthetic construct
  source 1..1569: mol_type = other DNA
atggaactgctgatcctgaaggccaacgccatcaccaccatcctgaccgccgtgaccttctgttttgccagcggccagaacatcaccgaggaattctaccagagcacctgtagcgccgtgtccaagggatatctgggcgcccttagaaccggctggtacaccagcgtgatcaccatcgagctgagcaacatcaaagaaaacaagtgcaacggcaccgacgccaaagtgaagctgatcaagcaagagctggacaagtacaagaatgccgtgaccgacctgcagctgctgatgcagtctacaccagccacaggctctggctctttcctgtgctttctgctcggagtgggcagcgccattgcctctggtgtcgccgtgtctaaagtgctgcacctggaaggcgaagtgaacaagatcaagagcgccctgctgagcaccaacaaggccgtggtgtctctgagcaatggcgtgtccgtgctgaccttcaaggtgctggacctgaagaactacatcgacaaacagctgctgcccatcctgaacaagcagtcctgcagcatccccaacatcgagacagtgatcgagttccagcagaagaacaaccggctgctggaaatcacccgcgagttctctgtgaatgccggcgtgaccacacctgtgtccacctacatgctgaccaacagcgagctgctgagcctgatcaacgacatgcccatcaccaacgaccagaaaaagctgatgagcaacaacgtgcagatcgtgcggcagcagagctacagcatcatgagcattatcaaagaagaggtgctggcctacgtggtgcagctgcctctgtatggcgtgatcgataccccttgctggaagctgcacacaagccctctgtgcaccaccaacaccaaagagggcagcaacatctgcctgaccagaaccgacagaggctggtactgcgataatgccggcagcgtctcattcttcccatgcgccgagacatgcaaggtgcagagcaaccgggtgttctgcgacaccatgaatagcagaaccctgccttccgaagtgaatctgtgcaacgtggacatcttcaaccctaagtacgactgcaagatcatgaccagcaagaccgacgtgtccagcagtgtgatcacctcactgggcgccatcgtgtcctgttacggcaagaccaagtgcaccgccagcaacaagaaccggggcatcatcaagaccttcagcaacggctgcgactacgtgtccaacaaaggcgtggacaccgtgtctgtgggcaacaccctgtactacgtgaacaaacaagagggccagtctctgtacgtgaagggcgagcccatcatcaacttctacgaccctctggtgttccccagcgacgagttcgatgccagcatcagccaagtgaacgagaagatcaatcagagcctggccttcatcagaaagtccgatgagctgctgcacaacgtgaacgccggcaagtccaccaccaatatcatgatcacgaccatcatcatcgtgattatcgtgatcctgctgtccctgatcgccgtgggcctgctgctttattgataatag

SEQ ID NO: 148 - protein, 520 aa, synthetic construct
MELLILKANAITTILTAVTFCFASGQNITEEFYQSTCSAVSKGYLGALRTGWYTSVITIELSNIKENKCNGTDAKVKLIKQELDKYKNAVTDLQLLMQSTPATGSGSFLCFLLGVGSAIASGVAVSKVLHLEGEVNKIKSALLSTNKAVVSLSNGVSVLTFKVLDLKNYIDKQLLPILNKQSCSIPNIETVIEFQQKNNRLLEITREFSVNAGVTTPVSTYMLTNSELLSLINDMPITNDQKKLMSNNVQIVRQQSYSIMSIIKEEVLAYVVQLPLYGVIDTPCWKLHTSPLCTTNTKEGSNICLTRTDRGWYCDNAGSVSFFPCAETCKVQSNRVFCDTMNSRTLPSEVNLCNVDIFNPKYDCKIMTSKTDVSSSVITSLGAIVSCYGKTKCTASNKNRGIIKTFSNGCDYVSNKGVDTVSVGNTLYYVNKQEGQSLYVKGEPIINFYDPLVFPSDEFDASISQVNEKINQSLAFIRKSDELLHNVNAGKSTTNIMITTIIIVIIVILLSLIAVGLLLY

SEQ ID NO: 149 - RNA, 1871 nt, synthetic construct
  source 1..1871: mol_type = other RNA
agcggctcggccattttgtcccagtcagtccggaggctgcggctgcagaagtaccgcctgcggagtaactgcaaaggccaccatggaactgctgatcctgaaggccaacgccatcaccaccatcctgaccgccgtgaccttctgttttgccagcggccagaacatcaccgaggaattctaccagagcacctgtagcgccgtgtccaagggatatctgggcgcccttagaaccggctggtacaccagcgtgatcaccatcgagctgagcaacatcaaagaaaacaagtgcaacggcaccgacgccaaagtgaagctgatcaagcaagagctggacaagtacaagaatgccgtgaccgacctgcagctgctgatgcagtctacaccagccacaggctctggctctttcctgtgctttctgctcggagtgggcagcgccattgcctctggtgtcgccgtgtctaaagtgctgcacctggaaggcgaagtgaacaagatcaagagcgccctgctgagcaccaacaaggccgtggtgtctctgagcaatggcgtgtccgtgctgaccttcaaggtgctggacctgaagaactacatcgacaaacagctgctgcccatcctgaacaagcagtcctgcagcatccccaacatcgagacagtgatcgagttccagcagaagaacaaccggctgctggaaatcacccgcgagttctctgtgaatgccggcgtgaccacacctgtgtccacctacatgctgaccaacagcgagctgctgagcctgatcaacgacatgcccatcaccaacgaccagaaaaagctgatgagcaacaacgtgcagatcgtgcggcagcagagctacagcatcatgagcattatcaaagaagaggtgctggcctacgtggtgcagctgcctctgtatggcgtgatcgataccccttgctggaagctgcacacaagccctctgtgcaccaccaacaccaaagagggcagcaacatctgcctgaccagaaccgacagaggctggtactgcgataatgccggcagcgtctcattcttcccatgcgccgagacatgcaaggtgcagagcaaccgggtgttctgcgacaccatgaatagcagaaccctgccttccgaagtgaatctgtgcaacgtggacatcttcaaccctaagtacgactgcaagatcatgaccagcaagaccgacgtgtccagcagtgtgatcacctcactgggcgccatcgtgtcctgttacggcaagaccaagtgcaccgccagcaacaagaaccggggcatcatcaagaccttcagcaacggctgcgactacgtgtccaacaaaggcgtggacaccgtgtctgtgggcaacaccctgtactacgtgaacaaacaagagggccagtctctgtacgtgaagggcgagcccatcatcaacttctacgaccctctggtgttccccagcgacgagttcgatgccagcatcagccaagtgaacgagaagatcaatcagagcctggccttcatcagaaagtccgatgagctgctgcacaacgtgaacgccggcaagtccaccaccaatatcatgatcacgaccatcatcatcgtgattatcgtgatcctgctgtccctgatcgccgtgggcctgctgctttattgataataggctggagcctcggtggccatgcttcttgccccttgggcctccccccagcccctcctccccttcctgcacccgtacccccgtggtctttgaataaagtctgagtgggcggcaaaaaaaaaaaaaaaaaaaaaaaaaaaaaaaaaaaaaaaaaaaaaaaaaaaaaaaaaaaaaaaaaaaaaaaaaaaaaaaaaaaaaaaaaaaaaaaaaaaaaaaaaaaaaa

SEQ ID NO: 150 - DNA, 1871 bp, synthetic construct
  source 1..1871: mol_type = other DNA
agcggctcggccattttgtcccagtcagtccggaggctgcggctgcagaagtaccgcctgcggagtaactgcaaaggccaccatggaactgctgatcctgaaggccaacgccatcaccaccatcctgaccgccgtgaccttctgttttgccagcggccagaacatcaccgaggaattctaccagagcacctgtagcgccgtgtccaagggatatctgggcgcccttagaaccggctggtacaccagcgtgatcaccatcgagctgagcaacatcaaagaaaacaagtgcaacggcaccgacgccaaagtgaagctgatcaagcaagagctggacaagtacaagaatgccgtgaccgacctgcagctgctgatgcagtctacaccagccacaggctctggctctttcctgggctttctgtgcggagtgggcagcgccattgcctctggtgtcgccgtgtctaaagtgctgcacctggaaggcgaagtgaacaagatcaagagcgccctgctgagcaccaacaaggccgtggtgtctctgagcaatggcgtgtccgtgctgaccttcaaggtgctggacctgaagaactacatcgacaaacagctgctgcccatcctgaacaagcagtcctgcagcatccccaacatcgagacagtgatcgagttccagcagaagaacaaccggctgctggaaatcacccgcgagttctctgtgaatgccggcgtgaccacacctgtgtccacctacatgctgaccaacagcgagctgctgagcctgatcaacgacatgcccatcaccaacgaccagaaaaagctgatgagcaacaacgtgcagatcgtgcggcagcagagctacagcatcatgagcattatcaaagaagaggtgctggcctacgtggtgcagctgcctctgtatggcgtgatcgataccccttgctggaagctgcacacaagccctctgtgcaccaccaacaccaaagagggcagcaacatctgcctgaccagaaccgacagaggctggtactgcgataatgccggcagcgtctcattcttcccacaagccgagacatgcaaggtgcagagcaaccgggtgttctgcgacaccatgtgcagcagaaccctgccttccgaagtgaatctgtgcaacgtggacatcttcaaccctaagtacgactgcaagatcatgaccagcaagaccgacgtgtccagcagtgtgatcacctcactgggcgccatcgtgtcctgttacggcaagaccaagtgcaccgccagcaacaagaaccggggcatcatcaagaccttcagcaacggctgcgactacgtgtccaacaaaggcgtggacaccgtgtctgtgggcaacaccctgtactacgtgaacaaacaagagggccagtctctgtacgtgaagggcgagcccatcatcaacttctacgaccctctggtgttccccagcgacgagttcgatgccagcatcagccaagtgaacgagaagatcaatcagagcctggccttcatcagaaagtccgatgagctgctgcacaacgtgaacgccggcaagtccaccaccaatatcatgatcacgaccatcatcatcgtgattatcgtgatcctgctgtccctgatcgccgtgggcctgctgctttattgataataggctggagcctcggtggccatgcttcttgccccttgggcctccccccagcccctcctccccttcctgcacccgtacccccgtggtctttgaataaagtctgagtgggcggcaaaaaaaaaaaaaaaaaaaaaaaaaaaaaaaaaaaaaaaaaaaaaaaaaaaaaaaaaaaaaaaaaaaaaaaaaaaaaaaaaaaaaaaaaaaaaaaaaaaaaaaaaaaaaa

SEQ ID NO: 151 - DNA, 1569 bp, synthetic construct
  source 1..1569: mol_type = other DNA
atggaactgctgatcctgaaggccaacgccatcaccaccatcctgaccgccgtgaccttctgttttgccagcggccagaacatcaccgaggaattctaccagagcacctgtagcgccgtgtccaagggatatctgggcgcccttagaaccggctggtacaccagcgtgatcaccatcgagctgagcaacatcaaagaaaacaagtgcaacggcaccgacgccaaagtgaagctgatcaagcaagagctggacaagtacaagaatgccgtgaccgacctgcagctgctgatgcagtctacaccagccacaggctctggctctttcctgggctttctgtgcggagtgggcagcgccattgcctctggtgtcgccgtgtctaaagtgctgcacctggaaggcgaagtgaacaagatcaagagcgccctgctgagcaccaacaaggccgtggtgtctctgagcaatggcgtgtccgtgctgaccttcaaggtgctggacctgaagaactacatcgacaaacagctgctgcccatcctgaacaagcagtcctgcagcatccccaacatcgagacagtgatcgagttccagcagaagaacaaccggctgctggaaatcacccgcgagttctctgtgaatgccggcgtgaccacacctgtgtccacctacatgctgaccaacagcgagctgctgagcctgatcaacgacatgcccatcaccaacgaccagaaaaagctgatgagcaacaacgtgcagatcgtgcggcagcagagctacagcatcatgagcattatcaaagaagaggtgctggcctacgtggtgcagctgcctctgtatggcgtgatcgataccccttgctggaagctgcacacaagccctctgtgcaccaccaacaccaaagagggcagcaacatctgcctgaccagaaccgacagaggctggtactgcgataatgccggcagcgtctcattcttcccacaagccgagacatgcaaggtgcagagcaaccgggtgttctgcgacaccatgtgcagcagaaccctgccttccgaagtgaatctgtgcaacgtggacatcttcaaccctaagtacgactgcaagatcatgaccagcaagaccgacgtgtccagcagtgtgatcacctcactgggcgccatcgtgtcctgttacggcaagaccaagtgcaccgccagcaacaagaaccggggcatcatcaagaccttcagcaacggctgcgactacgtgtccaacaaaggcgtggacaccgtgtctgtgggcaacaccctgtactacgtgaacaaacaagagggccagtctctgtacgtgaagggcgagcccatcatcaacttctacgaccctctggtgttccccagcgacgagttcgatgccagcatcagccaagtgaacgagaagatcaatcagagcctggccttcatcagaaagtccgatgagctgctgcacaacgtgaacgccggcaagtccaccaccaatatcatgatcacgaccatcatcatcgtgattatcgtgatcctgctgtccctgatcgccgtgggcctgctgctttattgataatag

SEQ ID NO: 152 - protein, 520 aa, synthetic construct
MELLILKANAITTILTAVTFCFASGQNITEEFYQSTCSAVSKGYLGALRTGWYTSVITIELSNIKENKCNGTDAKVKLIKQELDKYKNAVTDLQLLMQSTPATGSGSFLGFLCGVGSAIASGVAVSKVLHLEGEVNKIKSALLSTNKAVVSLSNGVSVLTFKVLDLKNYIDKQLLPILNKQSCSIPNIETVIEFQQKNNRLLEITREFSVNAGVTTPVSTYMLTNSELLSLINDMPITNDQKKLMSNNVQIVRQQSYSIMSIIKEEVLAYVVQLPLYGVIDTPCWKLHTSPLCTTNTKEGSNICLTRTDRGWYCDNAGSVSFFPQAETCKVQSNRVFCDTMCSRTLPSEVNLCNVDIFNPKYDCKIMTSKTDVSSSVITSLGAIVSCYGKTKCTASNKNRGIIKTFSNGCDYVSNKGVDTVSVGNTLYYVNKQEGQSLYVKGEPIINFYDPLVFPSDEFDASISQVNEKINQSLAFIRKSDELLHNVNAGKSTTNIMITTIIIVIIVILLSLIAVGLLLY

SEQ ID NO: 153 - RNA, 1871 nt, synthetic construct
  source 1..1871: mol_type = other RNA
agcggctcggccattttgtcccagtcagtccggaggctgcggctgcagaagtaccgcctgcggagtaactgcaaaggccaccatggaactgctgatcctgaaggccaacgccatcaccaccatcctgaccgccgtgaccttctgttttgccagcggccagaacatcaccgaggaattctaccagagcacctgtagcgccgtgtccaagggatatctgggcgcccttagaaccggctggtacaccagcgtgatcaccatcgagctgagcaacatcaaagaaaacaagtgcaacggcaccgacgccaaagtgaagctgatcaagcaagagctggacaagtacaagaatgccgtgaccgacctgcagctgctgatgcagtctacaccagccacaggctctggctctttcctgggctttctgtgcggagtgggcagcgccattgcctctggtgtcgccgtgtctaaagtgctgcacctggaaggcgaagtgaacaagatcaagagcgccctgctgagcaccaacaaggccgtggtgtctctgagcaatggcgtgtccgtgctgaccttcaaggtgctggacctgaagaactacatcgacaaacagctgctgcccatcctgaacaagcagtcctgcagcatccccaacatcgagacagtgatcgagttccagcagaagaacaaccggctgctggaaatcacccgcgagttctctgtgaatgccggcgtgaccacacctgtgtccacctacatgctgaccaacagcgagctgctgagcctgatcaacgacatgcccatcaccaacgaccagaaaaagctgatgagcaacaacgtgcagatcgtgcggcagcagagctacagcatcatgagcattatcaaagaagaggtgctggcctacgtggtgcagctgcctctgtatggcgtgatcgataccccttgctggaagctgcacacaagccctctgtgcaccaccaacaccaaagagggcagcaacatctgcctgaccagaaccgacagaggctggtactgcgataatgccggcagcgtctcattcttcccacaagccgagacatgcaaggtgcagagcaaccgggtgttctgcgacaccatgtgcagcagaaccctgccttccgaagtgaatctgtgcaacgtggacatcttcaaccctaagtacgactgcaagatcatgaccagcaagaccgacgtgtccagcagtgtgatcacctcactgggcgccatcgtgtcctgttacggcaagaccaagtgcaccgccagcaacaagaaccggggcatcatcaagaccttcagcaacggctgcgactacgtgtccaacaaaggcgtggacaccgtgtctgtgggcaacaccctgtactacgtgaacaaacaagagggccagtctctgtacgtgaagggcgagcccatcatcaacttctacgaccctctggtgttccccagcgacgagttcgatgccagcatcagccaagtgaacgagaagatcaatcagagcctggccttcatcagaaagtccgatgagctgctgcacaacgtgaacgccggcaagtccaccaccaatatcatgatcacgaccatcatcatcgtgattatcgtgatcctgctgtccctgatcgccgtgggcctgctgctttattgataataggctggagcctcggtggccatgcttcttgccccttgggcctccccccagcccctcctccccttcctgcacccgtacccccgtggtctttgaataaagtctgagtgggcggcaaaaaaaaaaaaaaaaaaaaaaaaaaaaaaaaaaaaaaaaaaaaaaaaaaaaaaaaaaaaaaaaaaaaaaaaaaaaaaaaaaaaaaaaaaaaaaaaaaaaaaaaaaaaaa

SEQ ID NO: 154 - DNA, 1871 bp, synthetic construct
  source 1..1871: mol_type = other DNA
agcggctcggccattttgtcccagtcagtccggaggctgcggctgcagaagtaccgcctgcggagtaactgcaaaggccaccatggaactgctgatcctgaaggccaacgccatcaccaccatcctgaccgccgtgaccttctgttttgccagcggccagaacatcaccgaggaattctaccagagcacctgtagcgccgtgtccaagggatatctgggcgcccttagaaccggctggtacaccagcgtgatcaccatcgagctgagcaacatcaaagaaaacaagtgcaacggcaccgacgccaaagtgaagctgatcaagcaagagctggacaagtacaagaatgccgtgaccgacctgcagctgctgatgcagtctacaccagccacaggctctggctctttcctgggctttctgctcggagtgtgcagcgccattgcctctggtgtcgccgtgtctaaagtgctgcacctggaaggcgaagtgaacaagatcaagagcgccctgctgagcaccaacaaggccgtggtgtctctgagcaatggcgtgtccgtgctgaccttcaaggtgctggacctgaagaactacatcgacaaacagctgctgcccatcctgaacaagcagtcctgcagcatccccaacatcgagacagtgatcgagttccagcagaagaacaaccggctgctggaaatcacccgcgagttctctgtgaatgccggcgtgaccacacctgtgtccacctacatgctgaccaacagcgagctgctgagcctgatcaacgacatgcccatcaccaacgaccagaaaaagctgatgagcaacaacgtgcagatcgtgcggcagcagagctacagcatcatgagcattatcaaagaagaggtgctggcctacgtggtgcagctgcctctgtatggcgtgatcgataccccttgctggaagctgcacacaagccctctgtgcaccaccaacaccaaagagggcagcaacatctgcctgaccagaaccgacagaggctggtactgcgataatgccggcagcgtctcattcttcccacaagccgagacatgcaaggtgcagagcaaccgggtgttctgcgacacctgcaatagcagaaccctgccttccgaagtgaatctgtgcaacgtggacatcttcaaccctaagtacgactgcaagatcatgaccagcaagaccgacgtgtccagcagtgtgatcacctcactgggcgccatcgtgtcctgttacggcaagaccaagtgcaccgccagcaacaagaaccggggcatcatcaagaccttcagcaacggctgcgactacgtgtccaacaaaggcgtggacaccgtgtctgtgggcaacaccctgtactacgtgaacaaacaagagggccagtctctgtacgtgaagggcgagcccatcatcaacttctacgaccctctggtgttccccagcgacgagttcgatgccagcatcagccaagtgaacgagaagatcaatcagagcctggccttcatcagaaagtccgatgagctgctgcacaacgtgaacgccggcaagtccaccaccaatatcatgatcacgaccatcatcatcgtgattatcgtgatcctgctgtccctgatcgccgtgggcctgctgctttattgataataggctggagcctcggtggccatgcttcttgccccttgggcctccccccagcccctcctccccttcctgcacccgtacccccgtggtctttgaataaagtctgagtgggcggcaaaaaaaaaaaaaaaaaaaaaaaaaaaaaaaaaaaaaaaaaaaaaaaaaaaaaaaaaaaaaaaaaaaaaaaaaaaaaaaaaaaaaaaaaaaaaaaaaaaaaaaaaaaaaa

SEQ ID NO: 155 - DNA, 1569 bp, synthetic construct
  source 1..1569: mol_type = other DNA
atggaactgctgatcctgaaggccaacgccatcaccaccatcctgaccgccgtgaccttctgttttgccagcggccagaacatcaccgaggaattctaccagagcacctgtagcgccgtgtccaagggatatctgggcgcccttagaaccggctggtacaccagcgtgatcaccatcgagctgagcaacatcaaagaaaacaagtgcaacggcaccgacgccaaagtgaagctgatcaagcaagagctggacaagtacaagaatgccgtgaccgacctgcagctgctgatgcagtctacaccagccacaggctctggctctttcctgggctttctgctcggagtgtgcagcgccattgcctctggtgtcgccgtgtctaaagtgctgcacctggaaggcgaagtgaacaagatcaagagcgccctgctgagcaccaacaaggccgtggtgtctctgagcaatggcgtgtccgtgctgaccttcaaggtgctggacctgaagaactacatcgacaaacagctgctgcccatcctgaacaagcagtcctgcagcatccccaacatcgagacagtgatcgagttccagcagaagaacaaccggctgctggaaatcacccgcgagttctctgtgaatgccggcgtgaccacacctgtgtccacctacatgctgaccaacagcgagctgctgagcctgatcaacgacatgcccatcaccaacgaccagaaaaagctgatgagcaacaacgtgcagatcgtgcggcagcagagctacagcatcatgagcattatcaaagaagaggtgctggcctacgtggtgcagctgcctctgtatggcgtgatcgataccccttgctggaagctgcacacaagccctctgtgcaccaccaacaccaaagagggcagcaacatctgcctgaccagaaccgacagaggctggtactgcgataatgccggcagcgtctcattcttcccacaagccgagacatgcaaggtgcagagcaaccgggtgttctgcgacacctgcaatagcagaaccctgccttccgaagtgaatctgtgcaacgtggacatcttcaaccctaagtacgactgcaagatcatgaccagcaagaccgacgtgtccagcagtgtgatcacctcactgggcgccatcgtgtcctgttacggcaagaccaagtgcaccgccagcaacaagaaccggggcatcatcaagaccttcagcaacggctgcgactacgtgtccaacaaaggcgtggacaccgtgtctgtgggcaacaccctgtactacgtgaacaaacaagagggccagtctctgtacgtgaagggcgagcccatcatcaacttctacgaccctctggtgttccccagcgacgagttcgatgccagcatcagccaagtgaacgagaagatcaatcagagcctggccttcatcagaaagtccgatgagctgctgcacaacgtgaacgccggcaagtccaccaccaatatcatgatcacgaccatcatcatcgtgattatcgtgatcctgctgtccctgatcgccgtgggcctgctgctttattgataatag

SEQ ID NO: 156 - protein, 520 aa, synthetic construct
MELLILKANAITTILTAVTFCFASGQNITEEFYQSTCSAVSKGYLGALRTGWYTSVITIELSNIKENKCNGTDAKVKLIKQELDKYKNAVTDLQLLMQSTPATGSGSFLGFLLGVCSAIASGVAVSKVLHLEGEVNKIKSALLSTNKAVVSLSNGVSVLTFKVLDLKNYIDKQLLPILNKQSCSIPNIETVIEFQQKNNRLLEITREFSVNAGVTTPVSTYMLTNSELLSLINDMPITNDQKKLMSNNVQIVRQQSYSIMSIIKEEVLAYVVQLPLYGVIDTPCWKLHTSPLCTTNTKEGSNICLTRTDRGWYCDNAGSVSFFPQAETCKVQSNRVFCDTCNSRTLPSEVNLCNVDIFNPKYDCKIMTSKTDVSSSVITSLGAIVSCYGKTKCTASNKNRGIIKTFSNGCDYVSNKGVDTVSVGNTLYYVNKQEGQSLYVKGEPIINFYDPLVFPSDEFDASISQVNEKINQSLAFIRKSDELLHNVNAGKSTTNIMITTIIIVIIVILLSLIAVGLLLY

SEQ ID NO: 157 - RNA, 1871 nt, synthetic construct
  source 1..1871: mol_type = other RNA
agcggctcggccattttgtcccagtcagtccggaggctgcggctgcagaagtaccgcctgcggagtaactgcaaaggccaccatggaactgctgatcctgaaggccaacgccatcaccaccatcctgaccgccgtgaccttctgttttgccagcggccagaacatcaccgaggaattctaccagagcacctgtagcgccgtgtccaagggatatctgggcgcccttagaaccggctggtacaccagcgtgatcaccatcgagctgagcaacatcaaagaaaacaagtgcaacggcaccgacgccaaagtgaagctgatcaagcaagagctggacaagtacaagaatgccgtgaccgacctgcagctgctgatgcagtctacaccagccacaggctctggctctttcctgggctttctgctcggagtgtgcagcgccattgcctctggtgtcgccgtgtctaaagtgctgcacctggaaggcgaagtgaacaagatcaagagcgccctgctgagcaccaacaaggccgtggtgtctctgagcaatggcgtgtccgtgctgaccttcaaggtgctggacctgaagaactacatcgacaaacagctgctgcccatcctgaacaagcagtcctgcagcatccccaacatcgagacagtgatcgagttccagcagaagaacaaccggctgctggaaatcacccgcgagttctctgtgaatgccggcgtgaccacacctgtgtccacctacatgctgaccaacagcgagctgctgagcctgatcaacgacatgcccatcaccaacgaccagaaaaagctgatgagcaacaacgtgcagatcgtgcggcagcagagctacagcatcatgagcattatcaaagaagaggtgctggcctacgtggtgcagctgcctctgtatggcgtgatcgataccccttgctggaagctgcacacaagccctctgtgcaccaccaacaccaaagagggcagcaacatctgcctgaccagaaccgacagaggctggtactgcgataatgccggcagcgtctcattcttcccacaagccgagacatgcaaggtgcagagcaaccgggtgttctgcgacacctgcaatagcagaaccctgccttccgaagtgaatctgtgcaacgtggacatcttcaaccctaagtacgactgcaagatcatgaccagcaagaccgacgtgtccagcagtgtgatcacctcactgggcgccatcgtgtcctgttacggcaagaccaagtgcaccgccagcaacaagaaccggggcatcatcaagaccttcagcaacggctgcgactacgtgtccaacaaaggcgtggacaccgtgtctgtgggcaacaccctgtactacgtgaacaaacaagagggccagtctctgtacgtgaagggcgagcccatcatcaacttctacgaccctctggtgttccccagcgacgagttcgatgccagcatcagccaagtgaacgagaagatcaatcagagcctggccttcatcagaaagtccgatgagctgctgcacaacgtgaacgccggcaagtccaccaccaatatcatgatcacgaccatcatcatcgtgattatcgtgatcctgctgtccctgatcgccgtgggcctgctgctttattgataataggctggagcctcggtggccatgcttcttgccccttgggcctccccccagcccctcctccccttcctgcacccgtacccccgtggtctttgaataaagtctgagtgggcggcaaaaaaaaaaaaaaaaaaaaaaaaaaaaaaaaaaaaaaaaaaaaaaaaaaaaaaaaaaaaaaaaaaaaaaaaaaaaaaaaaaaaaaaaaaaaaaaaaaaaaaaaaaaaaa

SEQ ID NO: 158 - DNA, 1871 bp, synthetic construct
  source 1..1871: mol_type = other DNA
agcggctcggccattttgtcccagtcagtccggaggctgcggctgcagaagtaccgcctgcggagtaactgcaaaggccaccatggaactgctgatcctgaaggccaacgccatcaccaccatcctgaccgccgtgaccttctgttttgccagcggccagaacatcaccgaggaattctaccagagcacctgtagcgccgtgtccaagggatatctgggcgcccttagaaccggctggtacaccagcgtgatcaccatcgagctgagcaacatcaaagaaaacaagtgcaacggcaccgacgccaaagtgaagctgatcaagcaagagctggacaagtacaagaatgccgtgaccgacctgcagctgctgatgcagtctacaccagccacaggctctggctctttcctgggcttttgcctcggagtgggcagcgccattgcctctggtgtcgccgtgtctaaagtgctgcacctggaaggcgaagtgaacaagatcaagagcgccctgctgagcaccaacaaggccgtggtgtctctgagcaatggcgtgtccgtgctgaccttcaaggtgctggacctgaagaactacatcgacaaacagctgctgcccatcctgaacaagcagtcctgcagcatccccaacatcgagacagtgatcgagttccagcagaagaacaaccggctgctggaaatcacccgcgagttctctgtgaatgccggcgtgaccacacctgtgtccacctacatgctgaccaacagcgagctgctgagcctgatcaacgacatgcccatcaccaacgaccagaaaaagctgatgagcaacaacgtgcagatcgtgcggcagcagagctacagcatcatgagcattatcaaagaagaggtgctggcctacgtggtgcagctgcctctgtatggcgtgatcgataccccttgctggaagctgcacacaagccctctgtgcaccaccaacaccaaagagggcagcaacatctgcctgaccagaaccgacagaggctggtactgcgataatgccggcagcgtctcattcttcccacaagccgagacatgcaaggtgcagagcaaccgggtgttctgcgacaccatgtgcagcagaaccctgccttccgaagtgaatctgtgcaacgtggacatcttcaaccctaagtacgactgcaagatcatgaccagcaagaccgacgtgtccagcagtgtgatcacctcactgggcgccatcgtgtcctgttacggcaagaccaagtgcaccgccagcaacaagaaccggggcatcatcaagaccttcagcaacggctgcgactacgtgtccaacaaaggcgtggacaccgtgtctgtgggcaacaccctgtactacgtgaacaaacaagagggccagtctctgtacgtgaagggcgagcccatcatcaacttctacgaccctctggtgttccccagcgacgagttcgatgccagcatcagccaagtgaacgagaagatcaatcagagcctggccttcatcagaaagtccgatgagctgctgcacaacgtgaacgccggcaagtccaccaccaatatcatgatcacgaccatcatcatcgtgattatcgtgatcctgctgtccctgatcgccgtgggcctgctgctttattgataataggctggagcctcggtggccatgcttcttgccccttgggcctccccccagcccctcctccccttcctgcacccgtacccccgtggtctttgaataaagtctgagtgggcggcaaaaaaaaaaaaaaaaaaaaaaaaaaaaaaaaaaaaaaaaaaaaaaaaaaaaaaaaaaaaaaaaaaaaaaaaaaaaaaaaaaaaaaaaaaaaaaaaaaaaaaaaaaaaaa

SEQ ID NO: 159 - DNA, 1569 bp, synthetic construct
  source 1..1569: mol_type = other DNA
atggaactgctgatcctgaaggccaacgccatcaccaccatcctgaccgccgtgaccttctgttttgccagcggccagaacatcaccgaggaattctaccagagcacctgtagcgccgtgtccaagggatatctgggcgcccttagaaccggctggtacaccagcgtgatcaccatcgagctgagcaacatcaaagaaaacaagtgcaacggcaccgacgccaaagtgaagctgatcaagcaagagctggacaagtacaagaatgccgtgaccgacctgcagctgctgatgcagtctacaccagccacaggctctggctctttcctgggcttttgcctcggagtgggcagcgccattgcctctggtgtcgccgtgtctaaagtgctgcacctggaaggcgaagtgaacaagatcaagagcgccctgctgagcaccaacaaggccgtggtgtctctgagcaatggcgtgtccgtgctgaccttcaaggtgctggacctgaagaactacatcgacaaacagctgctgcccatcctgaacaagcagtcctgcagcatccccaacatcgagacagtgatcgagttccagcagaagaacaaccggctgctggaaatcacccgcgagttctctgtgaatgccggcgtgaccacacctgtgtccacctacatgctgaccaacagcgagctgctgagcctgatcaacgacatgcccatcaccaacgaccagaaaaagctgatgagcaacaacgtgcagatcgtgcggcagcagagctacagcatcatgagcattatcaaagaagaggtgctggcctacgtggtgcagctgcctctgtatggcgtgatcgataccccttgctggaagctgcacacaagccctctgtgcaccaccaacaccaaagagggcagcaacatctgcctgaccagaaccgacagaggctggtactgcgataatgccggcagcgtctcattcttcccacaagccgagacatgcaaggtgcagagcaaccgggtgttctgcgacaccatgtgcagcagaaccctgccttccgaagtgaatctgtgcaacgtggacatcttcaaccctaagtacgactgcaagatcatgaccagcaagaccgacgtgtccagcagtgtgatcacctcactgggcgccatcgtgtcctgttacggcaagaccaagtgcaccgccagcaacaagaaccggggcatcatcaagaccttcagcaacggctgcgactacgtgtccaacaaaggcgtggacaccgtgtctgtgggcaacaccctgtactacgtgaacaaacaagagggccagtctctgtacgtgaagggcgagcccatcatcaacttctacgaccctctggtgttccccagcgacgagttcgatgccagcatcagccaagtgaacgagaagatcaatcagagcctggccttcatcagaaagtccgatgagctgctgcacaacgtgaacgccggcaagtccaccaccaatatcatgatcacgaccatcatcatcgtgattatcgtgatcctgctgtccctgatcgccgtgggcctgctgctttattgataatag

SEQ ID NO: 160 - protein, 520 aa, synthetic construct
MELLILKANAITTILTAVTFCFASGQNITEEFYQSTCSAVSKGYLGALRTGWYTSVITIELSNIKENKCNGTDAKVKLIKQELDKYKNAVTDLQLLMQSTPATGSGSFLGFCLGVGSAIASGVAVSKVLHLEGEVNKIKSALLSTNKAVVSLSNGVSVLTFKVLDLKNYIDKQLLPILNKQSCSIPNIETVIEFQQKNNRLLEITREFSVNAGVTTPVSTYMLTNSELLSLINDMPITNDQKKLMSNNVQIVRQQSYSIMSIIKEEVLAYVVQLPLYGVIDTPCWKLHTSPLCTTNTKEGSNICLTRTDRGWYCDNAGSVSFFPQAETCKVQSNRVFCDTMCSRTLPSEVNLCNVDIFNPKYDCKIMTSKTDVSSSVITSLGAIVSCYGKTKCTASNKNRGIIKTFSNGCDYVSNKGVDTVSVGNTLYYVNKQEGQSLYVKGEPIINFYDPLVFPSDEFDASISQVNEKINQSLAFIRKSDELLHNVNAGKSTTNIMITTIIIVIIVILLSLIAVGLLLY

SEQ ID NO: 161 - RNA, 1871 nt, synthetic construct
  source 1..1871: mol_type = other RNA
agcggctcggccattttgtcccagtcagtccggaggctgcggctgcagaagtaccgcctgcggagtaactgcaaaggccaccatggaactgctgatcctgaaggccaacgccatcaccaccatcctgaccgccgtgaccttctgttttgccagcggccagaacatcaccgaggaattctaccagagcacctgtagcgccgtgtccaagggatatctgggcgcccttagaaccggctggtacaccagcgtgatcaccatcgagctgagcaacatcaaagaaaacaagtgcaacggcaccgacgccaaagtgaagctgatcaagcaagagctggacaagtacaagaatgccgtgaccgacctgcagctgctgatgcagtctacaccagccacaggctctggctctttcctgggcttttgcctcggagtgggcagcgccattgcctctggtgtcgccgtgtctaaagtgctgcacctggaaggcgaagtgaacaagatcaagagcgccctgctgagcaccaacaaggccgtggtgtctctgagcaatggcgtgtccgtgctgaccttcaaggtgctggacctgaagaactacatcgacaaacagctgctgcccatcctgaacaagcagtcctgcagcatccccaacatcgagacagtgatcgagttccagcagaagaacaaccggctgctggaaatcacccgcgagttctctgtgaatgccggcgtgaccacacctgtgtccacctacatgctgaccaacagcgagctgctgagcctgatcaacgacatgcccatcaccaacgaccagaaaaagctgatgagcaacaacgtgcagatcgtgcggcagcagagctacagcatcatgagcattatcaaagaagaggtgctggcctacgtggtgcagctgcctctgtatggcgtgatcgataccccttgctggaagctgcacacaagccctctgtgcaccaccaacaccaaagagggcagcaacatctgcctgaccagaaccgacagaggctggtactgcgataatgccggcagcgtctcattcttcccacaagccgagacatgcaaggtgcagagcaaccgggtgttctgcgacaccatgtgcagcagaaccctgccttccgaagtgaatctgtgcaacgtggacatcttcaaccctaagtacgactgcaagatcatgaccagcaagaccgacgtgtccagcagtgtgatcacctcactgggcgccatcgtgtcctgttacggcaagaccaagtgcaccgccagcaacaagaaccggggcatcatcaagaccttcagcaacggctgcgactacgtgtccaacaaaggcgtggacaccgtgtctgtgggcaacaccctgtactacgtgaacaaacaagagggccagtctctgtacgtgaagggcgagcccatcatcaacttctacgaccctctggtgttccccagcgacgagttcgatgccagcatcagccaagtgaacgagaagatcaatcagagcctggccttcatcagaaagtccgatgagctgctgcacaacgtgaacgccggcaagtccaccaccaatatcatgatcacgaccatcatcatcgtgattatcgtgatcctgctgtccctgatcgccgtgggcctgctgctttattgataataggctggagcctcggtggccatgcttcttgccccttgggcctccccccagcccctcctccccttcctgcacccgtacccccgtggtctttgaataaagtctgagtgggcggcaaaaaaaaaaaaaaaaaaaaaaaaaaaaaaaaaaaaaaaaaaaaaaaaaaaaaaaaaaaaaaaaaaaaaaaaaaaaaaaaaaaaaaaaaaaaaaaaaaaaaaaaaaaaaa

SEQ ID NO: 162 - DNA, 1871 bp, synthetic construct
  source 1..1871: mol_type = other DNA
agcggctcggccattttgtcccagtcagtccggaggctgcggctgcagaagtaccgcctgcggagtaactgcaaaggccaccatggaactgctgatcctgaaggccaacgccatcaccaccatcctgaccgccgtgaccttctgttttgccagcggccagaacatcaccgaggaattctaccagagcacctgtagcgccgtgtccaagggatatctgggcgcccttagaaccggctggtacaccagcgtgatcaccatcgagctgagcaacatcaaagaaaacaagtgcaacggcaccgacgccaaagtgaagctgatcaagcaagagctggacaagtacaagaatgccgtgaccgacctgcagctgctgatgcagtctacaccagccacaggctctggctctttcctgggctgcctgctcggagtgggcagcgccattgcctctggtgtcgccgtgtctaaagtgctgcacctggaaggcgaagtgaacaagatcaagagcgccctgctgagcaccaacaaggccgtggtgtctctgagcaatggcgtgtccgtgctgaccttcaaggtgctggacctgaagaactacatcgacaaacagctgctgcccatcctgaacaagcagtcctgcagcatccccaacatcgagacagtgatcgagttccagcagaagaacaaccggctgctggaaatcacccgcgagttctctgtgaatgccggcgtgaccacacctgtgtccacctacatgctgaccaacagcgagctgctgagcctgatcaacgacatgcccatcaccaacgaccagaaaaagctgatgagcaacaacgtgcagatcgtgcggcagcagagctacagcatcatgagcattatcaaagaagaggtgctggcctacgtggtgcagctgcctctgtatggcgtgatcgataccccttgctggaagctgcacacaagccctctgtgcaccaccaacaccaaagagggcagcaacatctgcctgaccagaaccgacagaggctggtactgcgataatgccggcagcgtctcattcttcccacaagccgagacatgcaaggtgcagagcaaccgggtgttctgcgactgcatgaatagcagaaccctgccttccgaagtgaatctgtgcaacgtggacatcttcaaccctaagtacgactgcaagatcatgaccagcaagaccgacgtgtccagcagtgtgatcacctcactgggcgccatcgtgtcctgttacggcaagaccaagtgcaccgccagcaacaagaaccggggcatcatcaagaccttcagcaacggctgcgactacgtgtccaacaaaggcgtggacaccgtgtctgtgggcaacaccctgtactacgtgaacaaacaagagggccagtctctgtacgtgaagggcgagcccatcatcaacttctacgaccctctggtgttccccagcgacgagttcgatgccagcatcagccaagtgaacgagaagatcaatcagagcctggccttcatcagaaagtccgatgagctgctgcacaacgtgaacgccggcaagtccaccaccaatatcatgatcacgaccatcatcatcgtgattatcgtgatcctgctgtccctgatcgccgtgggcctgctgctttattgataataggctggagcctcggtggccatgcttcttgccccttgggcctccccccagcccctcctccccttcctgcacccgtacccccgtggtctttgaataaagtctgagtgggcggcaaaaaaaaaaaaaaaaaaaaaaaaaaaaaaaaaaaaaaaaaaaaaaaaaaaaaaaaaaaaaaaaaaaaaaaaaaaaaaaaaaaaaaaaaaaaaaaaaaaaaaaaaaaaaa

SEQ ID NO: 163 - DNA, 1569 bp, synthetic construct
  source 1..1569: mol_type = other DNA
atggaactgctgatcctgaaggccaacgccatcaccaccatcctgaccgccgtgaccttctgttttgccagcggccagaacatcaccgaggaattctaccagagcacctgtagcgccgtgtccaagggatatctgggcgcccttagaaccggctggtacaccagcgtgatcaccatcgagctgagcaacatcaaagaaaacaagtgcaacggcaccgacgccaaagtgaagctgatcaagcaagagctggacaagtacaagaatgccgtgaccgacctgcagctgctgatgcagtctacaccagccacaggctctggctctttcctgggctgcctgctcggagtgggcagcgccattgcctctggtgtcgccgtgtctaaagtgctgcacctggaaggcgaagtgaacaagatcaagagcgccctgctgagcaccaacaaggccgtggtgtctctgagcaatggcgtgtccgtgctgaccttcaaggtgctggacctgaagaactacatcgacaaacagctgctgcccatcctgaacaagcagtcctgcagcatccccaacatcgagacagtgatcgagttccagcagaagaacaaccggctgctggaaatcacccgcgagttctctgtgaatgccggcgtgaccacacctgtgtccacctacatgctgaccaacagcgagctgctgagcctgatcaacgacatgcccatcaccaacgaccagaaaaagctgatgagcaacaacgtgcagatcgtgcggcagcagagctacagcatcatgagcattatcaaagaagaggtgctggcctacgtggtgcagctgcctctgtatggcgtgatcgataccccttgctggaagctgcacacaagccctctgtgcaccaccaacaccaaagagggcagcaacatctgcctgaccagaaccgacagaggctggtactgcgataatgccggcagcgtctcattcttcccacaagccgagacatgcaaggtgcagagcaaccgggtgttctgcgactgcatgaatagcagaaccctgccttccgaagtgaatctgtgcaacgtggacatcttcaaccctaagtacgactgcaagatcatgaccagcaagaccgacgtgtccagcagtgtgatcacctcactgggcgccatcgtgtcctgttacggcaagaccaagtgcaccgccagcaacaagaaccggggcatcatcaagaccttcagcaacggctgcgactacgtgtccaacaaaggcgtggacaccgtgtctgtgggcaacaccctgtactacgtgaacaaacaagagggccagtctctgtacgtgaagggcgagcccatcatcaacttctacgaccctctggtgttccccagcgacgagttcgatgccagcatcagccaagtgaacgagaagatcaatcagagcctggccttcatcagaaagtccgatgagctgctgcacaacgtgaacgccggcaagtccaccaccaatatcatgatcacgaccatcatcatcgtgattatcgtgatcctgctgtccctgatcgccgtgggcctgctgctttattgataatag

SEQ ID NO: 164 - protein, 520 aa, synthetic construct
MELLILKANAITTILTAVTFCFASGQNITEEFYQSTCSAVSKGYLGALRTGWYTSVITIELSNIKENKCNGTDAKVKLIKQELDKYKNAVTDLQLLMQSTPATGSGSFLGCLLGVGSAIASGVAVSKVLHLEGEVNKIKSALLSTNKAVVSLSNGVSVLTFKVLDLKNYIDKQLLPILNKQSCSIPNIETVIEFQQKNNRLLEITREFSVNAGVTTPVSTYMLTNSELLSLINDMPITNDQKKLMSNNVQIVRQQSYSIMSIIKEEVLAYVVQLPLYGVIDTPCWKLHTSPLCTTNTKEGSNICLTRTDRGWYCDNAGSVSFFPQAETCKVQSNRVFCDCMNSRTLPSEVNLCNVDIFNPKYDCKIMTSKTDVSSSVITSLGAIVSCYGKTKCTASNKNRGIIKTFSNGCDYVSNKGVDTVSVGNTLYYVNKQEGQSLYVKGEPIINFYDPLVFPSDEFDASISQVNEKINQSLAFIRKSDELLHNVNAGKSTTNIMITTIIIVIIVILLSLIAVGLLLY

SEQ ID NO: 165 - RNA, 1871 nt, synthetic construct
  source 1..1871: mol_type = other RNA
agcggctcggccattttgtcccagtcagtccggaggctgcggctgcagaagtaccgcctgcggagtaactgcaaaggccaccatggaactgctgatcctgaaggccaacgccatcaccaccatcctgaccgccgtgaccttctgttttgccagcggccagaacatcaccgaggaattctaccagagcacctgtagcgccgtgtccaagggatatctgggcgcccttagaaccggctggtacaccagcgtgatcaccatcgagctgagcaacatcaaagaaaacaagtgcaacggcaccgacgccaaagtgaagctgatcaagcaagagctggacaagtacaagaatgccgtgaccgacctgcagctgctgatgcagtctacaccagccacaggctctggctctttcctgggctgcctgctcggagtgggcagcgccattgcctctggtgtcgccgtgtctaaagtgctgcacctggaaggcgaagtgaacaagatcaagagcgccctgctgagcaccaacaaggccgtggtgtctctgagcaatggcgtgtccgtgctgaccttcaaggtgctggacctgaagaactacatcgacaaacagctgctgcccatcctgaacaagcagtcctgcagcatccccaacatcgagacagtgatcgagttccagcagaagaacaaccggctgctggaaatcacccgcgagttctctgtgaatgccggcgtgaccacacctgtgtccacctacatgctgaccaacagcgagctgctgagcctgatcaacgacatgcccatcaccaacgaccagaaaaagctgatgagcaacaacgtgcagatcgtgcggcagcagagctacagcatcatgagcattatcaaagaagaggtgctggcctacgtggtgcagctgcctctgtatggcgtgatcgataccccttgctggaagctgcacacaagccctctgtgcaccaccaacaccaaagagggcagcaacatctgcctgaccagaaccgacagaggctggtactgcgataatgccggcagcgtctcattcttcccacaagccgagacatgcaaggtgcagagcaaccgggtgttctgcgactgcatgaatagcagaaccctgccttccgaagtgaatctgtgcaacgtggacatcttcaaccctaagtacgactgcaagatcatgaccagcaagaccgacgtgtccagcagtgtgatcacctcactgggcgccatcgtgtcctgttacggcaagaccaagtgcaccgccagcaacaagaaccggggcatcatcaagaccttcagcaacggctgcgactacgtgtccaacaaaggcgtggacaccgtgtctgtgggcaacaccctgtactacgtgaacaaacaagagggccagtctctgtacgtgaagggcgagcccatcatcaacttctacgaccctctggtgttccccagcgacgagttcgatgccagcatcagccaagtgaacgagaagatcaatcagagcctggccttcatcagaaagtccgatgagctgctgcacaacgtgaacgccggcaagtccaccaccaatatcatgatcacgaccatcatcatcgtgattatcgtgatcctgctgtccctgatcgccgtgggcctgctgctttattgataataggctggagcctcggtggccatgcttcttgccccttgggcctccccccagcccctcctccccttcctgcacccgtacccccgtggtctttgaataaagtctgagtgggcggcaaaaaaaaaaaaaaaaaaaaaaaaaaaaaaaaaaaaaaaaaaaaaaaaaaaaaaaaaaaaaaaaaaaaaaaaaaaaaaaaaaaaaaaaaaaaaaaaaaaaaaaaaaaaaa

SEQ ID NO: 166 - DNA, 1841 bp, synthetic construct
  source 1..1841: mol_type = other DNA
agcggctcggccattttgtcccagtcagtccggaggctgcggctgcagaagtaccgcctgcggagtaactgcaaaggccaccatggaactgctgatcctgaaggccaacgccatcaccaccatcctgaccgccgtgaccttctgttttgccagcggccagaacatcaccgaggaattctaccagagcacctgtagcgccgtgtccaagggatatctgggcgcccttagaaccggctggtacaccagcgtgatcaccatcgagctgagcaacatcaaagaaaacaagtgcaacggcaccgacgccaaagtgaagctgatcaagcaagagctggacaagtacaagaatgccgtgaccgacctgcagctgctgatgcagtctacaccagccacaggctctggctgcgccattgcctctggtgtcgccgtgtctaaagtgctgcacctggaaggcgaagtgaacaagatcaagagcgccctgctgagcaccaacaaggccgtggtgtctctgagcaatggcgtgtccgtgctgaccttcaaggtgctggacctgaagaactacatcgacaaacagctgctgcccatcctgaacaagcagtcctgcagcatccccaacatcgagacagtgatcgagttccagcagaagaacaaccggctgctggaaatcacccgcgagttctctgtgaatgccggcgtgaccacacctgtgtccacctacatgctgaccaacagcgagctgctgagcctgatcaacgacatgcccatcaccaacgaccagaaaaagctgatgagcaacaacgtgcagatcgtgcggcagcagagctacagcatcatgagcattatcaaagaagaggtgctggcctacgtggtgcagctgccttgctatggcgtgatcgataccccttgctggaagctgcacacaagccctctgtgcaccaccaacaccaaagagggcagcaacatctgcctgaccagaaccgacagaggctggtactgcgataatgccggcagcgtctcattcttcccacaagccgagacatgcaaggtgcagagcaaccgggtgttctgcgacaccatgaatagcagaaccctgccttccgaagtgaatctgtgcaacgtggacatcttcaaccctaagtacgactgcaagatcatgaccagcaagaccgacgtgtccagcagtgtgatcacctcactgggcgccatcgtgtcctgttacggcaagaccaagtgcaccgccagcaacaagaaccggggcatcatcaagaccttcagcaacggctgcgactacgtgtccaacaaaggcgtggacaccgtgtctgtgggcaacaccctgtactacgtgaacaaacaagagggccagtctctgtacgtgaagggcgagcccatcatcaacttctacgaccctctggtgttccccagcgacgagttcgatgccagcatcagccaagtgaacgagaagatcaatcagagcctggccttcatcagaaagtccgatgagctgctgcacaacgtgaacgccggcaagtccaccaccaatatcatgatcacgaccatcatcatcgtgattatcgtgatcctgctgtccctgatcgccgtgggcctgctgctttattgataataggctggagcctcggtggccatgcttcttgccccttgggcctccccccagcccctcctccccttcctgcacccgtacccccgtggtctttgaataaagtctgagtgggcggcaaaaaaaaaaaaaaaaaaaaaaaaaaaaaaaaaaaaaaaaaaaaaaaaaaaaaaaaaaaaaaaaaaaaaaaaaaaaaaaaaaaaaaaaaaaaaaaaaaaaaaaaaaaaaa

SEQ ID NO: 167 - DNA, 1539 bp, synthetic construct
  source 1..1539: mol_type = other DNA
atggaactgctgatcctgaaggccaacgccatcaccaccatcctgaccgccgtgaccttctgttttgccagcggccagaacatcaccgaggaattctaccagagcacctgtagcgccgtgtccaagggatatctgggcgcccttagaaccggctggtacaccagcgtgatcaccatcgagctgagcaacatcaaagaaaacaagtgcaacggcaccgacgccaaagtgaagctgatcaagcaagagctggacaagtacaagaatgccgtgaccgacctgcagctgctgatgcagtctacaccagccacaggctctggctgcgccattgcctctggtgtcgccgtgtctaaagtgctgcacctggaaggcgaagtgaacaagatcaagagcgccctgctgagcaccaacaaggccgtggtgtctctgagcaatggcgtgtccgtgctgaccttcaaggtgctggacctgaagaactacatcgacaaacagctgctgcccatcctgaacaagcagtcctgcagcatccccaacatcgagacagtgatcgagttccagcagaagaacaaccggctgctggaaatcacccgcgagttctctgtgaatgccggcgtgaccacacctgtgtccacctacatgctgaccaacagcgagctgctgagcctgatcaacgacatgcccatcaccaacgaccagaaaaagctgatgagcaacaacgtgcagatcgtgcggcagcagagctacagcatcatgagcattatcaaagaagaggtgctggcctacgtggtgcagctgccttgctatggcgtgatcgataccccttgctggaagctgcacacaagccctctgtgcaccaccaacaccaaagagggcagcaacatctgcctgaccagaaccgacagaggctggtactgcgataatgccggcagcgtctcattcttcccacaagccgagacatgcaaggtgcagagcaaccgggtgttctgcgacaccatgaatagcagaaccctgccttccgaagtgaatctgtgcaacgtggacatcttcaaccctaagtacgactgcaagatcatgaccagcaagaccgacgtgtccagcagtgtgatcacctcactgggcgccatcgtgtcctgttacggcaagaccaagtgcaccgccagcaacaagaaccggggcatcatcaagaccttcagcaacggctgcgactacgtgtccaacaaaggcgtggacaccgtgtctgtgggcaacaccctgtactacgtgaacaaacaagagggccagtctctgtacgtgaagggcgagcccatcatcaacttctacgaccctctggtgttccccagcgacgagttcgatgccagcatcagccaagtgaacgagaagatcaatcagagcctggccttcatcagaaagtccgatgagctgctgcacaacgtgaacgccggcaagtccaccaccaatatcatgatcacgaccatcatcatcgtgattatcgtgatcctgctgtccctgatcgccgtgggcctgctgctttattgataatag

SEQ ID NO: 168 - protein, 510 aa, synthetic construct
MELLILKANAITTILTAVTFCFASGQNITEEFYQSTCSAVSKGYLGALRTGWYTSVITIELSNIKENKCNGTDAKVKLIKQELDKYKNAVTDLQLLMQSTPATGSGCAIASGVAVSKVLHLEGEVNKIKSALLSTNKAVVSLSNGVSVLTFKVLDLKNYIDKQLLPILNKQSCSIPNIETVIEFQQKNNRLLEITREFSVNAGVTTPVSTYMLTNSELLSLINDMPITNDQKKLMSNNVQIVRQQSYSIMSIIKEEVLAYVVQLPCYGVIDTPCWKLHTSPLCTTNTKEGSNICLTRTDRGWYCDNAGSVSFFPQAETCKVQSNRVFCDTMNSRTLPSEVNLCNVDIFNPKYDCKIMTSKTDVSSSVITSLGAIVSCYGKTKCTASNKNRGIIKTFSNGCDYVSNKGVDTVSVGNTLYYVNKQEGQSLYVKGEPIINFYDPLVFPSDEFDASISQVNEKINQSLAFIRKSDELLHNVNAGKSTTNIMITTIIIVIIVILLSLIAVGLLLY

SEQ ID NO: 169 - RNA, 1841 nt, synthetic construct
  source 1..1841: mol_type = other RNA
agcggctcggccattttgtcccagtcagtccggaggctgcggctgcagaagtaccgcctgcggagtaactgcaaaggccaccatggaactgctgatcctgaaggccaacgccatcaccaccatcctgaccgccgtgaccttctgttttgccagcggccagaacatcaccgaggaattctaccagagcacctgtagcgccgtgtccaagggatatctgggcgcccttagaaccggctggtacaccagcgtgatcaccatcgagctgagcaacatcaaagaaaacaagtgcaacggcaccgacgccaaagtgaagctgatcaagcaagagctggacaagtacaagaatgccgtgaccgacctgcagctgctgatgcagtctacaccagccacaggctctggctgcgccattgcctctggtgtcgccgtgtctaaagtgctgcacctggaaggcgaagtgaacaagatcaagagcgccctgctgagcaccaacaaggccgtggtgtctctgagcaatggcgtgtccgtgctgaccttcaaggtgctggacctgaagaactacatcgacaaacagctgctgcccatcctgaacaagcagtcctgcagcatccccaacatcgagacagtgatcgagttccagcagaagaacaaccggctgctggaaatcacccgcgagttctctgtgaatgccggcgtgaccacacctgtgtccacctacatgctgaccaacagcgagctgctgagcctgatcaacgacatgcccatcaccaacgaccagaaaaagctgatgagcaacaacgtgcagatcgtgcggcagcagagctacagcatcatgagcattatcaaagaagaggtgctggcctacgtggtgcagctgccttgctatggcgtgatcgataccccttgctggaagctgcacacaagccctctgtgcaccaccaacaccaaagagggcagcaacatctgcctgaccagaaccgacagaggctggtactgcgataatgccggcagcgtctcattcttcccacaagccgagacatgcaaggtgcagagcaaccgggtgttctgcgacaccatgaatagcagaaccctgccttccgaagtgaatctgtgcaacgtggacatcttcaaccctaagtacgactgcaagatcatgaccagcaagaccgacgtgtccagcagtgtgatcacctcactgggcgccatcgtgtcctgttacggcaagaccaagtgcaccgccagcaacaagaaccggggcatcatcaagaccttcagcaacggctgcgactacgtgtccaacaaaggcgtggacaccgtgtctgtgggcaacaccctgtactacgtgaacaaacaagagggccagtctctgtacgtgaagggcgagcccatcatcaacttctacgaccctctggtgttccccagcgacgagttcgatgccagcatcagccaagtgaacgagaagatcaatcagagcctggccttcatcagaaagtccgatgagctgctgcacaacgtgaacgccggcaagtccaccaccaatatcatgatcacgaccatcatcatcgtgattatcgtgatcctgctgtccctgatcgccgtgggcctgctgctttattgataataggctggagcctcggtggccatgcttcttgccccttgggcctccccccagcccctcctccccttcctgcacccgtacccccgtggtctttgaataaagtctgagtgggcggcaaaaaaaaaaaaaaaaaaaaaaaaaaaaaaaaaaaaaaaaaaaaaaaaaaaaaaaaaaaaaaaaaaaaaaaaaaaaaaaaaaaaaaaaaaaaaaaaaaaaaaaaaaaaaa

SEQ ID NO: 170 - DNA, 1841 bp, synthetic construct
  source 1..1841: mol_type = other DNA
agcggctcggccattttgtcccagtcagtccggaggctgcggctgcagaagtaccgcctgcggagtaactgcaaaggccaccatggaactgctgatcctgaaggccaacgccatcaccaccatcctgaccgccgtgaccttctgttttgccagcggccagaacatcaccgaggaattctaccagagcacctgtagcgccgtgtccaagggatatctgggcgcccttagaaccggctggtacaccagcgtgatcaccatcgagctgagcaacatcaaagaaaacaagtgcaacggcaccgacgccaaagtgaagctgatcaagcaagagctggacaagtacaagaatgccgtgaccgacctgcagctgctgatgcagtctacaccagccacaggctctggcagcgccatttgctctggtgtcgccgtgtctaaagtgctgcacctggaaggcgaagtgaacaagatcaagagcgccctgctgagcaccaacaaggccgtggtgtctctgagcaatggcgtgtccgtgctgaccttcaaggtgctggacctgaagaactacatcgacaaacagctgctgcccatcctgaacaagcagtcctgcagcatccccaacatcgagacagtgatcgagttccagcagaagaacaaccggctgctggaaatcacccgcgagttctctgtgaatgccggcgtgaccacacctgtgtccacctacatgctgaccaacagcgagctgctgagcctgatcaacgacatgcccatcaccaacgaccagaaaaagctgatgagcaacaacgtgcagatcgtgcggcagcagagctacagcatcatgagcattatcaaagaagaggtgctggcctacgtggtgcagctgcctctgtgcggcgtgatcgataccccttgctggaagctgcacacaagccctctgtgcaccaccaacaccaaagagggcagcaacatctgcctgaccagaaccgacagaggctggtactgcgataatgccggcagcgtctcattcttcccacaagccgagacatgcaaggtgcagagcaaccgggtgttctgcgacaccatgaatagcagaaccctgccttccgaagtgaatctgtgcaacgtggacatcttcaaccctaagtacgactgcaagatcatgaccagcaagaccgacgtgtccagcagtgtgatcacctcactgggcgccatcgtgtcctgttacggcaagaccaagtgcaccgccagcaacaagaaccggggcatcatcaagaccttcagcaacggctgcgactacgtgtccaacaaaggcgtggacaccgtgtctgtgggcaacaccctgtactacgtgaacaaacaagagggccagtctctgtacgtgaagggcgagcccatcatcaacttctacgaccctctggtgttccccagcgacgagttcgatgccagcatcagccaagtgaacgagaagatcaatcagagcctggccttcatcagaaagtccgatgagctgctgcacaacgtgaacgccggcaagtccaccaccaatatcatgatcacgaccatcatcatcgtgattatcgtgatcctgctgtccctgatcgccgtgggcctgctgctttattgataataggctggagcctcggtggccatgcttcttgccccttgggcctccccccagcccctcctccccttcctgcacccgtacccccgtggtctttgaataaagtctgagtgggcggcaaaaaaaaaaaaaaaaaaaaaaaaaaaaaaaaaaaaaaaaaaaaaaaaaaaaaaaaaaaaaaaaaaaaaaaaaaaaaaaaaaaaaaaaaaaaaaaaaaaaaaaaaaaaaa

SEQ ID NO: 171 - DNA, 1539 bp, synthetic construct
  source 1..1539: mol_type = other DNA
atggaactgctgatcctgaaggccaacgccatcaccaccatcctgaccgccgtgaccttctgttttgccagcggccagaacatcaccgaggaattctaccagagcacctgtagcgccgtgtccaagggatatctgggcgcccttagaaccggctggtacaccagcgtgatcaccatcgagctgagcaacatcaaagaaaacaagtgcaacggcaccgacgccaaagtgaagctgatcaagcaagagctggacaagtacaagaatgccgtgaccgacctgcagctgctgatgcagtctacaccagccacaggctctggcagcgccatttgctctggtgtcgccgtgtctaaagtgctgcacctggaaggcgaagtgaacaagatcaagagcgccctgctgagcaccaacaaggccgtggtgtctctgagcaatggcgtgtccgtgctgaccttcaaggtgctggacctgaagaactacatcgacaaacagctgctgcccatcctgaacaagcagtcctgcagcatccccaacatcgagacagtgatcgagttccagcagaagaacaaccggctgctggaaatcacccgcgagttctctgtgaatgccggcgtgaccacacctgtgtccacctacatgctgaccaacagcgagctgctgagcctgatcaacgacatgcccatcaccaacgaccagaaaaagctgatgagcaacaacgtgcagatcgtgcggcagcagagctacagcatcatgagcattatcaaagaagaggtgctggcctacgtggtgcagctgcctctgtgcggcgtgatcgataccccttgctggaagctgcacacaagccctctgtgcaccaccaacaccaaagagggcagcaacatctgcctgaccagaaccgacagaggctggtactgcgataatgccggcagcgtctcattcttcccacaagccgagacatgcaaggtgcagagcaaccgggtgttctgcgacaccatgaatagcagaaccctgccttccgaagtgaatctgtgcaacgtggacatcttcaaccctaagtacgactgcaagatcatgaccagcaagaccgacgtgtccagcagtgtgatcacctcactgggcgccatcgtgtcctgttacggcaagaccaagtgcaccgccagcaacaagaaccggggcatcatcaagaccttcagcaacggctgcgactacgtgtccaacaaaggcgtggacaccgtgtctgtgggcaacaccctgtactacgtgaacaaacaagagggccagtctctgtacgtgaagggcgagcccatcatcaacttctacgaccctctggtgttccccagcgacgagttcgatgccagcatcagccaagtgaacgagaagatcaatcagagcctggccttcatcagaaagtccgatgagctgctgcacaacgtgaacgccggcaagtccaccaccaatatcatgatcacgaccatcatcatcgtgattatcgtgatcctgctgtccctgatcgccgtgggcctgctgctttattgataatag

SEQ ID NO: 172 - protein, 510 aa, synthetic construct
MELLILKANAITTILTAVTFCFASGQNITEEFYQSTCSAVSKGYLGALRTGWYTSVITIELSNIKENKCNGTDAKVKLIKQELDKYKNAVTDLQLLMQSTPATGSGSAICSGVAVSKVLHLEGEVNKIKSALLSTNKAVVSLSNGVSVLTFKVLDLKNYIDKQLLPILNKQSCSIPNIETVIEFQQKNNRLLEITREFSVNAGVTTPVSTYMLTNSELLSLINDMPITNDQKKLMSNNVQIVRQQSYSIMSIIKEEVLAYVVQLPLCGVIDTPCWKLHTSPLCTTNTKEGSNICLTRTDRGWYCDNAGSVSFFPQAETCKVQSNRVFCDTMNSRTLPSEVNLCNVDIFNPKYDCKIMTSKTDVSSSVITSLGAIVSCYGKTKCTASNKNRGIIKTFSNGCDYVSNKGVDTVSVGNTLYYVNKQEGQSLYVKGEPIINFYDPLVFPSDEFDASISQVNEKINQSLAFIRKSDELLHNVNAGKSTTNIMITTIIIVIIVILLSLIAVGLLLY

SEQ ID NO: 173 - RNA, 1841 nt, synthetic construct
  source 1..1841: mol_type = other RNA
agcggctcggccattttgtcccagtcagtccggaggctgcggctgcagaagtaccgcctgcggagtaactgcaaaggccaccatggaactgctgatcctgaaggccaacgccatcaccaccatcctgaccgccgtgaccttctgttttgccagcggccagaacatcaccgaggaattctaccagagcacctgtagcgccgtgtccaagggatatctgggcgcccttagaaccggctggtacaccagcgtgatcaccatcgagctgagcaacatcaaagaaaacaagtgcaacggcaccgacgccaaagtgaagctgatcaagcaagagctggacaagtacaagaatgccgtgaccgacctgcagctgctgatgcagtctacaccagccacaggctctggcagcgccatttgctctggtgtcgccgtgtctaaagtgctgcacctggaaggcgaagtgaacaagatcaagagcgccctgctgagcaccaacaaggccgtggtgtctctgagcaatggcgtgtccgtgctgaccttcaaggtgctggacctgaagaactacatcgacaaacagctgctgcccatcctgaacaagcagtcctgcagcatccccaacatcgagacagtgatcgagttccagcagaagaacaaccggctgctggaaatcacccgcgagttctctgtgaatgccggcgtgaccacacctgtgtccacctacatgctgaccaacagcgagctgctgagcctgatcaacgacatgcccatcaccaacgaccagaaaaagctgatgagcaacaacgtgcagatcgtgcggcagcagagctacagcatcatgagcattatcaaagaagaggtgctggcctacgtggtgcagctgcctctgtgcggcgtgatcgataccccttgctggaagctgcacacaagccctctgtgcaccaccaacaccaaagagggcagcaacatctgcctgaccagaaccgacagaggctggtactgcgataatgccggcagcgtctcattcttcccacaagccgagacatgcaaggtgcagagcaaccgggtgttctgcgacaccatgaatagcagaaccctgccttccgaagtgaatctgtgcaacgtggacatcttcaaccctaagtacgactgcaagatcatgaccagcaagaccgacgtgtccagcagtgtgatcacctcactgggcgccatcgtgtcctgttacggcaagaccaagtgcaccgccagcaacaagaaccggggcatcatcaagaccttcagcaacggctgcgactacgtgtccaacaaaggcgtggacaccgtgtctgtgggcaacaccctgtactacgtgaacaaacaagagggccagtctctgtacgtgaagggcgagcccatcatcaacttctacgaccctctggtgttccccagcgacgagttcgatgccagcatcagccaagtgaacgagaagatcaatcagagcctggccttcatcagaaagtccgatgagctgctgcacaacgtgaacgccggcaagtccaccaccaatatcatgatcacgaccatcatcatcgtgattatcgtgatcctgctgtccctgatcgccgtgggcctgctgctttattgataataggctggagcctcggtggccatgcttcttgccccttgggcctccccccagcccctcctccccttcctgcacccgtacccccgtggtctttgaataaagtctgagtgggcggcaaaaaaaaaaaaaaaaaaaaaaaaaaaaaaaaaaaaaaaaaaaaaaaaaaaaaaaaaaaaaaaaaaaaaaaaaaaaaaaaaaaaaaaaaaaaaaaaaaaaaaaaaaaaaa

SEQ ID NO: 174 - DNA, 1841 bp, synthetic construct
  source 1..1841: mol_type = other DNA
agcggctcggccattttgtcccagtcagtccggaggctgcggctgcagaagtaccgcctgcggagtaactgcaaaggccaccatggaactgctgatcctgaaggccaacgccatcaccaccatcctgaccgccgtgaccttctgttttgccagcggccagaacatcaccgaggaattctaccagagcacctgtagcgccgtgtccaagggatatctgggcgcccttagaaccggctggtacaccagcgtgatcaccatcgagctgagcaacatcaaagaaaacaagtgcaacggcaccgacgccaaagtgaagctgatcaagcaagagctggacaagtacaagaatgccgtgaccgacctgcagctgctgatgcagtctacaccagccacaggctctggcagcgcctgcgcctctggtgtcgccgtgtctaaagtgctgcacctggaaggcgaagtgaacaagatcaagagcgccctgctgagcaccaacaaggccgtggtgtctctgagcaatggcgtgtccgtgctgaccttcaaggtgctggacctgaagaactacatcgacaaacagctgctgcccatcctgaacaagcagtcctgcagcatccccaacatcgagacagtgatcgagttccagcagaagaacaaccggctgctggaaatcacccgcgagttctctgtgaatgccggcgtgaccacacctgtgtccacctacatgctgaccaacagcgagctgctgagcctgatcaacgacatgcccatcaccaacgaccagaaaaagctgatgagcaacaacgtgcagatcgtgcggcagcagagctacagctgcatgagcattatcaaagaagaggtgctggcctacgtggtgcagctgcctctgtatggcgtgatcgataccccttgctggaagctgcacacaagccctctgtgcaccaccaacaccaaagagggcagcaacatctgcctgaccagaaccgacagaggctggtactgcgataatgccggcagcgtctcattcttcccacaagccgagacatgcaaggtgcagagcaaccgggtgttctgcgacaccatgaatagcagaaccctgccttccgaagtgaatctgtgcaacgtggacatcttcaaccctaagtacgactgcaagatcatgaccagcaagaccgacgtgtccagcagtgtgatcacctcactgggcgccatcgtgtcctgttacggcaagaccaagtgcaccgccagcaacaagaaccggggcatcatcaagaccttcagcaacggctgcgactacgtgtccaacaaaggcgtggacaccgtgtctgtgggcaacaccctgtactacgtgaacaaacaagagggccagtctctgtacgtgaagggcgagcccatcatcaacttctacgaccctctggtgttccccagcgacgagttcgatgccagcatcagccaagtgaacgagaagatcaatcagagcctggccttcatcagaaagtccgatgagctgctgcacaacgtgaacgccggcaagtccaccaccaatatcatgatcacgaccatcatcatcgtgattatcgtgatcctgctgtccctgatcgccgtgggcctgctgctttattgataataggctggagcctcggtggccatgcttcttgccccttgggcctccccccagcccctcctccccttcctgcacccgtacccccgtggtctttgaataaagtctgagtgggcggcaaaaaaaaaaaaaaaaaaaaaaaaaaaaaaaaaaaaaaaaaaaaaaaaaaaaaaaaaaaaaaaaaaaaaaaaaaaaaaaaaaaaaaaaaaaaaaaaaaaaaaaaaaaaaa

SEQ ID NO: 175 - DNA, 1539 bp, synthetic construct
  source 1..1539: mol_type = other DNA
atggaactgctgatcctgaaggccaacgccatcaccaccatcctgaccgccgtgaccttctgttttgccagcggccagaacatcaccgaggaattctaccagagcacctgtagcgccgtgtccaagggatatctgggcgcccttagaaccggctggtacaccagcgtgatcaccatcgagctgagcaacatcaaagaaaacaagtgcaacggcaccgacgccaaagtgaagctgatcaagcaagagctggacaagtacaagaatgccgtgaccgacctgcagctgctgatgcagtctacaccagccacaggctctggcagcgcctgcgcctctggtgtcgccgtgtctaaagtgctgcacctggaaggcgaagtgaacaagatcaagagcgccctgctgagcaccaacaaggccgtggtgtctctgagcaatggcgtgtccgtgctgaccttcaaggtgctggacctgaagaactacatcgacaaacagctgctgcccatcctgaacaagcagtcctgcagcatccccaacatcgagacagtgatcgagttccagcagaagaacaaccggctgctggaaatcacccgcgagttctctgtgaatgccggcgtgaccacacctgtgtccacctacatgctgaccaacagcgagctgctgagcctgatcaacgacatgcccatcaccaacgaccagaaaaagctgatgagcaacaacgtgcagatcgtgcggcagcagagctacagctgcatgagcattatcaaagaagaggtgctggcctacgtggtgcagctgcctctgtatggcgtgatcgataccccttgctggaagctgcacacaagccctctgtgcaccaccaacaccaaagagggcagcaacatctgcctgaccagaaccgacagaggctggtactgcgataatgccggcagcgtctcattcttcccacaagccgagacatgcaaggtgcagagcaaccgggtgttctgcgacaccatgaatagcagaaccctgccttccgaagtgaatctgtgcaacgtggacatcttcaaccctaagtacgactgcaagatcatgaccagcaagaccgacgtgtccagcagtgtgatcacctcactgggcgccatcgtgtcctgttacggcaagaccaagtgcaccgccagcaacaagaaccggggcatcatcaagaccttcagcaacggctgcgactacgtgtccaacaaaggcgtggacaccgtgtctgtgggcaacaccctgtactacgtgaacaaacaagagggccagtctctgtacgtgaagggcgagcccatcatcaacttctacgaccctctggtgttccccagcgacgagttcgatgccagcatcagccaagtgaacgagaagatcaatcagagcctggccttcatcagaaagtccgatgagctgctgcacaacgtgaacgccggcaagtccaccaccaatatcatgatcacgaccatcatcatcgtgattatcgtgatcctgctgtccctgatcgccgtgggcctgctgctttattgataatag

SEQ ID NO: 176 - protein, 510 aa, synthetic construct
MELLILKANAITTILTAVTFCFASGQNITEEFYQSTCSAVSKGYLGALRTGWYTSVITIELSNIKENKCNGTDAKVKLIKQELDKYKNAVTDLQLLMQSTPATGSGSACASGVAVSKVLHLEGEVNKIKSALLSTNKAVVSLSNGVSVLTFKVLDLKNYIDKQLLPILNKQSCSIPNIETVIEFQQKNNRLLEITREFSVNAGVTTPVSTYMLTNSELLSLINDMPITNDQKKLMSNNVQIVRQQSYSCMSIIKEEVLAYVVQLPLYGVIDTPCWKLHTSPLCTTNTKEGSNICLTRTDRGWYCDNAGSVSFFPQAETCKVQSNRVFCDTMNSRTLPSEVNLCNVDIFNPKYDCKIMTSKTDVSSSVITSLGAIVSCYGKTKCTASNKNRGIIKTFSNGCDYVSNKGVDTVSVGNTLYYVNKQEGQSLYVKGEPIINFYDPLVFPSDEFDASISQVNEKINQSLAFIRKSDELLHNVNAGKSTTNIMITTIIIVIIVILLSLIAVGLLLY

SEQ ID NO: 177 - RNA, 1841 nt, synthetic construct
  source 1..1841: mol_type = other RNA
agcggctcggccattttgtcccagtcagtccggaggctgcggctgcagaagtaccgcctgcggagtaactgcaaaggccaccatggaactgctgatcctgaaggccaacgccatcaccaccatcctgaccgccgtgaccttctgttttgccagcggccagaacatcaccgaggaattctaccagagcacctgtagcgccgtgtccaagggatatctgggcgcccttagaaccggctggtacaccagcgtgatcaccatcgagctgagcaacatcaaagaaaacaagtgcaacggcaccgacgccaaagtgaagctgatcaagcaagagctggacaagtacaagaatgccgtgaccgacctgcagctgctgatgcagtctacaccagccacaggctctggcagcgcctgcgcctctggtgtcgccgtgtctaaagtgctgcacctggaaggcgaagtgaacaagatcaagagcgccctgctgagcaccaacaaggccgtggtgtctctgagcaatggcgtgtccgtgctgaccttcaaggtgctggacctgaagaactacatcgacaaacagctgctgcccatcctgaacaagcagtcctgcagcatccccaacatcgagacagtgatcgagttccagcagaagaacaaccggctgctggaaatcacccgcgagttctctgtgaatgccggcgtgaccacacctgtgtccacctacatgctgaccaacagcgagctgctgagcctgatcaacgacatgcccatcaccaacgaccagaaaaagctgatgagcaacaacgtgcagatcgtgcggcagcagagctacagctgcatgagcattatcaaagaagaggtgctggcctacgtggtgcagctgcctctgtatggcgtgatcgataccccttgctggaagctgcacacaagccctctgtgcaccaccaacaccaaagagggcagcaacatctgcctgaccagaaccgacagaggctggtactgcgataatgccggcagcgtctcattcttcccacaagccgagacatgcaaggtgcagagcaaccgggtgttctgcgacaccatgaatagcagaaccctgccttccgaagtgaatctgtgcaacgtggacatcttcaaccctaagtacgactgcaagatcatgaccagcaagaccgacgtgtccagcagtgtgatcacctcactgggcgccatcgtgtcctgttacggcaagaccaagtgcaccgccagcaacaagaaccggggcatcatcaagaccttcagcaacggctgcgactacgtgtccaacaaaggcgtggacaccgtgtctgtgggcaacaccctgtactacgtgaacaaacaagagggccagtctctgtacgtgaagggcgagcccatcatcaacttctacgaccctctggtgttccccagcgacgagttcgatgccagcatcagccaagtgaacgagaagatcaatcagagcctggccttcatcagaaagtccgatgagctgctgcacaacgtgaacgccggcaagtccaccaccaatatcatgatcacgaccatcatcatcgtgattatcgtgatcctgctgtccctgatcgccgtgggcctgctgctttattgataataggctggagcctcggtggccatgcttcttgccccttgggcctccccccagcccctcctccccttcctgcacccgtacccccgtggtctttgaataaagtctgagtgggcggcaaaaaaaaaaaaaaaaaaaaaaaaaaaaaaaaaaaaaaaaaaaaaaaaaaaaaaaaaaaaaaaaaaaaaaaaaaaaaaaaaaaaaaaaaaaaaaaaaaaaaaaaaaaaaa

SEQ ID NO: 178 - DNA, 1841 bp, synthetic construct
  source 1..1841: mol_type = other DNA
agcggctcggccattttgtcccagtcagtccggaggctgcggctgcagaagtaccgcctgcggagtaactgcaaaggccaccatggaactgctgatcctgaaggccaacgccatcaccaccatcctgaccgccgtgaccttctgttttgccagcggccagaacatcaccgaggaattctaccagagcacctgtagcgccgtgtccaagggatatctgggcgcccttagaaccggctggtacaccagcgtgatcaccatcgagctgagcaacatcaaagaaaacaagtgcaacggcaccgacgccaaagtgaagctgatcaagcaagagctggacaagtacaagaatgccgtgaccgacctgcagctgctgatgcagtctacaccagccacaggctctggcagctgcattgcctctggtgtcgccgtgtctaaagtgctgcacctggaaggcgaagtgaacaagatcaagagcgccctgctgagcaccaacaaggccgtggtgtctctgagcaatggcgtgtccgtgctgaccttcaaggtgctggacctgaagaactacatcgacaaacagctgctgcccatcctgaacaagcagtcctgcagcatccccaacatcgagacagtgatcgagttccagcagaagaacaaccggctgctggaaatcacccgcgagttctctgtgaatgccggcgtgaccacacctgtgtccacctacatgctgaccaacagcgagctgctgagcctgatcaacgacatgcccatcaccaacgaccagaaaaagctgatgagcaacaacgtgcagatcgtgcggcagcagagctacagcatcatgagcatttgcaaagaagaggtgctggcctacgtggtgcagctgcctctgtatggcgtgatcgataccccttgctggaagctgcacacaagccctctgtgcaccaccaacaccaaagagggcagcaacatctgcctgaccagaaccgacagaggctggtactgcgataatgccggcagcgtctcattcttcccacaagccgagacatgcaaggtgcagagcaaccgggtgttctgcgacaccatgaatagcagaaccctgccttccgaagtgaatctgtgcaacgtggacatcttcaaccctaagtacgactgcaagatcatgaccagcaagaccgacgtgtccagcagtgtgatcacctcactgggcgccatcgtgtcctgttacggcaagaccaagtgcaccgccagcaacaagaaccggggcatcatcaagaccttcagcaacggctgcgactacgtgtccaacaaaggcgtggacaccgtgtctgtgggcaacaccctgtactacgtgaacaaacaagagggccagtctctgtacgtgaagggcgagcccatcatcaacttctacgaccctctggtgttccccagcgacgagttcgatgccagcatcagccaagtgaacgagaagatcaatcagagcctggccttcatcagaaagtccgatgagctgctgcacaacgtgaacgccggcaagtccaccaccaatatcatgatcacgaccatcatcatcgtgattatcgtgatcctgctgtccctgatcgccgtgggcctgctgctttattgataataggctggagcctcggtggccatgcttcttgccccttgggcctccccccagcccctcctccccttcctgcacccgtacccccgtggtctttgaataaagtctgagtgggcggcaaaaaaaaaaaaaaaaaaaaaaaaaaaaaaaaaaaaaaaaaaaaaaaaaaaaaaaaaaaaaaaaaaaaaaaaaaaaaaaaaaaaaaaaaaaaaaaaaaaaaaaaaaaaaa

SEQ ID NO: 179 - DNA, 1539 bp, synthetic construct
  source 1..1539: mol_type = other DNA
atggaactgctgatcctgaaggccaacgccatcaccaccatcctgaccgccgtgaccttctgttttgccagcggccagaacatcaccgaggaattctaccagagcacctgtagcgccgtgtccaagggatatctgggcgcccttagaaccggctggtacaccagcgtgatcaccatcgagctgagcaacatcaaagaaaacaagtgcaacggcaccgacgccaaagtgaagctgatcaagcaagagctggacaagtacaagaatgccgtgaccgacctgcagctgctgatgcagtctacaccagccacaggctctggcagctgcattgcctctggtgtcgccgtgtctaaagtgctgcacctggaaggcgaagtgaacaagatcaagagcgccctgctgagcaccaacaaggccgtggtgtctctgagcaatggcgtgtccgtgctgaccttcaaggtgctggacctgaagaactacatcgacaaacagctgctgcccatcctgaacaagcagtcctgcagcatccccaacatcgagacagtgatcgagttccagcagaagaacaaccggctgctggaaatcacccgcgagttctctgtgaatgccggcgtgaccacacctgtgtccacctacatgctgaccaacagcgagctgctgagcctgatcaacgacatgcccatcaccaacgaccagaaaaagctgatgagcaacaacgtgcagatcgtgcggcagcagagctacagcatcatgagcatttgcaaagaagaggtgctggcctacgtggtgcagctgcctctgtatggcgtgatcgataccccttgctggaagctgcacacaagccctctgtgcaccaccaacaccaaagagggcagcaacatctgcctgaccagaaccgacagaggctggtactgcgataatgccggcagcgtctcattcttcccacaagccgagacatgcaaggtgcagagcaaccgggtgttctgcgacaccatgaatagcagaaccctgccttccgaagtgaatctgtgcaacgtggacatcttcaaccctaagtacgactgcaagatcatgaccagcaagaccgacgtgtccagcagtgtgatcacctcactgggcgccatcgtgtcctgttacggcaagaccaagtgcaccgccagcaacaagaaccggggcatcatcaagaccttcagcaacggctgcgactacgtgtccaacaaaggcgtggacaccgtgtctgtgggcaacaccctgtactacgtgaacaaacaagagggccagtctctgtacgtgaagggcgagcccatcatcaacttctacgaccctctggtgttccccagcgacgagttcgatgccagcatcagccaagtgaacgagaagatcaatcagagcctggccttcatcagaaagtccgatgagctgctgcacaacgtgaacgccggcaagtccaccaccaatatcatgatcacgaccatcatcatcgtgattatcgtgatcctgctgtccctgatcgccgtgggcctgctgctttattgataatag

SEQ ID NO: 180 - protein, 510 aa, synthetic construct
MELLILKANAITTILTAVTFCFASGQNITEEFYQSTCSAVSKGYLGALRTGWYTSVITIELSNIKENKCNGTDAKVKLIKQELDKYKNAVTDLQLLMQSTPATGSGSCIASGVAVSKVLHLEGEVNKIKSALLSTNKAVVSLSNGVSVLTFKVLDLKNYIDKQLLPILNKQSCSIPNIETVIEFQQKNNRLLEITREFSVNAGVTTPVSTYMLTNSELLSLINDMPITNDQKKLMSNNVQIVRQQSYSIMSICKEEVLAYVVQLPLYGVIDTPCWKLHTSPLCTTNTKEGSNICLTRTDRGWYCDNAGSVSFFPQAETCKVQSNRVFCDTMNSRTLPSEVNLCNVDIFNPKYDCKIMTSKTDVSSSVITSLGAIVSCYGKTKCTASNKNRGIIKTFSNGCDYVSNKGVDTVSVGNTLYYVNKQEGQSLYVKGEPIINFYDPLVFPSDEFDASISQVNEKINQSLAFIRKSDELLHNVNAGKSTTNIMITTIIIVIIVILLSLIAVGLLLY

SEQ ID NO: 181 - RNA, 1841 nt, synthetic construct
  source 1..1841: mol_type = other RNA
agcggctcggccattttgtcccagtcagtccggaggctgcggctgcagaagtaccgcctgcggagtaactgcaaaggccaccatggaactgctgatcctgaaggccaacgccatcaccaccatcctgaccgccgtgaccttctgttttgccagcggccagaacatcaccgaggaattctaccagagcacctgtagcgccgtgtccaagggatatctgggcgcccttagaaccggctggtacaccagcgtgatcaccatcgagctgagcaacatcaaagaaaacaagtgcaacggcaccgacgccaaagtgaagctgatcaagcaagagctggacaagtacaagaatgccgtgaccgacctgcagctgctgatgcagtctacaccagccacaggctctggcagctgcattgcctctggtgtcgccgtgtctaaagtgctgcacctggaaggcgaagtgaacaagatcaagagcgccctgctgagcaccaacaaggccgtggtgtctctgagcaatggcgtgtccgtgctgaccttcaaggtgctggacctgaagaactacatcgacaaacagctgctgcccatcctgaacaagcagtcctgcagcatccccaacatcgagacagtgatcgagttccagcagaagaacaaccggctgctggaaatcacccgcgagttctctgtgaatgccggcgtgaccacacctgtgtccacctacatgctgaccaacagcgagctgctgagcctgatcaacgacatgcccatcaccaacgaccagaaaaagctgatgagcaacaacgtgcagatcgtgcggcagcagagctacagcatcatgagcatttgcaaagaagaggtgctggcctacgtggtgcagctgcctctgtatggcgtgatcgataccccttgctggaagctgcacacaagccctctgtgcaccaccaacaccaaagagggcagcaacatctgcctgaccagaaccgacagaggctggtactgcgataatgccggcagcgtctcattcttcccacaagccgagacatgcaaggtgcagagcaaccgggtgttctgcgacaccatgaatagcagaaccctgccttccgaagtgaatctgtgcaacgtggacatcttcaaccctaagtacgactgcaagatcatgaccagcaagaccgacgtgtccagcagtgtgatcacctcactgggcgccatcgtgtcctgttacggcaagaccaagtgcaccgccagcaacaagaaccggggcatcatcaagaccttcagcaacggctgcgactacgtgtccaacaaaggcgtggacaccgtgtctgtgggcaacaccctgtactacgtgaacaaacaagagggccagtctctgtacgtgaagggcgagcccatcatcaacttctacgaccctctggtgttccccagcgacgagttcgatgccagcatcagccaagtgaacgagaagatcaatcagagcctggccttcatcagaaagtccgatgagctgctgcacaacgtgaacgccggcaagtccaccaccaatatcatgatcacgaccatcatcatcgtgattatcgtgatcctgctgtccctgatcgccgtgggcctgctgctttattgataataggctggagcctcggtggccatgcttcttgccccttgggcctccccccagcccctcctccccttcctgcacccgtacccccgtggtctttgaataaagtctgagtgggcggcaaaaaaaaaaaaaaaaaaaaaaaaaaaaaaaaaaaaaaaaaaaaaaaaaaaaaaaaaaaaaaaaaaaaaaaaaaaaaaaaaaaaaaaaaaaaaaaaaaaaaaaaaaaaaa

SEQ ID NO: 182 - DNA, 1841 bp, synthetic construct
  source 1..1841: mol_type = other DNA
agcggctcggccattttgtcccagtcagtccggaggctgcggctgcagaagtaccgcctgcggagtaactgcaaaggccaccatggaactgctgatcctgaaggccaacgccatcaccaccatcctgaccgccgtgaccttctgttttgccagcggccagaacatcaccgaggaattctaccagagcacctgtagcgccgtgtccaagggatatctgggcgcccttagaaccggctggtacaccagcgtgatcaccatcgagctgagcaacatcaaagaaaacaagtgcaacggcaccgacgccaaagtgaagctgatcaagcaagagctggacaagtacaagaatgccgtgaccgacctgcagctgctgatgcagtctacaccagccacaggctctggcagctgcattgcctctggtgtcgccgtgtctaaagtgctgcacctggaaggcgaagtgaacaagatcaagagcgccctgctgagcaccaacaaggccgtggtgtctctgagcaatggcgtgtccgtgctgaccttcaaggtgctggacctgaagaactacatcgacaaacagctgctgcccatcctgaacaagcagtcctgcagcatccccaacatcgagacagtgatcgagttccagcagaagaacaaccggctgctggaaatcacccgcgagttctctgtgaatgccggcgtgaccacacctgtgtccacctacatgctgaccaacagcgagctgctgagcctgatcaacgacatgcccatcaccaacgaccagaaaaagctgatgagcaacaacgtgcagatcgtgcggcagcagagctactgcatcatgagcattatcaaagaagaggtgctggcctacgtggtgcagctgcctctgtatggcgtgatcgataccccttgctggaagctgcacacaagccctctgtgcaccaccaacaccaaagagggcagcaacatctgcctgaccagaaccgacagaggctggtactgcgataatgccggcagcgtctcattcttcccacaagccgagacatgcaaggtgcagagcaaccgggtgttctgcgacaccatgaatagcagaaccctgccttccgaagtgaatctgtgcaacgtggacatcttcaaccctaagtacgactgcaagatcatgaccagcaagaccgacgtgtccagcagtgtgatcacctcactgggcgccatcgtgtcctgttacggcaagaccaagtgcaccgccagcaacaagaaccggggcatcatcaagaccttcagcaacggctgcgactacgtgtccaacaaaggcgtggacaccgtgtctgtgggcaacaccctgtactacgtgaacaaacaagagggccagtctctgtacgtgaagggcgagcccatcatcaacttctacgaccctctggtgttccccagcgacgagttcgatgccagcatcagccaagtgaacgagaagatcaatcagagcctggccttcatcagaaagtccgatgagctgctgcacaacgtgaacgccggcaagtccaccaccaatatcatgatcacgaccatcatcatcgtgattatcgtgatcctgctgtccctgatcgccgtgggcctgctgctttattgataataggctggagcctcggtggccatgcttcttgccccttgggcctccccccagcccctcctccccttcctgcacccgtacccccgtggtctttgaataaagtctgagtgggcggcaaaaaaaaaaaaaaaaaaaaaaaaaaaaaaaaaaaaaaaaaaaaaaaaaaaaaaaaaaaaaaaaaaaaaaaaaaaaaaaaaaaaaaaaaaaaaaaaaaaaaaaaaaaaaa

SEQ ID NO: 183 - DNA, 1539 bp, synthetic construct
  source 1..1539: mol_type = other DNA
atggaactgctgatcctgaaggccaacgccatcaccaccatcctgaccgccgtgaccttctgttttgccagcggccagaacatcaccgaggaattctaccagagcacctgtagcgccgtgtccaagggatatctgggcgcccttagaaccggctggtacaccagcgtgatcaccatcgagctgagcaacatcaaagaaaacaagtgcaacggcaccgacgccaaagtgaagctgatcaagcaagagctggacaagtacaagaatgccgtgaccgacctgcagctgctgatgcagtctacaccagccacaggctctggcagctgcattgcctctggtgtcgccgtgtctaaagtgctgcacctggaaggcgaagtgaacaagatcaagagcgccctgctgagcaccaacaaggccgtggtgtctctgagcaatggcgtgtccgtgctgaccttcaaggtgctggacctgaagaactacatcgacaaacagctgctgcccatcctgaacaagcagtcctgcagcatccccaacatcgagacagtgatcgagttccagcagaagaacaaccggctgctggaaatcacccgcgagttctctgtgaatgccggcgtgaccacacctgtgtccacctacatgctgaccaacagcgagctgctgagcctgatcaacgacatgcccatcaccaacgaccagaaaaagctgatgagcaacaacgtgcagatcgtgcggcagcagagctactgcatcatgagcattatcaaagaagaggtgctggcctacgtggtgcagctgcctctgtatggcgtgatcgataccccttgctggaagctgcacacaagccctctgtgcaccaccaacaccaaagagggcagcaacatctgcctgaccagaaccgacagaggctggtactgcgataatgccggcagcgtctcattcttcccacaagccgagacatgcaaggtgcagagcaaccgggtgttctgcgacaccatgaatagcagaaccctgccttccgaagtgaatctgtgcaacgtggacatcttcaaccctaagtacgactgcaagatcatgaccagcaagaccgacgtgtccagcagtgtgatcacctcactgggcgccatcgtgtcctgttacggcaagaccaagtgcaccgccagcaacaagaaccggggcatcatcaagaccttcagcaacggctgcgactacgtgtccaacaaaggcgtggacaccgtgtctgtgggcaacaccctgtactacgtgaacaaacaagagggccagtctctgtacgtgaagggcgagcccatcatcaacttctacgaccctctggtgttccccagcgacgagttcgatgccagcatcagccaagtgaacgagaagatcaatcagagcctggccttcatcagaaagtccgatgagctgctgcacaacgtgaacgccggcaagtccaccaccaatatcatgatcacgaccatcatcatcgtgattatcgtgatcctgctgtccctgatcgccgtgggcctgctgctttattgataatag

SEQ ID NO: 184 - protein, 510 aa, synthetic construct
MELLILKANAITTILTAVTFCFASGQNITEEFYQSTCSAVSKGYLGALRTGWYTSVITIELSNIKENKCNGTDAKVKLIKQELDKYKNAVTDLQLLMQSTPATGSGSCIASGVAVSKVLHLEGEVNKIKSALLSTNKAVVSLSNGVSVLTFKVLDLKNYIDKQLLPILNKQSCSIPNIETVIEFQQKNNRLLEITREFSVNAGVTTPVSTYMLTNSELLSLINDMPITNDQKKLMSNNVQIVRQQSYCIMSIIKEEVLAYVVQLPLYGVIDTPCWKLHTSPLCTTNTKEGSNICLTRTDRGWYCDNAGSVSFFPQAETCKVQSNRVFCDTMNSRTLPSEVNLCNVDIFNPKYDCKIMTSKTDVSSSVITSLGAIVSCYGKTKCTASNKNRGIIKTFSNGCDYVSNKGVDTVSVGNTLYYVNKQEGQSLYVKGEPIINFYDPLVFPSDEFDASISQVNEKINQSLAFIRKSDELLHNVNAGKSTTNIMITTIIIVIIVILLSLIAVGLLLY

SEQ ID NO: 185 - RNA, 1841 nt, synthetic construct
  source 1..1841: mol_type = other RNA
agcggctcggccattttgtcccagtcagtccggaggctgcggctgcagaagtaccgcctgcggagtaactgcaaaggccaccatggaactgctgatcctgaaggccaacgccatcaccaccatcctgaccgccgtgaccttctgttttgccagcggccagaacatcaccgaggaattctaccagagcacctgtagcgccgtgtccaagggatatctgggcgcccttagaaccggctggtacaccagcgtgatcaccatcgagctgagcaacatcaaagaaaacaagtgcaacggcaccgacgccaaagtgaagctgatcaagcaagagctggacaagtacaagaatgccgtgaccgacctgcagctgctgatgcagtctacaccagccacaggctctggcagctgcattgcctctggtgtcgccgtgtctaaagtgctgcacctggaaggcgaagtgaacaagatcaagagcgccctgctgagcaccaacaaggccgtggtgtctctgagcaatggcgtgtccgtgctgaccttcaaggtgctggacctgaagaactacatcgacaaacagctgctgcccatcctgaacaagcagtcctgcagcatccccaacatcgagacagtgatcgagttccagcagaagaacaaccggctgctggaaatcacccgcgagttctctgtgaatgccggcgtgaccacacctgtgtccacctacatgctgaccaacagcgagctgctgagcctgatcaacgacatgcccatcaccaacgaccagaaaaagctgatgagcaacaacgtgcagatcgtgcggcagcagagctactgcatcatgagcattatcaaagaagaggtgctggcctacgtggtgcagctgcctctgtatggcgtgatcgataccccttgctggaagctgcacacaagccctctgtgcaccaccaacaccaaagagggcagcaacatctgcctgaccagaaccgacagaggctggtactgcgataatgccggcagcgtctcattcttcccacaagccgagacatgcaaggtgcagagcaaccgggtgttctgcgacaccatgaatagcagaaccctgccttccgaagtgaatctgtgcaacgtggacatcttcaaccctaagtacgactgcaagatcatgaccagcaagaccgacgtgtccagcagtgtgatcacctcactgggcgccatcgtgtcctgttacggcaagaccaagtgcaccgccagcaacaagaaccggggcatcatcaagaccttcagcaacggctgcgactacgtgtccaacaaaggcgtggacaccgtgtctgtgggcaacaccctgtactacgtgaacaaacaagagggccagtctctgtacgtgaagggcgagcccatcatcaacttctacgaccctctggtgttccccagcgacgagttcgatgccagcatcagccaagtgaacgagaagatcaatcagagcctggccttcatcagaaagtccgatgagctgctgcacaacgtgaacgccggcaagtccaccaccaatatcatgatcacgaccatcatcatcgtgattatcgtgatcctgctgtccctgatcgccgtgggcctgctgctttattgataataggctggagcctcggtggccatgcttcttgccccttgggcctccccccagcccctcctccccttcctgcacccgtacccccgtggtctttgaataaagtctgagtgggcggcaaaaaaaaaaaaaaaaaaaaaaaaaaaaaaaaaaaaaaaaaaaaaaaaaaaaaaaaaaaaaaaaaaaaaaaaaaaaaaaaaaaaaaaaaaaaaaaaaaaaaaaaaaaaaa

SEQ ID NO: 186 - DNA, 1841 bp, synthetic construct
  source 1..1841: mol_type = other DNA
agcggctcggccattttgtcccagtcagtccggaggctgcggctgcagaagtaccgcctgcggagtaactgcaaaggccaccatggaactgctgatcctgaaggccaacgccatcaccaccatcctgaccgccgtgaccttctgttttgccagcggccagaacatcaccgaggaattctaccagagcacctgtagcgccgtgtccaagggatatctgggcgcccttagaaccggctggtacaccagcgtgatcaccatcgagctgagcaacatcaaagaaaacaagtgcaacggcaccgacgccaaagtgaagctgatcaagcaagagctggacaagtacaagaatgccgtgaccgacctgcagctgctgatgcagtctacaccagccacaggctctggcagctgcattgcctctggtgtcgccgtgtctaaagtgctgcacctggaaggcgaagtgaacaagatcaagagcgccctgctgagcaccaacaaggccgtggtgtctctgagcaatggcgtgtccgtgctgaccttcaaggtgctggacctgaagaactacatcgacaaacagctgctgcccatcctgaacaagcagtcctgcagcatccccaacatcgagacagtgatcgagttccagcagaagaacaaccggctgctggaaatcacccgcgagttctctgtgaatgccggcgtgaccacacctgtgtccacctacatgctgaccaacagcgagctgctgagcctgatcaacgacatgcccatcaccaacgaccagaaaaagctgatgagcaacaacgtgcagatcgtgcggcagcagagctacagcatcatgagctgcatcaaagaagaggtgctggcctacgtggtgcagctgcctctgtatggcgtgatcgataccccttgctggaagctgcacacaagccctctgtgcaccaccaacaccaaagagggcagcaacatctgcctgaccagaaccgacagaggctggtactgcgataatgccggcagcgtctcattcttcccacaagccgagacatgcaaggtgcagagcaaccgggtgttctgcgacaccatgaatagcagaaccctgccttccgaagtgaatctgtgcaacgtggacatcttcaaccctaagtacgactgcaagatcatgaccagcaagaccgacgtgtccagcagtgtgatcacctcactgggcgccatcgtgtcctgttacggcaagaccaagtgcaccgccagcaacaagaaccggggcatcatcaagaccttcagcaacggctgcgactacgtgtccaacaaaggcgtggacaccgtgtctgtgggcaacaccctgtactacgtgaacaaacaagagggccagtctctgtacgtgaagggcgagcccatcatcaacttctacgaccctctggtgttccccagcgacgagttcgatgccagcatcagccaagtgaacgagaagatcaatcagagcctggccttcatcagaaagtccgatgagctgctgcacaacgtgaacgccggcaagtccaccaccaatatcatgatcacgaccatcatcatcgtgattatcgtgatcctgctgtccctgatcgccgtgggcctgctgctttattgataataggctggagcctcggtggccatgcttcttgccccttgggcctccccccagcccctcctccccttcctgcacccgtacccccgtggtctttgaataaagtctgagtgggcggcaaaaaaaaaaaaaaaaaaaaaaaaaaaaaaaaaaaaaaaaaaaaaaaaaaaaaaaaaaaaaaaaaaaaaaaaaaaaaaaaaaaaaaaaaaaaaaaaaaaaaaaaaaaaaa

SEQ ID NO: 187 - DNA, 1539 bp, synthetic construct
  source 1..1539: mol_type = other DNA
atggaactgctgatcctgaaggccaacgccatcaccaccatcctgaccgccgtgaccttctgttttgccagcggccagaacatcaccgaggaattctaccagagcacctgtagcgccgtgtccaagggatatctgggcgcccttagaaccggctggtacaccagcgtgatcaccatcgagctgagcaacatcaaagaaaacaagtgcaacggcaccgacgccaaagtgaagctgatcaagcaagagctggacaagtacaagaatgccgtgaccgacctgcagctgctgatgcagtctacaccagccacaggctctggcagctgcattgcctctggtgtcgccgtgtctaaagtgctgcacctggaaggcgaagtgaacaagatcaagagcgccctgctgagcaccaacaaggccgtggtgtctctgagcaatggcgtgtccgtgctgaccttcaaggtgctggacctgaagaactacatcgacaaacagctgctgcccatcctgaacaagcagtcctgcagcatccccaacatcgagacagtgatcgagttccagcagaagaacaaccggctgctggaaatcacccgcgagttctctgtgaatgccggcgtgaccacacctgtgtccacctacatgctgaccaacagcgagctgctgagcctgatcaacgacatgcccatcaccaacgaccagaaaaagctgatgagcaacaacgtgcagatcgtgcggcagcagagctacagcatcatgagctgcatcaaagaagaggtgctggcctacgtggtgcagctgcctctgtatggcgtgatcgataccccttgctggaagctgcacacaagccctctgtgcaccaccaacaccaaagagggcagcaacatctgcctgaccagaaccgacagaggctggtactgcgataatgccggcagcgtctcattcttcccacaagccgagacatgcaaggtgcagagcaaccgggtgttctgcgacaccatgaatagcagaaccctgccttccgaagtgaatctgtgcaacgtggacatcttcaaccctaagtacgactgcaagatcatgaccagcaagaccgacgtgtccagcagtgtgatcacctcactgggcgccatcgtgtcctgttacggcaagaccaagtgcaccgccagcaacaagaaccggggcatcatcaagaccttcagcaacggctgcgactacgtgtccaacaaaggcgtggacaccgtgtctgtgggcaacaccctgtactacgtgaacaaacaagagggccagtctctgtacgtgaagggcgagcccatcatcaacttctacgaccctctggtgttccccagcgacgagttcgatgccagcatcagccaagtgaacgagaagatcaatcagagcctggccttcatcagaaagtccgatgagctgctgcacaacgtgaacgccggcaagtccaccaccaatatcatgatcacgaccatcatcatcgtgattatcgtgatcctgctgtccctgatcgccgtgggcctgctgctttattgataatag

SEQ ID NO: 188 - protein, 510 aa, synthetic construct
MELLILKANAITTILTAVTFCFASGQNITEEFYQSTCSAVSKGYLGALRTGWYTSVITIELSNIKENKCNGTDAKVKLIKQELDKYKNAVTDLQLLMQSTPATGSGSCIASGVAVSKVLHLEGEVNKIKSALLSTNKAVVSLSNGVSVLTFKVLDLKNYIDKQLLPILNKQSCSIPNIETVIEFQQKNNRLLEITREFSVNAGVTTPVSTYMLTNSELLSLINDMPITNDQKKLMSNNVQIVRQQSYSIMSCIKEEVLAYVVQLPLYGVIDTPCWKLHTSPLCTTNTKEGSNICLTRTDRGWYCDNAGSVSFFPQAETCKVQSNRVFCDTMNSRTLPSEVNLCNVDIFNPKYDCKIMTSKTDVSSSVITSLGAIVSCYGKTKCTASNKNRGIIKTFSNGCDYVSNKGVDTVSVGNTLYYVNKQEGQSLYVKGEPIINFYDPLVFPSDEFDASISQVNEKINQSLAFIRKSDELLHNVNAGKSTTNIMITTIIIVIIVILLSLIAVGLLLY

SEQ ID NO: 189 - RNA, 1841 nt, synthetic construct
  source 1..1841: mol_type = other RNA
agcggctcggccattttgtcccagtcagtccggaggctgcggctgcagaagtaccgcctgcggagtaactgcaaaggccaccatggaactgctgatcctgaaggccaacgccatcaccaccatcctgaccgccgtgaccttctgttttgccagcggccagaacatcaccgaggaattctaccagagcacctgtagcgccgtgtccaagggatatctgggcgcccttagaaccggctggtacaccagcgtgatcaccatcgagctgagcaacatcaaagaaaacaagtgcaacggcaccgacgccaaagtgaagctgatcaagcaagagctggacaagtacaagaatgccgtgaccgacctgcagctgctgatgcagtctacaccagccacaggctctggcagctgcattgcctctggtgtcgccgtgtctaaagtgctgcacctggaaggcgaagtgaacaagatcaagagcgccctgctgagcaccaacaaggccgtggtgtctctgagcaatggcgtgtccgtgctgaccttcaaggtgctggacctgaagaactacatcgacaaacagctgctgcccatcctgaacaagcagtcctgcagcatccccaacatcgagacagtgatcgagttccagcagaagaacaaccggctgctggaaatcacccgcgagttctctgtgaatgccggcgtgaccacacctgtgtccacctacatgctgaccaacagcgagctgctgagcctgatcaacgacatgcccatcaccaacgaccagaaaaagctgatgagcaacaacgtgcagatcgtgcggcagcagagctacagcatcatgagctgcatcaaagaagaggtgctggcctacgtggtgcagctgcctctgtatggcgtgatcgataccccttgctggaagctgcacacaagccctctgtgcaccaccaacaccaaagagggcagcaacatctgcctgaccagaaccgacagaggctggtactgcgataatgccggcagcgtctcattcttcccacaagccgagacatgcaaggtgcagagcaaccgggtgttctgcgacaccatgaatagcagaaccctgccttccgaagtgaatctgtgcaacgtggacatcttcaaccctaagtacgactgcaagatcatgaccagcaagaccgacgtgtccagcagtgtgatcacctcactgggcgccatcgtgtcctgttacggcaagaccaagtgcaccgccagcaacaagaaccggggcatcatcaagaccttcagcaacggctgcgactacgtgtccaacaaaggcgtggacaccgtgtctgtgggcaacaccctgtactacgtgaacaaacaagagggccagtctctgtacgtgaagggcgagcccatcatcaacttctacgaccctctggtgttccccagcgacgagttcgatgccagcatcagccaagtgaacgagaagatcaatcagagcctggccttcatcagaaagtccgatgagctgctgcacaacgtgaacgccggcaagtccaccaccaatatcatgatcacgaccatcatcatcgtgattatcgtgatcctgctgtccctgatcgccgtgggcctgctgctttattgataataggctggagcctcggtggccatgcttcttgccccttgggcctccccccagcccctcctccccttcctgcacccgtacccccgtggtctttgaataaagtctgagtgggcggcaaaaaaaaaaaaaaaaaaaaaaaaaaaaaaaaaaaaaaaaaaaaaaaaaaaaaaaaaaaaaaaaaaaaaaaaaaaaaaaaaaaaaaaaaaaaaaaaaaaaaaaaaaaaaa

SEQ ID NO: 190 - DNA, 1841 bp, synthetic construct
  source 1..1841: mol_type = other DNA
agcggctcggccattttgtcccagtcagtccggaggctgcggctgcagaagtaccgcctgcggagtaactgcaaaggccaccatggaactgctgatcctgaaggccaacgccatcaccaccatcctgaccgccgtgaccttctgttttgccagcggccagaacatcaccgaggaattctaccagagcacctgtagcgccgtgtccaagggatatctgggcgcccttagaaccggctggtacaccagcgtgatcaccatcgagctgagcaacatcaaagaaaacaagtgcaacggcaccgacgccaaagtgaagctgatcaagcaagagctggacaagtacaagaatgccgtgaccgacctgcagctgctgatgcagtctacaccagccacaggctctggcagcgccattgcctctggtgtcgccgtgtctaaagtgctgcacctggaaggcgaagtgaacaagatcaagagcgccctgctgagcaccaacaaggccgtggtgtctctgagcaatggcgtgtccgtgctgaccttcaaggtgctggacctgaagaactacatcgacaaacagctgctgcccatcctgaacaagcagtcctgcagcatccccaacatcgagacagtgatcgagttccagcagaagaacaaccggctgctggaaatcacccgcgagttctctgtgaatgccggcgtgaccacacctgtgtccacctacatgctgaccaacagcgagctgctgagcctgatcaacgacatgcccatcaccaacgaccagaaaaagctgatgagcaacaacgtgcagatcgtgcggcagcagagctacagcatcatgagcattatcaaagaagaggtgctggcctacgtggtgcagctgcctctgtatggcgtgatcgataccccttgctggaagctgcacacaagccctctgtgcaccaccaacaccaaagagggctgcaacatctgcctgaccagaaccgacagaggctggtactgcgataatgccggcagcgtctcattcttcccacaagccgagacatgcaaggtgcagagcaaccgggtgttctgcgacaccatgaatagcagaaccctgccttccgaagtgaatctgtgcaacgtggacatcttcaaccctaagtacgactgcaagatcatgaccagcaagaccgacgtgtccagcagtgtgatcacctcactgggcgccatcgtgtcctgttacggcaagaccaagtgcaccgccagcaacaagaaccggggcatcatcaagaccttcagcaacggctgcgactacgtgtccaacaaaggcgtggacaccgtgtctgtgggcaacaccctgtactacgtgaacaaacaagagggccagtctctgtacgtgaagtgcgagcccatcatcaacttctacgaccctctggtgttccccagcgacgagttcgatgccagcatcagccaagtgaacgagaagatcaatcagagcctggccttcatcagaaagtccgatgagctgctgcacaacgtgaacgccggcaagtccaccaccaatatcatgatcacgaccatcatcatcgtgattatcgtgatcctgctgtccctgatcgccgtgggcctgctgctttattgataataggctggagcctcggtggccatgcttcttgccccttgggcctccccccagcccctcctccccttcctgcacccgtacccccgtggtctttgaataaagtctgagtgggcggcaaaaaaaaaaaaaaaaaaaaaaaaaaaaaaaaaaaaaaaaaaaaaaaaaaaaaaaaaaaaaaaaaaaaaaaaaaaaaaaaaaaaaaaaaaaaaaaaaaaaaaaaaaaaaa

SEQ ID NO: 191 - DNA, 1539 bp, synthetic construct
  source 1..1539: mol_type = other DNA
atggaactgctgatcctgaaggccaacgccatcaccaccatcctgaccgccgtgaccttctgttttgccagcggccagaacatcaccgaggaattctaccagagcacctgtagcgccgtgtccaagggatatctgggcgcccttagaaccggctggtacaccagcgtgatcaccatcgagctgagcaacatcaaagaaaacaagtgcaacggcaccgacgccaaagtgaagctgatcaagcaagagctggacaagtacaagaatgccgtgaccgacctgcagctgctgatgcagtctacaccagccacaggctctggcagcgccattgcctctggtgtcgccgtgtctaaagtgctgcacctggaaggcgaagtgaacaagatcaagagcgccctgctgagcaccaacaaggccgtggtgtctctgagcaatggcgtgtccgtgctgaccttcaaggtgctggacctgaagaactacatcgacaaacagctgctgcccatcctgaacaagcagtcctgcagcatccccaacatcgagacagtgatcgagttccagcagaagaacaaccggctgctggaaatcacccgcgagttctctgtgaatgccggcgtgaccacacctgtgtccacctacatgctgaccaacagcgagctgctgagcctgatcaacgacatgcccatcaccaacgaccagaaaaagctgatgagcaacaacgtgcagatcgtgcggcagcagagctacagcatcatgagcattatcaaagaagaggtgctggcctacgtggtgcagctgcctctgtatggcgtgatcgataccccttgctggaagctgcacacaagccctctgtgcaccaccaacaccaaagagggctgcaacatctgcctgaccagaaccgacagaggctggtactgcgataatgccggcagcgtctcattcttcccacaagccgagacatgcaaggtgcagagcaaccgggtgttctgcgacaccatgaatagcagaaccctgccttccgaagtgaatctgtgcaacgtggacatcttcaaccctaagtacgactgcaagatcatgaccagcaagaccgacgtgtccagcagtgtgatcacctcactgggcgccatcgtgtcctgttacggcaagaccaagtgcaccgccagcaacaagaaccggggcatcatcaagaccttcagcaacggctgcgactacgtgtccaacaaaggcgtggacaccgtgtctgtgggcaacaccctgtactacgtgaacaaacaagagggccagtctctgtacgtgaagtgcgagcccatcatcaacttctacgaccctctggtgttccccagcgacgagttcgatgccagcatcagccaagtgaacgagaagatcaatcagagcctggccttcatcagaaagtccgatgagctgctgcacaacgtgaacgccggcaagtccaccaccaatatcatgatcacgaccatcatcatcgtgattatcgtgatcctgctgtccctgatcgccgtgggcctgctgctttattgataatag

SEQ ID NO: 192 - protein, 510 aa, synthetic construct
MELLILKANAITTILTAVTFCFASGQNITEEFYQSTCSAVSKGYLGALRTGWYTSVITIELSNIKENKCNGTDAKVKLIKQELDKYKNAVTDLQLLMQSTPATGSGSAIASGVAVSKVLHLEGEVNKIKSALLSTNKAVVSLSNGVSVLTFKVLDLKNYIDKQLLPILNKQSCSIPNIETVIEFQQKNNRLLEITREFSVNAGVTTPVSTYMLTNSELLSLINDMPITNDQKKLMSNNVQIVRQQSYSIMSIIKEEVLAYVVQLPLYGVIDTPCWKLHTSPLCTTNTKEGCNICLTRTDRGWYCDNAGSVSFFPQAETCKVQSNRVFCDTMNSRTLPSEVNLCNVDIFNPKYDCKIMTSKTDVSSSVITSLGAIVSCYGKTKCTASNKNRGIIKTFSNGCDYVSNKGVDTVSVGNTLYYVNKQEGQSLYVKCEPIINFYDPLVFPSDEFDASISQVNEKINQSLAFIRKSDELLHNVNAGKSTTNIMITTIIIVIIVILLSLIAVGLLLY

SEQ ID NO: 193 - RNA, 1841 nt, synthetic construct
  source 1..1841: mol_type = other RNA
agcggctcggccattttgtcccagtcagtccggaggctgcggctgcagaagtaccgcctgcggagtaactgcaaaggccaccatggaactgctgatcctgaaggccaacgccatcaccaccatcctgaccgccgtgaccttctgttttgccagcggccagaacatcaccgaggaattctaccagagcacctgtagcgccgtgtccaagggatatctgggcgcccttagaaccggctggtacaccagcgtgatcaccatcgagctgagcaacatcaaagaaaacaagtgcaacggcaccgacgccaaagtgaagctgatcaagcaagagctggacaagtacaagaatgccgtgaccgacctgcagctgctgatgcagtctacaccagccacaggctctggcagcgccattgcctctggtgtcgccgtgtctaaagtgctgcacctggaaggcgaagtgaacaagatcaagagcgccctgctgagcaccaacaaggccgtggtgtctctgagcaatggcgtgtccgtgctgaccttcaaggtgctggacctgaagaactacatcgacaaacagctgctgcccatcctgaacaagcagtcctgcagcatccccaacatcgagacagtgatcgagttccagcagaagaacaaccggctgctggaaatcacccgcgagttctctgtgaatgccggcgtgaccacacctgtgtccacctacatgctgaccaacagcgagctgctgagcctgatcaacgacatgcccatcaccaacgaccagaaaaagctgatgagcaacaacgtgcagatcgtgcggcagcagagctacagcatcatgagcattatcaaagaagaggtgctggcctacgtggtgcagctgcctctgtatggcgtgatcgataccccttgctggaagctgcacacaagccctctgtgcaccaccaacaccaaagagggctgcaacatctgcctgaccagaaccgacagaggctggtactgcgataatgccggcagcgtctcattcttcccacaagccgagacatgcaaggtgcagagcaaccgggtgttctgcgacaccatgaatagcagaaccctgccttccgaagtgaatctgtgcaacgtggacatcttcaaccctaagtacgactgcaagatcatgaccagcaagaccgacgtgtccagcagtgtgatcacctcactgggcgccatcgtgtcctgttacggcaagaccaagtgcaccgccagcaacaagaaccggggcatcatcaagaccttcagcaacggctgcgactacgtgtccaacaaaggcgtggacaccgtgtctgtgggcaacaccctgtactacgtgaacaaacaagagggccagtctctgtacgtgaagtgcgagcccatcatcaacttctacgaccctctggtgttccccagcgacgagttcgatgccagcatcagccaagtgaacgagaagatcaatcagagcctggccttcatcagaaagtccgatgagctgctgcacaacgtgaacgccggcaagtccaccaccaatatcatgatcacgaccatcatcatcgtgattatcgtgatcctgctgtccctgatcgccgtgggcctgctgctttattgataataggctggagcctcggtggccatgcttcttgccccttgggcctccccccagcccctcctccccttcctgcacccgtacccccgtggtctttgaataaagtctgagtgggcggcaaaaaaaaaaaaaaaaaaaaaaaaaaaaaaaaaaaaaaaaaaaaaaaaaaaaaaaaaaaaaaaaaaaaaaaaaaaaaaaaaaaaaaaaaaaaaaaaaaaaaaaaaaaaaa

SEQ ID NO: 194 - DNA, 1841 bp, synthetic construct
  source 1..1841: mol_type = other DNA
agcggctcggccattttgtcccagtcagtccggaggctgcggctgcagaagtaccgcctgcggagtaactgcaaaggccaccatggaactgctgatcctgaaggccaacgccatcaccaccatcctgaccgccgtgaccttctgttttgccagcggccagaacatcaccgaggaattctaccagagcacctgtagcgccgtgtccaagggatatctgggcgcccttagaaccggctggtacaccagcgtgatcaccatcgagctgagcaacatcaaagaaaacaagtgcaacggcaccgacgccaaagtgaagctgatcaagcaagagctggacaagtacaagaatgccgtgaccgacctgcagctgctgatgcagtctacaccagccacaggctctggcagcgccattgcctctggtgtcgccgtgtctaaagtgctgcacctggaaggcgaagtgaacaagatcaagagcgccctgctgagcaccaacaaggccgtggtgtctctgagcaatggcgtgtccgtgctgaccttcaaggtgctggacctgaagaactacatcgacaaacagctgctgcccatcctgaacaagcagtcctgcagcatccccaacatcgagacagtgatcgagttccagcagaagaacaaccggctgctggaaatcacccgcgagttctctgtgaatgccggcgtgaccacacctgtgtccacctacatgctgaccaacagcgagctgctgagcctgatcaacgacatgcccatcaccaacgaccagaaaaagctgatgagcaacaacgtgcagatcgtgcggcagcagagctacagcatcatgagcattatcaaagaagaggtgctggcctacgtggtgcagctgcctctgtatggcgtgatcgataccccttgctggaagctgcacacaagccctctgtgcaccacctgcaccaaagagggcagcaacatctgcctgaccagaaccgacagaggctggtactgcgataatgccggcagcgtctcattcttcccacaagccgagacatgcaaggtgcagagcaaccgggtgttctgcgacaccatgaatagcagaaccctgccttccgaagtgaatctgtgcaacgtggacatcttcaaccctaagtacgactgcaagatcatgaccagcaagaccgacgtgtccagcagtgtgatcacctcactgggcgccatcgtgtcctgttacggcaagaccaagtgcaccgccagcaacaagaaccggggcatcatcaagaccttcagcaacggctgcgactacgtgtccaacaaaggcgtggacaccgtgtctgtgggcaacaccctgtactacgtgaacaaacaagagggccagtctctgtacgtgaagtgcgagcccatcatcaacttctacgaccctctggtgttccccagcgacgagttcgatgccagcatcagccaagtgaacgagaagatcaatcagagcctggccttcatcagaaagtccgatgagctgctgcacaacgtgaacgccggcaagtccaccaccaatatcatgatcacgaccatcatcatcgtgattatcgtgatcctgctgtccctgatcgccgtgggcctgctgctttattgataataggctggagcctcggtggccatgcttcttgccccttgggcctccccccagcccctcctccccttcctgcacccgtacccccgtggtctttgaataaagtctgagtgggcggcaaaaaaaaaaaaaaaaaaaaaaaaaaaaaaaaaaaaaaaaaaaaaaaaaaaaaaaaaaaaaaaaaaaaaaaaaaaaaaaaaaaaaaaaaaaaaaaaaaaaaaaaaaaaaa

SEQ ID NO: 195 - DNA, 1539 bp, synthetic construct
  source 1..1539: mol_type = other DNA
atggaactgctgatcctgaaggccaacgccatcaccaccatcctgaccgccgtgaccttctgttttgccagcggccagaacatcaccgaggaattctaccagagcacctgtagcgccgtgtccaagggatatctgggcgcccttagaaccggctggtacaccagcgtgatcaccatcgagctgagcaacatcaaagaaaacaagtgcaacggcaccgacgccaaagtgaagctgatcaagcaagagctggacaagtacaagaatgccgtgaccgacctgcagctgctgatgcagtctacaccagccacaggctctggcagcgccattgcctctggtgtcgccgtgtctaaagtgctgcacctggaaggcgaagtgaacaagatcaagagcgccctgctgagcaccaacaaggccgtggtgtctctgagcaatggcgtgtccgtgctgaccttcaaggtgctggacctgaagaactacatcgacaaacagctgctgcccatcctgaacaagcagtcctgcagcatccccaacatcgagacagtgatcgagttccagcagaagaacaaccggctgctggaaatcacccgcgagttctctgtgaatgccggcgtgaccacacctgtgtccacctacatgctgaccaacagcgagctgctgagcctgatcaacgacatgcccatcaccaacgaccagaaaaagctgatgagcaacaacgtgcagatcgtgcggcagcagagctacagcatcatgagcattatcaaagaagaggtgctggcctacgtggtgcagctgcctctgtatggcgtgatcgataccccttgctggaagctgcacacaagccctctgtgcaccacctgcaccaaagagggcagcaacatctgcctgaccagaaccgacagaggctggtactgcgataatgccggcagcgtctcattcttcccacaagccgagacatgcaaggtgcagagcaaccgggtgttctgcgacaccatgaatagcagaaccctgccttccgaagtgaatctgtgcaacgtggacatcttcaaccctaagtacgactgcaagatcatgaccagcaagaccgacgtgtccagcagtgtgatcacctcactgggcgccatcgtgtcctgttacggcaagaccaagtgcaccgccagcaacaagaaccggggcatcatcaagaccttcagcaacggctgcgactacgtgtccaacaaaggcgtggacaccgtgtctgtgggcaacaccctgtactacgtgaacaaacaagagggccagtctctgtacgtgaagtgcgagcccatcatcaacttctacgaccctctggtgttccccagcgacgagttcgatgccagcatcagccaagtgaacgagaagatcaatcagagcctggccttcatcagaaagtccgatgagctgctgcacaacgtgaacgccggcaagtccaccaccaatatcatgatcacgaccatcatcatcgtgattatcgtgatcctgctgtccctgatcgccgtgggcctgctgctttattgataatag

SEQ ID NO: 196 - protein, 510 aa, synthetic construct
MELLILKANAITTILTAVTFCFASGQNITEEFYQSTCSAVSKGYLGALRTGWYTSVITIELSNIKENKCNGTDAKVKLIKQELDKYKNAVTDLQLLMQSTPATGSGSAIASGVAVSKVLHLEGEVNKIKSALLSTNKAVVSLSNGVSVLTFKVLDLKNYIDKQLLPILNKQSCSIPNIETVIEFQQKNNRLLEITREFSVNAGVTTPVSTYMLTNSELLSLINDMPITNDQKKLMSNNVQIVRQQSYSIMSIIKEEVLAYVVQLPLYGVIDTPCWKLHTSPLCTTCTKEGSNICLTRTDRGWYCDNAGSVSFFPQAETCKVQSNRVFCDTMNSRTLPSEVNLCNVDIFNPKYDCKIMTSKTDVSSSVITSLGAIVSCYGKTKCTASNKNRGIIKTFSNGCDYVSNKGVDTVSVGNTLYYVNKQEGQSLYVKCEPIINFYDPLVFPSDEFDASISQVNEKINQSLAFIRKSDELLHNVNAGKSTTNIMITTIIIVIIVILLSLIAVGLLLY

SEQ ID NO: 197 - RNA, 1841 nt, synthetic construct
  source 1..1841: mol_type = other RNA
agcggctcggccattttgtcccagtcagtccggaggctgcggctgcagaagtaccgcctgcggagtaactgcaaaggccaccatggaactgctgatcctgaaggccaacgccatcaccaccatcctgaccgccgtgaccttctgttttgccagcggccagaacatcaccgaggaattctaccagagcacctgtagcgccgtgtccaagggatatctgggcgcccttagaaccggctggtacaccagcgtgatcaccatcgagctgagcaacatcaaagaaaacaagtgcaacggcaccgacgccaaagtgaagctgatcaagcaagagctggacaagtacaagaatgccgtgaccgacctgcagctgctgatgcagtctacaccagccacaggctctggcagcgccattgcctctggtgtcgccgtgtctaaagtgctgcacctggaaggcgaagtgaacaagatcaagagcgccctgctgagcaccaacaaggccgtggtgtctctgagcaatggcgtgtccgtgctgaccttcaaggtgctggacctgaagaactacatcgacaaacagctgctgcccatcctgaacaagcagtcctgcagcatccccaacatcgagacagtgatcgagttccagcagaagaacaaccggctgctggaaatcacccgcgagttctctgtgaatgccggcgtgaccacacctgtgtccacctacatgctgaccaacagcgagctgctgagcctgatcaacgacatgcccatcaccaacgaccagaaaaagctgatgagcaacaacgtgcagatcgtgcggcagcagagctacagcatcatgagcattatcaaagaagaggtgctggcctacgtggtgcagctgcctctgtatggcgtgatcgataccccttgctggaagctgcacacaagccctctgtgcaccacctgcaccaaagagggcagcaacatctgcctgaccagaaccgacagaggctggtactgcgataatgccggcagcgtctcattcttcccacaagccgagacatgcaaggtgcagagcaaccgggtgttctgcgacaccatgaatagcagaaccctgccttccgaagtgaatctgtgcaacgtggacatcttcaaccctaagtacgactgcaagatcatgaccagcaagaccgacgtgtccagcagtgtgatcacctcactgggcgccatcgtgtcctgttacggcaagaccaagtgcaccgccagcaacaagaaccggggcatcatcaagaccttcagcaacggctgcgactacgtgtccaacaaaggcgtggacaccgtgtctgtgggcaacaccctgtactacgtgaacaaacaagagggccagtctctgtacgtgaagtgcgagcccatcatcaacttctacgaccctctggtgttccccagcgacgagttcgatgccagcatcagccaagtgaacgagaagatcaatcagagcctggccttcatcagaaagtccgatgagctgctgcacaacgtgaacgccggcaagtccaccaccaatatcatgatcacgaccatcatcatcgtgattatcgtgatcctgctgtccctgatcgccgtgggcctgctgctttattgataataggctggagcctcggtggccatgcttcttgccccttgggcctccccccagcccctcctccccttcctgcacccgtacccccgtggtctttgaataaagtctgagtgggcggcaaaaaaaaaaaaaaaaaaaaaaaaaaaaaaaaaaaaaaaaaaaaaaaaaaaaaaaaaaaaaaaaaaaaaaaaaaaaaaaaaaaaaaaaaaaaaaaaaaaaaaaaaaaaaa

SEQ ID NO: 198 - DNA, 1841 bp, synthetic construct
  source 1..1841: mol_type = other DNA
agcggctcggccattttgtcccagtcagtccggaggctgcggctgcagaagtaccgcctgcggagtaactgcaaaggccaccatggaactgctgatcctgaaggccaacgccatcaccaccatcctgaccgccgtgaccttctgttttgccagcggccagaacatcaccgaggaattctaccagagcacctgtagcgccgtgtccaagggatatctgggcgcccttagaaccggctggtacaccagcgtgatcaccatcgagctgagcaacatcaaagaaaacaagtgcaacggcaccgacgccaaagtgaagctgatcaagcaagagctggacaagtacaagaatgccgtgaccgacctgcagctgctgatgcagtctacaccagccacaggctctggcagcgccattgcctctggtgtcgccgtgtctaaagtgctgcacctggaaggcgaagtgaacaagatcaagagcgccctgctgagcaccaacaaggccgtggtgtctctgagcaatggcgtgtccgtgctgaccttcaaggtgctggacctgaagaactacatcgacaaacagctgctgcccatcctgaacaagcagtcctgcagcatccccaacatcgagacagtgatcgagttccagcagaagaacaaccggctgctggaaatcacccgcgagttctctgtgaatgccggcgtgaccacacctgtgtccacctacatgctgaccaacagcgagctgctgagcctgatcaacgacatgcccatcaccaacgaccagaaaaagctgatgagcaacaacgtgcagatcgtgcggcagcagagctacagcatcatgagcattatcaaagaagaggtgctggcctacgtggtgcagctgcctctgtatggcgtgatcgataccccttgctggaagctgcacacaagccctctgtgcaccaccaacaccaaagagggcagcaacatctgcctgaccagaaccgactgcggctggtactgcgataatgccggcagcgtctcattcttcccacaagccgagacatgcaaggtgcagagcaaccgggtgttctgcgacaccatgaatagcagaaccctgccttgcgaagtgaatctgtgcaacgtggacatcttcaaccctaagtacgactgcaagatcatgaccagcaagaccgacgtgtccagcagtgtgatcacctcactgggcgccatcgtgtcctgttacggcaagaccaagtgcaccgccagcaacaagaaccggggcatcatcaagaccttcagcaacggctgcgactacgtgtccaacaaaggcgtggacaccgtgtctgtgggcaacaccctgtactacgtgaacaaacaagagggccagtctctgtacgtgaagggcgagcccatcatcaacttctacgaccctctggtgttccccagcgacgagttcgatgccagcatcagccaagtgaacgagaagatcaatcagagcctggccttcatcagaaagtccgatgagctgctgcacaacgtgaacgccggcaagtccaccaccaatatcatgatcacgaccatcatcatcgtgattatcgtgatcctgctgtccctgatcgccgtgggcctgctgctttattgataataggctggagcctcggtggccatgcttcttgccccttgggcctccccccagcccctcctccccttcctgcacccgtacccccgtggtctttgaataaagtctgagtgggcggcaaaaaaaaaaaaaaaaaaaaaaaaaaaaaaaaaaaaaaaaaaaaaaaaaaaaaaaaaaaaaaaaaaaaaaaaaaaaaaaaaaaaaaaaaaaaaaaaaaaaaaaaaaaaaa

SEQ ID NO: 199 - DNA, 1539 bp, synthetic construct
  source 1..1539: mol_type = other DNA
atggaactgctgatcctgaaggccaacgccatcaccaccatcctgaccgccgtgaccttctgttttgccagcggccagaacatcaccgaggaattctaccagagcacctgtagcgccgtgtccaagggatatctgggcgcccttagaaccggctggtacaccagcgtgatcaccatcgagctgagcaacatcaaagaaaacaagtgcaacggcaccgacgccaaagtgaagctgatcaagcaagagctggacaagtacaagaatgccgtgaccgacctgcagctgctgatgcagtctacaccagccacaggctctggcagcgccattgcctctggtgtcgccgtgtctaaagtgctgcacctggaaggcgaagtgaacaagatcaagagcgccctgctgagcaccaacaaggccgtggtgtctctgagcaatggcgtgtccgtgctgaccttcaaggtgctggacctgaagaactacatcgacaaacagctgctgcccatcctgaacaagcagtcctgcagcatccccaacatcgagacagtgatcgagttccagcagaagaacaaccggctgctggaaatcacccgcgagttctctgtgaatgccggcgtgaccacacctgtgtccacctacatgctgaccaacagcgagctgctgagcctgatcaacgacatgcccatcaccaacgaccagaaaaagctgatgagcaacaacgtgcagatcgtgcggcagcagagctacagcatcatgagcattatcaaagaagaggtgctggcctacgtggtgcagctgcctctgtatggcgtgatcgataccccttgctggaagctgcacacaagccctctgtgcaccaccaacaccaaagagggcagcaacatctgcctgaccagaaccgactgcggctggtactgcgataatgccggcagcgtctcattcttcccacaagccgagacatgcaaggtgcagagcaaccgggtgttctgcgacaccatgaatagcagaaccctgccttgcgaagtgaatctgtgcaacgtggacatcttcaaccctaagtacgactgcaagatcatgaccagcaagaccgacgtgtccagcagtgtgatcacctcactgggcgccatcgtgtcctgttacggcaagaccaagtgcaccgccagcaacaagaaccggggcatcatcaagaccttcagcaacggctgcgactacgtgtccaacaaaggcgtggacaccgtgtctgtgggcaacaccctgtactacgtgaacaaacaagagggccagtctctgtacgtgaagggcgagcccatcatcaacttctacgaccctctggtgttccccagcgacgagttcgatgccagcatcagccaagtgaacgagaagatcaatcagagcctggccttcatcagaaagtccgatgagctgctgcacaacgtgaacgccggcaagtccaccaccaatatcatgatcacgaccatcatcatcgtgattatcgtgatcctgctgtccctgatcgccgtgggcctgctgctttattgataatag

SEQ ID NO: 200 - protein, 510 aa, synthetic construct
MELLILKANAITTILTAVTFCFASGQNITEEFYQSTCSAVSKGYLGALRTGWYTSVITIELSNIKENKCNGTDAKVKLIKQELDKYKNAVTDLQLLMQSTPATGSGSAIASGVAVSKVLHLEGEVNKIKSALLSTNKAVVSLSNGVSVLTFKVLDLKNYIDKQLLPILNKQSCSIPNIETVIEFQQKNNRLLEITREFSVNAGVTTPVSTYMLTNSELLSLINDMPITNDQKKLMSNNVQIVRQQSYSIMSIIKEEVLAYVVQLPLYGVIDTPCWKLHTSPLCTTNTKEGSNICLTRTDCGWYCDNAGSVSFFPQAETCKVQSNRVFCDTMNSRTLPCEVNLCNVDIFNPKYDCKIMTSKTDVSSSVITSLGAIVSCYGKTKCTASNKNRGIIKTFSNGCDYVSNKGVDTVSVGNTLYYVNKQEGQSLYVKGEPIINFYDPLVFPSDEFDASISQVNEKINQSLAFIRKSDELLHNVNAGKSTTNIMITTIIIVIIVILLSLIAVGLLLY

SEQ ID NO: 201 - RNA, 1841 nt, synthetic construct
  source 1..1841: mol_type = other RNA
agcggctcggccattttgtcccagtcagtccggaggctgcggctgcagaagtaccgcctgcggagtaactgcaaaggccaccatggaactgctgatcctgaaggccaacgccatcaccaccatcctgaccgccgtgaccttctgttttgccagcggccagaacatcaccgaggaattctaccagagcacctgtagcgccgtgtccaagggatatctgggcgcccttagaaccggctggtacaccagcgtgatcaccatcgagctgagcaacatcaaagaaaacaagtgcaacggcaccgacgccaaagtgaagctgatcaagcaagagctggacaagtacaagaatgccgtgaccgacctgcagctgctgatgcagtctacaccagccacaggctctggcagcgccattgcctctggtgtcgccgtgtctaaagtgctgcacctggaaggcgaagtgaacaagatcaagagcgccctgctgagcaccaacaaggccgtggtgtctctgagcaatggcgtgtccgtgctgaccttcaaggtgctggacctgaagaactacatcgacaaacagctgctgcccatcctgaacaagcagtcctgcagcatccccaacatcgagacagtgatcgagttccagcagaagaacaaccggctgctggaaatcacccgcgagttctctgtgaatgccggcgtgaccacacctgtgtccacctacatgctgaccaacagcgagctgctgagcctgatcaacgacatgcccatcaccaacgaccagaaaaagctgatgagcaacaacgtgcagatcgtgcggcagcagagctacagcatcatgagcattatcaaagaagaggtgctggcctacgtggtgcagctgcctctgtatggcgtgatcgataccccttgctggaagctgcacacaagccctctgtgcaccaccaacaccaaagagggcagcaacatctgcctgaccagaaccgactgcggctggtactgcgataatgccggcagcgtctcattcttcccacaagccgagacatgcaaggtgcagagcaaccgggtgttctgcgacaccatgaatagcagaaccctgccttgcgaagtgaatctgtgcaacgtggacatcttcaaccctaagtacgactgcaagatcatgaccagcaagaccgacgtgtccagcagtgtgatcacctcactgggcgccatcgtgtcctgttacggcaagaccaagtgcaccgccagcaacaagaaccggggcatcatcaagaccttcagcaacggctgcgactacgtgtccaacaaaggcgtggacaccgtgtctgtgggcaacaccctgtactacgtgaacaaacaagagggccagtctctgtacgtgaagggcgagcccatcatcaacttctacgaccctctggtgttccccagcgacgagttcgatgccagcatcagccaagtgaacgagaagatcaatcagagcctggccttcatcagaaagtccgatgagctgctgcacaacgtgaacgccggcaagtccaccaccaatatcatgatcacgaccatcatcatcgtgattatcgtgatcctgctgtccctgatcgccgtgggcctgctgctttattgataataggctggagcctcggtggccatgcttcttgccccttgggcctccccccagcccctcctccccttcctgcacccgtacccccgtggtctttgaataaagtctgagtgggcggcaaaaaaaaaaaaaaaaaaaaaaaaaaaaaaaaaaaaaaaaaaaaaaaaaaaaaaaaaaaaaaaaaaaaaaaaaaaaaaaaaaaaaaaaaaaaaaaaaaaaaaaaaaaaaa

SEQ ID NO: 202 - DNA, 1841 bp, synthetic construct
  source 1..1841: mol_type = other DNA
agcggctcggccattttgtcccagtcagtccggaggctgcggctgcagaagtaccgcctgcggagtaactgcaaaggccaccatggaactgctgatcctgaaggccaacgccatcaccaccatcctgaccgccgtgaccttctgttttgccagcggccagaacatcaccgaggaattctaccagagcacctgtagcgccgtgtccaagggatatctgggcgcccttagaaccggctggtacaccagcgtgatcaccatcgagctgagcaacatcaaagaaaacaagtgcaacggcaccgacgccaaagtgaagctgatcaagcaagagctggacaagtacaagaatgccgtgaccgacctgcagctgctgatgcagtctacaccagccacaggctctggcagcgccatttgttctggtatcgccgtgtgcaaagtgctgcacctggaaggcgaagtgaacaagatcaagagcgccctgctgagcaccaacaaggccgtggtgtctctgagcaatggcgtgtccgtgctgaccttcaaggtgctggacctgaagaactacatcgacaaacagctgctgcccatcgtcaacaagcagtcctgcagcatccccaacatcgagacagtgatcgagttccagcagaagaacaaccggctgctggaaatcacccgcgagttctctgtgaatgccggcgtgaccacacctgtgtccacctacatgctgaccaacagcgagctgctgagcctgatcaacgacatgcccatcaccaacgaccagaaaaagctgatgagcaacaacgtgcagatcgtgcggcagcagagctacagcatcatgtgcattatcaaagaagagatcctggcctacgtggtgcagctgcctctgtatggcgtgatcgataccccttgctggaagctgcacacaagccctctgtgcaccaccaacaccaaagagggcagcaacatctgcctgaccagaaccgacagaggctggtactgcgataatgccggcagcgtctcattcttcccacaagccgagacatgcaaggtgcagagcaaccgggtgttctgcgacaccatgaatagcagaaccctgccttccgaagtgaatctgtgcaacgtggacatcttcaaccctaagtacgactgcaagatcatgaccagcaagaccgacgtgtccagcagtgtgatcacctcactgggcgccatcgtgtcctgttacggcaagaccaagtgcaccgccagcaacaagaaccggggcatcatcaagaccttcagcaacggctgcgactacgtgtccaacaaaggcgtggacaccgtgtctgtgggcaacaccctgtactgcgtgaacaaacaagagggccagtctctgtacgtgaagggcgagcccatcatcaacttctacgaccctctggtgttccccagcagcgagttcgatgccagcatcagccaagtgaacgagaagatcaatcagagcctggccttcatcagaaagtccgatgagctgctgcacaacgtgaacgccggcaagtccaccaccaatatcatgatcacgaccatcatcatcgtgattatcgtgatcctgctgtccctgatcgccgtgggcctgctgctttattgataataggctggagcctcggtggccatgcttcttgccccttgggcctccccccagcccctcctccccttcctgcacccgtacccccgtggtctttgaataaagtctgagtgggcggcaaaaaaaaaaaaaaaaaaaaaaaaaaaaaaaaaaaaaaaaaaaaaaaaaaaaaaaaaaaaaaaaaaaaaaaaaaaaaaaaaaaaaaaaaaaaaaaaaaaaaaaaaaaaaa

SEQ ID NO: 203 - DNA, 1539 bp, synthetic construct
  source 1..1539: mol_type = other DNA
atggaactgctgatcctgaaggccaacgccatcaccaccatcctgaccgccgtgaccttctgttttgccagcggccagaacatcaccgaggaattctaccagagcacctgtagcgccgtgtccaagggatatctgggcgcccttagaaccggctggtacaccagcgtgatcaccatcgagctgagcaacatcaaagaaaacaagtgcaacggcaccgacgccaaagtgaagctgatcaagcaagagctggacaagtacaagaatgccgtgaccgacctgcagctgctgatgcagtctacaccagccacaggctctggcagcgccatttgttctggtatcgccgtgtgcaaagtgctgcacctggaaggcgaagtgaacaagatcaagagcgccctgctgagcaccaacaaggccgtggtgtctctgagcaatggcgtgtccgtgctgaccttcaaggtgctggacctgaagaactacatcgacaaacagctgctgcccatcgtcaacaagcagtcctgcagcatccccaacatcgagacagtgatcgagttccagcagaagaacaaccggctgctggaaatcacccgcgagttctctgtgaatgccggcgtgaccacacctgtgtccacctacatgctgaccaacagcgagctgctgagcctgatcaacgacatgcccatcaccaacgaccagaaaaagctgatgagcaacaacgtgcagatcgtgcggcagcagagctacagcatcatgtgcattatcaaagaagagatcctggcctacgtggtgcagctgcctctgtatggcgtgatcgataccccttgctggaagctgcacacaagccctctgtgcaccaccaacaccaaagagggcagcaacatctgcctgaccagaaccgacagaggctggtactgcgataatgccggcagcgtctcattcttcccacaagccgagacatgcaaggtgcagagcaaccgggtgttctgcgacaccatgaatagcagaaccctgccttccgaagtgaatctgtgcaacgtggacatcttcaaccctaagtacgactgcaagatcatgaccagcaagaccgacgtgtccagcagtgtgatcacctcactgggcgccatcgtgtcctgttacggcaagaccaagtgcaccgccagcaacaagaaccggggcatcatcaagaccttcagcaacggctgcgactacgtgtccaacaaaggcgtggacaccgtgtctgtgggcaacaccctgtactgcgtgaacaaacaagagggccagtctctgtacgtgaagggcgagcccatcatcaacttctacgaccctctggtgttccccagcagcgagttcgatgccagcatcagccaagtgaacgagaagatcaatcagagcctggccttcatcagaaagtccgatgagctgctgcacaacgtgaacgccggcaagtccaccaccaatatcatgatcacgaccatcatcatcgtgattatcgtgatcctgctgtccctgatcgccgtgggcctgctgctttattgataatag

SEQ ID NO: 204 - protein, 510 aa, synthetic construct
MELLILKANAITTILTAVTFCFASGQNITEEFYQSTCSAVSKGYLGALRTGWYTSVITIELSNIKENKCNGTDAKVKLIKQELDKYKNAVTDLQLLMQSTPATGSGSAICSGIAVCKVLHLEGEVNKIKSALLSTNKAVVSLSNGVSVLTFKVLDLKNYIDKQLLPIVNKQSCSIPNIETVIEFQQKNNRLLEITREFSVNAGVTTPVSTYMLTNSELLSLINDMPITNDQKKLMSNNVQIVRQQSYSIMCIIKEEILAYVVQLPLYGVIDTPCWKLHTSPLCTTNTKEGSNICLTRTDRGWYCDNAGSVSFFPQAETCKVQSNRVFCDTMNSRTLPSEVNLCNVDIFNPKYDCKIMTSKTDVSSSVITSLGAIVSCYGKTKCTASNKNRGIIKTFSNGCDYVSNKGVDTVSVGNTLYCVNKQEGQSLYVKGEPIINFYDPLVFPSSEFDASISQVNEKINQSLAFIRKSDELLHNVNAGKSTTNIMITTIIIVIIVILLSLIAVGLLLY

SEQ ID NO: 205 - RNA, 1841 nt, synthetic construct
  source 1..1841: mol_type = other RNA
agcggctcggccattttgtcccagtcagtccggaggctgcggctgcagaagtaccgcctgcggagtaactgcaaaggccaccatggaactgctgatcctgaaggccaacgccatcaccaccatcctgaccgccgtgaccttctgttttgccagcggccagaacatcaccgaggaattctaccagagcacctgtagcgccgtgtccaagggatatctgggcgcccttagaaccggctggtacaccagcgtgatcaccatcgagctgagcaacatcaaagaaaacaagtgcaacggcaccgacgccaaagtgaagctgatcaagcaagagctggacaagtacaagaatgccgtgaccgacctgcagctgctgatgcagtctacaccagccacaggctctggcagcgccatttgttctggtatcgccgtgtgcaaagtgctgcacctggaaggcgaagtgaacaagatcaagagcgccctgctgagcaccaacaaggccgtggtgtctctgagcaatggcgtgtccgtgctgaccttcaaggtgctggacctgaagaactacatcgacaaacagctgctgcccatcgtcaacaagcagtcctgcagcatccccaacatcgagacagtgatcgagttccagcagaagaacaaccggctgctggaaatcacccgcgagttctctgtgaatgccggcgtgaccacacctgtgtccacctacatgctgaccaacagcgagctgctgagcctgatcaacgacatgcccatcaccaacgaccagaaaaagctgatgagcaacaacgtgcagatcgtgcggcagcagagctacagcatcatgtgcattatcaaagaagagatcctggcctacgtggtgcagctgcctctgtatggcgtgatcgataccccttgctggaagctgcacacaagccctctgtgcaccaccaacaccaaagagggcagcaacatctgcctgaccagaaccgacagaggctggtactgcgataatgccggcagcgtctcattcttcccacaagccgagacatgcaaggtgcagagcaaccgggtgttctgcgacaccatgaatagcagaaccctgccttccgaagtgaatctgtgcaacgtggacatcttcaaccctaagtacgactgcaagatcatgaccagcaagaccgacgtgtccagcagtgtgatcacctcactgggcgccatcgtgtcctgttacggcaagaccaagtgcaccgccagcaacaagaaccggggcatcatcaagaccttcagcaacggctgcgactacgtgtccaacaaaggcgtggacaccgtgtctgtgggcaacaccctgtactgcgtgaacaaacaagagggccagtctctgtacgtgaagggcgagcccatcatcaacttctacgaccctctggtgttccccagcagcgagttcgatgccagcatcagccaagtgaacgagaagatcaatcagagcctggccttcatcagaaagtccgatgagctgctgcacaacgtgaacgccggcaagtccaccaccaatatcatgatcacgaccatcatcatcgtgattatcgtgatcctgctgtccctgatcgccgtgggcctgctgctttattgataataggctggagcctcggtggccatgcttcttgccccttgggcctccccccagcccctcctccccttcctgcacccgtacccccgtggtctttgaataaagtctgagtgggcggcaaaaaaaaaaaaaaaaaaaaaaaaaaaaaaaaaaaaaaaaaaaaaaaaaaaaaaaaaaaaaaaaaaaaaaaaaaaaaaaaaaaaaaaaaaaaaaaaaaaaaaaaaaaaaa

SEQ ID NO: 206 - DNA, 1841 bp, synthetic construct
  source 1..1841: mol_type = other DNA
agcggctcggccattttgtcccagtcagtccggaggctgcggctgcagaagtaccgcctgcggagtaactgcaaaggccaccatggaactgctgatcctgaaggccaacgccatcaccaccatcctgaccgccgtgaccttctgttttgccagcggccagaacatcaccgaggaattctaccagagcacctgtagcgccgtgtccaagggatatctgggcgcccttagaaccggctggtacaccagcgtgatcaccatcgagctgagcaacatcaaagaaaacaagtacaacggcaccgaggtgaaagtgaagctgatcaagcaagagctggacaagtacaagagcgccgtgaccgacctgcagctgctgatgcagtctacaccagccacaggctctggcagcgccatttgttctggtatcgccgtgtgcaaagtgctgcacctggaaggcgaagtgaacaagatcaagagcgccctgctgagcaccaacaaggccgtggtgtctctgagcaatggcgtgtccgtgctgaccttcaaggtgctggacctgaagaactacatcgacaaacagctgctgcccatcgtcaacaagcagtcctgcagcatccccaacatcgagacagtgatcgagttccagcagaagaacaaccggctgctggaaatcacccgcgagttctctgtgaatgccggcgtgaccacacctgtgtccacctacatgctgaccaacagcgagctgctgagcctgatcaacgacatgcccatcaccaacgaccagaaaaagctgatgagcaacaacgtgcagatcgtgcggcagcagagctacagcatcatgtgcattatcaaagaagagatcctggcctacgtggtgcagctgcctctgtatggcgtgatcgataccccttgctggaagctgcacacaagccctctgtgcaccaccaacaccaaagagggcagcaacatctgcctgaccagaaccgacagaggctggtactgcgataatgccggcagcgtctcattcttcccacaagccgagacatgcaaggtgcagagcaaccgggtgttctgcgacaccatgaatagcagaaccctgccttccgaagtgaatctgtgcaacgtggacatcttcaaccctaagtacgactgcaagatcatgaccagcaagaccgacgtgtccagcagtgtgatcacctcactgggcgccatcgtgtcctgttacggcaagaccaagtgcaccgccagcaacaagaaccggggcatcatcaagaccttcagcaacggctgcgactacgtgtccaacaaaggcgtggacaccgtgtctgtgggcaacaccctgtactgcgtgaacaaacaagagggccagtctctgtacgtgaagggcgagcccatcatcaacttctacgaccctctggtgttccccagcagcgagttcgatgccagcatcagccaagtgaacgagaagatcaatcagagcctggccttcatcagaaagtccgatgagctgctgcacaacgtgaacgccggcaagtccaccaccaatatcatgatcacgaccatcatcatcgtgattatcgtgatcctgctgtccctgatcgccgtgggcctgctgctttattgataataggctggagcctcggtggccatgcttcttgccccttgggcctccccccagcccctcctccccttcctgcacccgtacccccgtggtctttgaataaagtctgagtgggcggcaaaaaaaaaaaaaaaaaaaaaaaaaaaaaaaaaaaaaaaaaaaaaaaaaaaaaaaaaaaaaaaaaaaaaaaaaaaaaaaaaaaaaaaaaaaaaaaaaaaaaaaaaaaaaa

SEQ ID NO: 207 - DNA, 1539 bp, synthetic construct
  source 1..1539: mol_type = other DNA
atggaactgctgatcctgaaggccaacgccatcaccaccatcctgaccgccgtgaccttctgttttgccagcggccagaacatcaccgaggaattctaccagagcacctgtagcgccgtgtccaagggatatctgggcgcccttagaaccggctggtacaccagcgtgatcaccatcgagctgagcaacatcaaagaaaacaagtacaacggcaccgaggtgaaagtgaagctgatcaagcaagagctggacaagtacaagagcgccgtgaccgacctgcagctgctgatgcagtctacaccagccacaggctctggcagcgccatttgttctggtatcgccgtgtgcaaagtgctgcacctggaaggcgaagtgaacaagatcaagagcgccctgctgagcaccaacaaggccgtggtgtctctgagcaatggcgtgtccgtgctgaccttcaaggtgctggacctgaagaactacatcgacaaacagctgctgcccatcgtcaacaagcagtcctgcagcatccccaacatcgagacagtgatcgagttccagcagaagaacaaccggctgctggaaatcacccgcgagttctctgtgaatgccggcgtgaccacacctgtgtccacctacatgctgaccaacagcgagctgctgagcctgatcaacgacatgcccatcaccaacgaccagaaaaagctgatgagcaacaacgtgcagatcgtgcggcagcagagctacagcatcatgtgcattatcaaagaagagatcctggcctacgtggtgcagctgcctctgtatggcgtgatcgataccccttgctggaagctgcacacaagccctctgtgcaccaccaacaccaaagagggcagcaacatctgcctgaccagaaccgacagaggctggtactgcgataatgccggcagcgtctcattcttcccacaagccgagacatgcaaggtgcagagcaaccgggtgttctgcgacaccatgaatagcagaaccctgccttccgaagtgaatctgtgcaacgtggacatcttcaaccctaagtacgactgcaagatcatgaccagcaagaccgacgtgtccagcagtgtgatcacctcactgggcgccatcgtgtcctgttacggcaagaccaagtgcaccgccagcaacaagaaccggggcatcatcaagaccttcagcaacggctgcgactacgtgtccaacaaaggcgtggacaccgtgtctgtgggcaacaccctgtactgcgtgaacaaacaagagggccagtctctgtacgtgaagggcgagcccatcatcaacttctacgaccctctggtgttccccagcagcgagttcgatgccagcatcagccaagtgaacgagaagatcaatcagagcctggccttcatcagaaagtccgatgagctgctgcacaacgtgaacgccggcaagtccaccaccaatatcatgatcacgaccatcatcatcgtgattatcgtgatcctgctgtccctgatcgccgtgggcctgctgctttattgataatag

SEQ ID NO: 208 - protein, 510 aa, synthetic construct
MELLILKANAITTILTAVTFCFASGQNITEEFYQSTCSAVSKGYLGALRTGWYTSVITIELSNIKENKYNGTEVKVKLIKQELDKYKSAVTDLQLLMQSTPATGSGSAICSGIAVCKVLHLEGEVNKIKSALLSTNKAVVSLSNGVSVLTFKVLDLKNYIDKQLLPIVNKQSCSIPNIETVIEFQQKNNRLLEITREFSVNAGVTTPVSTYMLTNSELLSLINDMPITNDQKKLMSNNVQIVRQQSYSIMCIIKEEILAYVVQLPLYGVIDTPCWKLHTSPLCTTNTKEGSNICLTRTDRGWYCDNAGSVSFFPQAETCKVQSNRVFCDTMNSRTLPSEVNLCNVDIFNPKYDCKIMTSKTDVSSSVITSLGAIVSCYGKTKCTASNKNRGIIKTFSNGCDYVSNKGVDTVSVGNTLYCVNKQEGQSLYVKGEPIINFYDPLVFPSSEFDASISQVNEKINQSLAFIRKSDELLHNVNAGKSTTNIMITTIIIVIIVILLSLIAVGLLLY

SEQ ID NO: 209 - RNA, 1841 nt, synthetic construct
  source 1..1841: mol_type = other RNA
agcggctcggccattttgtcccagtcagtccggaggctgcggctgcagaagtaccgcctgcggagtaactgcaaaggccaccatggaactgctgatcctgaaggccaacgccatcaccaccatcctgaccgccgtgaccttctgttttgccagcggccagaacatcaccgaggaattctaccagagcacctgtagcgccgtgtccaagggatatctgggcgcccttagaaccggctggtacaccagcgtgatcaccatcgagctgagcaacatcaaagaaaacaagtacaacggcaccgaggtgaaagtgaagctgatcaagcaagagctggacaagtacaagagcgccgtgaccgacctgcagctgctgatgcagtctacaccagccacaggctctggcagcgccatttgttctggtatcgccgtgtgcaaagtgctgcacctggaaggcgaagtgaacaagatcaagagcgccctgctgagcaccaacaaggccgtggtgtctctgagcaatggcgtgtccgtgctgaccttcaaggtgctggacctgaagaactacatcgacaaacagctgctgcccatcgtcaacaagcagtcctgcagcatccccaacatcgagacagtgatcgagttccagcagaagaacaaccggctgctggaaatcacccgcgagttctctgtgaatgccggcgtgaccacacctgtgtccacctacatgctgaccaacagcgagctgctgagcctgatcaacgacatgcccatcaccaacgaccagaaaaagctgatgagcaacaacgtgcagatcgtgcggcagcagagctacagcatcatgtgcattatcaaagaagagatcctggcctacgtggtgcagctgcctctgtatggcgtgatcgataccccttgctggaagctgcacacaagccctctgtgcaccaccaacaccaaagagggcagcaacatctgcctgaccagaaccgacagaggctggtactgcgataatgccggcagcgtctcattcttcccacaagccgagacatgcaaggtgcagagcaaccgggtgttctgcgacaccatgaatagcagaaccctgccttccgaagtgaatctgtgcaacgtggacatcttcaaccctaagtacgactgcaagatcatgaccagcaagaccgacgtgtccagcagtgtgatcacctcactgggcgccatcgtgtcctgttacggcaagaccaagtgcaccgccagcaacaagaaccggggcatcatcaagaccttcagcaacggctgcgactacgtgtccaacaaaggcgtggacaccgtgtctgtgggcaacaccctgtactgcgtgaacaaacaagagggccagtctctgtacgtgaagggcgagcccatcatcaacttctacgaccctctggtgttccccagcagcgagttcgatgccagcatcagccaagtgaacgagaagatcaatcagagcctggccttcatcagaaagtccgatgagctgctgcacaacgtgaacgccggcaagtccaccaccaatatcatgatcacgaccatcatcatcgtgattatcgtgatcctgctgtccctgatcgccgtgggcctgctgctttattgataataggctggagcctcggtggccatgcttcttgccccttgggcctccccccagcccctcctccccttcctgcacccgtacccccgtggtctttgaataaagtctgagtgggcggcaaaaaaaaaaaaaaaaaaaaaaaaaaaaaaaaaaaaaaaaaaaaaaaaaaaaaaaaaaaaaaaaaaaaaaaaaaaaaaaaaaaaaaaaaaaaaaaaaaaaaaaaaaaaaa

SEQ ID NO: 210 - protein, 574 aa, Orthopneumovirus hominis
MELLILKANAITTILTAVTFCFASGQNITEEFYQSTCSAVSKGYLSALRTGWYTSVITIELSNIKENKCNGTDAKVKLIKQELDKYKNAVTELQLLMQSTPATNNRARRELPRFMNYTLNNAKKTNVTLSKKRKRRFLGFLLGVGSAIASGVAVSKVLHLEGEVNKIKSALLSTNKAVVSLSNGVSVLTSKVLDLKNYIDKQLLPIVNKQSCSISNIETVIEFQQKNNRLLEITREFSVNAGVTTPVSTYMLTNSELLSLINDMPITNDQKKLMSNNVQIVRQQSYSIMSIIKEEVLAYVVQLPLYGVIDTPCWKLHTSPLCTTNTKEGSNICLTRTDRGWYCDNAGSVSFFPQAETCKVQSNRVFCDTMNSLTLPSEVNLCNVDIFNPKYDCKIMTSKTDVSSSVITSLGAIVSCYGKTKCTASNKNRGIIKTFSNGCDYVSNKGVDTVSVGNTLYYVNKQEGKSLYVKGEPIINFYDPLVFPSDEFDASISQVNEKINQSLAFIRKSDELLHNVNAGKSTTNIMITTIIIVIIVILLSLIAVGLLLYCKARSTPVTLSKDQLSGINNIAFSN

SEQ ID NO: 211 - protein, 510 aa, synthetic construct
MELLILKANAITTILTAVTFCFASGQNITEEFYQSTCSAVSKGYLGALRTGWYTSVITIELSNIKENKCNGTDAKVKLIKQELDKYKNAVTDLQLLMQSTPATGSGSAICSGVAVCKVLHLEGEVNKIKSALLSTNKAVVSLSNGVSVLTFKVLDLKNYIDKQLLPILNKQSCSIPNIETVIEFQQKNNRLLEITREFSVNAGVTTPVSTYMLTNSELLSLINDMPITNDQKKLMSNNVQIVRQQSYSIMCIIKEEVLAYVVQLPLYGVIDTPCWKLHTSPLCTTNTKEGSNICLTRTDRGWYCDNAGSVSFFPQAETCKVQSNRVFCDTMNSRTLPSEVNLCNVDIFNPKYDCKIMTSKTDVSSSVITSLGAIVSCYGKTKCTASNKNRGIIKTFSNGCDYVSNKGVDTVSVGNTLYCVNKQEGQSLYVKGEPIINFYDPLVFPSDEFDASISQVNEKINQSLAFIRKSDELLHNVNAGKSTTNIMITTIIIVIIVILLSLIAVGLLLY

SEQ ID NO: 212 - protein, 510 aa, synthetic construct
MELLILKANAITTILTAVTFCFASGQNITEEFYQSTCSAVSKGYLGALRTGWYTSVITIELSNIKENKCNGTDAKVKLIKQELDKYKNAVTDLQLLMQSTPATGSGSAICSGIAVCKVLHLEGEVNKIKSALLSTNKAVVSLSNGVSVLTFKVLDLKNYIDKQLLPIVNKQSCSIPNIETVIEFQQKNNRLLEITREFSVNAGVTTPVSTYMLTNSELLSLINDMPITNDQKKLMSNNVQIVRQQSYSIMCIIKEEVLAYVVQLPLYGVIDTPCWKLHTSPLCTTNTKEGSNICLTRTDRGWYCDNAGSVSFFPQAETCKVQSNRVFCDTMNSRTLPSEVNLCNVDIFNPKYDCKIMTSKTDVSSSVITSLGAIVSCYGKTKCTASNKNRGIIKTFSNGCDYVSNKGVDTVSVGNTLYCVNKQEGQSLYVKGEPIINFYDPLVFPSDEFDASISQVNEKINQSLAFIRKSDELLHNVNAGKSTTNIMITTIIIVIIVILLSLIAVGLLLY

SEQ ID NO: 213 - protein, 510 aa, synthetic construct
MELLILKANAITTILTAVTFCFASGQNITEEFYQSTCSAVSKGYLGALRTGWYTSVITIELSNIKENKCNGTDAKVKLIKQELDKYKNAVTDLQLLMQSTPATGSGSAICSGIAVCKVLHLEGEVNKIKSALLSTNKAVVSLSNGVSVLTFKVLDLKNYIDKQLLPIVNKQSCSIPNIETVIEFQQKNNRLLEITREFSVNAGVTTPVSTYMLTNSELLSLINDMPITNDQKKLMSNNVQIVRQQSYSIMCIIKEEILAYVVQLPLYGVIDTPCWKLHTSPLCTTNTKEGSNICLTRTDRGWYCDNAGSVSFFPQAETCKVQSNRVFCDTMNSRTLPSEVNLCNVDIFNPKYDCKIMTSKTDVSSSVITSLGAIVSCYGKTKCTASNKNRGIIKTFSNGCDYVSNKGVDTVSVGNTLYCVNKQEGQSLYVKGEPIINFYDPLVFPSDEFDASISQVNEKINQSLAFIRKSDELLHNVNAGKSTTNIMITTIIIVIIVILLSLIAVGLLLY

SEQ ID NO: 214 - protein, 510 aa, synthetic construct
MELLILKANAITTILTAVTFCFASGQNITEEFYQSTCSAVSKGYLGALRTGWYTSVITIELSNIKENKCNGTDAKVKLIKQELDKYKNAVTDLQLLMQSTPATGSGSAICSGIAVCKVLHLEGEVNKIKSALLSTNKAVVSLSNGVSVLTFKVLDLKNYIDKQLLPIVNKQSCSIPNIETVIEFQQKNNRLLEITREFSVNAGVTTPVSTYMLTNSELLSLINDMPITNDQKKLMSNNVQIVRQQSYSIMCIIKEEVLAYVVQLPLYGVIDTPCWKLHTSPLCTTNTKEGSNICLTRTDRGWYCDNAGSVSFFPQAETCKVQSNRVFCDTMNSRTLPSEVNLCNVDIFNPKYDCKIMTSKTDVSSSVITSLGAIVSCYGKTKCTASNKNRGIIKTFSNGCDYVSNKGVDTVSVGNTLYCVNKQEGQSLYVKGEPIINFYDPLVFPSSEFDASISQVNEKINQSLAFIRKSDELLHNVNAGKSTTNIMITTIIIVIIVILLSLIAVGLLLY

SEQ ID NO: 215 - protein, 510 aa, synthetic construct
MELLILKANAITTILTAVTFCFASGQNITEEFYQSTCSAVSKGYLGALRTGWYTSVITIELSNIKENKCNGTDAKVKLIKQELDKYKNAVTDLQLLMQSTPACGSGSACASGIAVSKVLHLEGEVNKIKSALLSTNKAVVSLSNGVSVLTFKVLDLKNYIDKQLLPIVNKQSCSIPNIETVIEFQQKNNRLLEITREFSVNAGVTTPVSTYMLTNSELLSLINDMPITNDQKKLMSNNVQIVRQQSYSIMSIIKEEILAYVVQLPLYGVIDTPCWKLHTSPLCTTNTKEGSNICLTRTDRGWYCDNAGSVSFFPQAETCKVQSNRVFCDTMNSRTLPSEVNLCNVDIFNPKYDCKIMTSKTDVSSSVITSLGAIVSCYGKTKCTASNKNRGIIKTFSNGCDYVSNKGVDTVSVGNTLYYVNKQEGQSLYVKGEPIINFYDPLVFPSSEFDASISQVNEKINQSLAFIRKSDELLHNVNAGKSTTNIMITTIIIVIIVILLSLIAVGLLLY

SEQ ID NO: 216 - protein, 510 aa, synthetic construct
MELLILKANAITTILTAVTFCFASGQNITEEFYQSTCSAVSKGYLGALRTGWYTCVITIELSNIKENKCNGTDAKVKLIKQELDKYKNAVTDLQLLMQSTPATGSGSAIASGIAVSKVLHLEGEVNKIKSALLSTNKAVVSLSNGVSVCTFKVLDLKNYIDKQLLPIVNKQSCSIPNIETVIEFQQKNNRLLEITREFSVNAGVTTPVSTYMLTNSELLSLINDMPITNDQKKLMSNNVQIVRQQSYSIMSIIKEEILAYVVQLPLYGVIDTPCWKLHTSPLCTTNTKEGSNICLTRTDRGWYCDNAGSVSFFPQAETCKVQSNRVFCDTMNSRTLPSEVNLCNVDIFNPKYDCKIMTSKTDVSSSVITSLGAIVSCYGKTKCTASNKNRGIIKTFSNGCDYVSNKGVDTVSVGNTLYYVNKQEGQSLYVKGEPIINFYDPLVFPSSEFDASISQVNEKINQSLAFIRKSDELLHNVNAGKSTTNIMITTIIIVIIVILLSLIAVGLLLY

SEQ ID NO: 217 - RNA, 82 nt, synthetic construct
  source 1..82: mol_type = other RNA
agcggctcggccattttgtcccagtcagtccggaggctgcggctgcagaagtaccgcctgcggagtaactgcaaaggccacc

SEQ ID NO: 218 - RNA, 69 nt, synthetic construct
  source 1..69: mol_type = other RNA
agactcctccccatcctctccctctgtccctctgtccctctgaccctgcactgtcccagcaccgccacc

SEQ ID NO: 219 - RNA, 57 nt, synthetic construct
  source 1..57: mol_type = other RNA
gggaaataagagagaaaagaagagtaagaagaaatataagaccccggcgccgccacc

SEQ ID NO: 220 - RNA, 54 nt, synthetic construct
  source 1..54: mol_type = other RNA
gagaataaactagtattcttctggtccccacagactcagagagaacccgccacc

SEQ ID NO: 221 - RNA, 47 nt, synthetic construct
  source 1..47: mol_type = other RNA
gggaaataagagagaaaagaagagtaagaagaaatataagagccacc

SEQ ID NO: 222 - RNA, 110 nt, synthetic construct
  source 1..110: mol_type = other RNA
gctggagcctcggtggccatgcttcttgccccttgggcctccccccagcccctcctccccttcctgcacccgtacccccgtggtctttgaataaagtctgagtgggcggc

SEQ ID NO: 223 - RNA, 110 nt, synthetic construct
  source 1..110: mol_type = other RNA
gctggagcctcggtggcctagcttcttgccccttgggcctccccccagcccctcctccccttcctgcacccgtacccccgtggtctttgaataaagtctgagtgggcggc

SEQ ID NO: 224 - RNA, 295 nt, synthetic construct
  source 1..295: mol_type = other RNA
ctcgagctggtactgcatgcacgcaatgctagctgcccctttcccgtcctgggtaccccgagtctcccccgacctcgggtcccaggtatgctcccacctccacctgccccactcaccacctctgctagttccagacacctcccaagcacgcagcaatgcagctcaaaacgcttagcctagccacacccccacgggaaacagcagtgattaacctttagcaataaacgaaagtttaactaagctatactaaccccagggttggtcaatttcgtgccagccacaccctggagctagc

SEQ ID NO: 225 - RNA, 110 nt, synthetic construct
  source 1..110: mol_type = other RNA
tgataataggctggagcctcggtggccatgcttcttgccccttgggcctccccccagcccctcctccccttcctgcacccgtacccccgtggtctttgaataaagtctga